European Patent Application EP 4 736 871 A1, published May 6, 2026. Title: 呼吸道合胞病毒（RSV）疫苗. Applicant: 深圳深信生物科技有限公司. The sequence listing filed with the application follows.

SEQUENCE LISTING (293 sequences)

SEQ ID NO: 1 - protein, 544 aa, synthetic construct
MELPILKTNAITTILAAVTLCFASSQNITEEFYQSTCSAVSKGYLSCLRTGWYHSVITIELSNIKENKCNGTDAKVKLIKQELDKYKNAVTELQLLMQSTPAANSRARRELPRFMNYTLNNTKNTNVTLSKKRKRRFLGFLLGCGSAIASGIAVSKVLHLEGEVNKIKSALLSTNKAVVSLSNGVSVLTSKVLDLKNYIDKQLLPIVNKQSCSISNIETVIEFQQKNNRLLEITREFSVNAGVTTPVSTYMLTNSELLSLINDMPITNDQKKLMSSNVQIVRQQSYSIMSIIKEEVLAYVVQLPLYGVCDTPCWKLHTSPLCTTNTKEGSNICLTRTDRGWYCDNAGSVSFFPQAETCKVQSNRVFCDTMNSLTLPSEVNLCNIDIFNPKYDCKIMTSKTDVSSSCITSLGAIVSCYGKTKCTASNKNRGIIKTFSNGCDYVSNKGVDTVSVGNTLYYVNKQEGKSLYVKGEPIINFYDPLVFPSSEFDASISQVNEKINQSLAFIRKSDELLSAIGGYIPEAPRDGQAYVRKDGEWVLLSTFL

SEQ ID NO: 2 - protein, 544 aa, synthetic construct
MELLIHRSSAIFLTLAINALYLTSSQNITEEFYQSTCSAVSRGYFSCLRTGWYHSVITIELSNIKETKCNGTDTKVKLIKQELDKYKNAVTELQLLMQNTPAANNRARREAPQYMNYTINTTKNLNVSISKKRKRRFLGFLLGCGSAIASGIAVSKVLHLEGEVNKIKNALLSTNKAVVSLSNGVSVLTSKVLDLKNYINNQLLPIVNQQSCRISNIETVIEFQQKNSRLLEITREFSVNAGVTTPLSTYMLTNSELLSLINDMPITNDQKKLMSSNVQIVRQQSYSIMSIIKEEVLAYVVQLPIYGVCDTPCWKLHTSPLCTTNIKEGSNICLTRTDRGWYCDNAGSVSFFPQADTCKVQSNRVFCDTMNSLTLPSEVSLCNTDIFNSKYDCKIMTSKTDISSSCITSLGAIVSCYGKTKCTASNKNRGIIKTFSNGCDYVSNKGVDTVSVGNTLYYVNKLEGKNLYVKGEPIINYYDPLVFPSSEFDASISQVNEKINQSLAFIRRSDELLSAIGGYIPEAPRDGQAYVRKDGEWVLLSTFL

SEQ ID NO: 3 - protein, 544 aa, synthetic construct
MELPILKTNAITTILAAVTLCFASSQNITEEFYQSTCSAVSKGYLSCLRTGWYHSVITIELSNIKENKCNGTDAKVKLIKQELDKYKNAVTELQLLMQSTPAANSRARRELPRFMNYTLNNTKNTNVTLSKKRKRRFLGFLLGVGSAIASGIAVSKVLHLEGEVNKIKSALLSTNKAVVSLSNGVSVLTSKVLDLKNYIDKQLLPIVNKQSCSISNIETVIEFQQKNNRLLEITREFSVNAGVTTPVSTYMLTNSELLSLINDMPITNDQKKLMSSNVQIVRQQSYSIMSIIKEEVLAYVVQLPLYGVCDTPCWKLHTSPLCTTNTKEGSNICLTRTDRGWYCDNAGSVSFFPQAETCKVQSNRVFCDTMNSLTLPSEVNLCNIDIFNPKYDCKIMTSKTDVSSSVITSLGAIVSCYGKTKCTASNKNRGIIKTFSNGCDYVSNKGVDTVSVGNTLYYVNKQEGKSLYVKGEPIINFYDPLVFPSSEFDASISQVNEKINQSLAFIRKSDELLSAIGGYIPEAPRDGQAYVRKDGEWVLLSTFL

SEQ ID NO: 4 - protein, 544 aa, synthetic construct
MELLIHRSSAIFLTLAINALYLTSSQNITEEFYQSTCSAVSRGYFSCLRTGWYHSVITIELSNIKETKCNGTDTKVKLIKQELDKYKNAVTELQLLMQNTPAANNRARREAPQYMNYTINTTKNLNVSISKKRKRRFLGFLLGVGSAIASGIAVSKVLHLEGEVNKIKNALLSTNKAVVSLSNGVSVLTSKVLDLKNYINNQLLPIVNQQSCRISNIETVIEFQQKNSRLLEITREFSVNAGVTTPLSTYMLTNSELLSLINDMPITNDQKKLMSSNVQIVRQQSYSIMSIIKEEVLAYVVQLPIYGVCDTPCWKLHTSPLCTTNIKEGSNICLTRTDRGWYCDNAGSVSFFPQADTCKVQSNRVFCDTMNSLTLPSEVSLCNTDIFNSKYDCKIMTSKTDISSSVITSLGAIVSCYGKTKCTASNKNRGIIKTFSNGCDYVSNKGVDTVSVGNTLYYVNKLEGKNLYVKGEPIINYYDPLVFPSSEFDASISQVNEKINQSLAFIRRSDELLSAIGGYIPEAPRDGQAYVRKDGEWVLLSTFL

SEQ ID NO: 5 - protein, 544 aa, synthetic construct
MELPILKTNAITTILAAVTLCFASSQNITEEFYQSTCSAVSKGYLSACRTGWYHSVITIELSNIKENKCNGTDAKVKLIKQELDKYKNAVTELQLLMQSTPAANSRARRELPRFMNYTLNNTKNTNVTLSKKRKRRFLGFLLGCGSAIASGIAVSKVLHLEGEVNKIKSALLSTNKAVVSLSNGVSVLTSKVLDLKNYIDKQLLPIVNKQSCSISNIETVIEFQQKNNRLLEITREFSVNAGVTTPVSTYMLTNSELLSLINDMPITNDQKKLMSSNVQIVRQQSYSIMSIIKEEVLAYVVQLPLYGCIDTPCWKLHTSPLCTTNTKEGSNICLTRTDRGWYCDNAGSVSFFPQAETCKVQSNRVFCDTMNSLTLPSEVNLCNIDIFNPKYDCKIMTSKTDVSSSCITSLGAIVSCYGKTKCTASNKNRGIIKTFSNGCDYVSNKGVDTVSVGNTLYYVNKQEGKSLYVKGEPIINFYDPLVFPSSEFDASISQVNEKINQSLAFIRKSDELLSAIGGYIPEAPRDGQAYVRKDGEWVLLSTFL

SEQ ID NO: 6 - protein, 544 aa, synthetic construct
MELLIHRSSAIFLTLAINALYLTSSQNITEEFYQSTCSAVSRGYFSACRTGWYHSVITIELSNIKETKCNGTDTKVKLIKQELDKYKNAVTELQLLMQNTPAANNRARREAPQYMNYTINTTKNLNVSISKKRKRRFLGFLLGCGSAIASGIAVSKVLHLEGEVNKIKNALLSTNKAVVSLSNGVSVLTSKVLDLKNYINNQLLPIVNQQSCRISNIETVIEFQQKNSRLLEITREFSVNAGVTTPLSTYMLTNSELLSLINDMPITNDQKKLMSSNVQIVRQQSYSIMSIIKEEVLAYVVQLPIYGCIDTPCWKLHTSPLCTTNIKEGSNICLTRTDRGWYCDNAGSVSFFPQADTCKVQSNRVFCDTMNSLTLPSEVSLCNTDIFNSKYDCKIMTSKTDISSSCITSLGAIVSCYGKTKCTASNKNRGIIKTFSNGCDYVSNKGVDTVSVGNTLYYVNKLEGKNLYVKGEPIINYYDPLVFPSSEFDASISQVNEKINQSLAFIRRSDELLSAIGGYIPEAPRDGQAYVRKDGEWVLLSTFL

SEQ ID NO: 7 - protein, 544 aa, synthetic construct
MELPILKTNAITTILAAVTLCFASSQNITEEFYQSTCSAVSKGYLSACRTGWYHSVITIELSNIKENKCNGTDAKVKLIKQELDKYKNAVTELQLLMQSTPAANSRARRELPRFMNYTLNNTKNTNVTLSKKRKRRFLGFLLGVGSAIASGIAVSKVLHLEGEVNKIKSALLSTNKAVVSLSNGVSVLTSKVLDLKNYIDKQLLPIVNKQSCSISNIETVIEFQQKNNRLLEITREFSVNAGVTTPVSTYMLTNSELLSLINDMPITNDQKKLMSSNVQIVRQQSYSIMSIIKEEVLAYVVQLPLYGCIDTPCWKLHTSPLCTTNTKEGSNICLTRTDRGWYCDNAGSVSFFPQAETCKVQSNRVFCDTMNSLTLPSEVNLCNIDIFNPKYDCKIMTSKTDVSSSVITSLGAIVSCYGKTKCTASNKNRGIIKTFSNGCDYVSNKGVDTVSVGNTLYYVNKQEGKSLYVKGEPIINFYDPLVFPSSEFDASISQVNEKINQSLAFIRKSDELLSAIGGYIPEAPRDGQAYVRKDGEWVLLSTFL

SEQ ID NO: 8 - protein, 544 aa, synthetic construct
MELLIHRSSAIFLTLAINALYLTSSQNITEEFYQSTCSAVSRGYFSACRTGWYHSVITIELSNIKETKCNGTDTKVKLIKQELDKYKNAVTELQLLMQNTPAANNRARREAPQYMNYTINTTKNLNVSISKKRKRRFLGFLLGVGSAIASGIAVSKVLHLEGEVNKIKNALLSTNKAVVSLSNGVSVLTSKVLDLKNYINNQLLPIVNQQSCRISNIETVIEFQQKNSRLLEITREFSVNAGVTTPLSTYMLTNSELLSLINDMPITNDQKKLMSSNVQIVRQQSYSIMSIIKEEVLAYVVQLPIYGCIDTPCWKLHTSPLCTTNIKEGSNICLTRTDRGWYCDNAGSVSFFPQADTCKVQSNRVFCDTMNSLTLPSEVSLCNTDIFNSKYDCKIMTSKTDISSSVITSLGAIVSCYGKTKCTASNKNRGIIKTFSNGCDYVSNKGVDTVSVGNTLYYVNKLEGKNLYVKGEPIINYYDPLVFPSSEFDASISQVNEKINQSLAFIRRSDELLSAIGGYIPEAPRDGQAYVRKDGEWVLLSTFL

SEQ ID NO: 9 - protein, 544 aa, synthetic construct
MELPILKTNAITTILAAVTLCFASSQNITEEFYQSTCSAVSKGYLCALRTGWYHSVITIELSNIKENKCNGTDAKVKLIKQELDKYKNAVTELQLLMQSTPAANSRARRELPRFMNYTLNNTKNTNVTLSKKRKRRFLGFLLGCGSAIASGIAVSKVLHLEGEVNKIKSALLSTNKAVVSLSNGVSVLTSKVLDLKNYIDKQLLPIVNKQSCSISNIETVIEFQQKNNRLLEITREFSVNAGVTTPVSTYMLTNSELLSLINDMPITNDQKKLMSSNVQIVRQQSYSIMSIIKEEVLAYVVQLPLYGVIDCPCWKLHTSPLCTTNTKEGSNICLTRTDRGWYCDNAGSVSFFPQAETCKVQSNRVFCDTMNSLTLPSEVNLCNIDIFNPKYDCKIMTSKTDVSSSCITSLGAIVSCYGKTKCTASNKNRGIIKTFSNGCDYVSNKGVDTVSVGNTLYYVNKQEGKSLYVKGEPIINFYDPLVFPSSEFDASISQVNEKINQSLAFIRKSDELLSAIGGYIPEAPRDGQAYVRKDGEWVLLSTFL

SEQ ID NO: 10 - protein, 546 aa, synthetic construct
NOMELLIHRSSAIFLTLAINALYLTSSQNITEEFYQSTCSAVSRGYFCALRTGWYHSVITIELSNIKETKCNGTDTKVKLIKQELDKYKNAVTELQLLMQNTPAANNRARREAPQYMNYTINTTKNLNVSISKKRKRRFLGFLLGCGSAIASGIAVSKVLHLEGEVNKIKNALLSTNKAVVSLSNGVSVLTSKVLDLKNYINNQLLPIVNQQSCRISNIETVIEFQQKNSRLLEITREFSVNAGVTTPLSTYMLTNSELLSLINDMPITNDQKKLMSSNVQIVRQQSYSIMSIIKEEVLAYVVQLPIYGVIDCPCWKLHTSPLCTTNIKEGSNICLTRTDRGWYCDNAGSVSFFPQADTCKVQSNRVFCDTMNSLTLPSEVSLCNTDIFNSKYDCKIMTSKTDISSSCITSLGAIVSCYGKTKCTASNKNRGIIKTFSNGCDYVSNKGVDTVSVGNTLYYVNKLEGKNLYVKGEPIINYYDPLVFPSSEFDASISQVNEKINQSLAFIRRSDELLSAIGGYIPEAPRDGQAYVRKDGEWVLLSTFL

SEQ ID NO: 11 - protein, 544 aa, synthetic construct
MELPILKTNAITTILAAVTLCFASSQNITEEFYQSTCSAVSKGYLCALRTGWYHSVITIELSNIKENKCNGTDAKVKLIKQELDKYKNAVTELQLLMQSTPAANSRARRELPRFMNYTLNNTKNTNVTLSKKRKRRFLGFLLGVGSAIASGIAVSKVLHLEGEVNKIKSALLSTNKAVVSLSNGVSVLTSKVLDLKNYIDKQLLPIVNKQSCSISNIETVIEFQQKNNRLLEITREFSVNAGVTTPVSTYMLTNSELLSLINDMPITNDQKKLMSSNVQIVRQQSYSIMSIIKEEVLAYVVQLPLYGVIDCPCWKLHTSPLCTTNTKEGSNICLTRTDRGWYCDNAGSVSFFPQAETCKVQSNRVFCDTMNSLTLPSEVNLCNIDIFNPKYDCKIMTSKTDVSSSVITSLGAIVSCYGKTKCTASNKNRGIIKTFSNGCDYVSNKGVDTVSVGNTLYYVNKQEGKSLYVKGEPIINFYDPLVFPSSEFDASISQVNEKINQSLAFIRKSDELLSAIGGYIPEAPRDGQAYVRKDGEWVLLSTFL

SEQ ID NO: 12 - protein, 544 aa, synthetic construct
MELLIHRSSAIFLTLAINALYLTSSQNITEEFYQSTCSAVSRGYFCALRTGWYHSVITIELSNIKETKCNGTDTKVKLIKQELDKYKNAVTELQLLMQNTPAANNRARREAPQYMNYTINTTKNLNVSISKKRKRRFLGFLLGVGSAIASGIAVSKVLHLEGEVNKIKNALLSTNKAVVSLSNGVSVLTSKVLDLKNYINNQLLPIVNQQSCRISNIETVIEFQQKNSRLLEITREFSVNAGVTTPLSTYMLTNSELLSLINDMPITNDQKKLMSSNVQIVRQQSYSIMSIIKEEVLAYVVQLPIYGVIDCPCWKLHTSPLCTTNIKEGSNICLTRTDRGWYCDNAGSVSFFPQADTCKVQSNRVFCDTMNSLTLPSEVSLCNTDIFNSKYDCKIMTSKTDISSSVITSLGAIVSCYGKTKCTASNKNRGIIKTFSNGCDYVSNKGVDTVSVGNTLYYVNKLEGKNLYVKGEPIINYYDPLVFPSSEFDASISQVNEKINQSLAFIRRSDELLSAIGGYIPEAPRDGQAYVRKDGEWVLLSTFL

SEQ ID NO: 13 - protein, 544 aa, synthetic construct
MELPILKTNAITTILAAVTLCFASSQNITEEFYQSTCSAVSKGYLSALRTGWYHSVITIELSNIKENKCNGTDAKVKLIKQELDKYKNAVTELQLLMQSTPCANSRARRELPRFMNYTLNNTKNTNVTLSKKRKRRFLGFLLGVGSACASGIAVSKVLHLEGEVNKIKSALLSTNKAVVSLSNGVSVLTIKVLDLKNYIDKQLLPIVNKQSCSISNIETVIEFQQKNNRLLEITREFSVNAGVTTPVSTYMLTNSELLSLINDMPITNDQKKLMSSNVQIVRQQSYSIMSIIKEEILAYVVQLPLYGVIDTPCWKLHTSPLCTTNTKEGSNICLTRTDRGWYCDNAGSVSFFPQAETCKVQSNRVFCDTMNSLTLPSEVNLCNIDIFNPKYDCKIMTSKTDVSSSVITSLGAIVSCYGKTKCTASNKNRGIIKTFSNGCDYVSNKGVDTVSVGNTLYYVNKQEGKSLYVKGEPIINFYDPLVFPSSEFDASISQVNEKINQSLAFIRKSDELLSAIGGYIPEAPRDGQAYVRKDGEWVLLSTFL

SEQ ID NO: 14 - protein, 544 aa, synthetic construct
MELLIHRSSAIFLTLAINALYLTSSQNITEEFYQSTCSAVSRGYFSALRTGWYHSVITIELSNIKETKCNGTDTKVKLIKQELDKYKNAVTELQLLMQNTPCANNRARREAPQYMNYTINTTKNLNVSISKKRKRRFLGFLLGVGSACASGIAVSKVLHLEGEVNKIKNALLSTNKAVVSLSNGVSVLTIKVLDLKNYINNQLLPIVNQQSCRISNIETVIEFQQKNSRLLEITREFSVNAGVTTPLSTYMLTNSELLSLINDMPITNDQKKLMSSNVQIVRQQSYSIMSIIKEEILAYVVQLPIYGVIDTPCWKLHTSPLCTTNIKEGSNICLTRTDRGWYCDNAGSVSFFPQADTCKVQSNRVFCDTMNSLTLPSEVSLCNTDIFNSKYDCKIMTSKTDISSSVITSLGAIVSCYGKTKCTASNKNRGIIKTFSNGCDYVSNKGVDTVSVGNTLYYVNKLEGKNLYVKGEPIINYYDPLVFPSSEFDASISQVNEKINQSLAFIRRSDELLSAIGGYIPEAPRDGQAYVRKDGEWVLLSTFL

SEQ ID NO: 15 - protein, 544 aa, synthetic construct
MELPILKTNAITTILAAVTLCFASSQNITEEFYQSTCSAVSKGYLSALRTGWYHSVITIELSNIKENKCNGTDAKVKLIKQELDKYKNAVTELQLLMQSTPCANSRARRELPRFMNYTLNNTKNTNVTLSKKRKRRFLGFLLGVGSAIASGCAVSKVLHLEGEVNKIKSALLSTNKAVVSLSNGVSVLTIKVLDLKNYIDKQLLPIVNKQSCSISNIETVIEFQQKNNRLLEITREFSVNAGVTTPVSTYMLTNSELLSLINDMPITNDQKKLMSSNVQIVRQQSYSIMSIIKEEILAYVVQLPLYGVIDTPCWKLHTSPLCTTNTKEGSNICLTRTDRGWYCDNAGSVSFFPQAETCKVQSNRVFCDTMNSLTLPSEVNLCNIDIFNPKYDCKIMTSKTDVSSSVITSLGAIVSCYGKTKCTASNKNRGIIKTFSNGCDYVSNKGVDTVSVGNTLYYVNKQEGKSLYVKGEPIINFYDPLVFPSSEFDASISQVNEKINQSLAFIRKSDELLSAIGGYIPEAPRDGQAYVRKDGEWVLLSTFL

SEQ ID NO: 16 - protein, 544 aa, synthetic construct
MELLIHRSSAIFLTLAINALYLTSSQNITEEFYQSTCSAVSRGYFSALRTGWYHSVITIELSNIKETKCNGTDTKVKLIKQELDKYKNAVTELQLLMQNTPCANNRARREAPQYMNYTINTTKNLNVSISKKRKRRFLGFLLGVGSAIASGCAVSKVLHLEGEVNKIKNALLSTNKAVVSLSNGVSVLTIKVLDLKNYINNQLLPIVNQQSCRISNIETVIEFQQKNSRLLEITREFSVNAGVTTPLSTYMLTNSELLSLINDMPITNDQKKLMSSNVQIVRQQSYSIMSIIKEEILAYVVQLPIYGVIDTPCWKLHTSPLCTTNIKEGSNICLTRTDRGWYCDNAGSVSFFPQADTCKVQSNRVFCDTMNSLTLPSEVSLCNTDIFNSKYDCKIMTSKTDISSSVITSLGAIVSCYGKTKCTASNKNRGIIKTFSNGCDYVSNKGVDTVSVGNTLYYVNKLEGKNLYVKGEPIINYYDPLVFPSSEFDASISQVNEKINQSLAFIRRSDELLSAIGGYIPEAPRDGQAYVRKDGEWVLLSTFL

SEQ ID NO: 17 - protein, 544 aa, synthetic construct
MELPILKTNAITTILAAVTLCFASSQNITEEFYQSTCSAVSKGYLSALRTGWYHSVITIELSNIKENKCNGTDAKVKLIKQELDKYKNAVTELQLLMQSTPAACSRARRELPRFMNYTLNNTKNTNVTLSKKRKRRFLGFLLGVCSAIASGIAVSKVLHLEGEVNKIKSALLSTNKAVVSLSNGVSVLTIKVLDLKNYIDKQLLPIVNKQSCSISNIETVIEFQQKNNRLLEITREFSVNAGVTTPVSTYMLTNSELLSLINDMPITNDQKKLMSSNVQIVRQQSYSIMSIIKEEILAYVVQLPLYGVIDTPCWKLHTSPLCTTNTKEGSNICLTRTDRGWYCDNAGSVSFFPQAETCKVQSNRVFCDTMNSLTLPSEVNLCNIDIFNPKYDCKIMTSKTDVSSSVITSLGAIVSCYGKTKCTASNKNRGIIKTFSNGCDYVSNKGVDTVSVGNTLYYVNKQEGKSLYVKGEPIINFYDPLVFPSSEFDASISQVNEKINQSLAFIRKSDELLSAIGGYIPEAPRDGQAYVRKDGEWVLLSTFL

SEQ ID NO: 18 - protein, 544 aa, synthetic construct
MELLIHRSSAIFLTLAINALYLTSSQNITEEFYQSTCSAVSRGYFSALRTGWYHSVITIELSNIKETKCNGTDTKVKLIKQELDKYKNAVTELQLLMQNTPAACNRARREAPQYMNYTINTTKNLNVSISKKRKRRFLGFLLGVCSAIASGIAVSKVLHLEGEVNKIKNALLSTNKAVVSLSNGVSVLTIKVLDLKNYINNQLLPIVNQQSCRISNIETVIEFQQKNSRLLEITREFSVNAGVTTPLSTYMLTNSELLSLINDMPITNDQKKLMSSNVQIVRQQSYSIMSIIKEEILAYVVQLPIYGVIDTPCWKLHTSPLCTTNIKEGSNICLTRTDRGWYCDNAGSVSFFPQADTCKVQSNRVFCDTMNSLTLPSEVSLCNTDIFNSKYDCKIMTSKTDISSSVITSLGAIVSCYGKTKCTASNKNRGIIKTFSNGCDYVSNKGVDTVSVGNTLYYVNKLEGKNLYVKGEPIINYYDPLVFPSSEFDASISQVNEKINQSLAFIRRSDELLSAIGGYIPEAPRDGQAYVRKDGEWVLLSTFL

SEQ ID NO: 19 - protein, 544 aa, synthetic construct
MELPILKTNAITTILAAVTLCFASSQNITEEFYQSTCSAVSKGYLSALRTGWYHSVITIELSNIKENKCNGTDAKVKLIKQELDKYKNAVTELQLLMQSTPAACSRARRELPRFMNYTLNNTKNTNVTLSKKRKRRFLGFLLGVGCAIASGIAVSKVLHLEGEVNKIKSALLSTNKAVVSLSNGVSVLTIKVLDLKNYIDKQLLPIVNKQSCSISNIETVIEFQQKNNRLLEITREFSVNAGVTTPVSTYMLTNSELLSLINDMPITNDQKKLMSSNVQIVRQQSYSIMSIIKEEILAYVVQLPLYGVIDTPCWKLHTSPLCTTNTKEGSNICLTRTDRGWYCDNAGSVSFFPQAETCKVQSNRVFCDTMNSLTLPSEVNLCNIDIFNPKYDCKIMTSKTDVSSSVITSLGAIVSCYGKTKCTASNKNRGIIKTFSNGCDYVSNKGVDTVSVGNTLYYVNKQEGKSLYVKGEPIINFYDPLVFPSSEFDASISQVNEKINQSLAFIRKSDELLSAIGGYIPEAPRDGQAYVRKDGEWVLLSTFL

SEQ ID NO: 20 - protein, 544 aa, synthetic construct
MELLIHRSSAIFLTLAINALYLTSSQNITEEFYQSTCSAVSRGYFSALRTGWYHSVITIELSNIKETKCNGTDTKVKLIKQELDKYKNAVTELQLLMQNTPAACNRARREAPQYMNYTINTTKNLNVSISKKRKRRFLGFLLGVGCAIASGIAVSKVLHLEGEVNKIKNALLSTNKAVVSLSNGVSVLTIKVLDLKNYINNQLLPIVNQQSCRISNIETVIEFQQKNSRLLEITREFSVNAGVTTPLSTYMLTNSELLSLINDMPITNDQKKLMSSNVQIVRQQSYSIMSIIKEEILAYVVQLPIYGVIDTPCWKLHTSPLCTTNIKEGSNICLTRTDRGWYCDNAGSVSFFPQADTCKVQSNRVFCDTMNSLTLPSEVSLCNTDIFNSKYDCKIMTSKTDISSSVITSLGAIVSCYGKTKCTASNKNRGIIKTFSNGCDYVSNKGVDTVSVGNTLYYVNKLEGKNLYVKGEPIINYYDPLVFPSSEFDASISQVNEKINQSLAFIRRSDELLSAIGGYIPEAPRDGQAYVRKDGEWVLLSTFL

SEQ ID NO: 21 - protein, 544 aa, synthetic construct
MELPILKTNAITTILAAVTLCFASSQNITEEFYQSTCSAVSKGYLSALRTGWYHSVITIELSNIKENKCNGTDAKVKLIKQELDKYKNAVTELQLLMQSTPAANCRARRELPRFMNYTLNNTKNTNVTLSKKRKRRFLGFLLGVGSCIASGIAVSKVLHLEGEVNKIKSALLSTNKAVVSLSNGVSVLTIKVLDLKNYIDKQLLPIVNKQSCSISNIETVIEFQQKNNRLLEITREFSVNAGVTTPVSTYMLTNSELLSLINDMPITNDQKKLMSSNVQIVRQQSYSIMSIIKEEILAYVVQLPLYGVIDTPCWKLHTSPLCTTNTKEGSNICLTRTDRGWYCDNAGSVSFFPQAETCKVQSNRVFCDTMNSLTLPSEVNLCNIDIFNPKYDCKIMTSKTDVSSSVITSLGAIVSCYGKTKCTASNKNRGIIKTFSNGCDYVSNKGVDTVSVGNTLYYVNKQEGKSLYVKGEPIINFYDPLVFPSSEFDASISQVNEKINQSLAFIRKSDELLSAIGGYIPEAPRDGQAYVRKDGEWVLLSTFL

SEQ ID NO: 22 - protein, 544 aa, synthetic construct
MELLIHRSSAIFLTLAINALYLTSSQNITEEFYQSTCSAVSRGYFSALRTGWYHSVITIELSNIKETKCNGTDTKVKLIKQELDKYKNAVTELQLLMQNTPAANCRARREAPQYMNYTINTTKNLNVSISKKRKRRFLGFLLGVGSCIASGIAVSKVLHLEGEVNKIKNALLSTNKAVVSLSNGVSVLTIKVLDLKNYINNQLLPIVNQQSCRISNIETVIEFQQKNSRLLEITREFSVNAGVTTPLSTYMLTNSELLSLINDMPITNDQKKLMSSNVQIVRQQSYSIMSIIKEEILAYVVQLPIYGVIDTPCWKLHTSPLCTTNIKEGSNICLTRTDRGWYCDNAGSVSFFPQADTCKVQSNRVFCDTMNSLTLPSEVSLCNTDIFNSKYDCKIMTSKTDISSSVITSLGAIVSCYGKTKCTASNKNRGIIKTFSNGCDYVSNKGVDTVSVGNTLYYVNKLEGKNLYVKGEPIINYYDPLVFPSSEFDASISQVNEKINQSLAFIRRSDELLSAIGGYIPEAPRDGQAYVRKDGEWVLLSTFL

SEQ ID NO: 23 - protein, 544 aa, synthetic construct
MELPILKTNAITTILAAVTLCFASSQNITEEFYQSTCSAVSKGYLSALRTGWYHSVITIELSNIKENKCNGTDAKVKLIKQELDKYKNAVTELQLLMQSTPAANCRARRELPRFMNYTLNNTKNTNVTLSKKRKRRFLGFLLGVCSAIASGIAVSKVLHLEGEVNKIKSALLSTNKAVVSLSNGVSVLTIKVLDLKNYIDKQLLPIVNKQSCSISNIETVIEFQQKNNRLLEITREFSVNAGVTTPVSTYMLTNSELLSLINDMPITNDQKKLMSSNVQIVRQQSYSIMSIIKEEILAYVVQLPLYGVIDTPCWKLHTSPLCTTNTKEGSNICLTRTDRGWYCDNAGSVSFFPQAETCKVQSNRVFCDTMNSLTLPSEVNLCNIDIFNPKYDCKIMTSKTDVSSSVITSLGAIVSCYGKTKCTASNKNRGIIKTFSNGCDYVSNKGVDTVSVGNTLYYVNKQEGKSLYVKGEPIINFYDPLVFPSSEFDASISQVNEKINQSLAFIRKSDELLSAIGGYIPEAPRDGQAYVRKDGEWVLLSTFL

SEQ ID NO: 24 - protein, 544 aa, synthetic construct
MELLIHRSSAIFLTLAINALYLTSSQNITEEFYQSTCSAVSRGYFSALRTGWYHSVITIELSNIKETKCNGTDTKVKLIKQELDKYKNAVTELQLLMQNTPAANCRARREAPQYMNYTINTTKNLNVSISKKRKRRFLGFLLGVCSAIASGIAVSKVLHLEGEVNKIKNALLSTNKAVVSLSNGVSVLTIKVLDLKNYINNQLLPIVNQQSCRISNIETVIEFQQKNSRLLEITREFSVNAGVTTPLSTYMLTNSELLSLINDMPITNDQKKLMSSNVQIVRQQSYSIMSIIKEEILAYVVQLPIYGVIDTPCWKLHTSPLCTTNIKEGSNICLTRTDRGWYCDNAGSVSFFPQADTCKVQSNRVFCDTMNSLTLPSEVSLCNTDIFNSKYDCKIMTSKTDISSSVITSLGAIVSCYGKTKCTASNKNRGIIKTFSNGCDYVSNKGVDTVSVGNTLYYVNKLEGKNLYVKGEPIINYYDPLVFPSSEFDASISQVNEKINQSLAFIRRSDELLSAIGGYIPEAPRDGQAYVRKDGEWVLLSTFL

SEQ ID NO: 25 - protein, 544 aa, synthetic construct
MELPILKTNAITTILAAVTLCFASSQNITEEFYQSTCSAVSKGYLSALRTGWYHSVITIELSNIKENKCNGTDAKVKLIKQELDKYKNAVTELQLLMQSTPAANCRARRELPRFMNYTLNNTKNTNVTLSKKRKRRFLGFLLGVGCAIASGIAVSKVLHLEGEVNKIKSALLSTNKAVVSLSNGVSVLTIKVLDLKNYIDKQLLPIVNKQSCSISNIETVIEFQQKNNRLLEITREFSVNAGVTTPVSTYMLTNSELLSLINDMPITNDQKKLMSSNVQIVRQQSYSIMSIIKEEILAYVVQLPLYGVIDTPCWKLHTSPLCTTNTKEGSNICLTRTDRGWYCDNAGSVSFFPQAETCKVQSNRVFCDTMNSLTLPSEVNLCNIDIFNPKYDCKIMTSKTDVSSSVITSLGAIVSCYGKTKCTASNKNRGIIKTFSNGCDYVSNKGVDTVSVGNTLYYVNKQEGKSLYVKGEPIINFYDPLVFPSSEFDASISQVNEKINQSLAFIRKSDELLSAIGGYIPEAPRDGQAYVRKDGEWVLLSTFL

SEQ ID NO: 26 - protein, 544 aa, synthetic construct
MELLIHRSSAIFLTLAINALYLTSSQNITEEFYQSTCSAVSRGYFSALRTGWYHSVITIELSNIKETKCNGTDTKVKLIKQELDKYKNAVTELQLLMQNTPAANCRARREAPQYMNYTINTTKNLNVSISKKRKRRFLGFLLGVGCAIASGIAVSKVLHLEGEVNKIKNALLSTNKAVVSLSNGVSVLTIKVLDLKNYINNQLLPIVNQQSCRISNIETVIEFQQKNSRLLEITREFSVNAGVTTPLSTYMLTNSELLSLINDMPITNDQKKLMSSNVQIVRQQSYSIMSIIKEEILAYVVQLPIYGVIDTPCWKLHTSPLCTTNIKEGSNICLTRTDRGWYCDNAGSVSFFPQADTCKVQSNRVFCDTMNSLTLPSEVSLCNTDIFNSKYDCKIMTSKTDISSSVITSLGAIVSCYGKTKCTASNKNRGIIKTFSNGCDYVSNKGVDTVSVGNTLYYVNKLEGKNLYVKGEPIINYYDPLVFPSSEFDASISQVNEKINQSLAFIRRSDELLSAIGGYIPEAPRDGQAYVRKDGEWVLLSTFL

SEQ ID NO: 27 - protein, 544 aa, synthetic construct
MELPILKTNAITTILAAVTLCFASSQNITEEFYQSTCSAVSKGYLSALRTGWYHSVITIELSNIKENKCNGTDAKVKLIKQELDKYKNAVTELQLLMQSTCAANSRARRELPRFMNYTLNNTKNTNVTLSKKRKRRFLGFLLGVGSAIASGCAVSKVLHLEGEVNKIKSALLSTNKAVVSLSNGVSVLTIKVLDLKNYIDKQLLPIVNKQSCSISNIETVIEFQQKNNRLLEITREFSVNAGVTTPVSTYMLTNSELLSLINDMPITNDQKKLMSSNVQIVRQQSYSIMSIIKEEILAYVVQLPLYGVIDTPCWKLHTSPLCTTNTKEGSNICLTRTDRGWYCDNAGSVSFFPQAETCKVQSNRVFCDTMNSLTLPSEVNLCNIDIFNPKYDCKIMTSKTDVSSSVITSLGAIVSCYGKTKCTASNKNRGIIKTFSNGCDYVSNKGVDTVSVGNTLYYVNKQEGKSLYVKGEPIINFYDPLVFPSSEFDASISQVNEKINQSLAFIRKSDELLSAIGGYIPEAPRDGQAYVRKDGEWVLLSTFL

SEQ ID NO: 28 - protein, 544 aa, synthetic construct
MELLIHRSSAIFLTLAINALYLTSSQNITEEFYQSTCSAVSRGYFSALRTGWYHSVITIELSNIKETKCNGTDTKVKLIKQELDKYKNAVTELQLLMQNTCAANNRARREAPQYMNYTINTTKNLNVSISKKRKRRFLGFLLGVGSAIASGCAVSKVLHLEGEVNKIKNALLSTNKAVVSLSNGVSVLTIKVLDLKNYINNQLLPIVNQQSCRISNIETVIEFQQKNSRLLEITREFSVNAGVTTPLSTYMLTNSELLSLINDMPITNDQKKLMSSNVQIVRQQSYSIMSIIKEEILAYVVQLPIYGVIDTPCWKLHTSPLCTTNIKEGSNICLTRTDRGWYCDNAGSVSFFPQADTCKVQSNRVFCDTMNSLTLPSEVSLCNTDIFNSKYDCKIMTSKTDISSSVITSLGAIVSCYGKTKCTASNKNRGIIKTFSNGCDYVSNKGVDTVSVGNTLYYVNKLEGKNLYVKGEPIINYYDPLVFPSSEFDASISQVNEKINQSLAFIRRSDELLSAIGGYIPEAPRDGQAYVRKDGEWVLLSTFL

SEQ ID NO: 29 - protein, 544 aa, synthetic construct
MELPILKTNAITTILAAVTLCFASSQNITEEFYQSTCSAVSKGYLSALRTGWYHSVITIELSNIKENKCNGTDAKVKLIKQELDKYKNAVTELQLLMQSTPACNSRARRELPRFMNYTLNNTKNTNVTLSKKRKRRFLGFLLGVGCAIASGIAVSKVLHLEGEVNKIKSALLSTNKAVVSLSNGVSVLTIKVLDLKNYIDKQLLPIVNKQSCSISNIETVIEFQQKNNRLLEITREFSVNAGVTTPVSTYMLTNSELLSLINDMPITNDQKKLMSSNVQIVRQQSYSIMSIIKEEILAYVVQLPLYGVIDTPCWKLHTSPLCTTNTKEGSNICLTRTDRGWYCDNAGSVSFFPQAETCKVQSNRVFCDTMNSLTLPSEVNLCNIDIFNPKYDCKIMTSKTDVSSSVITSLGAIVSCYGKTKCTASNKNRGIIKTFSNGCDYVSNKGVDTVSVGNTLYYVNKQEGKSLYVKGEPIINFYDPLVFPSSEFDASISQVNEKINQSLAFIRKSDELLSAIGGYIPEAPRDGQAYVRKDGEWVLLSTFL

SEQ ID NO: 30 - protein, 544 aa, synthetic construct
MELLIHRSSAIFLTLAINALYLTSSQNITEEFYQSTCSAVSRGYFSALRTGWYHSVITIELSNIKETKCNGTDTKVKLIKQELDKYKNAVTELQLLMQNTPACNNRARREAPQYMNYTINTTKNLNVSISKKRKRRFLGFLLGVGCAIASGIAVSKVLHLEGEVNKIKNALLSTNKAVVSLSNGVSVLTIKVLDLKNYINNQLLPIVNQQSCRISNIETVIEFQQKNSRLLEITREFSVNAGVTTPLSTYMLTNSELLSLINDMPITNDQKKLMSSNVQIVRQQSYSIMSIIKEEILAYVVQLPIYGVIDTPCWKLHTSPLCTTNIKEGSNICLTRTDRGWYCDNAGSVSFFPQADTCKVQSNRVFCDTMNSLTLPSEVSLCNTDIFNSKYDCKIMTSKTDISSSVITSLGAIVSCYGKTKCTASNKNRGIIKTFSNGCDYVSNKGVDTVSVGNTLYYVNKLEGKNLYVKGEPIINYYDPLVFPSSEFDASISQVNEKINQSLAFIRRSDELLSAIGGYIPEAPRDGQAYVRKDGEWVLLSTFL

SEQ ID NO: 31 - protein, 544 aa, synthetic construct
MELPILKTNAITTILAAVTLCFASSQNITEEFYQSTCSAVSKGYLSALRTGWYTSVITIELSNIKINKCNGTDAKVKLIKQELDKYKNAVTELQLLMQSTPAANSRARRELPRFMNYTLNNTKNTNVTLSKKRKRRFLGFLLGVGSAIASGIAVSKVLHLEGEVNKIKSALLSTNKAVVSLSNGVSVLTSKVLDLKNYIDKQLLPIVNKQSCSISPIETVIEFQQKNNRLLEITREFSVNAGVTTPVSTYMLTNSELLSLINDMPITNDQKKLMSSNVQIVRQQSYSIMSIIKEEVLAYVVQLPLYGVIDTPCWKLHTSPLCTTNTKEGSNICLTRTDRGWYCDNAGSVSFFPQAETCKVQSNRVFCDTMNSLTLPSEVNLCNIDIFNPKYDCKIMTSKTDVSSSVITSLGAIVSCYGKTKCTASNKNRGIIKTFSNGCDYVSNKGVDTVSVGNTLYYVNKQEGKSLYVKGEPIINFYDPLVFPSQEFDASISQVNEKINQSLAFIRKSDELLSAIGGYIPEAPRDGQAYVRKDGEWVLLSTFL

SEQ ID NO: 32 - protein, 544 aa, synthetic construct
MELLIHRSSAIFLTLAINALYLTSSQNITEEFYQSTCSAVSRGYFSALRTGWYTSVITIELSNIKITKCNGTDTKVKLIKQELDKYKNAVTELQLLMQNTPAANNRARREAPQYMNYTINTTKNLNVSISKKRKRRFLGFLLGVGSAIASGIAVSKVLHLEGEVNKIKNALLSTNKAVVSLSNGVSVLTSKVLDLKNYINNQLLPIVNQQSCRISPIETVIEFQQKNSRLLEITREFSVNAGVTTPLSTYMLTNSELLSLINDMPITNDQKKLMSSNVQIVRQQSYSIMSIIKEEVLAYVVQLPIYGVIDTPCWKLHTSPLCTTNIKEGSNICLTRTDRGWYCDNAGSVSFFPQADTCKVQSNRVFCDTMNSLTLPSEVSLCNTDIFNSKYDCKIMTSKTDISSSVITSLGAIVSCYGKTKCTASNKNRGIIKTFSNGCDYVSNKGVDTVSVGNTLYYVNKLEGKNLYVKGEPIINYYDPLVFPSQEFDASISQVNEKINQSLAFIRRSDELLSAIGGYIPEAPRDGQAYVRKDGEWVLLSTFL

SEQ ID NO: 33 - protein, 544 aa, synthetic construct
MELPILKTNAITTILAAVTLCFASSQNITEEFYQSTCSAVSKGYLSALRTGWYTSVITIELSNIKINKCNGTDAKVKLIKQELDKYKNAVTELQLLMQSTPAANSRARRELPRFMNYTLNNTKNTNVTLSKKRKRRFLGFLLGVGSAIASGIAVSKVLHLEGEVNKIKSALLSTNKAVVSLSNGVSVLTSKVLDLKNYIDKQLLPIVNKQSCSISPIETVIEFQQKNNRLLEITREFSVNAGVTTPVSTYMLTNSELLSLINDMPITNDQKKLMSSNVQIVRQQSYSIMSIIKEEVLAYVVQLPLYGVIDTPCWKLHTSPLCTTNTKEGSNICLTRTDRGWYCDNAGSVSFFPQAETCKVQSNRVFCDTMNSLTLPSEVNLCNIDIFNPKYDCKIMTSKTDVSSSVITSLGAIVSCYGKTKCTASNKNRGIIKTFSNGCDYVSNKGVDTVSVGNTLYYVNKQEGKSLYVKGEPIINFYDPLVFPSDTFDASISQVNEKINQSLAFIRKSDELLSAIGGYIPEAPRDGQAYVRKDGEWVLLSTFL

SEQ ID NO: 34 - protein, 544 aa, synthetic construct
MELLIHRSSAIFLTLAINALYLTSSQNITEEFYQSTCSAVSRGYFSALRTGWYTSVITIELSNIKITKCNGTDTKVKLIKQELDKYKNAVTELQLLMQNTPAANNRARREAPQYMNYTINTTKNLNVSISKKRKRRFLGFLLGVGSAIASGIAVSKVLHLEGEVNKIKNALLSTNKAVVSLSNGVSVLTSKVLDLKNYINNQLLPIVNQQSCRISPIETVIEFQQKNSRLLEITREFSVNAGVTTPLSTYMLTNSELLSLINDMPITNDQKKLMSSNVQIVRQQSYSIMSIIKEEVLAYVVQLPIYGVIDTPCWKLHTSPLCTTNIKEGSNICLTRTDRGWYCDNAGSVSFFPQADTCKVQSNRVFCDTMNSLTLPSEVSLCNTDIFNSKYDCKIMTSKTDISSSVITSLGAIVSCYGKTKCTASNKNRGIIKTFSNGCDYVSNKGVDTVSVGNTLYYVNKLEGKNLYVKGEPIINYYDPLVFPSDTFDASISQVNEKINQSLAFIRRSDELLSAIGGYIPEAPRDGQAYVRKDGEWVLLSTFL

SEQ ID NO: 35 - protein, 544 aa, synthetic construct
MELPILKTNAITTILAAVTLCFASSQNITEEFYQSTCSAVSKGYLSALRTGWYTSVITIELSNIKEIKCNGTDAKVKLIKQELDKYKNAVTELQLLMQSTPAANSRARRELPRFMNYTLNNTKNTNVTLSKKRKRRFLGFLLGVGSAIASGIAVSKVLHLEGEVNKIKSALLSTNKAVVSLSNGVSVLTSKVLDLKNYIDKQLLPIVNKQSCSISPIETVIEFQQKNNRLLEITREFSVNAGVTTPVSTYMLTNSELLSLINDMPITNDQKKLMSSNVQIVRQQSYSIMSIIKEEVLAYVVQLPLYGVIDTPCWKLHTSPLCTTNTKEGSNICLTRTDRGWYCDNAGSVSFFPQAETCKVQSNRVFCDTMNSLTLPSEVNLCNIDIFNPKYDCKIMTSKTDVSSSVITSLGAIVSCYGKTKCTASNKNRGIIKTFSNGCDYVSNKGVDTVSVGNTLYYVNKQEGKSLYVKGEPIINFYDPLVFPSDQFDASISQVNEKINQSLAFIRKSDELLSAIGGYIPEAPRDGQAYVRKDGEWVLLSTFL

SEQ ID NO: 36 - protein, 544 aa, synthetic construct
MELLIHRSSAIFLTLAINALYLTSSQNITEEFYQSTCSAVSRGYFSALRTGWYTSVITIELSNIKEIKCNGTDTKVKLIKQELDKYKNAVTELQLLMQNTPAANNRARREAPQYMNYTINTTKNLNVSISKKRKRRFLGFLLGVGSAIASGIAVSKVLHLEGEVNKIKNALLSTNKAVVSLSNGVSVLTSKVLDLKNYINNQLLPIVNQQSCRISPIETVIEFQQKNSRLLEITREFSVNAGVTTPLSTYMLTNSELLSLINDMPITNDQKKLMSSNVQIVRQQSYSIMSIIKEEVLAYVVQLPIYGVIDTPCWKLHTSPLCTTNIKEGSNICLTRTDRGWYCDNAGSVSFFPQADTCKVQSNRVFCDTMNSLTLPSEVSLCNTDIFNSKYDCKIMTSKTDISSSVITSLGAIVSCYGKTKCTASNKNRGIIKTFSNGCDYVSNKGVDTVSVGNTLYYVNKLEGKNLYVKGEPIINYYDPLVFPSDQFDASISQVNEKINQSLAFIRRSDELLSAIGGYIPEAPRDGQAYVRKDGEWVLLSTFL

SEQ ID NO: 37 - protein, 544 aa, synthetic construct
MELPILKTNAITTILAAVTLCFASSQNITEEFYQSTCSAVSKGYLSALRTGWYTSVITIELSNIKINKCNGTDAKVKLIKQELDKYKNAVTELQLLMQSTPAANSRARRELPRFMNYTLNNTKNTNVTLSKKRKRRFLGFLLGVGSAIASGIAVSKVLHLEGEVNKIKSALLSTNKAVVSLSNGVSVLTSKVLDLKNYIDKQLLPIVNKQSCPISNIETVIEFQQKNNRLLEITREFSVNAGVTTPVSTYMLTNSELLSLINDMPITNDQKKLMSSNVQIVRQQSYSIMSIIKEEVLAYVVQLPLYGVIDTPCWKLHTSPLCTTNTKEGSNICLTRTDRGWYCDNAGSVSFFPQAETCKVQSNRVFCDTMNSLTLPSEVNLCNIDIFNPKYDCKIMTSKTDVSSSVITSLGAIVSCYGKTKCTASNKNRGIIKTFSNGCDYVSNKGVDTVSVGNTLYYVNKQEGKSLYVKGEPIINFYDPLVFPSQEFDASISQVNEKINQSLAFIRKSDELLSAIGGYIPEAPRDGQAYVRKDGEWVLLSTFL

SEQ ID NO: 38 - protein, 544 aa, synthetic construct
MELLIHRSSAIFLTLAINALYLTSSQNITEEFYQSTCSAVSRGYFSALRTGWYTSVITIELSNIKITKCNGTDTKVKLIKQELDKYKNAVTELQLLMQNTPAANNRARREAPQYMNYTINTTKNLNVSISKKRKRRFLGFLLGVGSAIASGIAVSKVLHLEGEVNKIKNALLSTNKAVVSLSNGVSVLTSKVLDLKNYINNQLLPIVNQQSCPISNIETVIEFQQKNSRLLEITREFSVNAGVTTPLSTYMLTNSELLSLINDMPITNDQKKLMSSNVQIVRQQSYSIMSIIKEEVLAYVVQLPIYGVIDTPCWKLHTSPLCTTNIKEGSNICLTRTDRGWYCDNAGSVSFFPQADTCKVQSNRVFCDTMNSLTLPSEVSLCNTDIFNSKYDCKIMTSKTDISSSVITSLGAIVSCYGKTKCTASNKNRGIIKTFSNGCDYVSNKGVDTVSVGNTLYYVNKLEGKNLYVKGEPIINYYDPLVFPSQEFDASISQVNEKINQSLAFIRRSDELLSAIGGYIPEAPRDGQAYVRKDGEWVLLSTFL

SEQ ID NO: 39 - protein, 544 aa, synthetic construct
MELPILKTNAITTILAAVTLCFASSQNITEEFYQSTCSAVSKGYLSALRTGWYTSVITIELSNIKINKCNGTDAKVKLIKQELDKYKNAVTELQLLMQSTPAANSRARRELPRFMNYTLNNTKNTNVTLSKKRKRRFLGFLLGVGSAIASGIAVSKVLHLEGEVNKIKSALLSTNKAVVSLSNGVSVLTSKVLDLKNYIDKQLLPIVNKQSCPISNIETVIEFQQKNNRLLEITREFSVNAGVTTPVSTYMLTNSELLSLINDMPITNDQKKLMSSNVQIVRQQSYSIMSIIKEEVLAYVVQLPLYGVIDTPCWKLHTSPLCTTNTKEGSNICLTRTDRGWYCDNAGSVSFFPQAETCKVQSNRVFCDTMNSLTLPSEVNLCNIDIFNPKYDCKIMTSKTDVSSSVITSLGAIVSCYGKTKCTASNKNRGIIKTFSNGCDYVSNKGVDTVSVGNTLYYVNKQEGKSLYVKGEPIINFYDPLVFPSDTFDASISQVNEKINQSLAFIRKSDELLSAIGGYIPEAPRDGQAYVRKDGEWVLLSTFL

SEQ ID NO: 40 - protein, 544 aa, synthetic construct
MELLIHRSSAIFLTLAINALYLTSSQNITEEFYQSTCSAVSRGYFSALRTGWYTSVITIELSNIKITKCNGTDTKVKLIKQELDKYKNAVTELQLLMQNTPAANNRARREAPQYMNYTINTTKNLNVSISKKRKRRFLGFLLGVGSAIASGIAVSKVLHLEGEVNKIKNALLSTNKAVVSLSNGVSVLTSKVLDLKNYINNQLLPIVNQQSCPISNIETVIEFQQKNSRLLEITREFSVNAGVTTPLSTYMLTNSELLSLINDMPITNDQKKLMSSNVQIVRQQSYSIMSIIKEEVLAYVVQLPIYGVIDTPCWKLHTSPLCTTNIKEGSNICLTRTDRGWYCDNAGSVSFFPQADTCKVQSNRVFCDTMNSLTLPSEVSLCNTDIFNSKYDCKIMTSKTDISSSVITSLGAIVSCYGKTKCTASNKNRGIIKTFSNGCDYVSNKGVDTVSVGNTLYYVNKLEGKNLYVKGEPIINYYDPLVFPSDTFDASISQVNEKINQSLAFIRRSDELLSAIGGYIPEAPRDGQAYVRKDGEWVLLSTFL

SEQ ID NO: 41 - protein, 544 aa, synthetic construct
MELPILKTNAITTILAAVTLCFASSQNITEEFYQSTCSAVSKGYLSALRTGWYTSVITIELSNIKEIKCNGTDAKVKLIKQELDKYKNAVTELQLLMQSTPAANSRARRELPRFMNYTLNNTKNTNVTLSKKRKRRFLGFLLGVGSAIASGIAVSKVLHLEGEVNKIKSALLSTNKAVVSLSNGVSVLTSKVLDLKNYIDKQLLPIVNKQSCPISNIETVIEFQQKNNRLLEITREFSVNAGVTTPVSTYMLTNSELLSLINDMPITNDQKKLMSSNVQIVRQQSYSIMSIIKEEVLAYVVQLPLYGVIDTPCWKLHTSPLCTTNTKEGSNICLTRTDRGWYCDNAGSVSFFPQAETCKVQSNRVFCDTMNSLTLPSEVNLCNIDIFNPKYDCKIMTSKTDVSSSVITSLGAIVSCYGKTKCTASNKNRGIIKTFSNGCDYVSNKGVDTVSVGNTLYYVNKQEGKSLYVKGEPIINFYDPLVFPSDQFDASISQVNEKINQSLAFIRKSDELLSAIGGYIPEAPRDGQAYVRKDGEWVLLSTFL

SEQ ID NO: 42 - protein, 544 aa, synthetic construct
MELLIHRSSAIFLTLAINALYLTSSQNITEEFYQSTCSAVSRGYFSALRTGWYTSVITIELSNIKEIKCNGTDTKVKLIKQELDKYKNAVTELQLLMQNTPAANNRARREAPQYMNYTINTTKNLNVSISKKRKRRFLGFLLGVGSAIASGIAVSKVLHLEGEVNKIKNALLSTNKAVVSLSNGVSVLTSKVLDLKNYINNQLLPIVNQQSCPISNIETVIEFQQKNSRLLEITREFSVNAGVTTPLSTYMLTNSELLSLINDMPITNDQKKLMSSNVQIVRQQSYSIMSIIKEEVLAYVVQLPIYGVIDTPCWKLHTSPLCTTNIKEGSNICLTRTDRGWYCDNAGSVSFFPQADTCKVQSNRVFCDTMNSLTLPSEVSLCNTDIFNSKYDCKIMTSKTDISSSVITSLGAIVSCYGKTKCTASNKNRGIIKTFSNGCDYVSNKGVDTVSVGNTLYYVNKLEGKNLYVKGEPIINYYDPLVFPSDQFDASISQVNEKINQSLAFIRRSDELLSAIGGYIPEAPRDGQAYVRKDGEWVLLSTFL

SEQ ID NO: 43 - protein, 544 aa, synthetic construct
MELPILKTNAITTILAAVTLCFASSQNITEEFYQSTCSAVSKGYLSALRTGWYTSVITIELSNIKEIKCNGTDAKVKLIKQELDKYKNAVTELQLLMQSTPAANSRARRELPRFMNYTLNNTKNTNVTLSKKRKRRFLGFLLGVGSAIASGIAVSKVLHLEGEVNKIKSALLSTNKAVVSLSNGVSVLTSKVLDLKNYIDKQLLPIVNKQSCSIPNIETVIEFQQKNNRLLEITREFSVNAGVTTPVSTYMLTNSELLSLINDMPITNDQKKLMSSNVQIVRQQSYSIMSIIKEEVLAYVVQLPLYGVIDTPCWKLHTSPLCTTNTKEGSNICLTRTDRGWYCDNAGSVSFFPQAETCKVQSNRVFCDTMNSLTLPSEVNLCNIDIFNPKYDCKIMTSKTDVSSSVITSLGAIVSCYGKTKCTASNKNRGIIKTFSNGCDYVSNKGVDTVSVGNTLYYVNKQEGKSLYVKGEPIINFYDPLVFPSDQFDASISQVNEKINQSLAFIRKSDELLSAIGGYIPEAPRDGQAYVRKDGEWVLLSTFL

SEQ ID NO: 44 - protein, 544 aa, synthetic construct
MELLIHRSSAIFLTLAINALYLTSSQNITEEFYQSTCSAVSRGYFSALRTGWYTSVITIELSNIKEIKCNGTDTKVKLIKQELDKYKNAVTELQLLMQNTPAANNRARREAPQYMNYTINTTKNLNVSISKKRKRRFLGFLLGVGSAIASGIAVSKVLHLEGEVNKIKNALLSTNKAVVSLSNGVSVLTSKVLDLKNYINNQLLPIVNQQSCRIPNIETVIEFQQKNSRLLEITREFSVNAGVTTPLSTYMLTNSELLSLINDMPITNDQKKLMSSNVQIVRQQSYSIMSIIKEEVLAYVVQLPIYGVIDTPCWKLHTSPLCTTNIKEGSNICLTRTDRGWYCDNAGSVSFFPQADTCKVQSNRVFCDTMNSLTLPSEVSLCNTDIFNSKYDCKIMTSKTDISSSVITSLGAIVSCYGKTKCTASNKNRGIIKTFSNGCDYVSNKGVDTVSVGNTLYYVNKLEGKNLYVKGEPIINYYDPLVFPSDQFDASISQVNEKINQSLAFIRRSDELLSAIGGYIPEAPRDGQAYVRKDGEWVLLSTFL

SEQ ID NO: 45 - protein, 544 aa, synthetic construct
MELPILKTNAITTILAAVTLCFASSQNITEEFYQSTCSAVSKGYLSALRTGWYTSVITIELSNIKINKCNGTDAKVKLIKQELDKYKNAVTELQLLMQSTPAANSRARRELPRFMNYTLNNTKNTNVTLSKKRKRRFLGFLLGVGSAIASGIAVSKVLHLEGEVNKIKSALLSTNKAVVSLSNGVSVLTSKVLDLKNYIDKQLLPIVNKQSCSISNPETVIEFQQKNNRLLEITREFSVNAGVTTPVSTYMLTNSELLSLINDMPITNDQKKLMSSNVQIVRQQSYSIMSIIKEEVLAYVVQLPLYGVIDTPCWKLHTSPLCTTNTKEGSNICLTRTDRGWYCDNAGSVSFFPQAETCKVQSNRVFCDTMNSLTLPSEVNLCNIDIFNPKYDCKIMTSKTDVSSSVITSLGAIVSCYGKTKCTASNKNRGIIKTFSNGCDYVSNKGVDTVSVGNTLYYVNKQEGKSLYVKGEPIINFYDPLVFPSDTFDASISQVNEKINQSLAFIRKSDELLSAIGGYIPEAPRDGQAYVRKDGEWVLLSTFL

SEQ ID NO: 46 - protein, 544 aa, synthetic construct
MELLIHRSSAIFLTLAINALYLTSSQNITEEFYQSTCSAVSRGYFSALRTGWYTSVITIELSNIKITKCNGTDTKVKLIKQELDKYKNAVTELQLLMQNTPAANNRARREAPQYMNYTINTTKNLNVSISKKRKRRFLGFLLGVGSAIASGIAVSKVLHLEGEVNKIKNALLSTNKAVVSLSNGVSVLTSKVLDLKNYINNQLLPIVNQQSCRISNPETVIEFQQKNSRLLEITREFSVNAGVTTPLSTYMLTNSELLSLINDMPITNDQKKLMSSNVQIVRQQSYSIMSIIKEEVLAYVVQLPIYGVIDTPCWKLHTSPLCTTNIKEGSNICLTRTDRGWYCDNAGSVSFFPQADTCKVQSNRVFCDTMNSLTLPSEVSLCNTDIFNSKYDCKIMTSKTDISSSVITSLGAIVSCYGKTKCTASNKNRGIIKTFSNGCDYVSNKGVDTVSVGNTLYYVNKLEGKNLYVKGEPIINYYDPLVFPSDTFDASISQVNEKINQSLAFIRRSDELLSAIGGYIPEAPRDGQAYVRKDGEWVLLSTFL

SEQ ID NO: 47 - protein, 544 aa, synthetic construct
MELPILKTNAITTILAAVTLCFASSQNITEEFYQSTCSAVSKGYLSALRTGWYTSVITIELSNIKEIKCNGTDAKVKLIKQELDKYKNAVTELQLLMQSTPAANSRARRELPRFMNYTLNNTKNTNVTLSKKRKRRFLGFLLGVGSAIASGIAVSKVLHLEGEVNKIKSALLSTNKAVVSLSNGVSVLTSKVLDLKNYIDKQLLPIVNKQSCSISNPETVIEFQQKNNRLLEITREFSVNAGVTTPVSTYMLTNSELLSLINDMPITNDQKKLMSSNVQIVRQQSYSIMSIIKEEVLAYVVQLPLYGVIDTPCWKLHTSPLCTTNTKEGSNICLTRTDRGWYCDNAGSVSFFPQAETCKVQSNRVFCDTMNSLTLPSEVNLCNIDIFNPKYDCKIMTSKTDVSSSVITSLGAIVSCYGKTKCTASNKNRGIIKTFSNGCDYVSNKGVDTVSVGNTLYYVNKQEGKSLYVKGEPIINFYDPLVFPSDQFDASISQVNEKINQSLAFIRKSDELLSAIGGYIPEAPRDGQAYVRKDGEWVLLSTFL

SEQ ID NO: 48 - protein, 544 aa, synthetic construct
MELLIHRSSAIFLTLAINALYLTSSQNITEEFYQSTCSAVSRGYFSALRTGWYTSVITIELSNIKEIKCNGTDTKVKLIKQELDKYKNAVTELQLLMQNTPAANNRARREAPQYMNYTINTTKNLNVSISKKRKRRFLGFLLGVGSAIASGIAVSKVLHLEGEVNKIKNALLSTNKAVVSLSNGVSVLTSKVLDLKNYINNQLLPIVNQQSCRISNPETVIEFQQKNSRLLEITREFSVNAGVTTPLSTYMLTNSELLSLINDMPITNDQKKLMSSNVQIVRQQSYSIMSIIKEEVLAYVVQLPIYGVIDTPCWKLHTSPLCTTNIKEGSNICLTRTDRGWYCDNAGSVSFFPQADTCKVQSNRVFCDTMNSLTLPSEVSLCNTDIFNSKYDCKIMTSKTDISSSVITSLGAIVSCYGKTKCTASNKNRGIIKTFSNGCDYVSNKGVDTVSVGNTLYYVNKLEGKNLYVKGEPIINYYDPLVFPSDQFDASISQVNEKINQSLAFIRRSDELLSAIGGYIPEAPRDGQAYVRKDGEWVLLSTFL

SEQ ID NO: 49 - protein, 544 aa, synthetic construct
MELPILKTNAITTILAAVTLCFASSQNITEEFYQSTCSAVSKGYLSALRTGWYTSVITIELSNIKINKCNGTDAKVKLIKQELDKYKNAVTELQLLMQSTPAANSRARRELPRFMNYTLNNTKNTNVTLSKKRKRRFLGFLLGVGSAIASGIAVSKVLHLEGEVNKIKSALLSTNKAVVSLSNGVSVLTSKVLDLKNYIDKQLLPIVNKQSCSISNPETVIEFQQKNNRLLEITREFSVNAGVTTPVSTYMLTNSELLSLINDMPITNDQKKLMSSNVQIVRQQSYSIMSIIKEEVLAYVVQLPLYGVIDTPCWKLHTSPLCTTNTKEGSNICLTRTDRGWYCDNAGSVSFFPQAETCKVQSNRVFCDTMNSLTLPSEVNLCNIDIFNPKYDCKIMTSKTDVSSSVITSLGAIVSCYGKTKCTASNKNRGIIKTFSNGCDYVSNKGVDTVSVGNTLYYVNKQEGKSLYVKGEPIINFYDPLVFPSQEFDASISQVNEKINQSLAFIRKSDELLSAIGGYIPEAPRDGQAYVRKDGEWVLLSTFL

SEQ ID NO: 50 - protein, 544 aa, synthetic construct
MELLIHRSSAIFLTLAINALYLTSSQNITEEFYQSTCSAVSRGYFSALRTGWYTSVITIELSNIKITKCNGTDTKVKLIKQELDKYKNAVTELQLLMQNTPAANNRARREAPQYMNYTINTTKNLNVSISKKRKRRFLGFLLGVGSAIASGIAVSKVLHLEGEVNKIKNALLSTNKAVVSLSNGVSVLTSKVLDLKNYINNQLLPIVNQQSCRISNPETVIEFQQKNSRLLEITREFSVNAGVTTPLSTYMLTNSELLSLINDMPITNDQKKLMSSNVQIVRQQSYSIMSIIKEEVLAYVVQLPIYGVIDTPCWKLHTSPLCTTNIKEGSNICLTRTDRGWYCDNAGSVSFFPQADTCKVQSNRVFCDTMNSLTLPSEVSLCNTDIFNSKYDCKIMTSKTDISSSVITSLGAIVSCYGKTKCTASNKNRGIIKTFSNGCDYVSNKGVDTVSVGNTLYYVNKLEGKNLYVKGEPIINYYDPLVFPSQEFDASISQVNEKINQSLAFIRRSDELLSAIGGYIPEAPRDGQAYVRKDGEWVLLSTFL

SEQ ID NO: 51 - protein, 549 aa, synthetic construct
MELPILKTNAITTILAAVTLCFASSQNITEEFYQSTCSAVSKGYLSALRTGWYTSVITIELSNIKINKCNGTDAKVKLIKQELDKYKNAVTELQLLMQSTPAANSRARRELPRFMNYTLNNTKNTNVTLSKKRKRRFLGFLLGVGSAIASGIAVSKVLHLEGEVNKIKSALLSTNKAVVSLSNGVSVLTSKVLDLKNYIDKQLLPIVNKQSCPISNIETVIEFQQKNNRLLEITREFSVNAGVTTPVSTYMLTNSELLSLINDMPITNDQKKLMSSNVQIVRQQSYSIMSIIKEEVLAYVVQLPLYGVIDTPCWKLHTSPLCTTNTKEGSNICLTRTDRGWYCDNAGSVSFFPQAETCKVQSNRVFCDTMNSLTLPSEVNLCNIDIFNPKYDCKIMTSKTDVSSSVITSLGAIVSCYGKTKCTASNKNRGIIKTFSNGCDYVSNKGVDTVSVGNTLYYVNKQEGKSLYVKGEPIINFYDPLVFPSDTFDASISQVNEKINQSLAFIRKSDELLHNVNAGKSTTNIMITTIIIVIIVILLALIAVGLLLY

SEQ ID NO: 52 - protein, 549 aa, synthetic construct
MELLIHRSSAIFLTLAINALYLTSSQNITEEFYQSTCSAVSRGYFSALRTGWYTSVITIELSNIKITKCNGTDTKVKLIKQELDKYKNAVTELQLLMQNTPAANNRARREAPQYMNYTINTTKNLNVSISKKRKRRFLGFLLGVGSAIASGIAVSKVLHLEGEVNKIKNALLSTNKAVVSLSNGVSVLTSKVLDLKNYINNQLLPIVNQQSCPISNIETVIEFQQKNSRLLEITREFSVNAGVTTPLSTYMLTNSELLSLINDMPITNDQKKLMSSNVQIVRQQSYSIMSIIKEEVLAYVVQLPIYGVIDTPCWKLHTSPLCTTNIKEGSNICLTRTDRGWYCDNAGSVSFFPQADTCKVQSNRVFCDTMNSLTLPSEVSLCNTDIFNSKYDCKIMTSKTDISSSVITSLGAIVSCYGKTKCTASNKNRGIIKTFSNGCDYVSNKGVDTVSVGNTLYYVNKLEGKNLYVKGEPIINYYDPLVFPSDTFDASISQVNEKINQSLAFIRRSDELLHNVNTGKSTTNIMITAIIIVIIVVLLSLIAIGLLLY

SEQ ID NO: 53 - protein, 549 aa, synthetic construct
MELPILKTNAITTILAAVTLCFASSQNITEEFYQSTCSAVSKGYLSALRTGWYTSVITIELSNIKINKCNGTDAKVKLIKQELDKYKNAVTELQLLMQSTPAANSRARRELPRFMNYTLNNTKNTNVTLSKKRKRRFLGFLLGVGSAIASGIAVSKVLHLEGEVNKIKSALLSTNKAVVSLSNGVSVLTSKVLDLKNYIDKQLLPIVNKQSCPISNIETVIEFQQKNNRLLEITREFSVNAGVTTPVSTYMLTNSELLSLINDMPITNDQKKLMSSNVQIVRQQSYSIMSIIKEEVLAYVVQLPLYGVIDTPCWKLHTSPLCTTNTKEGSNICLTRTDRGWYCDNAGSVSFFPQAETCKVQSNRVFCDTMNSLTLPSEVNLCNIDIFNPKYDCKIMTSKTDVSSSVITSLGAIVSCYGKTKCTASNKNRGIIKTFSNGCDYVSNKGVDTVSVGNTLYYVNKQEGKSLYVKGEPIINFYDPLVFPSQEFDASISQVNEKINQSLAFIRKSDELLHNVNAGKSTTNIMITTIIIVIIVILLALIAVGLLLY

SEQ ID NO: 54 - protein, 549 aa, synthetic construct
MELLIHRSSAIFLTLAINALYLTSSQNITEEFYQSTCSAVSRGYFSALRTGWYTSVITIELSNIKITKCNGTDTKVKLIKQELDKYKNAVTELQLLMQNTPAANNRARREAPQYMNYTINTTKNLNVSISKKRKRRFLGFLLGVGSAIASGIAVSKVLHLEGEVNKIKNALLSTNKAVVSLSNGVSVLTSKVLDLKNYINNQLLPIVNQQSCPISNIETVIEFQQKNSRLLEITREFSVNAGVTTPLSTYMLTNSELLSLINDMPITNDQKKLMSSNVQIVRQQSYSIMSIIKEEVLAYVVQLPIYGVIDTPCWKLHTSPLCTTNIKEGSNICLTRTDRGWYCDNAGSVSFFPQADTCKVQSNRVFCDTMNSLTLPSEVSLCNTDIFNSKYDCKIMTSKTDISSSVITSLGAIVSCYGKTKCTASNKNRGIIKTFSNGCDYVSNKGVDTVSVGNTLYYVNKLEGKNLYVKGEPIINYYDPLVFPSQEFDASISQVNEKINQSLAFIRRSDELLHNVNTGKSTTNIMITAIIIVIIVVLLSLIAIGLLLY

SEQ ID NO: 55 - protein, 549 aa, synthetic construct
MELPILKTNAITTILAAVTLCFASSQNITEEFYQSTCSAVSKGYLSALRTGWYTSVITIELSNIKINKCNGTDAKVKLIKQELDKYKNAVTELQLLMQSTPCANSRARRELPRFMNYTLNNTKNTNVTLSKKRKRRFLGFLLGVGSAIASGCAVSKVLHLEGEVNKIKSALLSTNKAVVSLSNGVSVLTSKVLDLKNYIDKQLLPIVNKQSCPISNIETVIEFQQKNNRLLEITREFSVNAGVTTPVSTYMLTNSELLSLINDMPITNDQKKLMSSNVQIVRQQSYSIMSIIKEEVLAYVVQLPLYGVIDTPCWKLHTSPLCTTNTKEGSNICLTRTDRGWYCDNAGSVSFFPQAETCKVQSNRVFCDTMNSLTLPSEVNLCNIDIFNPKYDCKIMTSKTDVSSSVITSLGAIVSCYGKTKCTASNKNRGIIKTFSNGCDYVSNKGVDTVSVGNTLYYVNKQEGKSLYVKGEPIINFYDPLVFPSDEFDASISQVNEKINQSLAFIRKSDELLHNVNAGKSTTNIMITTIIIVIIVILLALIAVGLLLY

SEQ ID NO: 56 - protein, 549 aa, synthetic construct
MELLIHRSSAIFLTLAINALYLTSSQNITEEFYQSTCSAVSRGYFSALRTGWYTSVITIELSNIKITKCNGTDTKVKLIKQELDKYKNAVTELQLLMQNTPCANNRARREAPQYMNYTINTTKNLNVSISKKRKRRFLGFLLGVGSAIASGCAVSKVLHLEGEVNKIKNALLSTNKAVVSLSNGVSVLTSKVLDLKNYINNQLLPIVNQQSCPISNIETVIEFQQKNSRLLEITREFSVNAGVTTPLSTYMLTNSELLSLINDMPITNDQKKLMSSNVQIVRQQSYSIMSIIKEEVLAYVVQLPIYGVIDTPCWKLHTSPLCTTNIKEGSNICLTRTDRGWYCDNAGSVSFFPQADTCKVQSNRVFCDTMNSLTLPSEVSLCNTDIFNSKYDCKIMTSKTDISSSVITSLGAIVSCYGKTKCTASNKNRGIIKTFSNGCDYVSNKGVDTVSVGNTLYYVNKLEGKNLYVKGEPIINYYDPLVFPSDEFDASISQVNEKINQSLAFIRRSDELLHNVNTGKSTTNIMITAIIIVIIVVLLSLIAIGLLLY

SEQ ID NO: 57 - protein, 549 aa, synthetic construct
MELPILKTNAITTILAAVTLCFASSQNITEEFYQSTCSAVSKGYLSALRTGWYTSVITIELSNIKINKCNGTDAKVKLIKQELDKYKNAVTELQLLMQSTCAANSRARRELPRFMNYTLNNTKNTNVTLSKKRKRRFLGFLLGVGSAIASGCAVSKVLHLEGEVNKIKSALLSTNKAVVSLSNGVSVLTSKVLDLKNYIDKQLLPIVNKQSCPISNIETVIEFQQKNNRLLEITREFSVNAGVTTPVSTYMLTNSELLSLINDMPITNDQKKLMSSNVQIVRQQSYSIMSIIKEEVLAYVVQLPLYGVIDTPCWKLHTSPLCTTNTKEGSNICLTRTDRGWYCDNAGSVSFFPQAETCKVQSNRVFCDTMNSLTLPSEVNLCNIDIFNPKYDCKIMTSKTDVSSSVITSLGAIVSCYGKTKCTASNKNRGIIKTFSNGCDYVSNKGVDTVSVGNTLYYVNKQEGKSLYVKGEPIINFYDPLVFPSDEFDASISQVNEKINQSLAFIRKSDELLHNVNAGKSTTNIMITTIIIVIIVILLALIAVGLLLY

SEQ ID NO: 58 - protein, 549 aa, synthetic construct
MELLIHRSSAIFLTLAINALYLTSSQNITEEFYQSTCSAVSRGYFSALRTGWYTSVITIELSNIKITKCNGTDTKVKLIKQELDKYKNAVTELQLLMQNTCAANNRARREAPQYMNYTINTTKNLNVSISKKRKRRFLGFLLGVGSAIASGCAVSKVLHLEGEVNKIKNALLSTNKAVVSLSNGVSVLTSKVLDLKNYINNQLLPIVNQQSCPISNIETVIEFQQKNSRLLEITREFSVNAGVTTPLSTYMLTNSELLSLINDMPITNDQKKLMSSNVQIVRQQSYSIMSIIKEEVLAYVVQLPIYGVIDTPCWKLHTSPLCTTNIKEGSNICLTRTDRGWYCDNAGSVSFFPQADTCKVQSNRVFCDTMNSLTLPSEVSLCNTDIFNSKYDCKIMTSKTDISSSVITSLGAIVSCYGKTKCTASNKNRGIIKTFSNGCDYVSNKGVDTVSVGNTLYYVNKLEGKNLYVKGEPIINYYDPLVFPSDEFDASISQVNEKINQSLAFIRRSDELLHNVNTGKSTTNIMITAIIIVIIVVLLSLIAIGLLLY

SEQ ID NO: 59 - protein, 549 aa, synthetic construct
MELPILKTNAITTILAAVTLCFASSQNITEEFYQSTCSAVSKGYLSALRTGWYTSVITIELSNIKINKCNGTDAKVKLIKQELDKYKNAVTELQLLMQSTPAANSRARRELPRFMNYTLNNTKNTNVTLSKKRKRRFLGFLLGVGSAIASGIAVSKVLHLEGEVNKIKSALLSTNKAVVSLSNGVSVLTSKVLDLKNYIDKQLLPIVNKQSCPISNIETVIEFQQKNNRLLEITREFSVNAGVTTPVSTYMLTNSELLSLINDMPITNDQKKLMSSNVQIVRQQSYSIMSIIKEEVLAYVVQLPLYGVIDTPCWKLHTSPLCTTNTKEGSNICLTRTDRGWYCDNAGSVSFFPQAETCKVQSNRVFCDTMNSLTLPSEVNLCNIDIFNPKYDCKIMTSKTDVSSSVITSLGAIVSCYGKTKCTASNKNRGIIKTFSNGCDYVSNKGVDTVSVGNTLYYVNKQEGKSLYVKGEPIINFYDPLVFPSDEFDASISQVNEKINQSLAFIRKSDELLHNVNAGKSTTNIMITTIIIVIIVILLALIAVGLLLY

SEQ ID NO: 60 - protein, 549 aa, synthetic construct
MELLIHRSSAIFLTLAINALYLTSSQNITEEFYQSTCSAVSRGYFSALRTGWYTSVITIELSNIKITKCNGTDTKVKLIKQELDKYKNAVTELQLLMQNTPAANNRARREAPQYMNYTINTTKNLNVSISKKRKRRFLGFLLGVGSAIASGIAVSKVLHLEGEVNKIKNALLSTNKAVVSLSNGVSVLTSKVLDLKNYINNQLLPIVNQQSCPISNIETVIEFQQKNSRLLEITREFSVNAGVTTPLSTYMLTNSELLSLINDMPITNDQKKLMSSNVQIVRQQSYSIMSIIKEEVLAYVVQLPIYGVIDTPCWKLHTSPLCTTNIKEGSNICLTRTDRGWYCDNAGSVSFFPQADTCKVQSNRVFCDTMNSLTLPSEVSLCNTDIFNSKYDCKIMTSKTDISSSVITSLGAIVSCYGKTKCTASNKNRGIIKTFSNGCDYVSNKGVDTVSVGNTLYYVNKLEGKNLYVKGEPIINYYDPLVFPSDEFDASISQVNEKINQSLAFIRRSDELLHNVNTGKSTTNIMITAIIIVIIVVLLSLIAIGLLLY

SEQ ID NO: 61 - protein, 549 aa, synthetic construct
MELPILKTNAITTILAAVTLCFASSQNITEEFYQSTCSAVSKGYLSALRTGWYVSVITIELSNIKENKCNGTDAKVKLIKQELDKYKNAVTELQLLMQSTPCANSRARRELPRFMNYTLNNTKNTNVTLSKKRKRRFLGFLLGVGSAIASGCAVSKVLHLEGEVNKIKSALLSTNKAVVSLSNGVSVLTMKVLDLKNYIDKQLLPIVNKQSCSISNIETVIEFQQKNNRLLEITREFSVNAGVTTPVSTYMLTNSELLSLINDMPITNDQKKLMSSNVQIVRQQSYSIMSIIKEELLAYVVQLPLYGVIDTPCWKLHTSPLCTTNTKEGSNICLTRTDRGWYCDNAGSVSFFPQAETCKVQSNRVFCDTMNSLTLPSEVNLCNIDIFNPKYDCKIMTSKTDVSSSVITSLGAIVSCYGKTKCTASNKNRGIIKTFSNGCDYVSNKGVDTVSVGNTLYYVNKQEGKSLYVKGEPIINFYDPLVFPSDEFDASISQVNEKINQSLAFIRKSDELLHNVNAGKSTTNIMITTIIIVIIVILLALIAVGLLLY

SEQ ID NO: 62 - protein, 549 aa, synthetic construct
MELLIHRSSAIFLTLAINALYLTSSQNITEEFYQSTCSAVSRGYFSALRTGWYVSVITIELSNIKETKCNGTDTKVKLIKQELDKYKNAVTELQLLMQNTPCANNRARREAPQYMNYTINTTKNLNVSISKKRKRRFLGFLLGVGSAIASGCAVSKVLHLEGEVNKIKNALLSTNKAVVSLSNGVSVLTMKVLDLKNYINNQLLPIVNQQSCRISNIETVIEFQQKNSRLLEITREFSVNAGVTTPLSTYMLTNSELLSLINDMPITNDQKKLMSSNVQIVRQQSYSIMSIIKEELLAYVVQLPIYGVIDTPCWKLHTSPLCTTNIKEGSNICLTRTDRGWYCDNAGSVSFFPQADTCKVQSNRVFCDTMNSLTLPSEVSLCNTDIFNSKYDCKIMTSKTDISSSVITSLGAIVSCYGKTKCTASNKNRGIIKTFSNGCDYVSNKGVDTVSVGNTLYYVNKLEGKNLYVKGEPIINYYDPLVFPSDEFDASISQVNEKINQSLAFIRRSDELLHNVNTGKSTTNIMITAIIIVIIVVLLSLIAIGLLLY

SEQ ID NO: 63 - protein, 549 aa, synthetic construct
MELPILKTNAITTILAAVTLCFASSQNITEEFYQSTCSAVSKGYLSALRTGWYFSVITIELSNIKENKCNGTDAKVKLIKQELDKYKNAVTELQLLMQSTPCANSRARRELPRFMNYTLNNTKNTNVTLSKKRKRRFLGFLLGVGSAIASGCAVSKVLHLEGEVNKIKSALLSTNKAVVSLSNGVSVLTMKVLDLKNYIDKQLLPIVNKQSCSISNIETVIEFQQKNNRLLEITREFSVNAGVTTPVSTYMLTNSELLSLINDMPITNDQKKLMSSNVQIVRQQSYSIMSIIKEELLAYVVQLPLYGVIDTPCWKLHTSPLCTTNTKEGSNICLTRTDRGWYCDNAGSVSFFPQAETCKVQSNRVFCDTMNSLTLPSEVNLCNIDIFNPKYDCKIMTSKTDVSSSVITSLGAIVSCYGKTKCTASNKNRGIIKTFSNGCDYVSNKGVDTVSVGNTLYYVNKQEGKSLYVKGEPIINFYDPLVFPSDEFDASISQVNEKINQSLAFIRKSDELLHNVNAGKSTTNIMITTIIIVIIVILLALIAVGLLLY

SEQ ID NO: 64 - protein, 549 aa, synthetic construct
MELLIHRSSAIFLTLAINALYLTSSQNITEEFYQSTCSAVSRGYFSALRTGWYFSVITIELSNIKETKCNGTDTKVKLIKQELDKYKNAVTELQLLMQNTPCANNRARREAPQYMNYTINTTKNLNVSISKKRKRRFLGFLLGVGSAIASGCAVSKVLHLEGEVNKIKNALLSTNKAVVSLSNGVSVLTMKVLDLKNYINNQLLPIVNQQSCRISNIETVIEFQQKNSRLLEITREFSVNAGVTTPLSTYMLTNSELLSLINDMPITNDQKKLMSSNVQIVRQQSYSIMSIIKEELLAYVVQLPIYGVIDTPCWKLHTSPLCTTNIKEGSNICLTRTDRGWYCDNAGSVSFFPQADTCKVQSNRVFCDTMNSLTLPSEVSLCNTDIFNSKYDCKIMTSKTDISSSVITSLGAIVSCYGKTKCTASNKNRGIIKTFSNGCDYVSNKGVDTVSVGNTLYYVNKLEGKNLYVKGEPIINYYDPLVFPSDEFDASISQVNEKINQSLAFIRRSDELLHNVNTGKSTTNIMITAIIIVIIVVLLSLIAIGLLLY

SEQ ID NO: 65 - protein, 549 aa, synthetic construct
MELPILKTNAITTILAAVTLCFASSQNITEEFYQSTCSAVSKGYLSALRTGWYCSVITIELSNIKENKCNGTDAKVKLIKQELDKYKNAVTELQLLMQSTPCANSRARRELPRFMNYTLNNTKNTNVTLSKKRKRRFLGFLLGVGSAIASGCAVSKVLHLEGEVNKIKSALLSTNKAVVSLSNGVSVLTMKVLDLKNYIDKQLLPIVNKQSCSISNIETVIEFQQKNNRLLEITREFSVNAGVTTPVSTYMLTNSELLSLINDMPITNDQKKLMSSNVQIVRQQSYSIMSIIKEELLAYVVQLPLYGVIDTPCWKLHTSPLCTTNTKEGSNICLTRTDRGWYCDNAGSVSFFPQAETCKVQSNRVFCDTMNSLTLPSEVNLCNIDIFNPKYDCKIMTSKTDVSSSVITSLGAIVSCYGKTKCTASNKNRGIIKTFSNGCDYVSNKGVDTVSVGNTLYYVNKQEGKSLYVKGEPIINFYDPLVFPSDEFDASISQVNEKINQSLAFIRKSDELLHNVNAGKSTTNIMITTIIIVIIVILLALIAVGLLLY

SEQ ID NO: 66 - protein, 549 aa, synthetic construct
MELLIHRSSAIFLTLAINALYLTSSQNITEEFYQSTCSAVSRGYFSALRTGWYCSVITIELSNIKETKCNGTDTKVKLIKQELDKYKNAVTELQLLMQNTPCANNRARREAPQYMNYTINTTKNLNVSISKKRKRRFLGFLLGVGSAIASGCAVSKVLHLEGEVNKIKNALLSTNKAVVSLSNGVSVLTMKVLDLKNYINNQLLPIVNQQSCRISNIETVIEFQQKNSRLLEITREFSVNAGVTTPLSTYMLTNSELLSLINDMPITNDQKKLMSSNVQIVRQQSYSIMSIIKEELLAYVVQLPIYGVIDTPCWKLHTSPLCTTNIKEGSNICLTRTDRGWYCDNAGSVSFFPQADTCKVQSNRVFCDTMNSLTLPSEVSLCNTDIFNSKYDCKIMTSKTDISSSVITSLGAIVSCYGKTKCTASNKNRGIIKTFSNGCDYVSNKGVDTVSVGNTLYYVNKLEGKNLYVKGEPIINYYDPLVFPSDEFDASISQVNEKINQSLAFIRRSDELLHNVNTGKSTTNIMITAIIIVIIVVLLSLIAIGLLLY

SEQ ID NO: 67 - protein, 549 aa, synthetic construct
MELPILKTNAITTILAAVTLCFASSQNITEEFYQSTCSAVSKGYLSALRTGWYASVITIELSNIKENKCNGTDAKVKLIKQELDKYKNAVTELQLLMQSTPCANSRARRELPRFMNYTLNNTKNTNVTLSKKRKRRFLGFLLGVGSAIASGCAVSKVLHLEGEVNKIKSALLSTNKAVVSLSNGVSVLTMKVLDLKNYIDKQLLPIVNKQSCSISNIETVIEFQQKNNRLLEITREFSVNAGVTTPVSTYMLTNSELLSLINDMPITNDQKKLMSSNVQIVRQQSYSIMSIIKEELLAYVVQLPLYGVIDTPCWKLHTSPLCTTNTKEGSNICLTRTDRGWYCDNAGSVSFFPQAETCKVQSNRVFCDTMNSLTLPSEVNLCNIDIFNPKYDCKIMTSKTDVSSSVITSLGAIVSCYGKTKCTASNKNRGIIKTFSNGCDYVSNKGVDTVSVGNTLYYVNKQEGKSLYVKGEPIINFYDPLVFPSDEFDASISQVNEKINQSLAFIRKSDELLHNVNAGKSTTNIMITTIIIVIIVILLALIAVGLLLY

SEQ ID NO: 68 - protein, 549 aa, synthetic construct
MELLIHRSSAIFLTLAINALYLTSSQNITEEFYQSTCSAVSRGYFSALRTGWYASVITIELSNIKETKCNGTDTKVKLIKQELDKYKNAVTELQLLMQNTPCANNRARREAPQYMNYTINTTKNLNVSISKKRKRRFLGFLLGVGSAIASGCAVSKVLHLEGEVNKIKNALLSTNKAVVSLSNGVSVLTMKVLDLKNYINNQLLPIVNQQSCRISNIETVIEFQQKNSRLLEITREFSVNAGVTTPLSTYMLTNSELLSLINDMPITNDQKKLMSSNVQIVRQQSYSIMSIIKEELLAYVVQLPIYGVIDTPCWKLHTSPLCTTNIKEGSNICLTRTDRGWYCDNAGSVSFFPQADTCKVQSNRVFCDTMNSLTLPSEVSLCNTDIFNSKYDCKIMTSKTDISSSVITSLGAIVSCYGKTKCTASNKNRGIIKTFSNGCDYVSNKGVDTVSVGNTLYYVNKLEGKNLYVKGEPIINYYDPLVFPSDEFDASISQVNEKINQSLAFIRRSDELLHNVNTGKSTTNIMITAIIIVIIVVLLSLIAIGLLLY

SEQ ID NO: 69 - protein, 549 aa, synthetic construct
MELPILKTNAITTILAAVTLCFASSQNITEEFYQSTCSAVSKGYLSALRTGWYVSVITIELSNIKENKCNGTDAKVKLIKQELDKYKNAVTELQLLMQSTPCANSRARRELPRFMNYTLNNTKNTNVTLSKKRKRRFLGFLLGVGSAIASGCAVSKVLHLEGEVNKIKSALLSTNKAVVSLSNGVSVLTFKVLDLKNYIDKQLLPIVNKQSCSISNIETVIEFQQKNNRLLEITREFSVNAGVTTPVSTYMLTNSELLSLINDMPITNDQKKLMSSNVQIVRQQSYSIMSIIKEELLAYVVQLPLYGVIDTPCWKLHTSPLCTTNTKEGSNICLTRTDRGWYCDNAGSVSFFPQAETCKVQSNRVFCDTMNSLTLPSEVNLCNIDIFNPKYDCKIMTSKTDVSSSVITSLGAIVSCYGKTKCTASNKNRGIIKTFSNGCDYVSNKGVDTVSVGNTLYYVNKQEGKSLYVKGEPIINFYDPLVFPSDEFDASISQVNEKINQSLAFIRKSDELLHNVNAGKSTTNIMITTIIIVIIVILLALIAVGLLLY

SEQ ID NO: 70 - protein, 549 aa, synthetic construct
MELLIHRSSAIFLTLAINALYLTSSQNITEEFYQSTCSAVSRGYFSALRTGWYVSVITIELSNIKETKCNGTDTKVKLIKQELDKYKNAVTELQLLMQNTPCANNRARREAPQYMNYTINTTKNLNVSISKKRKRRFLGFLLGVGSAIASGCAVSKVLHLEGEVNKIKNALLSTNKAVVSLSNGVSVLTFKVLDLKNYINNQLLPIVNQQSCRISNIETVIEFQQKNSRLLEITREFSVNAGVTTPLSTYMLTNSELLSLINDMPITNDQKKLMSSNVQIVRQQSYSIMSIIKEELLAYVVQLPIYGVIDTPCWKLHTSPLCTTNIKEGSNICLTRTDRGWYCDNAGSVSFFPQADTCKVQSNRVFCDTMNSLTLPSEVSLCNTDIFNSKYDCKIMTSKTDISSSVITSLGAIVSCYGKTKCTASNKNRGIIKTFSNGCDYVSNKGVDTVSVGNTLYYVNKLEGKNLYVKGEPIINYYDPLVFPSDEFDASISQVNEKINQSLAFIRRSDELLHNVNTGKSTTNIMITAIIIVIIVVLLSLIAIGLLLY

SEQ ID NO: 71 - protein, 549 aa, synthetic construct
MELPILKTNAITTILAAVTLCFASSQNITEEFYQSTCSAVSKGYLSALRTGWYFSVITIELSNIKENKCNGTDAKVKLIKQELDKYKNAVTELQLLMQSTPCANSRARRELPRFMNYTLNNTKNTNVTLSKKRKRRFLGFLLGVGSAIASGCAVSKVLHLEGEVNKIKSALLSTNKAVVSLSNGVSVLTFKVLDLKNYIDKQLLPIVNKQSCSISNIETVIEFQQKNNRLLEITREFSVNAGVTTPVSTYMLTNSELLSLINDMPITNDQKKLMSSNVQIVRQQSYSIMSIIKEELLAYVVQLPLYGVIDTPCWKLHTSPLCTTNTKEGSNICLTRTDRGWYCDNAGSVSFFPQAETCKVQSNRVFCDTMNSLTLPSEVNLCNIDIFNPKYDCKIMTSKTDVSSSVITSLGAIVSCYGKTKCTASNKNRGIIKTFSNGCDYVSNKGVDTVSVGNTLYYVNKQEGKSLYVKGEPIINFYDPLVFPSDEFDASISQVNEKINQSLAFIRKSDELLHNVNAGKSTTNIMITTIIIVIIVILLALIAVGLLLY

SEQ ID NO: 72 - protein, 549 aa, synthetic construct
MELLIHRSSAIFLTLAINALYLTSSQNITEEFYQSTCSAVSRGYFSALRTGWYFSVITIELSNIKETKCNGTDTKVKLIKQELDKYKNAVTELQLLMQNTPCANNRARREAPQYMNYTINTTKNLNVSISKKRKRRFLGFLLGVGSAIASGCAVSKVLHLEGEVNKIKNALLSTNKAVVSLSNGVSVLTFKVLDLKNYINNQLLPIVNQQSCRISNIETVIEFQQKNSRLLEITREFSVNAGVTTPLSTYMLTNSELLSLINDMPITNDQKKLMSSNVQIVRQQSYSIMSIIKEELLAYVVQLPIYGVIDTPCWKLHTSPLCTTNIKEGSNICLTRTDRGWYCDNAGSVSFFPQADTCKVQSNRVFCDTMNSLTLPSEVSLCNTDIFNSKYDCKIMTSKTDISSSVITSLGAIVSCYGKTKCTASNKNRGIIKTFSNGCDYVSNKGVDTVSVGNTLYYVNKLEGKNLYVKGEPIINYYDPLVFPSDEFDASISQVNEKINQSLAFIRRSDELLHNVNTGKSTTNIMITAIIIVIIVVLLSLIAIGLLLY

SEQ ID NO: 73 - protein, 549 aa, synthetic construct
MELPILKTNAITTILAAVTLCFASSQNITEEFYQSTCSAVSKGYLSALRTGWYCSVITIELSNIKENKCNGTDAKVKLIKQELDKYKNAVTELQLLMQSTPCANSRARRELPRFMNYTLNNTKNTNVTLSKKRKRRFLGFLLGVGSAIASGCAVSKVLHLEGEVNKIKSALLSTNKAVVSLSNGVSVLTFKVLDLKNYIDKQLLPIVNKQSCSISNIETVIEFQQKNNRLLEITREFSVNAGVTTPVSTYMLTNSELLSLINDMPITNDQKKLMSSNVQIVRQQSYSIMSIIKEELLAYVVQLPLYGVIDTPCWKLHTSPLCTTNTKEGSNICLTRTDRGWYCDNAGSVSFFPQAETCKVQSNRVFCDTMNSLTLPSEVNLCNIDIFNPKYDCKIMTSKTDVSSSVITSLGAIVSCYGKTKCTASNKNRGIIKTFSNGCDYVSNKGVDTVSVGNTLYYVNKQEGKSLYVKGEPIINFYDPLVFPSDEFDASISQVNEKINQSLAFIRKSDELLHNVNAGKSTTNIMITTIIIVIIVILLALIAVGLLLY

SEQ ID NO: 74 - protein, 549 aa, synthetic construct
MELLIHRSSAIFLTLAINALYLTSSQNITEEFYQSTCSAVSRGYFSALRTGWYCSVITIELSNIKETKCNGTDTKVKLIKQELDKYKNAVTELQLLMQNTPCANNRARREAPQYMNYTINTTKNLNVSISKKRKRRFLGFLLGVGSAIASGCAVSKVLHLEGEVNKIKNALLSTNKAVVSLSNGVSVLTFKVLDLKNYINNQLLPIVNQQSCRISNIETVIEFQQKNSRLLEITREFSVNAGVTTPLSTYMLTNSELLSLINDMPITNDQKKLMSSNVQIVRQQSYSIMSIIKEELLAYVVQLPIYGVIDTPCWKLHTSPLCTTNIKEGSNICLTRTDRGWYCDNAGSVSFFPQADTCKVQSNRVFCDTMNSLTLPSEVSLCNTDIFNSKYDCKIMTSKTDISSSVITSLGAIVSCYGKTKCTASNKNRGIIKTFSNGCDYVSNKGVDTVSVGNTLYYVNKLEGKNLYVKGEPIINYYDPLVFPSDEFDASISQVNEKINQSLAFIRRSDELLHNVNTGKSTTNIMITAIIIVIIVVLLSLIAIGLLLY

SEQ ID NO: 75 - protein, 549 aa, synthetic construct
MELPILKTNAITTILAAVTLCFASSQNITEEFYQSTCSAVSKGYLSALRTGWYASVITIELSNIKENKCNGTDAKVKLIKQELDKYKNAVTELQLLMQSTPCANSRARRELPRFMNYTLNNTKNTNVTLSKKRKRRFLGFLLGVGSAIASGCAVSKVLHLEGEVNKIKSALLSTNKAVVSLSNGVSVLTFKVLDLKNYIDKQLLPIVNKQSCSISNIETVIEFQQKNNRLLEITREFSVNAGVTTPVSTYMLTNSELLSLINDMPITNDQKKLMSSNVQIVRQQSYSIMSIIKEELLAYVVQLPLYGVIDTPCWKLHTSPLCTTNTKEGSNICLTRTDRGWYCDNAGSVSFFPQAETCKVQSNRVFCDTMNSLTLPSEVNLCNIDIFNPKYDCKIMTSKTDVSSSVITSLGAIVSCYGKTKCTASNKNRGIIKTFSNGCDYVSNKGVDTVSVGNTLYYVNKQEGKSLYVKGEPIINFYDPLVFPSDEFDASISQVNEKINQSLAFIRKSDELLHNVNAGKSTTNIMITTIIIVIIVILLALIAVGLLLY

SEQ ID NO: 76 - protein, 549 aa, synthetic construct
MELLIHRSSAIFLTLAINALYLTSSQNITEEFYQSTCSAVSRGYFSALRTGWYASVITIELSNIKETKCNGTDTKVKLIKQELDKYKNAVTELQLLMQNTPCANNRARREAPQYMNYTINTTKNLNVSISKKRKRRFLGFLLGVGSAIASGCAVSKVLHLEGEVNKIKNALLSTNKAVVSLSNGVSVLTFKVLDLKNYINNQLLPIVNQQSCRISNIETVIEFQQKNSRLLEITREFSVNAGVTTPLSTYMLTNSELLSLINDMPITNDQKKLMSSNVQIVRQQSYSIMSIIKEELLAYVVQLPIYGVIDTPCWKLHTSPLCTTNIKEGSNICLTRTDRGWYCDNAGSVSFFPQADTCKVQSNRVFCDTMNSLTLPSEVSLCNTDIFNSKYDCKIMTSKTDISSSVITSLGAIVSCYGKTKCTASNKNRGIIKTFSNGCDYVSNKGVDTVSVGNTLYYVNKLEGKNLYVKGEPIINYYDPLVFPSDEFDASISQVNEKINQSLAFIRRSDELLHNVNTGKSTTNIMITAIIIVIIVVLLSLIAIGLLLY

SEQ ID NO: 77 - protein, 549 aa, synthetic construct
MELPILKTNAITTILAAVTLCFASSQNITEEFYQSTCSAVSKGYLSALRTGWYVSVITIELSNIKENKCNGTDAKVKLIKQELDKYKNAVTELQLLMQSTCAANSRARRELPRFMNYTLNNTKNTNVTLSKKRKRRFLGFLLGVGSAIASGCAVSKVLHLEGEVNKIKSALLSTNKAVVSLSNGVSVLTMKVLDLKNYIDKQLLPIVNKQSCSISNIETVIEFQQKNNRLLEITREFSVNAGVTTPVSTYMLTNSELLSLINDMPITNDQKKLMSSNVQIVRQQSYSIMSIIKEELLAYVVQLPLYGVIDTPCWKLHTSPLCTTNTKEGSNICLTRTDRGWYCDNAGSVSFFPQAETCKVQSNRVFCDTMNSLTLPSEVNLCNIDIFNPKYDCKIMTSKTDVSSSVITSLGAIVSCYGKTKCTASNKNRGIIKTFSNGCDYVSNKGVDTVSVGNTLYYVNKQEGKSLYVKGEPIINFYDPLVFPSDEFDASISQVNEKINQSLAFIRKSDELLHNVNAGKSTTNIMITTIIIVIIVILLALIAVGLLLY

SEQ ID NO: 78 - protein, 551 aa, synthetic construct
NOMELLIHRSSAIFLTLAINALYLTSSQNITEEFYQSTCSAVSRGYFSALRTGWYVSVITIELSNIKETKCNGTDTKVKLIKQELDKYKNAVTELQLLMQNTCAANNRARREAPQYMNYTINTTKNLNVSISKKRKRRFLGFLLGVGSAIASGCAVSKVLHLEGEVNKIKNALLSTNKAVVSLSNGVSVLTMKVLDLKNYINNQLLPIVNQQSCRISNIETVIEFQQKNSRLLEITREFSVNAGVTTPLSTYMLTNSELLSLINDMPITNDQKKLMSSNVQIVRQQSYSIMSIIKEELLAYVVQLPIYGVIDTPCWKLHTSPLCTTNIKEGSNICLTRTDRGWYCDNAGSVSFFPQADTCKVQSNRVFCDTMNSLTLPSEVSLCNTDIFNSKYDCKIMTSKTDISSSVITSLGAIVSCYGKTKCTASNKNRGIIKTFSNGCDYVSNKGVDTVSVGNTLYYVNKLEGKNLYVKGEPIINYYDPLVFPSDEFDASISQVNEKINQSLAFIRRSDELLHNVNTGKSTTNIMITAIIIVIIVVLLSLIAIGLLLY

SEQ ID NO: 79 - protein, 549 aa, synthetic construct
MELPILKTNAITTILAAVTLCFASSQNITEEFYQSTCSAVSKGYLSALRTGWYFSVITIELSNIKENKCNGTDAKVKLIKQELDKYKNAVTELQLLMQSTCAANSRARRELPRFMNYTLNNTKNTNVTLSKKRKRRFLGFLLGVGSAIASGCAVSKVLHLEGEVNKIKSALLSTNKAVVSLSNGVSVLTMKVLDLKNYIDKQLLPIVNKQSCSISNIETVIEFQQKNNRLLEITREFSVNAGVTTPVSTYMLTNSELLSLINDMPITNDQKKLMSSNVQIVRQQSYSIMSIIKEELLAYVVQLPLYGVIDTPCWKLHTSPLCTTNTKEGSNICLTRTDRGWYCDNAGSVSFFPQAETCKVQSNRVFCDTMNSLTLPSEVNLCNIDIFNPKYDCKIMTSKTDVSSSVITSLGAIVSCYGKTKCTASNKNRGIIKTFSNGCDYVSNKGVDTVSVGNTLYYVNKQEGKSLYVKGEPIINFYDPLVFPSDEFDASISQVNEKINQSLAFIRKSDELLHNVNAGKSTTNIMITTIIIVIIVILLALIAVGLLLY

SEQ ID NO: 80 - protein, 549 aa, synthetic construct
MELLIHRSSAIFLTLAINALYLTSSQNITEEFYQSTCSAVSRGYFSALRTGWYFSVITIELSNIKETKCNGTDTKVKLIKQELDKYKNAVTELQLLMQNTCAANNRARREAPQYMNYTINTTKNLNVSISKKRKRRFLGFLLGVGSAIASGCAVSKVLHLEGEVNKIKNALLSTNKAVVSLSNGVSVLTMKVLDLKNYINNQLLPIVNQQSCRISNIETVIEFQQKNSRLLEITREFSVNAGVTTPLSTYMLTNSELLSLINDMPITNDQKKLMSSNVQIVRQQSYSIMSIIKEELLAYVVQLPIYGVIDTPCWKLHTSPLCTTNIKEGSNICLTRTDRGWYCDNAGSVSFFPQADTCKVQSNRVFCDTMNSLTLPSEVSLCNTDIFNSKYDCKIMTSKTDISSSVITSLGAIVSCYGKTKCTASNKNRGIIKTFSNGCDYVSNKGVDTVSVGNTLYYVNKLEGKNLYVKGEPIINYYDPLVFPSDEFDASISQVNEKINQSLAFIRRSDELLHNVNTGKSTTNIMITAIIIVIIVVLLSLIAIGLLLY

SEQ ID NO: 81 - protein, 549 aa, synthetic construct
MELPILKTNAITTILAAVTLCFASSQNITEEFYQSTCSAVSKGYLSALRTGWYCSVITIELSNIKENKCNGTDAKVKLIKQELDKYKNAVTELQLLMQSTCAANSRARRELPRFMNYTLNNTKNTNVTLSKKRKRRFLGFLLGVGSAIASGCAVSKVLHLEGEVNKIKSALLSTNKAVVSLSNGVSVLTMKVLDLKNYIDKQLLPIVNKQSCSISNIETVIEFQQKNNRLLEITREFSVNAGVTTPVSTYMLTNSELLSLINDMPITNDQKKLMSSNVQIVRQQSYSIMSIIKEELLAYVVQLPLYGVIDTPCWKLHTSPLCTTNTKEGSNICLTRTDRGWYCDNAGSVSFFPQAETCKVQSNRVFCDTMNSLTLPSEVNLCNIDIFNPKYDCKIMTSKTDVSSSVITSLGAIVSCYGKTKCTASNKNRGIIKTFSNGCDYVSNKGVDTVSVGNTLYYVNKQEGKSLYVKGEPIINFYDPLVFPSDEFDASISQVNEKINQSLAFIRKSDELLHNVNAGKSTTNIMITTIIIVIIVILLALIAVGLLLY

SEQ ID NO: 82 - protein, 549 aa, synthetic construct
MELLIHRSSAIFLTLAINALYLTSSQNITEEFYQSTCSAVSRGYFSALRTGWYCSVITIELSNIKETKCNGTDTKVKLIKQELDKYKNAVTELQLLMQNTCAANNRARREAPQYMNYTINTTKNLNVSISKKRKRRFLGFLLGVGSAIASGCAVSKVLHLEGEVNKIKNALLSTNKAVVSLSNGVSVLTMKVLDLKNYINNQLLPIVNQQSCRISNIETVIEFQQKNSRLLEITREFSVNAGVTTPLSTYMLTNSELLSLINDMPITNDQKKLMSSNVQIVRQQSYSIMSIIKEELLAYVVQLPIYGVIDTPCWKLHTSPLCTTNIKEGSNICLTRTDRGWYCDNAGSVSFFPQADTCKVQSNRVFCDTMNSLTLPSEVSLCNTDIFNSKYDCKIMTSKTDISSSVITSLGAIVSCYGKTKCTASNKNRGIIKTFSNGCDYVSNKGVDTVSVGNTLYYVNKLEGKNLYVKGEPIINYYDPLVFPSDEFDASISQVNEKINQSLAFIRRSDELLHNVNTGKSTTNIMITAIIIVIIVVLLSLIAIGLLLY

SEQ ID NO: 83 - protein, 549 aa, synthetic construct
MELPILKTNAITTILAAVTLCFASSQNITEEFYQSTCSAVSKGYLSALRTGWYASVITIELSNIKENKCNGTDAKVKLIKQELDKYKNAVTELQLLMQSTCAANSRARRELPRFMNYTLNNTKNTNVTLSKKRKRRFLGFLLGVGSAIASGCAVSKVLHLEGEVNKIKSALLSTNKAVVSLSNGVSVLTMKVLDLKNYIDKQLLPIVNKQSCSISNIETVIEFQQKNNRLLEITREFSVNAGVTTPVSTYMLTNSELLSLINDMPITNDQKKLMSSNVQIVRQQSYSIMSIIKEELLAYVVQLPLYGVIDTPCWKLHTSPLCTTNTKEGSNICLTRTDRGWYCDNAGSVSFFPQAETCKVQSNRVFCDTMNSLTLPSEVNLCNIDIFNPKYDCKIMTSKTDVSSSVITSLGAIVSCYGKTKCTASNKNRGIIKTFSNGCDYVSNKGVDTVSVGNTLYYVNKQEGKSLYVKGEPIINFYDPLVFPSDEFDASISQVNEKINQSLAFIRKSDELLHNVNAGKSTTNIMITTIIIVIIVILLALIAVGLLLY

SEQ ID NO: 84 - protein, 549 aa, synthetic construct
MELLIHRSSAIFLTLAINALYLTSSQNITEEFYQSTCSAVSRGYFSALRTGWYASVITIELSNIKETKCNGTDTKVKLIKQELDKYKNAVTELQLLMQNTCAANNRARREAPQYMNYTINTTKNLNVSISKKRKRRFLGFLLGVGSAIASGCAVSKVLHLEGEVNKIKNALLSTNKAVVSLSNGVSVLTMKVLDLKNYINNQLLPIVNQQSCRISNIETVIEFQQKNSRLLEITREFSVNAGVTTPLSTYMLTNSELLSLINDMPITNDQKKLMSSNVQIVRQQSYSIMSIIKEELLAYVVQLPIYGVIDTPCWKLHTSPLCTTNIKEGSNICLTRTDRGWYCDNAGSVSFFPQADTCKVQSNRVFCDTMNSLTLPSEVSLCNTDIFNSKYDCKIMTSKTDISSSVITSLGAIVSCYGKTKCTASNKNRGIIKTFSNGCDYVSNKGVDTVSVGNTLYYVNKLEGKNLYVKGEPIINYYDPLVFPSDEFDASISQVNEKINQSLAFIRRSDELLHNVNTGKSTTNIMITAIIIVIIVVLLSLIAIGLLLY

SEQ ID NO: 85 - protein, 549 aa, unidentified
MELPILKTNAITTILAAVTLCFASSQNITEEFYQSTCSAVSKGYLSALRTGWYVSVITIELSNIKENKCNGTDAKVKLIKQELDKYKNAVTELQLLMQSTCAANSRARRELPRFMNYTLNNTKNTNVTLSKKRKRRFLGFLLGVGSAIASGCAVSKVLHLEGEVNKIKSALLSTNKAVVSLSNGVSVLTFKVLDLKNYIDKQLLPIVNKQSCSISNIETVIEFQQKNNRLLEITREFSVNAGVTTPVSTYMLTNSELLSLINDMPITNDQKKLMSSNVQIVRQQSYSIMSIIKEELLAYVVQLPLYGVIDTPCWKLHTSPLCTTNTKEGSNICLTRTDRGWYCDNAGSVSFFPQAETCKVQSNRVFCDTMNSLTLPSEVNLCNIDIFNPKYDCKIMTSKTDVSSSVITSLGAIVSCYGKTKCTASNKNRGIIKTFSNGCDYVSNKGVDTVSVGNTLYYVNKQEGKSLYVKGEPIINFYDPLVFPSDEFDASISQVNEKINQSLAFIRKSDELLHNVNAGKSTTNIMITTIIIVIIVILLALIAVGLLLY

SEQ ID NO: 86 - protein, 549 aa, synthetic construct
MELLIHRSSAIFLTLAINALYLTSSQNITEEFYQSTCSAVSRGYFSALRTGWYVSVITIELSNIKETKCNGTDTKVKLIKQELDKYKNAVTELQLLMQNTCAANNRARREAPQYMNYTINTTKNLNVSISKKRKRRFLGFLLGVGSAIASGCAVSKVLHLEGEVNKIKNALLSTNKAVVSLSNGVSVLTFKVLDLKNYINNQLLPIVNQQSCRISNIETVIEFQQKNSRLLEITREFSVNAGVTTPLSTYMLTNSELLSLINDMPITNDQKKLMSSNVQIVRQQSYSIMSIIKEELLAYVVQLPIYGVIDTPCWKLHTSPLCTTNIKEGSNICLTRTDRGWYCDNAGSVSFFPQADTCKVQSNRVFCDTMNSLTLPSEVSLCNTDIFNSKYDCKIMTSKTDISSSVITSLGAIVSCYGKTKCTASNKNRGIIKTFSNGCDYVSNKGVDTVSVGNTLYYVNKLEGKNLYVKGEPIINYYDPLVFPSDEFDASISQVNEKINQSLAFIRRSDELLHNVNTGKSTTNIMITAIIIVIIVVLLSLIAIGLLLY

SEQ ID NO: 87 - protein, 549 aa, synthetic construct
MELPILKTNAITTILAAVTLCFASSQNITEEFYQSTCSAVSKGYLSALRTGWYFSVITIELSNIKENKCNGTDAKVKLIKQELDKYKNAVTELQLLMQSTCAANSRARRELPRFMNYTLNNTKNTNVTLSKKRKRRFLGFLLGVGSAIASGCAVSKVLHLEGEVNKIKSALLSTNKAVVSLSNGVSVLTFKVLDLKNYIDKQLLPIVNKQSCSISNIETVIEFQQKNNRLLEITREFSVNAGVTTPVSTYMLTNSELLSLINDMPITNDQKKLMSSNVQIVRQQSYSIMSIIKEELLAYVVQLPLYGVIDTPCWKLHTSPLCTTNTKEGSNICLTRTDRGWYCDNAGSVSFFPQAETCKVQSNRVFCDTMNSLTLPSEVNLCNIDIFNPKYDCKIMTSKTDVSSSVITSLGAIVSCYGKTKCTASNKNRGIIKTFSNGCDYVSNKGVDTVSVGNTLYYVNKQEGKSLYVKGEPIINFYDPLVFPSDEFDASISQVNEKINQSLAFIRKSDELLHNVNAGKSTTNIMITTIIIVIIVILLALIAVGLLLY

SEQ ID NO: 88 - protein, 549 aa, synthetic construct
MELLIHRSSAIFLTLAINALYLTSSQNITEEFYQSTCSAVSRGYFSALRTGWYFSVITIELSNIKETKCNGTDTKVKLIKQELDKYKNAVTELQLLMQNTCAANNRARREAPQYMNYTINTTKNLNVSISKKRKRRFLGFLLGVGSAIASGCAVSKVLHLEGEVNKIKNALLSTNKAVVSLSNGVSVLTFKVLDLKNYINNQLLPIVNQQSCRISNIETVIEFQQKNSRLLEITREFSVNAGVTTPLSTYMLTNSELLSLINDMPITNDQKKLMSSNVQIVRQQSYSIMSIIKEELLAYVVQLPIYGVIDTPCWKLHTSPLCTTNIKEGSNICLTRTDRGWYCDNAGSVSFFPQADTCKVQSNRVFCDTMNSLTLPSEVSLCNTDIFNSKYDCKIMTSKTDISSSVITSLGAIVSCYGKTKCTASNKNRGIIKTFSNGCDYVSNKGVDTVSVGNTLYYVNKLEGKNLYVKGEPIINYYDPLVFPSDEFDASISQVNEKINQSLAFIRRSDELLHNVNTGKSTTNIMITAIIIVIIVVLLSLIAIGLLLY

SEQ ID NO: 89 - protein, 549 aa, synthetic construct
MELPILKTNAITTILAAVTLCFASSQNITEEFYQSTCSAVSKGYLSALRTGWYCSVITIELSNIKENKCNGTDAKVKLIKQELDKYKNAVTELQLLMQSTCAANSRARRELPRFMNYTLNNTKNTNVTLSKKRKRRFLGFLLGVGSAIASGCAVSKVLHLEGEVNKIKSALLSTNKAVVSLSNGVSVLTFKVLDLKNYIDKQLLPIVNKQSCSISNIETVIEFQQKNNRLLEITREFSVNAGVTTPVSTYMLTNSELLSLINDMPITNDQKKLMSSNVQIVRQQSYSIMSIIKEELLAYVVQLPLYGVIDTPCWKLHTSPLCTTNTKEGSNICLTRTDRGWYCDNAGSVSFFPQAETCKVQSNRVFCDTMNSLTLPSEVNLCNIDIFNPKYDCKIMTSKTDVSSSVITSLGAIVSCYGKTKCTASNKNRGIIKTFSNGCDYVSNKGVDTVSVGNTLYYVNKQEGKSLYVKGEPIINFYDPLVFPSDEFDASISQVNEKINQSLAFIRKSDELLHNVNAGKSTTNIMITTIIIVIIVILLALIAVGLLLY

SEQ ID NO: 90 - protein, 549 aa, synthetic construct
MELLIHRSSAIFLTLAINALYLTSSQNITEEFYQSTCSAVSRGYFSALRTGWYCSVITIELSNIKETKCNGTDTKVKLIKQELDKYKNAVTELQLLMQNTCAANNRARREAPQYMNYTINTTKNLNVSISKKRKRRFLGFLLGVGSAIASGCAVSKVLHLEGEVNKIKNALLSTNKAVVSLSNGVSVLTFKVLDLKNYINNQLLPIVNQQSCRISNIETVIEFQQKNSRLLEITREFSVNAGVTTPLSTYMLTNSELLSLINDMPITNDQKKLMSSNVQIVRQQSYSIMSIIKEELLAYVVQLPIYGVIDTPCWKLHTSPLCTTNIKEGSNICLTRTDRGWYCDNAGSVSFFPQADTCKVQSNRVFCDTMNSLTLPSEVSLCNTDIFNSKYDCKIMTSKTDISSSVITSLGAIVSCYGKTKCTASNKNRGIIKTFSNGCDYVSNKGVDTVSVGNTLYYVNKLEGKNLYVKGEPIINYYDPLVFPSDEFDASISQVNEKINQSLAFIRRSDELLHNVNTGKSTTNIMITAIIIVIIVVLLSLIAIGLLLY

SEQ ID NO: 91 - protein, 549 aa, synthetic construct
MELPILKTNAITTILAAVTLCFASSQNITEEFYQSTCSAVSKGYLSALRTGWYASVITIELSNIKENKCNGTDAKVKLIKQELDKYKNAVTELQLLMQSTCAANSRARRELPRFMNYTLNNTKNTNVTLSKKRKRRFLGFLLGVGSAIASGCAVSKVLHLEGEVNKIKSALLSTNKAVVSLSNGVSVLTFKVLDLKNYIDKQLLPIVNKQSCSISNIETVIEFQQKNNRLLEITREFSVNAGVTTPVSTYMLTNSELLSLINDMPITNDQKKLMSSNVQIVRQQSYSIMSIIKEELLAYVVQLPLYGVIDTPCWKLHTSPLCTTNTKEGSNICLTRTDRGWYCDNAGSVSFFPQAETCKVQSNRVFCDTMNSLTLPSEVNLCNIDIFNPKYDCKIMTSKTDVSSSVITSLGAIVSCYGKTKCTASNKNRGIIKTFSNGCDYVSNKGVDTVSVGNTLYYVNKQEGKSLYVKGEPIINFYDPLVFPSDEFDASISQVNEKINQSLAFIRKSDELLHNVNAGKSTTNIMITTIIIVIIVILLALIAVGLLLY

SEQ ID NO: 92 - protein, 549 aa, synthetic construct
MELLIHRSSAIFLTLAINALYLTSSQNITEEFYQSTCSAVSRGYFSALRTGWYASVITIELSNIKETKCNGTDTKVKLIKQELDKYKNAVTELQLLMQNTCAANNRARREAPQYMNYTINTTKNLNVSISKKRKRRFLGFLLGVGSAIASGCAVSKVLHLEGEVNKIKNALLSTNKAVVSLSNGVSVLTFKVLDLKNYINNQLLPIVNQQSCRISNIETVIEFQQKNSRLLEITREFSVNAGVTTPLSTYMLTNSELLSLINDMPITNDQKKLMSSNVQIVRQQSYSIMSIIKEELLAYVVQLPIYGVIDTPCWKLHTSPLCTTNIKEGSNICLTRTDRGWYCDNAGSVSFFPQADTCKVQSNRVFCDTMNSLTLPSEVSLCNTDIFNSKYDCKIMTSKTDISSSVITSLGAIVSCYGKTKCTASNKNRGIIKTFSNGCDYVSNKGVDTVSVGNTLYYVNKLEGKNLYVKGEPIINYYDPLVFPSDEFDASISQVNEKINQSLAFIRRSDELLHNVNTGKSTTNIMITAIIIVIIVVLLSLIAIGLLLY

SEQ ID NO: 93 - protein, 549 aa, synthetic construct
MELPILKTNAITTILAAVTLCFASSQNITEEFYQSTCSAVSKGYLSALRTGWYVSVITIELSNIKENKCNGTDAKVKLIKQELDKYKNAVTELQLLMQSTPCANSRARRELPRFMNYTLNNTKNTNVTLSKKRKRRFLGFLLGVGSAIASGCAVSKVLHLEGEVNKIKSALLSTNKAVVSLSNGVSVLTIKVLDLKNYIDKQLLPIVNKQSCSISNIETVIEFQQKNNRLLEITREFSVNAGVTTPVSTYMLTNSELLSLINDMPITNDQKKLMSSNVQIVRQQSYSIMSIIKEELLAYVVQLPLYGVIDTPCWKLHTSPLCTTNTKEGSNICLTRTDRGWYCDNAGSVSFFPQAETCKVQSNRVFCDTMNSLTLPSEVNLCNIDIFNPKYDCKIMTSKTDVSSSVITSLGAIVSCYGKTKCTASNKNRGIIKTFSNGCDYVSNKGVDTVSVGNTLYYVNKQEGKSLYVKGEPIINFYDPLVFPSDEFDASISQVNEKINQSLAFIRKSDELLHNVNAGKSTTNIMITTIIIVIIVILLALIAVGLLLY

SEQ ID NO: 94 - protein, 549 aa, synthetic construct
MELLIHRSSAIFLTLAINALYLTSSQNITEEFYQSTCSAVSRGYFSALRTGWYVSVITIELSNIKETKCNGTDTKVKLIKQELDKYKNAVTELQLLMQNTPCANNRARREAPQYMNYTINTTKNLNVSISKKRKRRFLGFLLGVGSAIASGCAVSKVLHLEGEVNKIKNALLSTNKAVVSLSNGVSVLTIKVLDLKNYINNQLLPIVNQQSCRISNIETVIEFQQKNSRLLEITREFSVNAGVTTPLSTYMLTNSELLSLINDMPITNDQKKLMSSNVQIVRQQSYSIMSIIKEELLAYVVQLPIYGVIDTPCWKLHTSPLCTTNIKEGSNICLTRTDRGWYCDNAGSVSFFPQADTCKVQSNRVFCDTMNSLTLPSEVSLCNTDIFNSKYDCKIMTSKTDISSSVITSLGAIVSCYGKTKCTASNKNRGIIKTFSNGCDYVSNKGVDTVSVGNTLYYVNKLEGKNLYVKGEPIINYYDPLVFPSDEFDASISQVNEKINQSLAFIRRSDELLHNVNTGKSTTNIMITAIIIVIIVVLLSLIAIGLLLY

SEQ ID NO: 95 - protein, 549 aa, synthetic construct
MELPILKTNAITTILAAVTLCFASSQNITEEFYQSTCSAVSKGYLSALRTGWYFSVITIELSNIKENKCNGTDAKVKLIKQELDKYKNAVTELQLLMQSTPCANSRARRELPRFMNYTLNNTKNTNVTLSKKRKRRFLGFLLGVGSAIASGCAVSKVLHLEGEVNKIKSALLSTNKAVVSLSNGVSVLTIKVLDLKNYIDKQLLPIVNKQSCSISNIETVIEFQQKNNRLLEITREFSVNAGVTTPVSTYMLTNSELLSLINDMPITNDQKKLMSSNVQIVRQQSYSIMSIIKEELLAYVVQLPLYGVIDTPCWKLHTSPLCTTNTKEGSNICLTRTDRGWYCDNAGSVSFFPQAETCKVQSNRVFCDTMNSLTLPSEVNLCNIDIFNPKYDCKIMTSKTDVSSSVITSLGAIVSCYGKTKCTASNKNRGIIKTFSNGCDYVSNKGVDTVSVGNTLYYVNKQEGKSLYVKGEPIINFYDPLVFPSDEFDASISQVNEKINQSLAFIRKSDELLHNVNAGKSTTNIMITTIIIVIIVILLALIAVGLLLY

SEQ ID NO: 96 - protein, 549 aa, synthetic construct
MELLIHRSSAIFLTLAINALYLTSSQNITEEFYQSTCSAVSRGYFSALRTGWYFSVITIELSNIKETKCNGTDTKVKLIKQELDKYKNAVTELQLLMQNTPCANNRARREAPQYMNYTINTTKNLNVSISKKRKRRFLGFLLGVGSAIASGCAVSKVLHLEGEVNKIKNALLSTNKAVVSLSNGVSVLTIKVLDLKNYINNQLLPIVNQQSCRISNIETVIEFQQKNSRLLEITREFSVNAGVTTPLSTYMLTNSELLSLINDMPITNDQKKLMSSNVQIVRQQSYSIMSIIKEELLAYVVQLPIYGVIDTPCWKLHTSPLCTTNIKEGSNICLTRTDRGWYCDNAGSVSFFPQADTCKVQSNRVFCDTMNSLTLPSEVSLCNTDIFNSKYDCKIMTSKTDISSSVITSLGAIVSCYGKTKCTASNKNRGIIKTFSNGCDYVSNKGVDTVSVGNTLYYVNKLEGKNLYVKGEPIINYYDPLVFPSDEFDASISQVNEKINQSLAFIRRSDELLHNVNTGKSTTNIMITAIIIVIIVVLLSLIAIGLLLY

SEQ ID NO: 97 - protein, 549 aa, synthetic construct
MELPILKTNAITTILAAVTLCFASSQNITEEFYQSTCSAVSKGYLSALRTGWYCSVITIELSNIKENKCNGTDAKVKLIKQELDKYKNAVTELQLLMQSTPCANSRARRELPRFMNYTLNNTKNTNVTLSKKRKRRFLGFLLGVGSAIASGCAVSKVLHLEGEVNKIKSALLSTNKAVVSLSNGVSVLTIKVLDLKNYIDKQLLPIVNKQSCSISNIETVIEFQQKNNRLLEITREFSVNAGVTTPVSTYMLTNSELLSLINDMPITNDQKKLMSSNVQIVRQQSYSIMSIIKEELLAYVVQLPLYGVIDTPCWKLHTSPLCTTNTKEGSNICLTRTDRGWYCDNAGSVSFFPQAETCKVQSNRVFCDTMNSLTLPSEVNLCNIDIFNPKYDCKIMTSKTDVSSSVITSLGAIVSCYGKTKCTASNKNRGIIKTFSNGCDYVSNKGVDTVSVGNTLYYVNKQEGKSLYVKGEPIINFYDPLVFPSDEFDASISQVNEKINQSLAFIRKSDELLHNVNAGKSTTNIMITTIIIVIIVILLALIAVGLLLY

SEQ ID NO: 98 - protein, 549 aa, synthetic construct
MELLIHRSSAIFLTLAINALYLTSSQNITEEFYQSTCSAVSRGYFSALRTGWYCSVITIELSNIKETKCNGTDTKVKLIKQELDKYKNAVTELQLLMQNTPCANNRARREAPQYMNYTINTTKNLNVSISKKRKRRFLGFLLGVGSAIASGCAVSKVLHLEGEVNKIKNALLSTNKAVVSLSNGVSVLTIKVLDLKNYINNQLLPIVNQQSCRISNIETVIEFQQKNSRLLEITREFSVNAGVTTPLSTYMLTNSELLSLINDMPITNDQKKLMSSNVQIVRQQSYSIMSIIKEELLAYVVQLPIYGVIDTPCWKLHTSPLCTTNIKEGSNICLTRTDRGWYCDNAGSVSFFPQADTCKVQSNRVFCDTMNSLTLPSEVSLCNTDIFNSKYDCKIMTSKTDISSSVITSLGAIVSCYGKTKCTASNKNRGIIKTFSNGCDYVSNKGVDTVSVGNTLYYVNKLEGKNLYVKGEPIINYYDPLVFPSDEFDASISQVNEKINQSLAFIRRSDELLHNVNTGKSTTNIMITAIIIVIIVVLLSLIAIGLLLY

SEQ ID NO: 99 - protein, 549 aa, synthetic construct
MELPILKTNAITTILAAVTLCFASSQNITEEFYQSTCSAVSKGYLSALRTGWYASVITIELSNIKENKCNGTDAKVKLIKQELDKYKNAVTELQLLMQSTPCANSRARRELPRFMNYTLNNTKNTNVTLSKKRKRRFLGFLLGVGSAIASGCAVSKVLHLEGEVNKIKSALLSTNKAVVSLSNGVSVLTIKVLDLKNYIDKQLLPIVNKQSCSISNIETVIEFQQKNNRLLEITREFSVNAGVTTPVSTYMLTNSELLSLINDMPITNDQKKLMSSNVQIVRQQSYSIMSIIKEELLAYVVQLPLYGVIDTPCWKLHTSPLCTTNTKEGSNICLTRTDRGWYCDNAGSVSFFPQAETCKVQSNRVFCDTMNSLTLPSEVNLCNIDIFNPKYDCKIMTSKTDVSSSVITSLGAIVSCYGKTKCTASNKNRGIIKTFSNGCDYVSNKGVDTVSVGNTLYYVNKQEGKSLYVKGEPIINFYDPLVFPSDEFDASISQVNEKINQSLAFIRKSDELLHNVNAGKSTTNIMITTIIIVIIVILLALIAVGLLLY

SEQ ID NO: 100 - protein, 549 aa, synthetic construct
MELLIHRSSAIFLTLAINALYLTSSQNITEEFYQSTCSAVSRGYFSALRTGWYASVITIELSNIKETKCNGTDTKVKLIKQELDKYKNAVTELQLLMQNTPCANNRARREAPQYMNYTINTTKNLNVSISKKRKRRFLGFLLGVGSAIASGCAVSKVLHLEGEVNKIKNALLSTNKAVVSLSNGVSVLTIKVLDLKNYINNQLLPIVNQQSCRISNIETVIEFQQKNSRLLEITREFSVNAGVTTPLSTYMLTNSELLSLINDMPITNDQKKLMSSNVQIVRQQSYSIMSIIKEELLAYVVQLPIYGVIDTPCWKLHTSPLCTTNIKEGSNICLTRTDRGWYCDNAGSVSFFPQADTCKVQSNRVFCDTMNSLTLPSEVSLCNTDIFNSKYDCKIMTSKTDISSSVITSLGAIVSCYGKTKCTASNKNRGIIKTFSNGCDYVSNKGVDTVSVGNTLYYVNKLEGKNLYVKGEPIINYYDPLVFPSDEFDASISQVNEKINQSLAFIRRSDELLHNVNTGKSTTNIMITAIIIVIIVVLLSLIAIGLLLY

SEQ ID NO: 101 - protein, 544 aa, synthetic construct
MELPILKTNAITTILAAVTLCFASSQNITEEFYQSTCSAVSKGYLSALRTGWYHSVITIELSNIKENKCNGTDAKVKLIKQELDKYKNAVTELQLLMQSTPACNSRARRELPRFMNYTLNNTKNTNVTLSKKRKRRFLGFLLGVGSACASGIAVSKVLHLEGEVNKIKSALLSTNKAVVSLSNGVSVLTIKVLDLKNYIDKQLLPIVNKQSCSISNIETVIEFQQKNNRLLEITREFSVNAGVTTPVSTYMLTNSELLSLINDMPITNDQKKLMSSNVQIVRQQSYSIMSIIKEEILAYVVQLPLYGVIDTPCWKLHTSPLCTTNTKEGSNICLTRTDRGWYCDNAGSVSFFPQAETCKVQSNRVFCDTMNSLTLPSEVNLCNIDIFNPKYDCKIMTSKTDVSSSVITSLGAIVSCYGKTKCTASNKNRGIIKTFSNGCDYVSNKGVDTVSVGNTLYYVNKQEGKSLYVKGEPIINFYDPLVFPSSEFDASISQVNEKINQSLAFIRKSDELLSAIGGYIPEAPRDGQAYVRKDGEWVLLSTFL

SEQ ID NO: 102 - protein, 544 aa, synthetic construct
MELLIHRSSAIFLTLAINALYLTSSQNITEEFYQSTCSAVSRGYFSALRTGWYHSVITIELSNIKETKCNGTDTKVKLIKQELDKYKNAVTELQLLMQNTPACNNRARREAPQYMNYTINTTKNLNVSISKKRKRRFLGFLLGVGSACASGIAVSKVLHLEGEVNKIKNALLSTNKAVVSLSNGVSVLTIKVLDLKNYINNQLLPIVNQQSCRISNIETVIEFQQKNSRLLEITREFSVNAGVTTPLSTYMLTNSELLSLINDMPITNDQKKLMSSNVQIVRQQSYSIMSIIKEEILAYVVQLPIYGVIDTPCWKLHTSPLCTTNIKEGSNICLTRTDRGWYCDNAGSVSFFPQADTCKVQSNRVFCDTMNSLTLPSEVSLCNTDIFNSKYDCKIMTSKTDISSSVITSLGAIVSCYGKTKCTASNKNRGIIKTFSNGCDYVSNKGVDTVSVGNTLYYVNKLEGKNLYVKGEPIINYYDPLVFPSSEFDASISQVNEKINQSLAFIRRSDELLSAIGGYIPEAPRDGQAYVRKDGEWVLLSTFL

SEQ ID NO: 103 - protein, 549 aa, synthetic construct
MELPILKTNAITTILAAVTLCFASSQNITEEFYQSTCSAVSKGYLSALRTGWYHSVITIELSNIKENKCNGTDAKVKLIKQELDKYKNAVTELQLLMQSTPACNSRARRELPRFMNYTLNNTKNTNVTLSKKRKRRFLGFLLGVGSACASGIAVSKVLHLEGEVNKIKSALLSTNKAVVSLSNGVSVLTIKVLDLKNYIDKQLLPIVNKQSCSISNIETVIEFQQKNNRLLEITREFSVNAGVTTPVSTYMLTNSELLSLINDMPITNDQKKLMSSNVQIVRQQSYSIMSIIKEEILAYVVQLPLYGVIDTPCWKLHTSPLCTTNTKEGSNICLTRTDRGWYCDNAGSVSFFPQAETCKVQSNRVFCDTMNSLTLPSEVNLCNIDIFNPKYDCKIMTSKTDVSSSVITSLGAIVSCYGKTKCTASNKNRGIIKTFSNGCDYVSNKGVDTVSVGNTLYYVNKQEGKSLYVKGEPIINFYDPLVFPSSEFDASISQVNEKINQSLAFIRKSDELLHNVNAGKSTTNIMITTIIIVIIVILLALIAVGLLLY

SEQ ID NO: 104 - protein, 549 aa, synthetic construct
MELLIHRSSAIFLTLAINALYLTSSQNITEEFYQSTCSAVSRGYFSALRTGWYHSVITIELSNIKETKCNGTDTKVKLIKQELDKYKNAVTELQLLMQNTPACNNRARREAPQYMNYTINTTKNLNVSISKKRKRRFLGFLLGVGSACASGIAVSKVLHLEGEVNKIKNALLSTNKAVVSLSNGVSVLTIKVLDLKNYINNQLLPIVNQQSCRISNIETVIEFQQKNSRLLEITREFSVNAGVTTPLSTYMLTNSELLSLINDMPITNDQKKLMSSNVQIVRQQSYSIMSIIKEEILAYVVQLPIYGVIDTPCWKLHTSPLCTTNIKEGSNICLTRTDRGWYCDNAGSVSFFPQADTCKVQSNRVFCDTMNSLTLPSEVSLCNTDIFNSKYDCKIMTSKTDISSSVITSLGAIVSCYGKTKCTASNKNRGIIKTFSNGCDYVSNKGVDTVSVGNTLYYVNKLEGKNLYVKGEPIINYYDPLVFPSSEFDASISQVNEKINQSLAFIRRSDELLHNVNTGKSTTNIMITAIIIVIIVVLLSLIAIGLLLY

SEQ ID NO: 105 - DNA, 1635 bp, synthetic construct
  source 1..1635: mol_type = other DNA
atggaactgcccatcctgaaaacaaacgccatcaccaccatcctggccgccgtgacactgtgttttgccagcagccagaacatcaccgaagagttctaccagagcacctgtagcgccgtgtctaagggctatctgtcttgcctgagaaccggctggtatcacagcgtgatcaccatcgagctgagcaacatcaaagaaaacaagtgcaacggcaccgacgccaaagtgaagctgatcaagcaagagctggacaagtacaagaacgccgtgaccgaactgcagctgctgatgcagtctacccctgccgccaatagcagagccagacgggaactgcctagattcatgaactacaccctgaacaacaccaagaacaccaacgtgaccctgagcaagaagcggaagcggagattcctgggctttctgctcggatgcggaagcgccattgcctctggaattgccgtgtccaaggtgctgcatctggaaggcgaagtgaacaagatcaagagcgccctgctgagcaccaacaaggccgtggtttctctgagcaatggcgtgtccgtgctgacctctaaggtgctggacctgaagaactacatcgacaaacagctgctgcccatcgtcaacaagcagagctgcagcatcagcaacatcgagacagtgatcgagttccagcagaagaacaaccggctgctggaaatcacccgcgagttttctgtgaatgccggcgtgaccacacctgtgtccacctacatgctgaccaacagcgagctgctgtccctgatcaacgacatgcccatcaccaacgaccagaaaaagctgatgagcagcaacgtgcagatcgtgcggcagcagagctactccatcatgagcattatcaaagaagaggtgctggcctacgtggtgcagctgcctctgtatggcgtgtgcgataccccttgctggaagctgcacacaagccctctgtgcaccaccaacaccaaagagggctccaacatctgcctgaccagaaccgatagaggctggtactgcgataatgccggcagcgtcagcttcttcccacaagccgagacatgcaaggtgcagagcaacagagtgttctgcgataccatgaacagcctgacactgccctccgaagtgaatctgtgcaatatcgacatcttcaacccgaagtacgactgcaagatcatgaccagcaagaccgacgtgtcaagctcctgcatcacatctctgggcgccatcgtgtcctgctacggcaagacaaagtgcaccgccagcaacaagaaccggggcatcatcaagaccttcagcaacggctgcgactacgtgtccaacaaaggcgtggacaccgtgtctgtgggcaacaccctgtactacgtgaacaagcaagaaggcaagagcctgtacgtgaagggcgagcccatcatcaacttctacgaccctctggtgttccccagcagcgagtttgatgccagcatctcccaagtgaacgagaagatcaaccagagcctggccttcatcagaaagtccgatgagctgctgagcgccatcggcggctatatccctgaagctcctagagatggacaggcctatgtgcggaaggatggcgaatgggtgctgctgtctaccttcctgtga

SEQ ID NO: 106 - DNA, 1635 bp, synthetic construct
  source 1..1635: mol_type = other DNA
atggaactgctgattcacagaagcagcgccatctttctgaccctggccatcaatgccctgtacctgaccagcagccagaacatcaccgaagagttctaccagagcacctgtagcgccgtgtccagaggctacttttcttgcctgagaaccggctggtatcacagcgtgatcaccatcgagctgagcaacatcaaagaaacaaagtgcaacggcaccgacaccaaagtgaagctgatcaagcaagagctggacaagtacaagaacgccgtgaccgaactgcagctgctgatgcagaatacccctgccgccaacaaccgggccagaagagaagcccctcagtacatgaactacaccatcaacaccaccaagaacctgaacgtgtccatcagcaagaagcggaagcggagattcctgggctttctgctcggatgcggaagcgccattgcctctggaattgccgtgtctaaggtgctgcacctggaaggcgaagtgaacaagatcaagaatgccctgctgagcaccaacaaggccgtggtgtctctgtctaatggcgtgtccgtgctgaccagcaaggtgctggacctgaagaactacatcaacaaccagctgctgcccatcgtgaaccagcagagctgccggatcagcaacatcgagacagtgatcgagttccagcagaagaacagcagactgctggaaatcacccgcgagttttccgtgaatgccggcgtgacaacacccctgagcacctacatgctgaccaacagcgagctgctgtccctgatcaacgacatgcccatcaccaacgaccagaaaaagctgatgagcagcaacgtgcagatcgtgcggcagcagtcctacagcatcatgagcattatcaaagaagaggtgctggcctacgtggtgcagctgcctatctacggcgtgtgcgataccccttgctggaagctgcacacaagccctctgtgcaccaccaatatcaaagagggctccaacatctgcctgaccagaaccgatagaggctggtactgcgataatgccggcagcgtcagcttcttcccacaagccgatacctgcaaggtgcagagcaacagagtgttctgcgataccatgaacagcctgacactgcccagcgaggtgtccctgtgcaacaccgacatcttcaactctaagtacgactgcaagatcatgacctccaagaccgacatcagctcctcctgcatcacatctctgggcgccatcgtgtcctgctacggcaagacaaagtgtaccgccagcaacaagaaccggggcatcatcaagaccttcagcaacggctgcgactacgtgtccaacaaaggcgtggacaccgtgtctgtgggcaacaccctgtactacgtgaacaagctggaaggcaagaatctgtacgtgaagggcgagcccatcatcaactactacgaccctctggtgttccccagcagcgagtttgatgccagcatcagccaagtgaacgagaagatcaaccagagcctggccttcatccgcagatccgatgaactgctgtctgccatcggcggctatatccccgaagctcctagagatggacaggcctatgtgcggaaggatggcgaatgggtgctgctgtctaccttcctgtga

SEQ ID NO: 107 - DNA, 1635 bp, synthetic construct
  source 1..1635: mol_type = other DNA
atggaactgcccatcctgaaaacaaacgccatcaccaccatcctggccgccgtgacactgtgttttgccagcagccagaacatcaccgaagagttctaccagagcacctgtagcgccgtgtctaagggctatctgtcttgcctgagaaccggctggtatcacagcgtgatcaccatcgagctgagcaacatcaaagaaaacaagtgcaacggcaccgacgccaaagtgaagctgatcaagcaagagctggacaagtacaagaacgccgtgaccgaactgcagctgctgatgcagtctacccctgccgccaatagcagagccagacgggaactgcctagattcatgaactacaccctgaacaacaccaagaacaccaacgtgaccctgagcaagaagcggaagcggagattcctgggctttctgctcggagtgggaagcgccattgcctctggaattgccgtgtccaaggtgctgcatctggaaggcgaagtgaacaagatcaagagcgccctgctgagcaccaacaaggccgtggtttctctgagcaatggcgtgtccgtgctgacctctaaggtgctggacctgaagaactacatcgacaaacagctgctgcccatcgtcaacaagcagagctgcagcatcagcaacatcgagacagtgatcgagttccagcagaagaacaaccggctgctggaaatcacccgcgagttttctgtgaatgccggcgtgaccacacctgtgtccacctacatgctgaccaacagcgagctgctgtccctgatcaacgacatgcccatcaccaacgaccagaaaaagctgatgagcagcaacgtgcagatcgtgcggcagcagagctactccatcatgagcattatcaaagaagaggtgctggcctacgtggtgcagctgcctctgtatggcgtgtgcgataccccttgctggaagctgcacacaagccctctgtgcaccaccaacaccaaagagggctccaacatctgcctgaccagaaccgatagaggctggtactgcgataatgccggcagcgtcagcttcttcccacaagccgagacatgcaaggtgcagagcaacagagtgttctgcgataccatgaacagcctgacactgccctccgaagtgaatctgtgcaatatcgacatcttcaacccgaagtacgactgcaagatcatgaccagcaagaccgacgtgtcaagctccgtgatcacatctctgggcgccatcgtgtcctgctacggcaagacaaagtgcaccgccagcaacaagaaccggggcatcatcaagaccttcagcaacggctgcgactacgtgtccaacaaaggcgtggacaccgtgtctgtgggcaacaccctgtactacgtgaacaagcaagaaggcaagagcctgtacgtgaagggcgagcccatcatcaacttctacgaccctctggtgttccccagcagcgagtttgatgccagcatctcccaagtgaacgagaagatcaaccagagcctggccttcatcagaaagtccgatgagctgctgagcgccatcggcggctatatccctgaagctcctagagatggacaggcctatgtgcggaaggatggcgaatgggtgctgctgtctaccttcctgtga

SEQ ID NO: 108 - DNA, 1635 bp, synthetic construct
  source 1..1635: mol_type = other DNA
atggaactgctgattcacagaagcagcgccatctttctgaccctggccatcaatgccctgtacctgaccagcagccagaacatcaccgaagagttctaccagagcacctgtagcgccgtgtccagaggctacttttcttgcctgagaaccggctggtatcacagcgtgatcaccatcgagctgagcaacatcaaagaaacaaagtgcaacggcaccgacaccaaagtgaagctgatcaagcaagagctggacaagtacaagaacgccgtgaccgaactgcagctgctgatgcagaatacccctgccgccaacaaccgggccagaagagaagcccctcagtacatgaactacaccatcaacaccaccaagaacctgaacgtgtccatcagcaagaagcggaagcggagattcctgggctttctgctcggagtgggaagcgccattgcctctggaattgccgtgtctaaggtgctgcacctggaaggcgaagtgaacaagatcaagaatgccctgctgagcaccaacaaggccgtggtgtctctgtctaatggcgtgtccgtgctgaccagcaaggtgctggacctgaagaactacatcaacaaccagctgctgcccatcgtgaaccagcagagctgccggatcagcaacatcgagacagtgatcgagttccagcagaagaacagcagactgctggaaatcacccgcgagttttccgtgaatgccggcgtgacaacacccctgagcacctacatgctgaccaacagcgagctgctgtccctgatcaacgacatgcccatcaccaacgaccagaaaaagctgatgagcagcaacgtgcagatcgtgcggcagcagtcctacagcatcatgagcattatcaaagaagaggtgctggcctacgtggtgcagctgcctatctacggcgtgtgcgataccccttgctggaagctgcacacaagccctctgtgcaccaccaatatcaaagagggctccaacatctgcctgaccagaaccgatagaggctggtactgcgataatgccggcagcgtcagcttcttcccacaagccgatacctgcaaggtgcagagcaacagagtgttctgcgataccatgaacagcctgacactgcccagcgaggtgtccctgtgcaacaccgacatcttcaactctaagtacgactgcaagatcatgacctccaagaccgacatcagctcctccgtgatcacatctctgggcgccatcgtgtcctgctacggcaagacaaagtgtaccgccagcaacaagaaccggggcatcatcaagaccttcagcaacggctgcgactacgtgtccaacaaaggcgtggacaccgtgtctgtgggcaacaccctgtactacgtgaacaagctggaaggcaagaatctgtacgtgaagggcgagcccatcatcaactactacgaccctctggtgttccccagcagcgagtttgatgccagcatcagccaagtgaacgagaagatcaaccagagcctggccttcatccgcagatccgatgaactgctgtctgccatcggcggctatatccccgaagctcctagagatggacaggcctatgtgcggaaggatggcgaatgggtgctgctgtctaccttcctgtga

SEQ ID NO: 109 - DNA, 1635 bp, synthetic construct
  source 1..1635: mol_type = other DNA
atggaactgcccatcctgaaaacaaacgccatcaccaccatcctggccgccgtgacactgtgttttgccagcagccagaacatcaccgaagagttctaccagagcacctgtagcgccgtgtctaagggctatctgtctgcctgcagaaccggctggtatcacagcgtgatcaccatcgagctgagcaacatcaaagaaaacaagtgcaacggcaccgacgccaaagtgaagctgatcaagcaagagctggacaagtacaagaacgccgtgaccgaactgcagctgctgatgcagtctacccctgccgccaatagcagagccagacgggaactgcctagattcatgaactacaccctgaacaacaccaagaacaccaacgtgaccctgagcaagaagcggaagcggagattcctgggctttctgctcggatgcggaagcgccattgcctctggaattgccgtgtccaaggtgctgcatctggaaggcgaagtgaacaagatcaagagcgccctgctgagcaccaacaaggccgtggtttctctgagcaatggcgtgtccgtgctgacctctaaggtgctggacctgaagaactacatcgacaaacagctgctgcccatcgtcaacaagcagagctgcagcatcagcaacatcgagacagtgatcgagttccagcagaagaacaaccggctgctggaaatcacccgcgagttttctgtgaatgccggcgtgaccacacctgtgtccacctacatgctgaccaacagcgagctgctgtccctgatcaacgacatgcccatcaccaacgaccagaaaaagctgatgagcagcaacgtgcagatcgtgcggcagcagagctactccatcatgagcattatcaaagaagaggtgctggcctacgtggtgcagctgcctctgtatggctgcatcgataccccttgctggaagctgcacacaagccctctgtgcaccaccaacaccaaagagggctccaacatctgcctgaccagaaccgatagaggctggtactgcgataatgccggcagcgtcagcttcttcccacaagccgagacatgcaaggtgcagagcaacagagtgttctgcgataccatgaacagcctgacactgccctccgaagtgaatctgtgcaatatcgacatcttcaacccgaagtacgactgcaagatcatgaccagcaagaccgacgtgtcaagctcctgcatcacatctctgggcgccatcgtgtcctgctacggcaagacaaagtgcaccgccagcaacaagaaccggggcatcatcaagaccttcagcaacggctgcgactacgtgtccaacaaaggcgtggacaccgtgtctgtgggcaacaccctgtactacgtgaacaagcaagaaggcaagagcctgtacgtgaagggcgagcccatcatcaacttctacgaccctctggtgttccccagcagcgagtttgatgccagcatctcccaagtgaacgagaagatcaaccagagcctggccttcatcagaaagtccgatgagctgctgagcgccatcggcggctatatccctgaagctcctagagatggacaggcctatgtgcggaaggatggcgaatgggtgctgctgtctaccttcctgtga

SEQ ID NO: 110 - DNA, 1635 bp, synthetic construct
  source 1..1635: mol_type = other DNA
atggaactgctgattcacagaagcagcgccatctttctgaccctggccatcaatgccctgtacctgaccagcagccagaacatcaccgaagagttctaccagagcacctgtagcgccgtgtccagaggctacttttctgcctgcagaaccggctggtatcacagcgtgatcaccatcgagctgagcaacatcaaagaaacaaagtgcaacggcaccgacaccaaagtgaagctgatcaagcaagagctggacaagtacaagaacgccgtgaccgaactgcagctgctgatgcagaatacccctgccgccaacaaccgggccagaagagaagcccctcagtacatgaactacaccatcaacaccaccaagaacctgaacgtgtccatcagcaagaagcggaagcggagattcctgggctttctgctcggatgcggaagcgccattgcctctggaattgccgtgtctaaggtgctgcacctggaaggcgaagtgaacaagatcaagaatgccctgctgagcaccaacaaggccgtggtgtctctgtctaatggcgtgtccgtgctgaccagcaaggtgctggacctgaagaactacatcaacaaccagctgctgcccatcgtgaaccagcagagctgccggatcagcaacatcgagacagtgatcgagttccagcagaagaacagcagactgctggaaatcacccgcgagttttccgtgaatgccggcgtgacaacacccctgagcacctacatgctgaccaacagcgagctgctgtccctgatcaacgacatgcccatcaccaacgaccagaaaaagctgatgagcagcaacgtgcagatcgtgcggcagcagtcctacagcatcatgagcattatcaaagaagaggtgctggcctacgtggtgcagctgcctatctacggctgcatcgataccccttgctggaagctgcacacaagccctctgtgcaccaccaatatcaaagagggctccaacatctgcctgaccagaaccgatagaggctggtactgcgataatgccggcagcgtcagcttcttcccacaagccgatacctgcaaggtgcagagcaacagagtgttctgcgataccatgaacagcctgacactgcccagcgaggtgtccctgtgcaacaccgacatcttcaactctaagtacgactgcaagatcatgacctccaagaccgacatcagctcctcctgcatcacatctctgggcgccatcgtgtcctgctacggcaagacaaagtgtaccgccagcaacaagaaccggggcatcatcaagaccttcagcaacggctgcgactacgtgtccaacaaaggcgtggacaccgtgtctgtgggcaacaccctgtactacgtgaacaagctggaaggcaagaatctgtacgtgaagggcgagcccatcatcaactactacgaccctctggtgttccccagcagcgagtttgatgccagcatcagccaagtgaacgagaagatcaaccagagcctggccttcatccgcagatccgatgaactgctgtctgccatcggcggctatatccccgaagctcctagagatggacaggcctatgtgcggaaggatggcgaatgggtgctgctgtctaccttcctgtga

SEQ ID NO: 111 - DNA, 1635 bp, synthetic construct
  source 1..1635: mol_type = other DNA
atggaactgcccatcctgaaaacaaacgccatcaccaccatcctggccgccgtgacactgtgttttgccagcagccagaacatcaccgaagagttctaccagagcacctgtagcgccgtgtctaagggctatctgtctgcctgcagaaccggctggtatcacagcgtgatcaccatcgagctgagcaacatcaaagaaaacaagtgcaacggcaccgacgccaaagtgaagctgatcaagcaagagctggacaagtacaagaacgccgtgaccgaactgcagctgctgatgcagtctacccctgccgccaatagcagagccagacgggaactgcctagattcatgaactacaccctgaacaacaccaagaacaccaacgtgaccctgagcaagaagcggaagcggagattcctgggctttctgctcggagtgggaagcgccattgcctctggaattgccgtgtccaaggtgctgcatctggaaggcgaagtgaacaagatcaagagcgccctgctgagcaccaacaaggccgtggtttctctgagcaatggcgtgtccgtgctgacctctaaggtgctggacctgaagaactacatcgacaaacagctgctgcccatcgtcaacaagcagagctgcagcatcagcaacatcgagacagtgatcgagttccagcagaagaacaaccggctgctggaaatcacccgcgagttttctgtgaatgccggcgtgaccacacctgtgtccacctacatgctgaccaacagcgagctgctgtccctgatcaacgacatgcccatcaccaacgaccagaaaaagctgatgagcagcaacgtgcagatcgtgcggcagcagagctactccatcatgagcattatcaaagaagaggtgctggcctacgtggtgcagctgcctctgtatggctgcatcgataccccttgctggaagctgcacacaagccctctgtgcaccaccaacaccaaagagggctccaacatctgcctgaccagaaccgatagaggctggtactgcgataatgccggcagcgtcagcttcttcccacaagccgagacatgcaaggtgcagagcaacagagtgttctgcgataccatgaacagcctgacactgccctccgaagtgaatctgtgcaatatcgacatcttcaacccgaagtacgactgcaagatcatgaccagcaagaccgacgtgtcaagctccgtgatcacatctctgggcgccatcgtgtcctgctacggcaagacaaagtgcaccgccagcaacaagaaccggggcatcatcaagaccttcagcaacggctgcgactacgtgtccaacaaaggcgtggacaccgtgtctgtgggcaacaccctgtactacgtgaacaagcaagaaggcaagagcctgtacgtgaagggcgagcccatcatcaacttctacgaccctctggtgttccccagcagcgagtttgatgccagcatctcccaagtgaacgagaagatcaaccagagcctggccttcatcagaaagtccgatgagctgctgagcgccatcggcggctatatccctgaagctcctagagatggacaggcctatgtgcggaaggatggcgaatgggtgctgctgtctaccttcctgtga

SEQ ID NO: 112 - DNA, 1635 bp, synthetic construct
  source 1..1635: mol_type = other DNA
atggaactgctgattcacagaagcagcgccatctttctgaccctggccatcaatgccctgtacctgaccagcagccagaacatcaccgaagagttctaccagagcacctgtagcgccgtgtccagaggctacttttctgcctgcagaaccggctggtatcacagcgtgatcaccatcgagctgagcaacatcaaagaaacaaagtgcaacggcaccgacaccaaagtgaagctgatcaagcaagagctggacaagtacaagaacgccgtgaccgaactgcagctgctgatgcagaatacccctgccgccaacaaccgggccagaagagaagcccctcagtacatgaactacaccatcaacaccaccaagaacctgaacgtgtccatcagcaagaagcggaagcggagattcctgggctttctgctcggagtgggaagcgccattgcctctggaattgccgtgtctaaggtgctgcacctggaaggcgaagtgaacaagatcaagaatgccctgctgagcaccaacaaggccgtggtgtctctgtctaatggcgtgtccgtgctgaccagcaaggtgctggacctgaagaactacatcaacaaccagctgctgcccatcgtgaaccagcagagctgccggatcagcaacatcgagacagtgatcgagttccagcagaagaacagcagactgctggaaatcacccgcgagttttccgtgaatgccggcgtgacaacacccctgagcacctacatgctgaccaacagcgagctgctgtccctgatcaacgacatgcccatcaccaacgaccagaaaaagctgatgagcagcaacgtgcagatcgtgcggcagcagtcctacagcatcatgagcattatcaaagaagaggtgctggcctacgtggtgcagctgcctatctacggctgcatcgataccccttgctggaagctgcacacaagccctctgtgcaccaccaatatcaaagagggctccaacatctgcctgaccagaaccgatagaggctggtactgcgataatgccggcagcgtcagcttcttcccacaagccgatacctgcaaggtgcagagcaacagagtgttctgcgataccatgaacagcctgacactgcccagcgaggtgtccctgtgcaacaccgacatcttcaactctaagtacgactgcaagatcatgacctccaagaccgacatcagctcctccgtgatcacatctctgggcgccatcgtgtcctgctacggcaagacaaagtgtaccgccagcaacaagaaccggggcatcatcaagaccttcagcaacggctgcgactacgtgtccaacaaaggcgtggacaccgtgtctgtgggcaacaccctgtactacgtgaacaagctggaaggcaagaatctgtacgtgaagggcgagcccatcatcaactactacgaccctctggtgttccccagcagcgagtttgatgccagcatcagccaagtgaacgagaagatcaaccagagcctggccttcatccgcagatccgatgaactgctgtctgccatcggcggctatatccccgaagctcctagagatggacaggcctatgtgcggaaggatggcgaatgggtgctgctgtctaccttcctgtga

SEQ ID NO: 113 - DNA, 1635 bp, synthetic construct
  source 1..1635: mol_type = other DNA
atggaactgcccatcctgaaaacaaacgccatcaccaccatcctggccgccgtgacactgtgttttgccagcagccagaacatcaccgaagagttctaccagagcacctgtagcgccgtgtctaagggctatctgtgcgccctgagaaccggctggtatcacagcgtgatcaccatcgagctgagcaacatcaaagaaaacaagtgcaacggcaccgacgccaaagtgaagctgatcaagcaagagctggacaagtacaagaacgccgtgaccgaactgcagctgctgatgcagtctacccctgccgccaatagcagagccagacgggaactgcctagattcatgaactacaccctgaacaacaccaagaacaccaacgtgaccctgagcaagaagcggaagcggagattcctgggctttctgctcggatgcggaagcgccattgcctctggaattgccgtgtccaaggtgctgcatctggaaggcgaagtgaacaagatcaagagcgccctgctgagcaccaacaaggccgtggtttctctgagcaatggcgtgtccgtgctgacctctaaggtgctggacctgaagaactacatcgacaaacagctgctgcccatcgtcaacaagcagagctgcagcatcagcaacatcgagacagtgatcgagttccagcagaagaacaaccggctgctggaaatcacccgcgagttttctgtgaatgccggcgtgaccacacctgtgtccacctacatgctgaccaacagcgagctgctgtccctgatcaacgacatgcccatcaccaacgaccagaaaaagctgatgagcagcaacgtgcagatcgtgcggcagcagagctactccatcatgagcattatcaaagaagaggtgctggcctacgtggtgcagctgcctctgtatggcgtgatcgattgcccttgctggaagctgcacacaagccctctgtgcaccaccaacaccaaagagggctccaacatctgcctgaccagaaccgatagaggctggtactgcgataatgccggcagcgtcagcttcttcccacaagccgagacatgcaaggtgcagagcaacagagtgttctgcgataccatgaacagcctgacactgccctccgaagtgaatctgtgcaatatcgacatcttcaacccgaagtacgactgcaagatcatgaccagcaagaccgacgtgtcaagctcctgcatcacatctctgggcgccatcgtgtcctgctacggcaagacaaagtgcaccgccagcaacaagaaccggggcatcatcaagaccttcagcaacggctgcgactacgtgtccaacaaaggcgtggacaccgtgtctgtgggcaacaccctgtactacgtgaacaagcaagaaggcaagagcctgtacgtgaagggcgagcccatcatcaacttctacgaccctctggtgttccccagcagcgagtttgatgccagcatctcccaagtgaacgagaagatcaaccagagcctggccttcatcagaaagtccgatgagctgctgagcgccatcggcggctatatccctgaagctcctagagatggacaggcctatgtgcggaaggatggcgaatgggtgctgctgtctaccttcctgtga

SEQ ID NO: 114 - DNA, 1635 bp, synthetic construct
  source 1..1635: mol_type = other DNA
atggaactgctgattcacagaagcagcgccatctttctgaccctggccatcaatgccctgtacctgaccagcagccagaacatcaccgaagagttctaccagagcacctgtagcgccgtgtccagaggctacttttgcgccctgagaaccggctggtatcacagcgtgatcaccatcgagctgagcaacatcaaagaaacaaagtgcaacggcaccgacaccaaagtgaagctgatcaagcaagagctggacaagtacaagaacgccgtgaccgaactgcagctgctgatgcagaatacccctgccgccaacaaccgggccagaagagaagcccctcagtacatgaactacaccatcaacaccaccaagaacctgaacgtgtccatcagcaagaagcggaagcggagattcctgggctttctgctcggatgcggaagcgccattgcctctggaattgccgtgtctaaggtgctgcacctggaaggcgaagtgaacaagatcaagaatgccctgctgagcaccaacaaggccgtggtgtctctgtctaatggcgtgtccgtgctgaccagcaaggtgctggacctgaagaactacatcaacaaccagctgctgcccatcgtgaaccagcagagctgccggatcagcaacatcgagacagtgatcgagttccagcagaagaacagcagactgctggaaatcacccgcgagttttccgtgaatgccggcgtgacaacacccctgagcacctacatgctgaccaacagcgagctgctgtccctgatcaacgacatgcccatcaccaacgaccagaaaaagctgatgagcagcaacgtgcagatcgtgcggcagcagtcctacagcatcatgagcattatcaaagaagaggtgctggcctacgtggtgcagctgcctatctacggcgtgatcgattgcccttgctggaagctgcacacaagccctctgtgcaccaccaatatcaaagagggctccaacatctgcctgaccagaaccgatagaggctggtactgcgataatgccggcagcgtcagcttcttcccacaagccgatacctgcaaggtgcagagcaacagagtgttctgcgataccatgaacagcctgacactgcccagcgaggtgtccctgtgcaacaccgacatcttcaactctaagtacgactgcaagatcatgacctccaagaccgacatcagctcctcctgcatcacatctctgggcgccatcgtgtcctgctacggcaagacaaagtgtaccgccagcaacaagaaccggggcatcatcaagaccttcagcaacggctgcgactacgtgtccaacaaaggcgtggacaccgtgtctgtgggcaacaccctgtactacgtgaacaagctggaaggcaagaatctgtacgtgaagggcgagcccatcatcaactactacgaccctctggtgttccccagcagcgagtttgatgccagcatcagccaagtgaacgagaagatcaaccagagcctggccttcatccgcagatccgatgaactgctgtctgccatcggcggctatatccccgaagctcctagagatggacaggcctatgtgcggaaggatggcgaatgggtgctgctgtctaccttcctgtga

SEQ ID NO: 115 - DNA, 1635 bp, synthetic construct
  source 1..1635: mol_type = other DNA
atggaactgcccatcctgaaaacaaacgccatcaccaccatcctggccgccgtgacactgtgttttgccagcagccagaacatcaccgaagagttctaccagagcacctgtagcgccgtgtctaagggctatctgtgcgccctgagaaccggctggtatcacagcgtgatcaccatcgagctgagcaacatcaaagaaaacaagtgcaacggcaccgacgccaaagtgaagctgatcaagcaagagctggacaagtacaagaacgccgtgaccgaactgcagctgctgatgcagtctacccctgccgccaatagcagagccagacgggaactgcctagattcatgaactacaccctgaacaacaccaagaacaccaacgtgaccctgagcaagaagcggaagcggagattcctgggctttctgctcggagtgggaagcgccattgcctctggaattgccgtgtccaaggtgctgcatctggaaggcgaagtgaacaagatcaagagcgccctgctgagcaccaacaaggccgtggtttctctgagcaatggcgtgtccgtgctgacctctaaggtgctggacctgaagaactacatcgacaaacagctgctgcccatcgtcaacaagcagagctgcagcatcagcaacatcgagacagtgatcgagttccagcagaagaacaaccggctgctggaaatcacccgcgagttttctgtgaatgccggcgtgaccacacctgtgtccacctacatgctgaccaacagcgagctgctgtccctgatcaacgacatgcccatcaccaacgaccagaaaaagctgatgagcagcaacgtgcagatcgtgcggcagcagagctactccatcatgagcattatcaaagaagaggtgctggcctacgtggtgcagctgcctctgtatggcgtgatcgattgcccttgctggaagctgcacacaagccctctgtgcaccaccaacaccaaagagggctccaacatctgcctgaccagaaccgatagaggctggtactgcgataatgccggcagcgtcagcttcttcccacaagccgagacatgcaaggtgcagagcaacagagtgttctgcgataccatgaacagcctgacactgccctccgaagtgaatctgtgcaatatcgacatcttcaacccgaagtacgactgcaagatcatgaccagcaagaccgacgtgtcaagctccgtgatcacatctctgggcgccatcgtgtcctgctacggcaagacaaagtgcaccgccagcaacaagaaccggggcatcatcaagaccttcagcaacggctgcgactacgtgtccaacaaaggcgtggacaccgtgtctgtgggcaacaccctgtactacgtgaacaagcaagaaggcaagagcctgtacgtgaagggcgagcccatcatcaacttctacgaccctctggtgttccccagcagcgagtttgatgccagcatctcccaagtgaacgagaagatcaaccagagcctggccttcatcagaaagtccgatgagctgctgagcgccatcggcggctatatccctgaagctcctagagatggacaggcctatgtgcggaaggatggcgaatgggtgctgctgtctaccttcctgtga

SEQ ID NO: 116 - DNA, 1635 bp, synthetic construct
  source 1..1635: mol_type = other DNA
atggaactgctgattcacagaagcagcgccatctttctgaccctggccatcaatgccctgtacctgaccagcagccagaacatcaccgaagagttctaccagagcacctgtagcgccgtgtccagaggctacttttgcgccctgagaaccggctggtatcacagcgtgatcaccatcgagctgagcaacatcaaagaaacaaagtgcaacggcaccgacaccaaagtgaagctgatcaagcaagagctggacaagtacaagaacgccgtgaccgaactgcagctgctgatgcagaatacccctgccgccaacaaccgggccagaagagaagcccctcagtacatgaactacaccatcaacaccaccaagaacctgaacgtgtccatcagcaagaagcggaagcggagattcctgggctttctgctcggagtgggaagcgccattgcctctggaattgccgtgtctaaggtgctgcacctggaaggcgaagtgaacaagatcaagaatgccctgctgagcaccaacaaggccgtggtgtctctgtctaatggcgtgtccgtgctgaccagcaaggtgctggacctgaagaactacatcaacaaccagctgctgcccatcgtgaaccagcagagctgccggatcagcaacatcgagacagtgatcgagttccagcagaagaacagcagactgctggaaatcacccgcgagttttccgtgaatgccggcgtgacaacacccctgagcacctacatgctgaccaacagcgagctgctgtccctgatcaacgacatgcccatcaccaacgaccagaaaaagctgatgagcagcaacgtgcagatcgtgcggcagcagtcctacagcatcatgagcattatcaaagaagaggtgctggcctacgtggtgcagctgcctatctacggcgtgatcgattgcccttgctggaagctgcacacaagccctctgtgcaccaccaatatcaaagagggctccaacatctgcctgaccagaaccgatagaggctggtactgcgataatgccggcagcgtcagcttcttcccacaagccgatacctgcaaggtgcagagcaacagagtgttctgcgataccatgaacagcctgacactgcccagcgaggtgtccctgtgcaacaccgacatcttcaactctaagtacgactgcaagatcatgacctccaagaccgacatcagctcctccgtgatcacatctctgggcgccatcgtgtcctgctacggcaagacaaagtgtaccgccagcaacaagaaccggggcatcatcaagaccttcagcaacggctgcgactacgtgtccaacaaaggcgtggacaccgtgtctgtgggcaacaccctgtactacgtgaacaagctggaaggcaagaatctgtacgtgaagggcgagcccatcatcaactactacgaccctctggtgttccccagcagcgagtttgatgccagcatcagccaagtgaacgagaagatcaaccagagcctggccttcatccgcagatccgatgaactgctgtctgccatcggcggctatatccccgaagctcctagagatggacaggcctatgtgcggaaggatggcgaatgggtgctgctgtctaccttcctgtga

SEQ ID NO: 117 - DNA, 1638 bp, synthetic construct
  source 1..1638: mol_type = other DNA
atggaactgcccatcctgaaaacaaacgccatcaccaccatcctggccgccgtgacactgtgttttgccagcagccagaacatcaccgaagagttctaccagagcacctgtagcgccgtgtctaagggctatctgtctgccctgagaaccggctggtatcacagcgtgatcaccatcgagctgagcaacatcaaagaaaacaagtgcaacggcaccgacgccaaagtgaagctgatcaagcaagagctggacaagtacaagaacgccgtgaccgaactgcagctgctgatgcagtctaccccttgcgccaatagcagagccagacgggaactgcctagattcatgaactacaccctgaacaacaccaagaacaccaacgtgaccctgagcaagaagcggaagcggagattcctgggctttctgctcggagtgggaagcgcctgcgcctctggaattgccgtgtccaaggtgctgcatctggaaggcgaagtgaacaagatcaagagcgccctgctgagcaccaacaaggccgtggtttctctgagcaatggcgtgtccgtgctgaccatcaaggtgctggacctgaagaactacatcgacaaacagctgctgcccatcgtcaacaagcagagctgcagcatcagcaacatcgagacagtgatcgagttccagcagaagaacaaccggctgctggaaatcacccgcgagttttctgtgaatgccggcgtgaccacacctgtgtccacctacatgctgaccaacagcgagctgctgtccctgatcaacgacatgcccatcaccaacgaccagaaaaagctgatgagcagcaacgtgcagatcgtgcggcagcagagctactccatcatgagcattatcaaagaagagatcctggcctacgtggtgcagctgcctctgtatggcgtgatcgataccccttgctggaagctgcacacaagccctctgtgcaccaccaacaccaaagagggctccaacatctgcctgaccagaaccgatagaggctggtactgcgataatgccggcagcgtcagcttcttcccacaagccgagacatgcaaggtgcagagcaacagagtgttctgcgataccatgaacagcctgacactgccctccgaagtgaatctgtgcaatatcgacatcttcaacccgaagtacgactgcaagatcatgaccagcaagaccgacgtgtcaagctccgtgatcacatctctgggcgccatcgtgtcctgctacggcaagacaaagtgcaccgccagcaacaagaaccggggcatcatcaagaccttcagcaacggctgcgactacgtgtccaacaaaggcgtggacaccgtgtctgtgggcaacaccctgtactacgtgaacaagcaagaaggcaagagcctgtacgtgaagggcgagcccatcatcaacttctacgaccctctggtgttccccagcagcgagtttgatgccagcatctcccaagtgaacgagaagatcaaccagagcctggccttcatcagaaagtccgatgagctgctgagcgccatcggcggctatatccctgaagctcctagagatggacaggcctatgtgcggaaggatggcgaatgggtgctgctgtctaccttcctgtgatga

SEQ ID NO: 118 - DNA, 1638 bp, synthetic construct; identical to SEQ ID NO: 117
  source 1..1638: mol_type = other DNA

SEQ ID NO: 119 - DNA, 1638 bp, synthetic construct
  source 1..1638: mol_type = other DNA
atggaactgcccatcctgaaaacaaacgccatcaccaccatcctggccgccgtgacactgtgttttgccagcagccagaacatcaccgaagagttctaccagagcacctgtagcgccgtgtctaagggctatctgtctgccctgagaaccggctggtatcacagcgtgatcaccatcgagctgagcaacatcaaagaaaacaagtgcaacggcaccgacgccaaagtgaagctgatcaagcaagagctggacaagtacaagaacgccgtgaccgaactgcagctgctgatgcagtctaccccttgcgccaatagcagagccagacgggaactgcctagattcatgaactacaccctgaacaacaccaagaacaccaacgtgaccctgagcaagaagcggaagcggagattcctgggctttctgctcggagtgggaagcgccattgcctctggatgcgccgtgtccaaggtgctgcatctggaaggcgaagtgaacaagatcaagagcgccctgctgagcaccaacaaggccgtggtttctctgagcaatggcgtgtccgtgctgaccatcaaggtgctggacctgaagaactacatcgacaaacagctgctgcccatcgtcaacaagcagagctgcagcatcagcaacatcgagacagtgatcgagttccagcagaagaacaaccggctgctggaaatcacccgcgagttttctgtgaatgccggcgtgaccacacctgtgtccacctacatgctgaccaacagcgagctgctgtccctgatcaacgacatgcccatcaccaacgaccagaaaaagctgatgagcagcaacgtgcagatcgtgcggcagcagagctactccatcatgagcattatcaaagaagagatcctggcctacgtggtgcagctgcctctgtatggcgtgatcgataccccttgctggaagctgcacacaagccctctgtgcaccaccaacaccaaagagggctccaacatctgcctgaccagaaccgatagaggctggtactgcgataatgccggcagcgtcagcttcttcccacaagccgagacatgcaaggtgcagagcaacagagtgttctgcgataccatgaacagcctgacactgccctccgaagtgaatctgtgcaatatcgacatcttcaacccgaagtacgactgcaagatcatgaccagcaagaccgacgtgtcaagctccgtgatcacatctctgggcgccatcgtgtcctgctacggcaagacaaagtgcaccgccagcaacaagaaccggggcatcatcaagaccttcagcaacggctgcgactacgtgtccaacaaaggcgtggacaccgtgtctgtgggcaacaccctgtactacgtgaacaagcaagaaggcaagagcctgtacgtgaagggcgagcccatcatcaacttctacgaccctctggtgttccccagcagcgagtttgatgccagcatctcccaagtgaacgagaagatcaaccagagcctggccttcatcagaaagtccgatgagctgctgagcgccatcggcggctatatccctgaagctcctagagatggacaggcctatgtgcggaaggatggcgaatgggtgctgctgtctaccttcctgtgatga

SEQ ID NO: 120 - DNA, 1638 bp, synthetic construct
  source 1..1638: mol_type = other DNA
atggaactgctgattcacagaagcagcgccatctttctgaccctggccatcaatgccctgtacctgaccagcagccagaacatcaccgaagagttctaccagagcacctgtagcgccgtgtccagaggctacttttctgccctgagaaccggctggtatcacagcgtgatcaccatcgagctgagcaacatcaaagaaacaaagtgcaacggcaccgacaccaaagtgaagctgatcaagcaagagctggacaagtacaagaacgccgtgaccgaactgcagctgctgatgcagaataccccttgcgccaacaaccgggccagaagagaagcccctcagtacatgaactacaccatcaacaccaccaagaacctgaacgtgtccatcagcaagaagcggaagcggagattcctgggctttctgctcggagtgggaagcgccattgcctctggatgcgccgtgtctaaggtgctgcacctggaaggcgaagtgaacaagatcaagaatgccctgctgagcaccaacaaggccgtggtgtctctgtctaatggcgtgtccgtgctgaccatcaaggtgctggacctgaagaactacatcaacaaccagctgctgcccatcgtgaaccagcagagctgccggatcagcaacatcgagacagtgatcgagttccagcagaagaacagcagactgctggaaatcacccgcgagttttccgtgaatgccggcgtgacaacacccctgagcacctacatgctgaccaacagcgagctgctgtccctgatcaacgacatgcccatcaccaacgaccagaaaaagctgatgagcagcaacgtgcagatcgtgcggcagcagtcctacagcatcatgagcattatcaaagaagagatcctggcctacgtggtgcagctgcctatctacggcgtgatcgataccccttgctggaagctgcacacaagccctctgtgcaccaccaatatcaaagagggctccaacatctgcctgaccagaaccgatagaggctggtactgcgataatgccggcagcgtcagcttcttcccacaagccgatacctgcaaggtgcagagcaacagagtgttctgcgataccatgaacagcctgacactgcccagcgaggtgtccctgtgcaacaccgacatcttcaactctaagtacgactgcaagatcatgacctccaagaccgacatcagctcctccgtgatcacatctctgggcgccatcgtgtcctgctacggcaagacaaagtgtaccgccagcaacaagaaccggggcatcatcaagaccttcagcaacggctgcgactacgtgtccaacaaaggcgtggacaccgtgtctgtgggcaacaccctgtactacgtgaacaagctggaaggcaagaatctgtacgtgaagggcgagcccatcatcaactactacgaccctctggtgttccccagcagcgagtttgatgccagcatcagccaagtgaacgagaagatcaaccagagcctggccttcatccgcagatccgatgaactgctgtctgccatcggcggctatatccccgaagctcctagagatggacaggcctatgtgcggaaggatggcgaatgggtgctgctgtctaccttcctgtgatga

SEQ ID NO: 121 - DNA, 1638 bp, synthetic construct
  source 1..1638: mol_type = other DNA
atggaactgcccatcctgaaaacaaacgccatcaccaccatcctggccgccgtgacactgtgttttgccagcagccagaacatcaccgaagagttctaccagagcacctgtagcgccgtgtctaagggctatctgtctgccctgagaaccggctggtatcacagcgtgatcaccatcgagctgagcaacatcaaagaaaacaagtgcaacggcaccgacgccaaagtgaagctgatcaagcaagagctggacaagtacaagaacgccgtgaccgaactgcagctgctgatgcagtctacccctgccgcctgcagcagagccagacgggaactgcctagattcatgaactacaccctgaacaacaccaagaacaccaacgtgaccctgagcaagaagcggaagcggagattcctgggctttctgctcggagtgtgcagcgccattgcctctggaattgccgtgtccaaggtgctgcatctggaaggcgaagtgaacaagatcaagagcgccctgctgagcaccaacaaggccgtggtttctctgagcaatggcgtgtccgtgctgaccatcaaggtgctggacctgaagaactacatcgacaaacagctgctgcccatcgtcaacaagcagagctgcagcatcagcaacatcgagacagtgatcgagttccagcagaagaacaaccggctgctggaaatcacccgcgagttttctgtgaatgccggcgtgaccacacctgtgtccacctacatgctgaccaacagcgagctgctgtccctgatcaacgacatgcccatcaccaacgaccagaaaaagctgatgagcagcaacgtgcagatcgtgcggcagcagagctactccatcatgagcattatcaaagaagagatcctggcctacgtggtgcagctgcctctgtatggcgtgatcgataccccttgctggaagctgcacacaagccctctgtgcaccaccaacaccaaagagggctccaacatctgcctgaccagaaccgatagaggctggtactgcgataatgccggcagcgtcagcttcttcccacaagccgagacatgcaaggtgcagagcaacagagtgttctgcgataccatgaacagcctgacactgccctccgaagtgaatctgtgcaatatcgacatcttcaacccgaagtacgactgcaagatcatgaccagcaagaccgacgtgtcaagctccgtgatcacatctctgggcgccatcgtgtcctgctacggcaagacaaagtgcaccgccagcaacaagaaccggggcatcatcaagaccttcagcaacggctgcgactacgtgtccaacaaaggcgtggacaccgtgtctgtgggcaacaccctgtactacgtgaacaagcaagaaggcaagagcctgtacgtgaagggcgagcccatcatcaacttctacgaccctctggtgttccccagcagcgagtttgatgccagcatctcccaagtgaacgagaagatcaaccagagcctggccttcatcagaaagtccgatgagctgctgagcgccatcggcggctatatccctgaagctcctagagatggacaggcctatgtgcggaaggatggcgaatgggtgctgctgtctaccttcctgtgatga

SEQ ID NO: 122 - DNA, 1638 bp, synthetic construct
  source 1..1638: mol_type = other DNA
atggaactgctgattcacagaagcagcgccatctttctgaccctggccatcaatgccctgtacctgaccagcagccagaacatcaccgaagagttctaccagagcacctgtagcgccgtgtccagaggctacttttctgccctgagaaccggctggtatcacagcgtgatcaccatcgagctgagcaacatcaaagaaacaaagtgcaacggcaccgacaccaaagtgaagctgatcaagcaagagctggacaagtacaagaacgccgtgaccgaactgcagctgctgatgcagaatacccctgccgcctgcaaccgggccagaagagaagcccctcagtacatgaactacaccatcaacaccaccaagaacctgaacgtgtccatcagcaagaagcggaagcggagattcctgggctttctgctcggagtgtgcagcgccattgcctctggaattgccgtgtctaaggtgctgcacctggaaggcgaagtgaacaagatcaagaatgccctgctgagcaccaacaaggccgtggtgtctctgtctaatggcgtgtccgtgctgaccatcaaggtgctggacctgaagaactacatcaacaaccagctgctgcccatcgtgaaccagcagagctgccggatcagcaacatcgagacagtgatcgagttccagcagaagaacagcagactgctggaaatcacccgcgagttttccgtgaatgccggcgtgacaacacccctgagcacctacatgctgaccaacagcgagctgctgtccctgatcaacgacatgcccatcaccaacgaccagaaaaagctgatgagcagcaacgtgcagatcgtgcggcagcagtcctacagcatcatgagcattatcaaagaagagatcctggcctacgtggtgcagctgcctatctacggcgtgatcgataccccttgctggaagctgcacacaagccctctgtgcaccaccaatatcaaagagggctccaacatctgcctgaccagaaccgatagaggctggtactgcgataatgccggcagcgtcagcttcttcccacaagccgatacctgcaaggtgcagagcaacagagtgttctgcgataccatgaacagcctgacactgcccagcgaggtgtccctgtgcaacaccgacatcttcaactctaagtacgactgcaagatcatgacctccaagaccgacatcagctcctccgtgatcacatctctgggcgccatcgtgtcctgctacggcaagacaaagtgtaccgccagcaacaagaaccggggcatcatcaagaccttcagcaacggctgcgactacgtgtccaacaaaggcgtggacaccgtgtctgtgggcaacaccctgtactacgtgaacaagctggaaggcaagaatctgtacgtgaagggcgagcccatcatcaactactacgaccctctggtgttccccagcagcgagtttgatgccagcatcagccaagtgaacgagaagatcaaccagagcctggccttcatccgcagatccgatgaactgctgtctgccatcggcggctatatccccgaagctcctagagatggacaggcctatgtgcggaaggatggcgaatgggtgctgctgtctaccttcctgtgatga

SEQ ID NO: 123 - DNA, 1638 bp, synthetic construct
  source 1..1638: mol_type = other DNA
atggaactgcccatcctgaaaacaaacgccatcaccaccatcctggccgccgtgacactgtgttttgccagcagccagaacatcaccgaagagttctaccagagcacctgtagcgccgtgtctaagggctatctgtctgccctgagaaccggctggtatcacagcgtgatcaccatcgagctgagcaacatcaaagaaaacaagtgcaacggcaccgacgccaaagtgaagctgatcaagcaagagctggacaagtacaagaacgccgtgaccgaactgcagctgctgatgcagtctacccctgccgcctgcagcagagccagacgggaactgcctagattcatgaactacaccctgaacaacaccaagaacaccaacgtgaccctgagcaagaagcggaagcggagattcctgggctttctgctcggagtgggatgcgccattgcctctggaattgccgtgtccaaggtgctgcatctggaaggcgaagtgaacaagatcaagagcgccctgctgagcaccaacaaggccgtggtttctctgagcaatggcgtgtccgtgctgaccatcaaggtgctggacctgaagaactacatcgacaaacagctgctgcccatcgtcaacaagcagagctgcagcatcagcaacatcgagacagtgatcgagttccagcagaagaacaaccggctgctggaaatcacccgcgagttttctgtgaatgccggcgtgaccacacctgtgtccacctacatgctgaccaacagcgagctgctgtccctgatcaacgacatgcccatcaccaacgaccagaaaaagctgatgagcagcaacgtgcagatcgtgcggcagcagagctactccatcatgagcattatcaaagaagagatcctggcctacgtggtgcagctgcctctgtatggcgtgatcgataccccttgctggaagctgcacacaagccctctgtgcaccaccaacaccaaagagggctccaacatctgcctgaccagaaccgatagaggctggtactgcgataatgccggcagcgtcagcttcttcccacaagccgagacatgcaaggtgcagagcaacagagtgttctgcgataccatgaacagcctgacactgccctccgaagtgaatctgtgcaatatcgacatcttcaacccgaagtacgactgcaagatcatgaccagcaagaccgacgtgtcaagctccgtgatcacatctctgggcgccatcgtgtcctgctacggcaagacaaagtgcaccgccagcaacaagaaccggggcatcatcaagaccttcagcaacggctgcgactacgtgtccaacaaaggcgtggacaccgtgtctgtgggcaacaccctgtactacgtgaacaagcaagaaggcaagagcctgtacgtgaagggcgagcccatcatcaacttctacgaccctctggtgttccccagcagcgagtttgatgccagcatctcccaagtgaacgagaagatcaaccagagcctggccttcatcagaaagtccgatgagctgctgagcgccatcggcggctatatccctgaagctcctagagatggacaggcctatgtgcggaaggatggcgaatgggtgctgctgtctaccttcctgtgatga

SEQ ID NO: 124 - DNA, 1638 bp, synthetic construct
  source 1..1638: mol_type = other DNA
atggaactgctgattcacagaagcagcgccatctttctgaccctggccatcaatgccctgtacctgaccagcagccagaacatcaccgaagagttctaccagagcacctgtagcgccgtgtccagaggctacttttctgccctgagaaccggctggtatcacagcgtgatcaccatcgagctgagcaacatcaaagaaacaaagtgcaacggcaccgacaccaaagtgaagctgatcaagcaagagctggacaagtacaagaacgccgtgaccgaactgcagctgctgatgcagaatacccctgccgcctgcaaccgggccagaagagaagcccctcagtacatgaactacaccatcaacaccaccaagaacctgaacgtgtccatcagcaagaagcggaagcggagattcctgggctttctgctcggagtgggatgcgccattgcctctggaattgccgtgtctaaggtgctgcacctggaaggcgaagtgaacaagatcaagaatgccctgctgagcaccaacaaggccgtggtgtctctgtctaatggcgtgtccgtgctgaccatcaaggtgctggacctgaagaactacatcaacaaccagctgctgcccatcgtgaaccagcagagctgccggatcagcaacatcgagacagtgatcgagttccagcagaagaacagcagactgctggaaatcacccgcgagttttccgtgaatgccggcgtgacaacacccctgagcacctacatgctgaccaacagcgagctgctgtccctgatcaacgacatgcccatcaccaacgaccagaaaaagctgatgagcagcaacgtgcagatcgtgcggcagcagtcctacagcatcatgagcattatcaaagaagagatcctggcctacgtggtgcagctgcctatctacggcgtgatcgataccccttgctggaagctgcacacaagccctctgtgcaccaccaatatcaaagagggctccaacatctgcctgaccagaaccgatagaggctggtactgcgataatgccggcagcgtcagcttcttcccacaagccgatacctgcaaggtgcagagcaacagagtgttctgcgataccatgaacagcctgacactgcccagcgaggtgtccctgtgcaacaccgacatcttcaactctaagtacgactgcaagatcatgacctccaagaccgacatcagctcctccgtgatcacatctctgggcgccatcgtgtcctgctacggcaagacaaagtgtaccgccagcaacaagaaccggggcatcatcaagaccttcagcaacggctgcgactacgtgtccaacaaaggcgtggacaccgtgtctgtgggcaacaccctgtactacgtgaacaagctggaaggcaagaatctgtacgtgaagggcgagcccatcatcaactactacgaccctctggtgttccccagcagcgagtttgatgccagcatcagccaagtgaacgagaagatcaaccagagcctggccttcatccgcagatccgatgaactgctgtctgccatcggcggctatatccccgaagctcctagagatggacaggcctatgtgcggaaggatggcgaatgggtgctgctgtctaccttcctgtgatga

SEQ ID NO: 125 - DNA, 1638 bp, synthetic construct
  source 1..1638: mol_type = other DNA
atggaactgcccatcctgaaaacaaacgccatcaccaccatcctggccgccgtgacactgtgttttgccagcagccagaacatcaccgaagagttctaccagagcacctgtagcgccgtgtctaagggctatctgtctgccctgagaaccggctggtatcacagcgtgatcaccatcgagctgagcaacatcaaagaaaacaagtgcaacggcaccgacgccaaagtgaagctgatcaagcaagagctggacaagtacaagaacgccgtgaccgaactgcagctgctgatgcagtctacccctgccgccaattgcagagccagacgggaactgcctagattcatgaactacaccctgaacaacaccaagaacaccaacgtgaccctgagcaagaagcggaagcggagattcctgggctttctgctcggagtgggaagctgcattgcctctggaattgccgtgtccaaggtgctgcatctggaaggcgaagtgaacaagatcaagagcgccctgctgagcaccaacaaggccgtggtttctctgagcaatggcgtgtccgtgctgaccatcaaggtgctggacctgaagaactacatcgacaaacagctgctgcccatcgtcaacaagcagagctgcagcatcagcaacatcgagacagtgatcgagttccagcagaagaacaaccggctgctggaaatcacccgcgagttttctgtgaatgccggcgtgaccacacctgtgtccacctacatgctgaccaacagcgagctgctgtccctgatcaacgacatgcccatcaccaacgaccagaaaaagctgatgagcagcaacgtgcagatcgtgcggcagcagagctactccatcatgagcattatcaaagaagagatcctggcctacgtggtgcagctgcctctgtatggcgtgatcgataccccttgctggaagctgcacacaagccctctgtgcaccaccaacaccaaagagggctccaacatctgcctgaccagaaccgatagaggctggtactgcgataatgccggcagcgtcagcttcttcccacaagccgagacatgcaaggtgcagagcaacagagtgttctgcgataccatgaacagcctgacactgccctccgaagtgaatctgtgcaatatcgacatcttcaacccgaagtacgactgcaagatcatgaccagcaagaccgacgtgtcaagctccgtgatcacatctctgggcgccatcgtgtcctgctacggcaagacaaagtgcaccgccagcaacaagaaccggggcatcatcaagaccttcagcaacggctgcgactacgtgtccaacaaaggcgtggacaccgtgtctgtgggcaacaccctgtactacgtgaacaagcaagaaggcaagagcctgtacgtgaagggcgagcccatcatcaacttctacgaccctctggtgttccccagcagcgagtttgatgccagcatctcccaagtgaacgagaagatcaaccagagcctggccttcatcagaaagtccgatgagctgctgagcgccatcggcggctatatccctgaagctcctagagatggacaggcctatgtgcggaaggatggcgaatgggtgctgctgtctaccttcctgtgatga

SEQ ID NO: 126 - DNA, 1638 bp, synthetic construct
  source 1..1638: mol_type = other DNA
atggaactgctgattcacagaagcagcgccatctttctgaccctggccatcaatgccctgtacctgaccagcagccagaacatcaccgaagagttctaccagagcacctgtagcgccgtgtccagaggctacttttctgccctgagaaccggctggtatcacagcgtgatcaccatcgagctgagcaacatcaaagaaacaaagtgcaacggcaccgacaccaaagtgaagctgatcaagcaagagctggacaagtacaagaacgccgtgaccgaactgcagctgctgatgcagaatacccctgccgccaactgccgggccagaagagaagcccctcagtacatgaactacaccatcaacaccaccaagaacctgaacgtgtccatcagcaagaagcggaagcggagattcctgggctttctgctcggagtgggaagctgcattgcctctggaattgccgtgtctaaggtgctgcacctggaaggcgaagtgaacaagatcaagaatgccctgctgagcaccaacaaggccgtggtgtctctgtctaatggcgtgtccgtgctgaccatcaaggtgctggacctgaagaactacatcaacaaccagctgctgcccatcgtgaaccagcagagctgccggatcagcaacatcgagacagtgatcgagttccagcagaagaacagcagactgctggaaatcacccgcgagttttccgtgaatgccggcgtgacaacacccctgagcacctacatgctgaccaacagcgagctgctgtccctgatcaacgacatgcccatcaccaacgaccagaaaaagctgatgagcagcaacgtgcagatcgtgcggcagcagtcctacagcatcatgagcattatcaaagaagagatcctggcctacgtggtgcagctgcctatctacggcgtgatcgataccccttgctggaagctgcacacaagccctctgtgcaccaccaatatcaaagagggctccaacatctgcctgaccagaaccgatagaggctggtactgcgataatgccggcagcgtcagcttcttcccacaagccgatacctgcaaggtgcagagcaacagagtgttctgcgataccatgaacagcctgacactgcccagcgaggtgtccctgtgcaacaccgacatcttcaactctaagtacgactgcaagatcatgacctccaagaccgacatcagctcctccgtgatcacatctctgggcgccatcgtgtcctgctacggcaagacaaagtgtaccgccagcaacaagaaccggggcatcatcaagaccttcagcaacggctgcgactacgtgtccaacaaaggcgtggacaccgtgtctgtgggcaacaccctgtactacgtgaacaagctggaaggcaagaatctgtacgtgaagggcgagcccatcatcaactactacgaccctctggtgttccccagcagcgagtttgatgccagcatcagccaagtgaacgagaagatcaaccagagcctggccttcatccgcagatccgatgaactgctgtctgccatcggcggctatatccccgaagctcctagagatggacaggcctatgtgcggaaggatggcgaatgggtgctgctgtctaccttcctgtgatga

SEQ ID NO: 127 - DNA, 1638 bp, synthetic construct
  source 1..1638: mol_type = other DNA
atggaactgcccatcctgaaaacaaacgccatcaccaccatcctggccgccgtgacactgtgttttgccagcagccagaacatcaccgaagagttctaccagagcacctgtagcgccgtgtctaagggctatctgtctgccctgagaaccggctggtatcacagcgtgatcaccatcgagctgagcaacatcaaagaaaacaagtgcaacggcaccgacgccaaagtgaagctgatcaagcaagagctggacaagtacaagaacgccgtgaccgaactgcagctgctgatgcagtctacccctgccgccaattgcagagccagacgggaactgcctagattcatgaactacaccctgaacaacaccaagaacaccaacgtgaccctgagcaagaagcggaagcggagattcctgggctttctgctcggagtgtgcagcgccattgcctctggaattgccgtgtccaaggtgctgcatctggaaggcgaagtgaacaagatcaagagcgccctgctgagcaccaacaaggccgtggtttctctgagcaatggcgtgtccgtgctgaccatcaaggtgctggacctgaagaactacatcgacaaacagctgctgcccatcgtcaacaagcagagctgcagcatcagcaacatcgagacagtgatcgagttccagcagaagaacaaccggctgctggaaatcacccgcgagttttctgtgaatgccggcgtgaccacacctgtgtccacctacatgctgaccaacagcgagctgctgtccctgatcaacgacatgcccatcaccaacgaccagaaaaagctgatgagcagcaacgtgcagatcgtgcggcagcagagctactccatcatgagcattatcaaagaagagatcctggcctacgtggtgcagctgcctctgtatggcgtgatcgataccccttgctggaagctgcacacaagccctctgtgcaccaccaacaccaaagagggctccaacatctgcctgaccagaaccgatagaggctggtactgcgataatgccggcagcgtcagcttcttcccacaagccgagacatgcaaggtgcagagcaacagagtgttctgcgataccatgaacagcctgacactgccctccgaagtgaatctgtgcaatatcgacatcttcaacccgaagtacgactgcaagatcatgaccagcaagaccgacgtgtcaagctccgtgatcacatctctgggcgccatcgtgtcctgctacggcaagacaaagtgcaccgccagcaacaagaaccggggcatcatcaagaccttcagcaacggctgcgactacgtgtccaacaaaggcgtggacaccgtgtctgtgggcaacaccctgtactacgtgaacaagcaagaaggcaagagcctgtacgtgaagggcgagcccatcatcaacttctacgaccctctggtgttccccagcagcgagtttgatgccagcatctcccaagtgaacgagaagatcaaccagagcctggccttcatcagaaagtccgatgagctgctgagcgccatcggcggctatatccctgaagctcctagagatggacaggcctatgtgcggaaggatggcgaatgggtgctgctgtctaccttcctgtgatga

SEQ ID NO: 128 - DNA, 1638 bp, synthetic construct
  source 1..1638: mol_type = other DNA
atggaactgctgattcacagaagcagcgccatctttctgaccctggccatcaatgccctgtacctgaccagcagccagaacatcaccgaagagttctaccagagcacctgtagcgccgtgtccagaggctacttttctgccctgagaaccggctggtatcacagcgtgatcaccatcgagctgagcaacatcaaagaaacaaagtgcaacggcaccgacaccaaagtgaagctgatcaagcaagagctggacaagtacaagaacgccgtgaccgaactgcagctgctgatgcagaatacccctgccgccaactgccgggccagaagagaagcccctcagtacatgaactacaccatcaacaccaccaagaacctgaacgtgtccatcagcaagaagcggaagcggagattcctgggctttctgctcggagtgtgcagcgccattgcctctggaattgccgtgtctaaggtgctgcacctggaaggcgaagtgaacaagatcaagaatgccctgctgagcaccaacaaggccgtggtgtctctgtctaatggcgtgtccgtgctgaccatcaaggtgctggacctgaagaactacatcaacaaccagctgctgcccatcgtgaaccagcagagctgccggatcagcaacatcgagacagtgatcgagttccagcagaagaacagcagactgctggaaatcacccgcgagttttccgtgaatgccggcgtgacaacacccctgagcacctacatgctgaccaacagcgagctgctgtccctgatcaacgacatgcccatcaccaacgaccagaaaaagctgatgagcagcaacgtgcagatcgtgcggcagcagtcctacagcatcatgagcattatcaaagaagagatcctggcctacgtggtgcagctgcctatctacggcgtgatcgataccccttgctggaagctgcacacaagccctctgtgcaccaccaatatcaaagagggctccaacatctgcctgaccagaaccgatagaggctggtactgcgataatgccggcagcgtcagcttcttcccacaagccgatacctgcaaggtgcagagcaacagagtgttctgcgataccatgaacagcctgacactgcccagcgaggtgtccctgtgcaacaccgacatcttcaactctaagtacgactgcaagatcatgacctccaagaccgacatcagctcctccgtgatcacatctctgggcgccatcgtgtcctgctacggcaagacaaagtgtaccgccagcaacaagaaccggggcatcatcaagaccttcagcaacggctgcgactacgtgtccaacaaaggcgtggacaccgtgtctgtgggcaacaccctgtactacgtgaacaagctggaaggcaagaatctgtacgtgaagggcgagcccatcatcaactactacgaccctctggtgttccccagcagcgagtttgatgccagcatcagccaagtgaacgagaagatcaaccagagcctggccttcatccgcagatccgatgaactgctgtctgccatcggcggctatatccccgaagctcctagagatggacaggcctatgtgcggaaggatggcgaatgggtgctgctgtctaccttcctgtgatga

SEQ ID NO: 129 - DNA, 1638 bp, synthetic construct
  source 1..1638: mol_type = other DNA
atggaactgcccatcctgaaaacaaacgccatcaccaccatcctggccgccgtgacactgtgttttgccagcagccagaacatcaccgaagagttctaccagagcacctgtagcgccgtgtctaagggctatctgtctgccctgagaaccggctggtatcacagcgtgatcaccatcgagctgagcaacatcaaagaaaacaagtgcaacggcaccgacgccaaagtgaagctgatcaagcaagagctggacaagtacaagaacgccgtgaccgaactgcagctgctgatgcagtctacccctgccgccaattgcagagccagacgggaactgcctagattcatgaactacaccctgaacaacaccaagaacaccaacgtgaccctgagcaagaagcggaagcggagattcctgggctttctgctcggagtgggatgcgccattgcctctggaattgccgtgtccaaggtgctgcatctggaaggcgaagtgaacaagatcaagagcgccctgctgagcaccaacaaggccgtggtttctctgagcaatggcgtgtccgtgctgaccatcaaggtgctggacctgaagaactacatcgacaaacagctgctgcccatcgtcaacaagcagagctgcagcatcagcaacatcgagacagtgatcgagttccagcagaagaacaaccggctgctggaaatcacccgcgagttttctgtgaatgccggcgtgaccacacctgtgtccacctacatgctgaccaacagcgagctgctgtccctgatcaacgacatgcccatcaccaacgaccagaaaaagctgatgagcagcaacgtgcagatcgtgcggcagcagagctactccatcatgagcattatcaaagaagagatcctggcctacgtggtgcagctgcctctgtatggcgtgatcgataccccttgctggaagctgcacacaagccctctgtgcaccaccaacaccaaagagggctccaacatctgcctgaccagaaccgatagaggctggtactgcgataatgccggcagcgtcagcttcttcccacaagccgagacatgcaaggtgcagagcaacagagtgttctgcgataccatgaacagcctgacactgccctccgaagtgaatctgtgcaatatcgacatcttcaacccgaagtacgactgcaagatcatgaccagcaagaccgacgtgtcaagctccgtgatcacatctctgggcgccatcgtgtcctgctacggcaagacaaagtgcaccgccagcaacaagaaccggggcatcatcaagaccttcagcaacggctgcgactacgtgtccaacaaaggcgtggacaccgtgtctgtgggcaacaccctgtactacgtgaacaagcaagaaggcaagagcctgtacgtgaagggcgagcccatcatcaacttctacgaccctctggtgttccccagcagcgagtttgatgccagcatctcccaagtgaacgagaagatcaaccagagcctggccttcatcagaaagtccgatgagctgctgagcgccatcggcggctatatccctgaagctcctagagatggacaggcctatgtgcggaaggatggcgaatgggtgctgctgtctaccttcctgtgatga

SEQ ID NO: 130 - DNA, 1638 bp, synthetic construct
  source 1..1638: mol_type = other DNA
atggaactgctgattcacagaagcagcgccatctttctgaccctggccatcaatgccctgtacctgaccagcagccagaacatcaccgaagagttctaccagagcacctgtagcgccgtgtccagaggctacttttctgccctgagaaccggctggtatcacagcgtgatcaccatcgagctgagcaacatcaaagaaacaaagtgcaacggcaccgacaccaaagtgaagctgatcaagcaagagctggacaagtacaagaacgccgtgaccgaactgcagctgctgatgcagaatacccctgccgccaactgccgggccagaagagaagcccctcagtacatgaactacaccatcaacaccaccaagaacctgaacgtgtccatcagcaagaagcggaagcggagattcctgggctttctgctcggagtgggatgcgccattgcctctggaattgccgtgtctaaggtgctgcacctggaaggcgaagtgaacaagatcaagaatgccctgctgagcaccaacaaggccgtggtgtctctgtctaatggcgtgtccgtgctgaccatcaaggtgctggacctgaagaactacatcaacaaccagctgctgcccatcgtgaaccagcagagctgccggatcagcaacatcgagacagtgatcgagttccagcagaagaacagcagactgctggaaatcacccgcgagttttccgtgaatgccggcgtgacaacacccctgagcacctacatgctgaccaacagcgagctgctgtccctgatcaacgacatgcccatcaccaacgaccagaaaaagctgatgagcagcaacgtgcagatcgtgcggcagcagtcctacagcatcatgagcattatcaaagaagagatcctggcctacgtggtgcagctgcctatctacggcgtgatcgataccccttgctggaagctgcacacaagccctctgtgcaccaccaatatcaaagagggctccaacatctgcctgaccagaaccgatagaggctggtactgcgataatgccggcagcgtcagcttcttcccacaagccgatacctgcaaggtgcagagcaacagagtgttctgcgataccatgaacagcctgacactgcccagcgaggtgtccctgtgcaacaccgacatcttcaactctaagtacgactgcaagatcatgacctccaagaccgacatcagctcctccgtgatcacatctctgggcgccatcgtgtcctgctacggcaagacaaagtgtaccgccagcaacaagaaccggggcatcatcaagaccttcagcaacggctgcgactacgtgtccaacaaaggcgtggacaccgtgtctgtgggcaacaccctgtactacgtgaacaagctggaaggcaagaatctgtacgtgaagggcgagcccatcatcaactactacgaccctctggtgttccccagcagcgagtttgatgccagcatcagccaagtgaacgagaagatcaaccagagcctggccttcatccgcagatccgatgaactgctgtctgccatcggcggctatatccccgaagctcctagagatggacaggcctatgtgcggaaggatggcgaatgggtgctgctgtctaccttcctgtgatga

SEQ ID NO: 131 - DNA, 1638 bp, synthetic construct
  source 1..1638: mol_type = other DNA
atggaactgcccatcctgaaaacaaacgccatcaccaccatcctggccgccgtgacactgtgttttgccagcagccagaacatcaccgaagagttctaccagagcacctgtagcgccgtgtctaagggctatctgtctgccctgagaaccggctggtatcacagcgtgatcaccatcgagctgagcaacatcaaagaaaacaagtgcaacggcaccgacgccaaagtgaagctgatcaagcaagagctggacaagtacaagaacgccgtgaccgaactgcagctgctgatgcagtctacctgcgccgccaatagcagagccagacgggaactgcctagattcatgaactacaccctgaacaacaccaagaacaccaacgtgaccctgagcaagaagcggaagcggagattcctgggctttctgctcggagtgggaagcgccattgcctctggatgcgccgtgtccaaggtgctgcatctggaaggcgaagtgaacaagatcaagagcgccctgctgagcaccaacaaggccgtggtttctctgagcaatggcgtgtccgtgctgaccatcaaggtgctggacctgaagaactacatcgacaaacagctgctgcccatcgtcaacaagcagagctgcagcatcagcaacatcgagacagtgatcgagttccagcagaagaacaaccggctgctggaaatcacccgcgagttttctgtgaatgccggcgtgaccacacctgtgtccacctacatgctgaccaacagcgagctgctgtccctgatcaacgacatgcccatcaccaacgaccagaaaaagctgatgagcagcaacgtgcagatcgtgcggcagcagagctactccatcatgagcattatcaaagaagagatcctggcctacgtggtgcagctgcctctgtatggcgtgatcgataccccttgctggaagctgcacacaagccctctgtgcaccaccaacaccaaagagggctccaacatctgcctgaccagaaccgatagaggctggtactgcgataatgccggcagcgtcagcttcttcccacaagccgagacatgcaaggtgcagagcaacagagtgttctgcgataccatgaacagcctgacactgccctccgaagtgaatctgtgcaatatcgacatcttcaacccgaagtacgactgcaagatcatgaccagcaagaccgacgtgtcaagctccgtgatcacatctctgggcgccatcgtgtcctgctacggcaagacaaagtgcaccgccagcaacaagaaccggggcatcatcaagaccttcagcaacggctgcgactacgtgtccaacaaaggcgtggacaccgtgtctgtgggcaacaccctgtactacgtgaacaagcaagaaggcaagagcctgtacgtgaagggcgagcccatcatcaacttctacgaccctctggtgttccccagcagcgagtttgatgccagcatctcccaagtgaacgagaagatcaaccagagcctggccttcatcagaaagtccgatgagctgctgagcgccatcggcggctatatccctgaagctcctagagatggacaggcctatgtgcggaaggatggcgaatgggtgctgctgtctaccttcctgtgatga

SEQ ID NO: 132 - DNA, 1638 bp, synthetic construct
  source 1..1638: mol_type = other DNA
atggaactgctgattcacagaagcagcgccatctttctgaccctggccatcaatgccctgtacctgaccagcagccagaacatcaccgaagagttctaccagagcacctgtagcgccgtgtccagaggctacttttctgccctgagaaccggctggtatcacagcgtgatcaccatcgagctgagcaacatcaaagaaacaaagtgcaacggcaccgacaccaaagtgaagctgatcaagcaagagctggacaagtacaagaacgccgtgaccgaactgcagctgctgatgcagaatacctgcgccgccaacaaccgggccagaagagaagcccctcagtacatgaactacaccatcaacaccaccaagaacctgaacgtgtccatcagcaagaagcggaagcggagattcctgggctttctgctcggagtgggaagcgccattgcctctggatgcgccgtgtctaaggtgctgcacctggaaggcgaagtgaacaagatcaagaatgccctgctgagcaccaacaaggccgtggtgtctctgtctaatggcgtgtccgtgctgaccatcaaggtgctggacctgaagaactacatcaacaaccagctgctgcccatcgtgaaccagcagagctgccggatcagcaacatcgagacagtgatcgagttccagcagaagaacagcagactgctggaaatcacccgcgagttttccgtgaatgccggcgtgacaacacccctgagcacctacatgctgaccaacagcgagctgctgtccctgatcaacgacatgcccatcaccaacgaccagaaaaagctgatgagcagcaacgtgcagatcgtgcggcagcagtcctacagcatcatgagcattatcaaagaagagatcctggcctacgtggtgcagctgcctatctacggcgtgatcgataccccttgctggaagctgcacacaagccctctgtgcaccaccaatatcaaagagggctccaacatctgcctgaccagaaccgatagaggctggtactgcgataatgccggcagcgtcagcttcttcccacaagccgatacctgcaaggtgcagagcaacagagtgttctgcgataccatgaacagcctgacactgcccagcgaggtgtccctgtgcaacaccgacatcttcaactctaagtacgactgcaagatcatgacctccaagaccgacatcagctcctccgtgatcacatctctgggcgccatcgtgtcctgctacggcaagacaaagtgtaccgccagcaacaagaaccggggcatcatcaagaccttcagcaacggctgcgactacgtgtccaacaaaggcgtggacaccgtgtctgtgggcaacaccctgtactacgtgaacaagctggaaggcaagaatctgtacgtgaagggcgagcccatcatcaactactacgaccctctggtgttccccagcagcgagtttgatgccagcatcagccaagtgaacgagaagatcaaccagagcctggccttcatccgcagatccgatgaactgctgtctgccatcggcggctatatccccgaagctcctagagatggacaggcctatgtgcggaaggatggcgaatgggtgctgctgtctaccttcctgtgatga

SEQ ID NO: 133 - DNA, 1638 bp, synthetic construct
  source 1..1638: mol_type = other DNA
atggaactgcccatcctgaaaacaaacgccatcaccaccatcctggccgccgtgacactgtgttttgccagcagccagaacatcaccgaagagttctaccagagcacctgtagcgccgtgtctaagggctatctgtctgccctgagaaccggctggtatcacagcgtgatcaccatcgagctgagcaacatcaaagaaaacaagtgcaacggcaccgacgccaaagtgaagctgatcaagcaagagctggacaagtacaagaacgccgtgaccgaactgcagctgctgatgcagtctacccctgcctgcaatagcagagccagacgggaactgcctagattcatgaactacaccctgaacaacaccaagaacaccaacgtgaccctgagcaagaagcggaagcggagattcctgggctttctgctcggagtgggatgcgccattgcctctggaattgccgtgtccaaggtgctgcatctggaaggcgaagtgaacaagatcaagagcgccctgctgagcaccaacaaggccgtggtttctctgagcaatggcgtgtccgtgctgaccatcaaggtgctggacctgaagaactacatcgacaaacagctgctgcccatcgtcaacaagcagagctgcagcatcagcaacatcgagacagtgatcgagttccagcagaagaacaaccggctgctggaaatcacccgcgagttttctgtgaatgccggcgtgaccacacctgtgtccacctacatgctgaccaacagcgagctgctgtccctgatcaacgacatgcccatcaccaacgaccagaaaaagctgatgagcagcaacgtgcagatcgtgcggcagcagagctactccatcatgagcattatcaaagaagagatcctggcctacgtggtgcagctgcctctgtatggcgtgatcgataccccttgctggaagctgcacacaagccctctgtgcaccaccaacaccaaagagggctccaacatctgcctgaccagaaccgatagaggctggtactgcgataatgccggcagcgtcagcttcttcccacaagccgagacatgcaaggtgcagagcaacagagtgttctgcgataccatgaacagcctgacactgccctccgaagtgaatctgtgcaatatcgacatcttcaacccgaagtacgactgcaagatcatgaccagcaagaccgacgtgtcaagctccgtgatcacatctctgggcgccatcgtgtcctgctacggcaagacaaagtgcaccgccagcaacaagaaccggggcatcatcaagaccttcagcaacggctgcgactacgtgtccaacaaaggcgtggacaccgtgtctgtgggcaacaccctgtactacgtgaacaagcaagaaggcaagagcctgtacgtgaagggcgagcccatcatcaacttctacgaccctctggtgttccccagcagcgagtttgatgccagcatctcccaagtgaacgagaagatcaaccagagcctggccttcatcagaaagtccgatgagctgctgagcgccatcggcggctatatccctgaagctcctagagatggacaggcctatgtgcggaaggatggcgaatgggtgctgctgtctaccttcctgtgatga

SEQ ID NO: 134 - DNA, 1638 bp, synthetic construct
  source 1..1638: mol_type = other DNA
atggaactgctgattcacagaagcagcgccatctttctgaccctggccatcaatgccctgtacctgaccagcagccagaacatcaccgaagagttctaccagagcacctgtagcgccgtgtccagaggctacttttctgccctgagaaccggctggtatcacagcgtgatcaccatcgagctgagcaacatcaaagaaacaaagtgcaacggcaccgacaccaaagtgaagctgatcaagcaagagctggacaagtacaagaacgccgtgaccgaactgcagctgctgatgcagaatacccctgcctgcaacaaccgggccagaagagaagcccctcagtacatgaactacaccatcaacaccaccaagaacctgaacgtgtccatcagcaagaagcggaagcggagattcctgggctttctgctcggagtgggatgcgccattgcctctggaattgccgtgtctaaggtgctgcacctggaaggcgaagtgaacaagatcaagaatgccctgctgagcaccaacaaggccgtggtgtctctgtctaatggcgtgtccgtgctgaccatcaaggtgctggacctgaagaactacatcaacaaccagctgctgcccatcgtgaaccagcagagctgccggatcagcaacatcgagacagtgatcgagttccagcagaagaacagcagactgctggaaatcacccgcgagttttccgtgaatgccggcgtgacaacacccctgagcacctacatgctgaccaacagcgagctgctgtccctgatcaacgacatgcccatcaccaacgaccagaaaaagctgatgagcagcaacgtgcagatcgtgcggcagcagtcctacagcatcatgagcattatcaaagaagagatcctggcctacgtggtgcagctgcctatctacggcgtgatcgataccccttgctggaagctgcacacaagccctctgtgcaccaccaatatcaaagagggctccaacatctgcctgaccagaaccgatagaggctggtactgcgataatgccggcagcgtcagcttcttcccacaagccgatacctgcaaggtgcagagcaacagagtgttctgcgataccatgaacagcctgacactgcccagcgaggtgtccctgtgcaacaccgacatcttcaactctaagtacgactgcaagatcatgacctccaagaccgacatcagctcctccgtgatcacatctctgggcgccatcgtgtcctgctacggcaagacaaagtgtaccgccagcaacaagaaccggggcatcatcaagaccttcagcaacggctgcgactacgtgtccaacaaaggcgtggacaccgtgtctgtgggcaacaccctgtactacgtgaacaagctggaaggcaagaatctgtacgtgaagggcgagcccatcatcaactactacgaccctctggtgttccccagcagcgagtttgatgccagcatcagccaagtgaacgagaagatcaaccagagcctggccttcatccgcagatccgatgaactgctgtctgccatcggcggctatatccccgaagctcctagagatggacaggcctatgtgcggaaggatggcgaatgggtgctgctgtctaccttcctgtgatga

SEQ ID NO: 135 - DNA, 1638 bp, synthetic construct
  source 1..1638: mol_type = other DNA
atggaactgcccatcctgaaaacaaacgccatcaccaccatcctggccgccgtgacactgtgttttgccagcagccagaacatcaccgaagagttctaccagagcacctgtagcgccgtgtctaagggctatctgtctgccctgagaaccggctggtataccagcgtgatcaccatcgagctgagcaacatcaaaatcaacaagtgcaacggcaccgacgccaaagtgaagctgatcaagcaagagctggacaagtacaagaacgccgtgaccgaactgcagctgctgatgcagtctacccctgccgccaatagcagagccagacgggaactgcctagattcatgaactacaccctgaacaacaccaagaacaccaacgtgaccctgagcaagaagcggaagcggagattcctgggctttctgctcggagtgggaagcgccattgcctctggaattgccgtgtccaaggtgctgcatctggaaggcgaagtgaacaagatcaagagcgccctgctgagcaccaacaaggccgtggtttctctgagcaatggcgtgtccgtgctgacctctaaggtgctggacctgaagaactacatcgacaaacagctgctgcccatcgtcaacaagcagagctgcagcatcagccccatcgagacagtgatcgagttccagcagaagaacaaccggctgctggaaatcacccgcgagttttctgtgaatgccggcgtgaccacacctgtgtccacctacatgctgaccaacagcgagctgctgtccctgatcaacgacatgcccatcaccaacgaccagaaaaagctgatgagcagcaacgtgcagatcgtgcggcagcagagctactccatcatgagcattatcaaagaagaggtgctggcctacgtggtgcagctgcctctgtatggcgtgatcgataccccttgctggaagctgcacacaagccctctgtgcaccaccaacaccaaagagggctccaacatctgcctgaccagaaccgatagaggctggtactgcgataatgccggcagcgtcagcttcttcccacaagccgagacatgcaaggtgcagagcaacagagtgttctgcgataccatgaacagcctgacactgccctccgaagtgaatctgtgcaatatcgacatcttcaacccgaagtacgactgcaagatcatgaccagcaagaccgacgtgtcaagctccgtgatcacatctctgggcgccatcgtgtcctgctacggcaagacaaagtgcaccgccagcaacaagaaccggggcatcatcaagaccttcagcaacggctgcgactacgtgtccaacaaaggcgtggacaccgtgtctgtgggcaacaccctgtactacgtgaacaagcaagaaggcaagagcctgtacgtgaagggcgagcccatcatcaacttctacgaccctctggtgttccccagccaggagtttgatgccagcatctcccaagtgaacgagaagatcaaccagagcctggccttcatcagaaagtccgatgagctgctgagcgccatcggcggctatatccctgaagctcctagagatggacaggcctatgtgcggaaggatggcgaatgggtgctgctgtctaccttcctgtgatga

SEQ ID NO: 136 - DNA, 1638 bp, synthetic construct
  source 1..1638: mol_type = other DNA
atggaactgctgattcacagaagcagcgccatctttctgaccctggccatcaatgccctgtacctgaccagcagccagaacatcaccgaagagttctaccagagcacctgtagcgccgtgtccagaggctacttttctgccctgagaaccggctggtataccagcgtgatcaccatcgagctgagcaacatcaaaatcacaaagtgcaacggcaccgacaccaaagtgaagctgatcaagcaagagctggacaagtacaagaacgccgtgaccgaactgcagctgctgatgcagaatacccctgccgccaacaaccgggccagaagagaagcccctcagtacatgaactacaccatcaacaccaccaagaacctgaacgtgtccatcagcaagaagcggaagcggagattcctgggctttctgctcggagtgggaagcgccattgcctctggaattgccgtgtctaaggtgctgcacctggaaggcgaagtgaacaagatcaagaatgccctgctgagcaccaacaaggccgtggtgtctctgtctaatggcgtgtccgtgctgaccagcaaggtgctggacctgaagaactacatcaacaaccagctgctgcccatcgtgaaccagcagagctgccggatcagccccatcgagacagtgatcgagttccagcagaagaacagcagactgctggaaatcacccgcgagttttccgtgaatgccggcgtgacaacacccctgagcacctacatgctgaccaacagcgagctgctgtccctgatcaacgacatgcccatcaccaacgaccagaaaaagctgatgagcagcaacgtgcagatcgtgcggcagcagtcctacagcatcatgagcattatcaaagaagaggtgctggcctacgtggtgcagctgcctatctacggcgtgatcgataccccttgctggaagctgcacacaagccctctgtgcaccaccaatatcaaagagggctccaacatctgcctgaccagaaccgatagaggctggtactgcgataatgccggcagcgtcagcttcttcccacaagccgatacctgcaaggtgcagagcaacagagtgttctgcgataccatgaacagcctgacactgcccagcgaggtgtccctgtgcaacaccgacatcttcaactctaagtacgactgcaagatcatgacctccaagaccgacatcagctcctccgtgatcacatctctgggcgccatcgtgtcctgctacggcaagacaaagtgtaccgccagcaacaagaaccggggcatcatcaagaccttcagcaacggctgcgactacgtgtccaacaaaggcgtggacaccgtgtctgtgggcaacaccctgtactacgtgaacaagctggaaggcaagaatctgtacgtgaagggcgagcccatcatcaactactacgaccctctggtgttccccagccaggagtttgatgccagcatcagccaagtgaacgagaagatcaaccagagcctggccttcatccgcagatccgatgaactgctgtctgccatcggcggctatatccccgaagctcctagagatggacaggcctatgtgcggaaggatggcgaatgggtgctgctgtctaccttcctgtgatga

SEQ ID NO: 137 - DNA, 1638 bp, synthetic construct
  source 1..1638: mol_type = other DNA
atggaactgcccatcctgaaaacaaacgccatcaccaccatcctggccgccgtgacactgtgttttgccagcagccagaacatcaccgaagagttctaccagagcacctgtagcgccgtgtctaagggctatctgtctgccctgagaaccggctggtataccagcgtgatcaccatcgagctgagcaacatcaaaatcaacaagtgcaacggcaccgacgccaaagtgaagctgatcaagcaagagctggacaagtacaagaacgccgtgaccgaactgcagctgctgatgcagtctacccctgccgccaatagcagagccagacgggaactgcctagattcatgaactacaccctgaacaacaccaagaacaccaacgtgaccctgagcaagaagcggaagcggagattcctgggctttctgctcggagtgggaagcgccattgcctctggaattgccgtgtccaaggtgctgcatctggaaggcgaagtgaacaagatcaagagcgccctgctgagcaccaacaaggccgtggtttctctgagcaatggcgtgtccgtgctgacctctaaggtgctggacctgaagaactacatcgacaaacagctgctgcccatcgtcaacaagcagagctgcagcatcagccccatcgagacagtgatcgagttccagcagaagaacaaccggctgctggaaatcacccgcgagttttctgtgaatgccggcgtgaccacacctgtgtccacctacatgctgaccaacagcgagctgctgtccctgatcaacgacatgcccatcaccaacgaccagaaaaagctgatgagcagcaacgtgcagatcgtgcggcagcagagctactccatcatgagcattatcaaagaagaggtgctggcctacgtggtgcagctgcctctgtatggcgtgatcgataccccttgctggaagctgcacacaagccctctgtgcaccaccaacaccaaagagggctccaacatctgcctgaccagaaccgatagaggctggtactgcgataatgccggcagcgtcagcttcttcccacaagccgagacatgcaaggtgcagagcaacagagtgttctgcgataccatgaacagcctgacactgccctccgaagtgaatctgtgcaatatcgacatcttcaacccgaagtacgactgcaagatcatgaccagcaagaccgacgtgtcaagctccgtgatcacatctctgggcgccatcgtgtcctgctacggcaagacaaagtgcaccgccagcaacaagaaccggggcatcatcaagaccttcagcaacggctgcgactacgtgtccaacaaaggcgtggacaccgtgtctgtgggcaacaccctgtactacgtgaacaagcaagaaggcaagagcctgtacgtgaagggcgagcccatcatcaacttctacgaccctctggtgttccccagcgacacctttgatgccagcatctcccaagtgaacgagaagatcaaccagagcctggccttcatcagaaagtccgatgagctgctgagcgccatcggcggctatatccctgaagctcctagagatggacaggcctatgtgcggaaggatggcgaatgggtgctgctgtctaccttcctgtgatga

SEQ ID NO: 138 - DNA, 1638 bp, synthetic construct
  source 1..1638: mol_type = other DNA
atggaactgctgattcacagaagcagcgccatctttctgaccctggccatcaatgccctgtacctgaccagcagccagaacatcaccgaagagttctaccagagcacctgtagcgccgtgtccagaggctacttttctgccctgagaaccggctggtataccagcgtgatcaccatcgagctgagcaacatcaaaatcacaaagtgcaacggcaccgacaccaaagtgaagctgatcaagcaagagctggacaagtacaagaacgccgtgaccgaactgcagctgctgatgcagaatacccctgccgccaacaaccgggccagaagagaagcccctcagtacatgaactacaccatcaacaccaccaagaacctgaacgtgtccatcagcaagaagcggaagcggagattcctgggctttctgctcggagtgggaagcgccattgcctctggaattgccgtgtctaaggtgctgcacctggaaggcgaagtgaacaagatcaagaatgccctgctgagcaccaacaaggccgtggtgtctctgtctaatggcgtgtccgtgctgaccagcaaggtgctggacctgaagaactacatcaacaaccagctgctgcccatcgtgaaccagcagagctgccggatcagccccatcgagacagtgatcgagttccagcagaagaacagcagactgctggaaatcacccgcgagttttccgtgaatgccggcgtgacaacacccctgagcacctacatgctgaccaacagcgagctgctgtccctgatcaacgacatgcccatcaccaacgaccagaaaaagctgatgagcagcaacgtgcagatcgtgcggcagcagtcctacagcatcatgagcattatcaaagaagaggtgctggcctacgtggtgcagctgcctatctacggcgtgatcgataccccttgctggaagctgcacacaagccctctgtgcaccaccaatatcaaagagggctccaacatctgcctgaccagaaccgatagaggctggtactgcgataatgccggcagcgtcagcttcttcccacaagccgatacctgcaaggtgcagagcaacagagtgttctgcgataccatgaacagcctgacactgcccagcgaggtgtccctgtgcaacaccgacatcttcaactctaagtacgactgcaagatcatgacctccaagaccgacatcagctcctccgtgatcacatctctgggcgccatcgtgtcctgctacggcaagacaaagtgtaccgccagcaacaagaaccggggcatcatcaagaccttcagcaacggctgcgactacgtgtccaacaaaggcgtggacaccgtgtctgtgggcaacaccctgtactacgtgaacaagctggaaggcaagaatctgtacgtgaagggcgagcccatcatcaactactacgaccctctggtgttccccagcgacacctttgatgccagcatcagccaagtgaacgagaagatcaaccagagcctggccttcatccgcagatccgatgaactgctgtctgccatcggcggctatatccccgaagctcctagagatggacaggcctatgtgcggaaggatggcgaatgggtgctgctgtctaccttcctgtgatga

SEQ ID NO: 139 - DNA, 1638 bp, synthetic construct
  source 1..1638: mol_type = other DNA
atggaactgcccatcctgaaaacaaacgccatcaccaccatcctggccgccgtgacactgtgttttgccagcagccagaacatcaccgaagagttctaccagagcacctgtagcgccgtgtctaagggctatctgtctgccctgagaaccggctggtataccagcgtgatcaccatcgagctgagcaacatcaaagaaatcaagtgcaacggcaccgacgccaaagtgaagctgatcaagcaagagctggacaagtacaagaacgccgtgaccgaactgcagctgctgatgcagtctacccctgccgccaatagcagagccagacgggaactgcctagattcatgaactacaccctgaacaacaccaagaacaccaacgtgaccctgagcaagaagcggaagcggagattcctgggctttctgctcggagtgggaagcgccattgcctctggaattgccgtgtccaaggtgctgcatctggaaggcgaagtgaacaagatcaagagcgccctgctgagcaccaacaaggccgtggtttctctgagcaatggcgtgtccgtgctgacctctaaggtgctggacctgaagaactacatcgacaaacagctgctgcccatcgtcaacaagcagagctgcagcatcagccccatcgagacagtgatcgagttccagcagaagaacaaccggctgctggaaatcacccgcgagttttctgtgaatgccggcgtgaccacacctgtgtccacctacatgctgaccaacagcgagctgctgtccctgatcaacgacatgcccatcaccaacgaccagaaaaagctgatgagcagcaacgtgcagatcgtgcggcagcagagctactccatcatgagcattatcaaagaagaggtgctggcctacgtggtgcagctgcctctgtatggcgtgatcgataccccttgctggaagctgcacacaagccctctgtgcaccaccaacaccaaagagggctccaacatctgcctgaccagaaccgatagaggctggtactgcgataatgccggcagcgtcagcttcttcccacaagccgagacatgcaaggtgcagagcaacagagtgttctgcgataccatgaacagcctgacactgccctccgaagtgaatctgtgcaatatcgacatcttcaacccgaagtacgactgcaagatcatgaccagcaagaccgacgtgtcaagctccgtgatcacatctctgggcgccatcgtgtcctgctacggcaagacaaagtgcaccgccagcaacaagaaccggggcatcatcaagaccttcagcaacggctgcgactacgtgtccaacaaaggcgtggacaccgtgtctgtgggcaacaccctgtactacgtgaacaagcaagaaggcaagagcctgtacgtgaagggcgagcccatcatcaacttctacgaccctctggtgttccccagcgaccagtttgatgccagcatctcccaagtgaacgagaagatcaaccagagcctggccttcatcagaaagtccgatgagctgctgagcgccatcggcggctatatccctgaagctcctagagatggacaggcctatgtgcggaaggatggcgaatgggtgctgctgtctaccttcctgtgatga

SEQ ID NO: 140 - DNA, 1638 bp, synthetic construct
  source 1..1638: mol_type = other DNA
atggaactgctgattcacagaagcagcgccatctttctgaccctggccatcaatgccctgtacctgaccagcagccagaacatcaccgaagagttctaccagagcacctgtagcgccgtgtccagaggctacttttctgccctgagaaccggctggtataccagcgtgatcaccatcgagctgagcaacatcaaagaaatcaagtgcaacggcaccgacaccaaagtgaagctgatcaagcaagagctggacaagtacaagaacgccgtgaccgaactgcagctgctgatgcagaatacccctgccgccaacaaccgggccagaagagaagcccctcagtacatgaactacaccatcaacaccaccaagaacctgaacgtgtccatcagcaagaagcggaagcggagattcctgggctttctgctcggagtgggaagcgccattgcctctggaattgccgtgtctaaggtgctgcacctggaaggcgaagtgaacaagatcaagaatgccctgctgagcaccaacaaggccgtggtgtctctgtctaatggcgtgtccgtgctgaccagcaaggtgctggacctgaagaactacatcaacaaccagctgctgcccatcgtgaaccagcagagctgccggatcagccccatcgagacagtgatcgagttccagcagaagaacagcagactgctggaaatcacccgcgagttttccgtgaatgccggcgtgacaacacccctgagcacctacatgctgaccaacagcgagctgctgtccctgatcaacgacatgcccatcaccaacgaccagaaaaagctgatgagcagcaacgtgcagatcgtgcggcagcagtcctacagcatcatgagcattatcaaagaagaggtgctggcctacgtggtgcagctgcctatctacggcgtgatcgataccccttgctggaagctgcacacaagccctctgtgcaccaccaatatcaaagagggctccaacatctgcctgaccagaaccgatagaggctggtactgcgataatgccggcagcgtcagcttcttcccacaagccgatacctgcaaggtgcagagcaacagagtgttctgcgataccatgaacagcctgacactgcccagcgaggtgtccctgtgcaacaccgacatcttcaactctaagtacgactgcaagatcatgacctccaagaccgacatcagctcctccgtgatcacatctctgggcgccatcgtgtcctgctacggcaagacaaagtgtaccgccagcaacaagaaccggggcatcatcaagaccttcagcaacggctgcgactacgtgtccaacaaaggcgtggacaccgtgtctgtgggcaacaccctgtactacgtgaacaagctggaaggcaagaatctgtacgtgaagggcgagcccatcatcaactactacgaccctctggtgttccccagcgaccagtttgatgccagcatcagccaagtgaacgagaagatcaaccagagcctggccttcatccgcagatccgatgaactgctgtctgccatcggcggctatatccccgaagctcctagagatggacaggcctatgtgcggaaggatggcgaatgggtgctgctgtctaccttcctgtgatga

SEQ ID NO: 141 - DNA, 1638 bp, synthetic construct
  source 1..1638: mol_type = other DNA
atggaactgcccatcctgaaaacaaacgccatcaccaccatcctggccgccgtgacactgtgttttgccagcagccagaacatcaccgaagagttctaccagagcacctgtagcgccgtgtctaagggctatctgtctgccctgagaaccggctggtataccagcgtgatcaccatcgagctgagcaacatcaaaatcaacaagtgcaacggcaccgacgccaaagtgaagctgatcaagcaagagctggacaagtacaagaacgccgtgaccgaactgcagctgctgatgcagtctacccctgccgccaatagcagagccagacgggaactgcctagattcatgaactacaccctgaacaacaccaagaacaccaacgtgaccctgagcaagaagcggaagcggagattcctgggctttctgctcggagtgggaagcgccattgcctctggaattgccgtgtccaaggtgctgcatctggaaggcgaagtgaacaagatcaagagcgccctgctgagcaccaacaaggccgtggtttctctgagcaatggcgtgtccgtgctgacctctaaggtgctggacctgaagaactacatcgacaaacagctgctgcccatcgtcaacaagcagagctgccccatcagcaacatcgagacagtgatcgagttccagcagaagaacaaccggctgctggaaatcacccgcgagttttctgtgaatgccggcgtgaccacacctgtgtccacctacatgctgaccaacagcgagctgctgtccctgatcaacgacatgcccatcaccaacgaccagaaaaagctgatgagcagcaacgtgcagatcgtgcggcagcagagctactccatcatgagcattatcaaagaagaggtgctggcctacgtggtgcagctgcctctgtatggcgtgatcgataccccttgctggaagctgcacacaagccctctgtgcaccaccaacaccaaagagggctccaacatctgcctgaccagaaccgatagaggctggtactgcgataatgccggcagcgtcagcttcttcccacaagccgagacatgcaaggtgcagagcaacagagtgttctgcgataccatgaacagcctgacactgccctccgaagtgaatctgtgcaatatcgacatcttcaacccgaagtacgactgcaagatcatgaccagcaagaccgacgtgtcaagctccgtgatcacatctctgggcgccatcgtgtcctgctacggcaagacaaagtgcaccgccagcaacaagaaccggggcatcatcaagaccttcagcaacggctgcgactacgtgtccaacaaaggcgtggacaccgtgtctgtgggcaacaccctgtactacgtgaacaagcaagaaggcaagagcctgtacgtgaagggcgagcccatcatcaacttctacgaccctctggtgttccccagccaggagtttgatgccagcatctcccaagtgaacgagaagatcaaccagagcctggccttcatcagaaagtccgatgagctgctgagcgccatcggcggctatatccctgaagctcctagagatggacaggcctatgtgcggaaggatggcgaatgggtgctgctgtctaccttcctgtgatga

SEQ ID NO: 142 - DNA, 1638 bp, synthetic construct
  source 1..1638: mol_type = other DNA
atggaactgctgattcacagaagcagcgccatctttctgaccctggccatcaatgccctgtacctgaccagcagccagaacatcaccgaagagttctaccagagcacctgtagcgccgtgtccagaggctacttttctgccctgagaaccggctggtataccagcgtgatcaccatcgagctgagcaacatcaaaatcacaaagtgcaacggcaccgacaccaaagtgaagctgatcaagcaagagctggacaagtacaagaacgccgtgaccgaactgcagctgctgatgcagaatacccctgccgccaacaaccgggccagaagagaagcccctcagtacatgaactacaccatcaacaccaccaagaacctgaacgtgtccatcagcaagaagcggaagcggagattcctgggctttctgctcggagtgggaagcgccattgcctctggaattgccgtgtctaaggtgctgcacctggaaggcgaagtgaacaagatcaagaatgccctgctgagcaccaacaaggccgtggtgtctctgtctaatggcgtgtccgtgctgaccagcaaggtgctggacctgaagaactacatcaacaaccagctgctgcccatcgtgaaccagcagagctgccccatcagcaacatcgagacagtgatcgagttccagcagaagaacagcagactgctggaaatcacccgcgagttttccgtgaatgccggcgtgacaacacccctgagcacctacatgctgaccaacagcgagctgctgtccctgatcaacgacatgcccatcaccaacgaccagaaaaagctgatgagcagcaacgtgcagatcgtgcggcagcagtcctacagcatcatgagcattatcaaagaagaggtgctggcctacgtggtgcagctgcctatctacggcgtgatcgataccccttgctggaagctgcacacaagccctctgtgcaccaccaatatcaaagagggctccaacatctgcctgaccagaaccgatagaggctggtactgcgataatgccggcagcgtcagcttcttcccacaagccgatacctgcaaggtgcagagcaacagagtgttctgcgataccatgaacagcctgacactgcccagcgaggtgtccctgtgcaacaccgacatcttcaactctaagtacgactgcaagatcatgacctccaagaccgacatcagctcctccgtgatcacatctctgggcgccatcgtgtcctgctacggcaagacaaagtgtaccgccagcaacaagaaccggggcatcatcaagaccttcagcaacggctgcgactacgtgtccaacaaaggcgtggacaccgtgtctgtgggcaacaccctgtactacgtgaacaagctggaaggcaagaatctgtacgtgaagggcgagcccatcatcaactactacgaccctctggtgttccccagccaggagtttgatgccagcatcagccaagtgaacgagaagatcaaccagagcctggccttcatccgcagatccgatgaactgctgtctgccatcggcggctatatccccgaagctcctagagatggacaggcctatgtgcggaaggatggcgaatgggtgctgctgtctaccttcctgtgatga

SEQ ID NO: 143 - DNA, 1638 bp, synthetic construct
  source 1..1638: mol_type = other DNA
atggaactgcccatcctgaaaacaaacgccatcaccaccatcctggccgccgtgacactgtgttttgccagcagccagaacatcaccgaagagttctaccagagcacctgtagcgccgtgtctaagggctatctgtctgccctgagaaccggctggtataccagcgtgatcaccatcgagctgagcaacatcaaaatcaacaagtgcaacggcaccgacgccaaagtgaagctgatcaagcaagagctggacaagtacaagaacgccgtgaccgaactgcagctgctgatgcagtctacccctgccgccaatagcagagccagacgggaactgcctagattcatgaactacaccctgaacaacaccaagaacaccaacgtgaccctgagcaagaagcggaagcggagattcctgggctttctgctcggagtgggaagcgccattgcctctggaattgccgtgtccaaggtgctgcatctggaaggcgaagtgaacaagatcaagagcgccctgctgagcaccaacaaggccgtggtttctctgagcaatggcgtgtccgtgctgacctctaaggtgctggacctgaagaactacatcgacaaacagctgctgcccatcgtcaacaagcagagctgccccatcagcaacatcgagacagtgatcgagttccagcagaagaacaaccggctgctggaaatcacccgcgagttttctgtgaatgccggcgtgaccacacctgtgtccacctacatgctgaccaacagcgagctgctgtccctgatcaacgacatgcccatcaccaacgaccagaaaaagctgatgagcagcaacgtgcagatcgtgcggcagcagagctactccatcatgagcattatcaaagaagaggtgctggcctacgtggtgcagctgcctctgtatggcgtgatcgataccccttgctggaagctgcacacaagccctctgtgcaccaccaacaccaaagagggctccaacatctgcctgaccagaaccgatagaggctggtactgcgataatgccggcagcgtcagcttcttcccacaagccgagacatgcaaggtgcagagcaacagagtgttctgcgataccatgaacagcctgacactgccctccgaagtgaatctgtgcaatatcgacatcttcaacccgaagtacgactgcaagatcatgaccagcaagaccgacgtgtcaagctccgtgatcacatctctgggcgccatcgtgtcctgctacggcaagacaaagtgcaccgccagcaacaagaaccggggcatcatcaagaccttcagcaacggctgcgactacgtgtccaacaaaggcgtggacaccgtgtctgtgggcaacaccctgtactacgtgaacaagcaagaaggcaagagcctgtacgtgaagggcgagcccatcatcaacttctacgaccctctggtgttccccagcgacacctttgatgccagcatctcccaagtgaacgagaagatcaaccagagcctggccttcatcagaaagtccgatgagctgctgagcgccatcggcggctatatccctgaagctcctagagatggacaggcctatgtgcggaaggatggcgaatgggtgctgctgtctaccttcctgtgatga

SEQ ID NO: 144 - DNA, 1638 bp, synthetic construct
  source 1..1638: mol_type = other DNA
atggaactgctgattcacagaagcagcgccatctttctgaccctggccatcaatgccctgtacctgaccagcagccagaacatcaccgaagagttctaccagagcacctgtagcgccgtgtccagaggctacttttctgccctgagaaccggctggtataccagcgtgatcaccatcgagctgagcaacatcaaaatcacaaagtgcaacggcaccgacaccaaagtgaagctgatcaagcaagagctggacaagtacaagaacgccgtgaccgaactgcagctgctgatgcagaatacccctgccgccaacaaccgggccagaagagaagcccctcagtacatgaactacaccatcaacaccaccaagaacctgaacgtgtccatcagcaagaagcggaagcggagattcctgggctttctgctcggagtgggaagcgccattgcctctggaattgccgtgtctaaggtgctgcacctggaaggcgaagtgaacaagatcaagaatgccctgctgagcaccaacaaggccgtggtgtctctgtctaatggcgtgtccgtgctgaccagcaaggtgctggacctgaagaactacatcaacaaccagctgctgcccatcgtgaaccagcagagctgccccatcagcaacatcgagacagtgatcgagttccagcagaagaacagcagactgctggaaatcacccgcgagttttccgtgaatgccggcgtgacaacacccctgagcacctacatgctgaccaacagcgagctgctgtccctgatcaacgacatgcccatcaccaacgaccagaaaaagctgatgagcagcaacgtgcagatcgtgcggcagcagtcctacagcatcatgagcattatcaaagaagaggtgctggcctacgtggtgcagctgcctatctacggcgtgatcgataccccttgctggaagctgcacacaagccctctgtgcaccaccaatatcaaagagggctccaacatctgcctgaccagaaccgatagaggctggtactgcgataatgccggcagcgtcagcttcttcccacaagccgatacctgcaaggtgcagagcaacagagtgttctgcgataccatgaacagcctgacactgcccagcgaggtgtccctgtgcaacaccgacatcttcaactctaagtacgactgcaagatcatgacctccaagaccgacatcagctcctccgtgatcacatctctgggcgccatcgtgtcctgctacggcaagacaaagtgtaccgccagcaacaagaaccggggcatcatcaagaccttcagcaacggctgcgactacgtgtccaacaaaggcgtggacaccgtgtctgtgggcaacaccctgtactacgtgaacaagctggaaggcaagaatctgtacgtgaagggcgagcccatcatcaactactacgaccctctggtgttccccagcgacacctttgatgccagcatcagccaagtgaacgagaagatcaaccagagcctggccttcatccgcagatccgatgaactgctgtctgccatcggcggctatatccccgaagctcctagagatggacaggcctatgtgcggaaggatggcgaatgggtgctgctgtctaccttcctgtgatga

SEQ ID NO: 145 - DNA, 1638 bp, synthetic construct
  source 1..1638: mol_type = other DNA
atggaactgcccatcctgaaaacaaacgccatcaccaccatcctggccgccgtgacactgtgttttgccagcagccagaacatcaccgaagagttctaccagagcacctgtagcgccgtgtctaagggctatctgtctgccctgagaaccggctggtataccagcgtgatcaccatcgagctgagcaacatcaaagaaatcaagtgcaacggcaccgacgccaaagtgaagctgatcaagcaagagctggacaagtacaagaacgccgtgaccgaactgcagctgctgatgcagtctacccctgccgccaatagcagagccagacgggaactgcctagattcatgaactacaccctgaacaacaccaagaacaccaacgtgaccctgagcaagaagcggaagcggagattcctgggctttctgctcggagtgggaagcgccattgcctctggaattgccgtgtccaaggtgctgcatctggaaggcgaagtgaacaagatcaagagcgccctgctgagcaccaacaaggccgtggtttctctgagcaatggcgtgtccgtgctgacctctaaggtgctggacctgaagaactacatcgacaaacagctgctgcccatcgtcaacaagcagagctgccccatcagcaacatcgagacagtgatcgagttccagcagaagaacaaccggctgctggaaatcacccgcgagttttctgtgaatgccggcgtgaccacacctgtgtccacctacatgctgaccaacagcgagctgctgtccctgatcaacgacatgcccatcaccaacgaccagaaaaagctgatgagcagcaacgtgcagatcgtgcggcagcagagctactccatcatgagcattatcaaagaagaggtgctggcctacgtggtgcagctgcctctgtatggcgtgatcgataccccttgctggaagctgcacacaagccctctgtgcaccaccaacaccaaagagggctccaacatctgcctgaccagaaccgatagaggctggtactgcgataatgccggcagcgtcagcttcttcccacaagccgagacatgcaaggtgcagagcaacagagtgttctgcgataccatgaacagcctgacactgccctccgaagtgaatctgtgcaatatcgacatcttcaacccgaagtacgactgcaagatcatgaccagcaagaccgacgtgtcaagctccgtgatcacatctctgggcgccatcgtgtcctgctacggcaagacaaagtgcaccgccagcaacaagaaccggggcatcatcaagaccttcagcaacggctgcgactacgtgtccaacaaaggcgtggacaccgtgtctgtgggcaacaccctgtactacgtgaacaagcaagaaggcaagagcctgtacgtgaagggcgagcccatcatcaacttctacgaccctctggtgttccccagcgaccagtttgatgccagcatctcccaagtgaacgagaagatcaaccagagcctggccttcatcagaaagtccgatgagctgctgagcgccatcggcggctatatccctgaagctcctagagatggacaggcctatgtgcggaaggatggcgaatgggtgctgctgtctaccttcctgtgatga

SEQ ID NO: 146 - DNA, 1638 bp, synthetic construct
  source 1..1638: mol_type = other DNA
atggaactgctgattcacagaagcagcgccatctttctgaccctggccatcaatgccctgtacctgaccagcagccagaacatcaccgaagagttctaccagagcacctgtagcgccgtgtccagaggctacttttctgccctgagaaccggctggtataccagcgtgatcaccatcgagctgagcaacatcaaagaaatcaagtgcaacggcaccgacaccaaagtgaagctgatcaagcaagagctggacaagtacaagaacgccgtgaccgaactgcagctgctgatgcagaatacccctgccgccaacaaccgggccagaagagaagcccctcagtacatgaactacaccatcaacaccaccaagaacctgaacgtgtccatcagcaagaagcggaagcggagattcctgggctttctgctcggagtgggaagcgccattgcctctggaattgccgtgtctaaggtgctgcacctggaaggcgaagtgaacaagatcaagaatgccctgctgagcaccaacaaggccgtggtgtctctgtctaatggcgtgtccgtgctgaccagcaaggtgctggacctgaagaactacatcaacaaccagctgctgcccatcgtgaaccagcagagctgccccatcagcaacatcgagacagtgatcgagttccagcagaagaacagcagactgctggaaatcacccgcgagttttccgtgaatgccggcgtgacaacacccctgagcacctacatgctgaccaacagcgagctgctgtccctgatcaacgacatgcccatcaccaacgaccagaaaaagctgatgagcagcaacgtgcagatcgtgcggcagcagtcctacagcatcatgagcattatcaaagaagaggtgctggcctacgtggtgcagctgcctatctacggcgtgatcgataccccttgctggaagctgcacacaagccctctgtgcaccaccaatatcaaagagggctccaacatctgcctgaccagaaccgatagaggctggtactgcgataatgccggcagcgtcagcttcttcccacaagccgatacctgcaaggtgcagagcaacagagtgttctgcgataccatgaacagcctgacactgcccagcgaggtgtccctgtgcaacaccgacatcttcaactctaagtacgactgcaagatcatgacctccaagaccgacatcagctcctccgtgatcacatctctgggcgccatcgtgtcctgctacggcaagacaaagtgtaccgccagcaacaagaaccggggcatcatcaagaccttcagcaacggctgcgactacgtgtccaacaaaggcgtggacaccgtgtctgtgggcaacaccctgtactacgtgaacaagctggaaggcaagaatctgtacgtgaagggcgagcccatcatcaactactacgaccctctggtgttccccagcgaccagtttgatgccagcatcagccaagtgaacgagaagatcaaccagagcctggccttcatccgcagatccgatgaactgctgtctgccatcggcggctatatccccgaagctcctagagatggacaggcctatgtgcggaaggatggcgaatgggtgctgctgtctaccttcctgtgatga

SEQ ID NO: 147 - DNA, 1638 bp, synthetic construct
  source 1..1638: mol_type = other DNA
atggaactgcccatcctgaaaacaaacgccatcaccaccatcctggccgccgtgacactgtgttttgccagcagccagaacatcaccgaagagttctaccagagcacctgtagcgccgtgtctaagggctatctgtctgccctgagaaccggctggtataccagcgtgatcaccatcgagctgagcaacatcaaagaaatcaagtgcaacggcaccgacgccaaagtgaagctgatcaagcaagagctggacaagtacaagaacgccgtgaccgaactgcagctgctgatgcagtctacccctgccgccaatagcagagccagacgggaactgcctagattcatgaactacaccctgaacaacaccaagaacaccaacgtgaccctgagcaagaagcggaagcggagattcctgggctttctgctcggagtgggaagcgccattgcctctggaattgccgtgtccaaggtgctgcatctggaaggcgaagtgaacaagatcaagagcgccctgctgagcaccaacaaggccgtggtttctctgagcaatggcgtgtccgtgctgacctctaaggtgctggacctgaagaactacatcgacaaacagctgctgcccatcgtcaacaagcagagctgcagcatccccaacatcgagacagtgatcgagttccagcagaagaacaaccggctgctggaaatcacccgcgagttttctgtgaatgccggcgtgaccacacctgtgtccacctacatgctgaccaacagcgagctgctgtccctgatcaacgacatgcccatcaccaacgaccagaaaaagctgatgagcagcaacgtgcagatcgtgcggcagcagagctactccatcatgagcattatcaaagaagaggtgctggcctacgtggtgcagctgcctctgtatggcgtgatcgataccccttgctggaagctgcacacaagccctctgtgcaccaccaacaccaaagagggctccaacatctgcctgaccagaaccgatagaggctggtactgcgataatgccggcagcgtcagcttcttcccacaagccgagacatgcaaggtgcagagcaacagagtgttctgcgataccatgaacagcctgacactgccctccgaagtgaatctgtgcaatatcgacatcttcaacccgaagtacgactgcaagatcatgaccagcaagaccgacgtgtcaagctccgtgatcacatctctgggcgccatcgtgtcctgctacggcaagacaaagtgcaccgccagcaacaagaaccggggcatcatcaagaccttcagcaacggctgcgactacgtgtccaacaaaggcgtggacaccgtgtctgtgggcaacaccctgtactacgtgaacaagcaagaaggcaagagcctgtacgtgaagggcgagcccatcatcaacttctacgaccctctggtgttccccagcgaccagtttgatgccagcatctcccaagtgaacgagaagatcaaccagagcctggccttcatcagaaagtccgatgagctgctgagcgccatcggcggctatatccctgaagctcctagagatggacaggcctatgtgcggaaggatggcgaatgggtgctgctgtctaccttcctgtgatga

SEQ ID NO: 148 - DNA, 1638 bp, synthetic construct
  source 1..1638: mol_type = other DNA
atggaactgctgattcacagaagcagcgccatctttctgaccctggccatcaatgccctgtacctgaccagcagccagaacatcaccgaagagttctaccagagcacctgtagcgccgtgtccagaggctacttttctgccctgagaaccggctggtataccagcgtgatcaccatcgagctgagcaacatcaaagaaatcaagtgcaacggcaccgacaccaaagtgaagctgatcaagcaagagctggacaagtacaagaacgccgtgaccgaactgcagctgctgatgcagaatacccctgccgccaacaaccgggccagaagagaagcccctcagtacatgaactacaccatcaacaccaccaagaacctgaacgtgtccatcagcaagaagcggaagcggagattcctgggctttctgctcggagtgggaagcgccattgcctctggaattgccgtgtctaaggtgctgcacctggaaggcgaagtgaacaagatcaagaatgccctgctgagcaccaacaaggccgtggtgtctctgtctaatggcgtgtccgtgctgaccagcaaggtgctggacctgaagaactacatcaacaaccagctgctgcccatcgtgaaccagcagagctgccggatccccaacatcgagacagtgatcgagttccagcagaagaacagcagactgctggaaatcacccgcgagttttccgtgaatgccggcgtgacaacacccctgagcacctacatgctgaccaacagcgagctgctgtccctgatcaacgacatgcccatcaccaacgaccagaaaaagctgatgagcagcaacgtgcagatcgtgcggcagcagtcctacagcatcatgagcattatcaaagaagaggtgctggcctacgtggtgcagctgcctatctacggcgtgatcgataccccttgctggaagctgcacacaagccctctgtgcaccaccaatatcaaagagggctccaacatctgcctgaccagaaccgatagaggctggtactgcgataatgccggcagcgtcagcttcttcccacaagccgatacctgcaaggtgcagagcaacagagtgttctgcgataccatgaacagcctgacactgcccagcgaggtgtccctgtgcaacaccgacatcttcaactctaagtacgactgcaagatcatgacctccaagaccgacatcagctcctccgtgatcacatctctgggcgccatcgtgtcctgctacggcaagacaaagtgtaccgccagcaacaagaaccggggcatcatcaagaccttcagcaacggctgcgactacgtgtccaacaaaggcgtggacaccgtgtctgtgggcaacaccctgtactacgtgaacaagctggaaggcaagaatctgtacgtgaagggcgagcccatcatcaactactacgaccctctggtgttccccagcgaccagtttgatgccagcatcagccaagtgaacgagaagatcaaccagagcctggccttcatccgcagatccgatgaactgctgtctgccatcggcggctatatccccgaagctcctagagatggacaggcctatgtgcggaaggatggcgaatgggtgctgctgtctaccttcctgtgatga

SEQ ID NO: 149 - DNA, 1638 bp, synthetic construct
  source 1..1638: mol_type = other DNA
atggaactgcccatcctgaaaacaaacgccatcaccaccatcctggccgccgtgacactgtgttttgccagcagccagaacatcaccgaagagttctaccagagcacctgtagcgccgtgtctaagggctatctgtctgccctgagaaccggctggtataccagcgtgatcaccatcgagctgagcaacatcaaaatcaacaagtgcaacggcaccgacgccaaagtgaagctgatcaagcaagagctggacaagtacaagaacgccgtgaccgaactgcagctgctgatgcagtctacccctgccgccaatagcagagccagacgggaactgcctagattcatgaactacaccctgaacaacaccaagaacaccaacgtgaccctgagcaagaagcggaagcggagattcctgggctttctgctcggagtgggaagcgccattgcctctggaattgccgtgtccaaggtgctgcatctggaaggcgaagtgaacaagatcaagagcgccctgctgagcaccaacaaggccgtggtttctctgagcaatggcgtgtccgtgctgacctctaaggtgctggacctgaagaactacatcgacaaacagctgctgcccatcgtcaacaagcagagctgcagcatcagcaaccccgagacagtgatcgagttccagcagaagaacaaccggctgctggaaatcacccgcgagttttctgtgaatgccggcgtgaccacacctgtgtccacctacatgctgaccaacagcgagctgctgtccctgatcaacgacatgcccatcaccaacgaccagaaaaagctgatgagcagcaacgtgcagatcgtgcggcagcagagctactccatcatgagcattatcaaagaagaggtgctggcctacgtggtgcagctgcctctgtatggcgtgatcgataccccttgctggaagctgcacacaagccctctgtgcaccaccaacaccaaagagggctccaacatctgcctgaccagaaccgatagaggctggtactgcgataatgccggcagcgtcagcttcttcccacaagccgagacatgcaaggtgcagagcaacagagtgttctgcgataccatgaacagcctgacactgccctccgaagtgaatctgtgcaatatcgacatcttcaacccgaagtacgactgcaagatcatgaccagcaagaccgacgtgtcaagctccgtgatcacatctctgggcgccatcgtgtcctgctacggcaagacaaagtgcaccgccagcaacaagaaccggggcatcatcaagaccttcagcaacggctgcgactacgtgtccaacaaaggcgtggacaccgtgtctgtgggcaacaccctgtactacgtgaacaagcaagaaggcaagagcctgtacgtgaagggcgagcccatcatcaacttctacgaccctctggtgttccccagcgacacctttgatgccagcatctcccaagtgaacgagaagatcaaccagagcctggccttcatcagaaagtccgatgagctgctgagcgccatcggcggctatatccctgaagctcctagagatggacaggcctatgtgcggaaggatggcgaatgggtgctgctgtctaccttcctgtgatga

SEQ ID NO: 150 - DNA, 1638 bp, synthetic construct
  source 1..1638: mol_type = other DNA
atggaactgctgattcacagaagcagcgccatctttctgaccctggccatcaatgccctgtacctgaccagcagccagaacatcaccgaagagttctaccagagcacctgtagcgccgtgtccagaggctacttttctgccctgagaaccggctggtataccagcgtgatcaccatcgagctgagcaacatcaaaatcacaaagtgcaacggcaccgacaccaaagtgaagctgatcaagcaagagctggacaagtacaagaacgccgtgaccgaactgcagctgctgatgcagaatacccctgccgccaacaaccgggccagaagagaagcccctcagtacatgaactacaccatcaacaccaccaagaacctgaacgtgtccatcagcaagaagcggaagcggagattcctgggctttctgctcggagtgggaagcgccattgcctctggaattgccgtgtctaaggtgctgcacctggaaggcgaagtgaacaagatcaagaatgccctgctgagcaccaacaaggccgtggtgtctctgtctaatggcgtgtccgtgctgaccagcaaggtgctggacctgaagaactacatcaacaaccagctgctgcccatcgtgaaccagcagagctgccggatcagcaaccccgagacagtgatcgagttccagcagaagaacagcagactgctggaaatcacccgcgagttttccgtgaatgccggcgtgacaacacccctgagcacctacatgctgaccaacagcgagctgctgtccctgatcaacgacatgcccatcaccaacgaccagaaaaagctgatgagcagcaacgtgcagatcgtgcggcagcagtcctacagcatcatgagcattatcaaagaagaggtgctggcctacgtggtgcagctgcctatctacggcgtgatcgataccccttgctggaagctgcacacaagccctctgtgcaccaccaatatcaaagagggctccaacatctgcctgaccagaaccgatagaggctggtactgcgataatgccggcagcgtcagcttcttcccacaagccgatacctgcaaggtgcagagcaacagagtgttctgcgataccatgaacagcctgacactgcccagcgaggtgtccctgtgcaacaccgacatcttcaactctaagtacgactgcaagatcatgacctccaagaccgacatcagctcctccgtgatcacatctctgggcgccatcgtgtcctgctacggcaagacaaagtgtaccgccagcaacaagaaccggggcatcatcaagaccttcagcaacggctgcgactacgtgtccaacaaaggcgtggacaccgtgtctgtgggcaacaccctgtactacgtgaacaagctggaaggcaagaatctgtacgtgaagggcgagcccatcatcaactactacgaccctctggtgttccccagcgacacctttgatgccagcatcagccaagtgaacgagaagatcaaccagagcctggccttcatccgcagatccgatgaactgctgtctgccatcggcggctatatccccgaagctcctagagatggacaggcctatgtgcggaaggatggcgaatgggtgctgctgtctaccttcctgtgatga

SEQ ID NO: 151 - DNA, 1638 bp, synthetic construct
  source 1..1638: mol_type = other DNA
atggaactgcccatcctgaaaacaaacgccatcaccaccatcctggccgccgtgacactgtgttttgccagcagccagaacatcaccgaagagttctaccagagcacctgtagcgccgtgtctaagggctatctgtctgccctgagaaccggctggtataccagcgtgatcaccatcgagctgagcaacatcaaagaaatcaagtgcaacggcaccgacgccaaagtgaagctgatcaagcaagagctggacaagtacaagaacgccgtgaccgaactgcagctgctgatgcagtctacccctgccgccaatagcagagccagacgggaactgcctagattcatgaactacaccctgaacaacaccaagaacaccaacgtgaccctgagcaagaagcggaagcggagattcctgggctttctgctcggagtgggaagcgccattgcctctggaattgccgtgtccaaggtgctgcatctggaaggcgaagtgaacaagatcaagagcgccctgctgagcaccaacaaggccgtggtttctctgagcaatggcgtgtccgtgctgacctctaaggtgctggacctgaagaactacatcgacaaacagctgctgcccatcgtcaacaagcagagctgcagcatcagcaaccccgagacagtgatcgagttccagcagaagaacaaccggctgctggaaatcacccgcgagttttctgtgaatgccggcgtgaccacacctgtgtccacctacatgctgaccaacagcgagctgctgtccctgatcaacgacatgcccatcaccaacgaccagaaaaagctgatgagcagcaacgtgcagatcgtgcggcagcagagctactccatcatgagcattatcaaagaagaggtgctggcctacgtggtgcagctgcctctgtatggcgtgatcgataccccttgctggaagctgcacacaagccctctgtgcaccaccaacaccaaagagggctccaacatctgcctgaccagaaccgatagaggctggtactgcgataatgccggcagcgtcagcttcttcccacaagccgagacatgcaaggtgcagagcaacagagtgttctgcgataccatgaacagcctgacactgccctccgaagtgaatctgtgcaatatcgacatcttcaacccgaagtacgactgcaagatcatgaccagcaagaccgacgtgtcaagctccgtgatcacatctctgggcgccatcgtgtcctgctacggcaagacaaagtgcaccgccagcaacaagaaccggggcatcatcaagaccttcagcaacggctgcgactacgtgtccaacaaaggcgtggacaccgtgtctgtgggcaacaccctgtactacgtgaacaagcaagaaggcaagagcctgtacgtgaagggcgagcccatcatcaacttctacgaccctctggtgttccccagcgaccagtttgatgccagcatctcccaagtgaacgagaagatcaaccagagcctggccttcatcagaaagtccgatgagctgctgagcgccatcggcggctatatccctgaagctcctagagatggacaggcctatgtgcggaaggatggcgaatgggtgctgctgtctaccttcctgtgatga

SEQ ID NO: 152 - DNA, 1638 bp, synthetic construct
  source 1..1638: mol_type = other DNA
atggaactgctgattcacagaagcagcgccatctttctgaccctggccatcaatgccctgtacctgaccagcagccagaacatcaccgaagagttctaccagagcacctgtagcgccgtgtccagaggctacttttctgccctgagaaccggctggtataccagcgtgatcaccatcgagctgagcaacatcaaagaaatcaagtgcaacggcaccgacaccaaagtgaagctgatcaagcaagagctggacaagtacaagaacgccgtgaccgaactgcagctgctgatgcagaatacccctgccgccaacaaccgggccagaagagaagcccctcagtacatgaactacaccatcaacaccaccaagaacctgaacgtgtccatcagcaagaagcggaagcggagattcctgggctttctgctcggagtgggaagcgccattgcctctggaattgccgtgtctaaggtgctgcacctggaaggcgaagtgaacaagatcaagaatgccctgctgagcaccaacaaggccgtggtgtctctgtctaatggcgtgtccgtgctgaccagcaaggtgctggacctgaagaactacatcaacaaccagctgctgcccatcgtgaaccagcagagctgccggatcagcaaccccgagacagtgatcgagttccagcagaagaacagcagactgctggaaatcacccgcgagttttccgtgaatgccggcgtgacaacacccctgagcacctacatgctgaccaacagcgagctgctgtccctgatcaacgacatgcccatcaccaacgaccagaaaaagctgatgagcagcaacgtgcagatcgtgcggcagcagtcctacagcatcatgagcattatcaaagaagaggtgctggcctacgtggtgcagctgcctatctacggcgtgatcgataccccttgctggaagctgcacacaagccctctgtgcaccaccaatatcaaagagggctccaacatctgcctgaccagaaccgatagaggctggtactgcgataatgccggcagcgtcagcttcttcccacaagccgatacctgcaaggtgcagagcaacagagtgttctgcgataccatgaacagcctgacactgcccagcgaggtgtccctgtgcaacaccgacatcttcaactctaagtacgactgcaagatcatgacctccaagaccgacatcagctcctccgtgatcacatctctgggcgccatcgtgtcctgctacggcaagacaaagtgtaccgccagcaacaagaaccggggcatcatcaagaccttcagcaacggctgcgactacgtgtccaacaaaggcgtggacaccgtgtctgtgggcaacaccctgtactacgtgaacaagctggaaggcaagaatctgtacgtgaagggcgagcccatcatcaactactacgaccctctggtgttccccagcgaccagtttgatgccagcatcagccaagtgaacgagaagatcaaccagagcctggccttcatccgcagatccgatgaactgctgtctgccatcggcggctatatccccgaagctcctagagatggacaggcctatgtgcggaaggatggcgaatgggtgctgctgtctaccttcctgtgatga

SEQ ID NO: 153 - DNA, 1638 bp, synthetic construct
  source 1..1638: mol_type = other DNA
atggaactgcccatcctgaaaacaaacgccatcaccaccatcctggccgccgtgacactgtgttttgccagcagccagaacatcaccgaagagttctaccagagcacctgtagcgccgtgtctaagggctatctgtctgccctgagaaccggctggtataccagcgtgatcaccatcgagctgagcaacatcaaaatcaacaagtgcaacggcaccgacgccaaagtgaagctgatcaagcaagagctggacaagtacaagaacgccgtgaccgaactgcagctgctgatgcagtctacccctgccgccaatagcagagccagacgggaactgcctagattcatgaactacaccctgaacaacaccaagaacaccaacgtgaccctgagcaagaagcggaagcggagattcctgggctttctgctcggagtgggaagcgccattgcctctggaattgccgtgtccaaggtgctgcatctggaaggcgaagtgaacaagatcaagagcgccctgctgagcaccaacaaggccgtggtttctctgagcaatggcgtgtccgtgctgacctctaaggtgctggacctgaagaactacatcgacaaacagctgctgcccatcgtcaacaagcagagctgcagcatcagcaaccccgagacagtgatcgagttccagcagaagaacaaccggctgctggaaatcacccgcgagttttctgtgaatgccggcgtgaccacacctgtgtccacctacatgctgaccaacagcgagctgctgtccctgatcaacgacatgcccatcaccaacgaccagaaaaagctgatgagcagcaacgtgcagatcgtgcggcagcagagctactccatcatgagcattatcaaagaagaggtgctggcctacgtggtgcagctgcctctgtatggcgtgatcgataccccttgctggaagctgcacacaagccctctgtgcaccaccaacaccaaagagggctccaacatctgcctgaccagaaccgatagaggctggtactgcgataatgccggcagcgtcagcttcttcccacaagccgagacatgcaaggtgcagagcaacagagtgttctgcgataccatgaacagcctgacactgccctccgaagtgaatctgtgcaatatcgacatcttcaacccgaagtacgactgcaagatcatgaccagcaagaccgacgtgtcaagctccgtgatcacatctctgggcgccatcgtgtcctgctacggcaagacaaagtgcaccgccagcaacaagaaccggggcatcatcaagaccttcagcaacggctgcgactacgtgtccaacaaaggcgtggacaccgtgtctgtgggcaacaccctgtactacgtgaacaagcaagaaggcaagagcctgtacgtgaagggcgagcccatcatcaacttctacgaccctctggtgttccccagccaggagtttgatgccagcatctcccaagtgaacgagaagatcaaccagagcctggccttcatcagaaagtccgatgagctgctgagcgccatcggcggctatatccctgaagctcctagagatggacaggcctatgtgcggaaggatggcgaatgggtgctgctgtctaccttcctgtgatga

SEQ ID NO: 154 - DNA, 1638 bp, synthetic construct
  source 1..1638: mol_type = other DNA
atggaactgctgattcacagaagcagcgccatctttctgaccctggccatcaatgccctgtacctgaccagcagccagaacatcaccgaagagttctaccagagcacctgtagcgccgtgtccagaggctacttttctgccctgagaaccggctggtataccagcgtgatcaccatcgagctgagcaacatcaaaatcacaaagtgcaacggcaccgacaccaaagtgaagctgatcaagcaagagctggacaagtacaagaacgccgtgaccgaactgcagctgctgatgcagaatacccctgccgccaacaaccgggccagaagagaagcccctcagtacatgaactacaccatcaacaccaccaagaacctgaacgtgtccatcagcaagaagcggaagcggagattcctgggctttctgctcggagtgggaagcgccattgcctctggaattgccgtgtctaaggtgctgcacctggaaggcgaagtgaacaagatcaagaatgccctgctgagcaccaacaaggccgtggtgtctctgtctaatggcgtgtccgtgctgaccagcaaggtgctggacctgaagaactacatcaacaaccagctgctgcccatcgtgaaccagcagagctgccggatcagcaaccccgagacagtgatcgagttccagcagaagaacagcagactgctggaaatcacccgcgagttttccgtgaatgccggcgtgacaacacccctgagcacctacatgctgaccaacagcgagctgctgtccctgatcaacgacatgcccatcaccaacgaccagaaaaagctgatgagcagcaacgtgcagatcgtgcggcagcagtcctacagcatcatgagcattatcaaagaagaggtgctggcctacgtggtgcagctgcctatctacggcgtgatcgataccccttgctggaagctgcacacaagccctctgtgcaccaccaatatcaaagagggctccaacatctgcctgaccagaaccgatagaggctggtactgcgataatgccggcagcgtcagcttcttcccacaagccgatacctgcaaggtgcagagcaacagagtgttctgcgataccatgaacagcctgacactgcccagcgaggtgtccctgtgcaacaccgacatcttcaactctaagtacgactgcaagatcatgacctccaagaccgacatcagctcctccgtgatcacatctctgggcgccatcgtgtcctgctacggcaagacaaagtgtaccgccagcaacaagaaccggggcatcatcaagaccttcagcaacggctgcgactacgtgtccaacaaaggcgtggacaccgtgtctgtgggcaacaccctgtactacgtgaacaagctggaaggcaagaatctgtacgtgaagggcgagcccatcatcaactactacgaccctctggtgttccccagccaggagtttgatgccagcatcagccaagtgaacgagaagatcaaccagagcctggccttcatccgcagatccgatgaactgctgtctgccatcggcggctatatccccgaagctcctagagatggacaggcctatgtgcggaaggatggcgaatgggtgctgctgtctaccttcctgtgatga

SEQ ID NO: 155 - DNA, 1653 bp, synthetic construct
  source 1..1653: mol_type = other DNA
atggaactgcccatcctgaaaacaaacgccatcaccaccatcctggccgccgtgacactgtgttttgccagcagccagaacatcaccgaagagttctaccagagcacctgtagcgccgtgtctaagggctatctgtctgccctgagaaccggctggtataccagcgtgatcaccatcgagctgagcaacatcaaaatcaacaagtgcaacggcaccgacgccaaagtgaagctgatcaagcaagagctggacaagtacaagaacgccgtgaccgaactgcagctgctgatgcagtctacccctgccgccaatagcagagccagacgggaactgcctagattcatgaactacaccctgaacaacaccaagaacaccaacgtgaccctgagcaagaagcggaagcggagattcctgggctttctgctcggagtgggaagcgccattgcctctggaattgccgtgtccaaggtgctgcatctggaaggcgaagtgaacaagatcaagagcgccctgctgagcaccaacaaggccgtggtttctctgagcaatggcgtgtccgtgctgacctctaaggtgctggacctgaagaactacatcgacaaacagctgctgcccatcgtcaacaagcagagctgccccatcagcaacatcgagacagtgatcgagttccagcagaagaacaaccggctgctggaaatcacccgcgagttttctgtgaatgccggcgtgaccacacctgtgtccacctacatgctgaccaacagcgagctgctgtccctgatcaacgacatgcccatcaccaacgaccagaaaaagctgatgagcagcaacgtgcagatcgtgcggcagcagagctactccatcatgagcattatcaaagaagaggtgctggcctacgtggtgcagctgcctctgtatggcgtgatcgataccccttgctggaagctgcacacaagccctctgtgcaccaccaacaccaaagagggctccaacatctgcctgaccagaaccgatagaggctggtactgcgataatgccggcagcgtcagcttcttcccacaagccgagacatgcaaggtgcagagcaacagagtgttctgcgataccatgaacagcctgacactgccctccgaagtgaatctgtgcaatatcgacatcttcaacccgaagtacgactgcaagatcatgaccagcaagaccgacgtgtcaagctccgtgatcacatctctgggcgccatcgtgtcctgctacggcaagacaaagtgcaccgccagcaacaagaaccggggcatcatcaagaccttcagcaacggctgcgactacgtgtccaacaaaggcgtggacaccgtgtctgtgggcaacaccctgtactacgtgaacaagcaagaaggcaagagcctgtacgtgaagggcgagcccatcatcaacttctacgaccctctggtgttccccagcgacacctttgatgccagcatctcccaagtgaacgagaagatcaaccagagcctggccttcatcagaaagtccgatgagctgctgcacaacgtgaacgccggcaagtccaccaccaatatcatgatcaccacgatcatcatcgtgatcatcgtcatcctgctggctctgatcgctgtgggcctgctgctgtattgatga

SEQ ID NO: 156 - DNA, 1653 bp, synthetic construct
  source 1..1653: mol_type = other DNA
atggaactgctgattcacagaagcagcgccatctttctgaccctggccatcaatgccctgtacctgaccagcagccagaacatcaccgaagagttctaccagagcacctgtagcgccgtgtccagaggctacttttctgccctgagaaccggctggtataccagcgtgatcaccatcgagctgagcaacatcaaaatcacaaagtgcaacggcaccgacaccaaagtgaagctgatcaagcaagagctggacaagtacaagaacgccgtgaccgaactgcagctgctgatgcagaatacccctgccgccaacaaccgggccagaagagaagcccctcagtacatgaactacaccatcaacaccaccaagaacctgaacgtgtccatcagcaagaagcggaagcggagattcctgggctttctgctcggagtgggaagcgccattgcctctggaattgccgtgtctaaggtgctgcacctggaaggcgaagtgaacaagatcaagaatgccctgctgagcaccaacaaggccgtggtgtctctgtctaatggcgtgtccgtgctgaccagcaaggtgctggacctgaagaactacatcaacaaccagctgctgcccatcgtgaaccagcagagctgccccatcagcaacatcgagacagtgatcgagttccagcagaagaacagcagactgctggaaatcacccgcgagttttccgtgaatgccggcgtgacaacacccctgagcacctacatgctgaccaacagcgagctgctgtccctgatcaacgacatgcccatcaccaacgaccagaaaaagctgatgagcagcaacgtgcagatcgtgcggcagcagtcctacagcatcatgagcattatcaaagaagaggtgctggcctacgtggtgcagctgcctatctacggcgtgatcgataccccttgctggaagctgcacacaagccctctgtgcaccaccaatatcaaagagggctccaacatctgcctgaccagaaccgatagaggctggtactgcgataatgccggcagcgtcagcttcttcccacaagccgatacctgcaaggtgcagagcaacagagtgttctgcgataccatgaacagcctgacactgcccagcgaggtgtccctgtgcaacaccgacatcttcaactctaagtacgactgcaagatcatgacctccaagaccgacatcagctcctccgtgatcacatctctgggcgccatcgtgtcctgctacggcaagacaaagtgtaccgccagcaacaagaaccggggcatcatcaagaccttcagcaacggctgcgactacgtgtccaacaaaggcgtggacaccgtgtctgtgggcaacaccctgtactacgtgaacaagctggaaggcaagaatctgtacgtgaagggcgagcccatcatcaactactacgaccctctggtgttccccagcgacacctttgatgccagcatcagccaagtgaacgagaagatcaaccagagcctggccttcatccgcagatccgatgaactgctgcacaatgtgaacaccggcaagagcaccacaaacatcatgatcaccgccatcatcatcgtgatcatcgtcgtgctgctgagcctgatcgctatcggcctgctgctgtactgatga

SEQ ID NO: 157 - DNA, 1653 bp, synthetic construct
  source 1..1653: mol_type = other DNA
atggaactgcccatcctgaaaacaaacgccatcaccaccatcctggccgccgtgacactgtgttttgccagcagccagaacatcaccgaagagttctaccagagcacctgtagcgccgtgtctaagggctatctgtctgccctgagaaccggctggtataccagcgtgatcaccatcgagctgagcaacatcaaaatcaacaagtgcaacggcaccgacgccaaagtgaagctgatcaagcaagagctggacaagtacaagaacgccgtgaccgaactgcagctgctgatgcagtctacccctgccgccaatagcagagccagacgggaactgcctagattcatgaactacaccctgaacaacaccaagaacaccaacgtgaccctgagcaagaagcggaagcggagattcctgggctttctgctcggagtgggaagcgccattgcctctggaattgccgtgtccaaggtgctgcatctggaaggcgaagtgaacaagatcaagagcgccctgctgagcaccaacaaggccgtggtttctctgagcaatggcgtgtccgtgctgacctctaaggtgctggacctgaagaactacatcgacaaacagctgctgcccatcgtcaacaagcagagctgccccatcagcaacatcgagacagtgatcgagttccagcagaagaacaaccggctgctggaaatcacccgcgagttttctgtgaatgccggcgtgaccacacctgtgtccacctacatgctgaccaacagcgagctgctgtccctgatcaacgacatgcccatcaccaacgaccagaaaaagctgatgagcagcaacgtgcagatcgtgcggcagcagagctactccatcatgagcattatcaaagaagaggtgctggcctacgtggtgcagctgcctctgtatggcgtgatcgataccccttgctggaagctgcacacaagccctctgtgcaccaccaacaccaaagagggctccaacatctgcctgaccagaaccgatagaggctggtactgcgataatgccggcagcgtcagcttcttcccacaagccgagacatgcaaggtgcagagcaacagagtgttctgcgataccatgaacagcctgacactgccctccgaagtgaatctgtgcaatatcgacatcttcaacccgaagtacgactgcaagatcatgaccagcaagaccgacgtgtcaagctccgtgatcacatctctgggcgccatcgtgtcctgctacggcaagacaaagtgcaccgccagcaacaagaaccggggcatcatcaagaccttcagcaacggctgcgactacgtgtccaacaaaggcgtggacaccgtgtctgtgggcaacaccctgtactacgtgaacaagcaagaaggcaagagcctgtacgtgaagggcgagcccatcatcaacttctacgaccctctggtgttccccagccaggagtttgatgccagcatctcccaagtgaacgagaagatcaaccagagcctggccttcatcagaaagtccgatgagctgctgcacaacgtgaacgccggcaagtccaccaccaatatcatgatcaccacgatcatcatcgtgatcatcgtcatcctgctggctctgatcgctgtgggcctgctgctgtattgatga

SEQ ID NO: 158 - DNA, 1653 bp, synthetic construct
  source 1..1653: mol_type = other DNA
atggaactgctgattcacagaagcagcgccatctttctgaccctggccatcaatgccctgtacctgaccagcagccagaacatcaccgaagagttctaccagagcacctgtagcgccgtgtccagaggctacttttctgccctgagaaccggctggtataccagcgtgatcaccatcgagctgagcaacatcaaaatcacaaagtgcaacggcaccgacaccaaagtgaagctgatcaagcaagagctggacaagtacaagaacgccgtgaccgaactgcagctgctgatgcagaatacccctgccgccaacaaccgggccagaagagaagcccctcagtacatgaactacaccatcaacaccaccaagaacctgaacgtgtccatcagcaagaagcggaagcggagattcctgggctttctgctcggagtgggaagcgccattgcctctggaattgccgtgtctaaggtgctgcacctggaaggcgaagtgaacaagatcaagaatgccctgctgagcaccaacaaggccgtggtgtctctgtctaatggcgtgtccgtgctgaccagcaaggtgctggacctgaagaactacatcaacaaccagctgctgcccatcgtgaaccagcagagctgccccatcagcaacatcgagacagtgatcgagttccagcagaagaacagcagactgctggaaatcacccgcgagttttccgtgaatgccggcgtgacaacacccctgagcacctacatgctgaccaacagcgagctgctgtccctgatcaacgacatgcccatcaccaacgaccagaaaaagctgatgagcagcaacgtgcagatcgtgcggcagcagtcctacagcatcatgagcattatcaaagaagaggtgctggcctacgtggtgcagctgcctatctacggcgtgatcgataccccttgctggaagctgcacacaagccctctgtgcaccaccaatatcaaagagggctccaacatctgcctgaccagaaccgatagaggctggtactgcgataatgccggcagcgtcagcttcttcccacaagccgatacctgcaaggtgcagagcaacagagtgttctgcgataccatgaacagcctgacactgcccagcgaggtgtccctgtgcaacaccgacatcttcaactctaagtacgactgcaagatcatgacctccaagaccgacatcagctcctccgtgatcacatctctgggcgccatcgtgtcctgctacggcaagacaaagtgtaccgccagcaacaagaaccggggcatcatcaagaccttcagcaacggctgcgactacgtgtccaacaaaggcgtggacaccgtgtctgtgggcaacaccctgtactacgtgaacaagctggaaggcaagaatctgtacgtgaagggcgagcccatcatcaactactacgaccctctggtgttccccagccaggagtttgatgccagcatcagccaagtgaacgagaagatcaaccagagcctggccttcatccgcagatccgatgaactgctgcacaatgtgaacaccggcaagagcaccacaaacatcatgatcaccgccatcatcatcgtgatcatcgtcgtgctgctgagcctgatcgctatcggcctgctgctgtactgatga

SEQ ID NO: 159 - DNA, 1653 bp, synthetic construct
  source 1..1653: mol_type = other DNA
atggaactgcccatcctgaaaacaaacgccatcaccaccatcctggccgccgtgacactgtgttttgccagcagccagaacatcaccgaagagttctaccagagcacctgtagcgccgtgtctaagggctatctgtctgccctgagaaccggctggtataccagcgtgatcaccatcgagctgagcaacatcaaaatcaacaagtgcaacggcaccgacgccaaagtgaagctgatcaagcaagagctggacaagtacaagaacgccgtgaccgaactgcagctgctgatgcagtctaccccttgcgccaatagcagagccagacgggaactgcctagattcatgaactacaccctgaacaacaccaagaacaccaacgtgaccctgagcaagaagcggaagcggagattcctgggctttctgctcggagtgggaagcgccattgcctctggatgcgccgtgtccaaggtgctgcatctggaaggcgaagtgaacaagatcaagagcgccctgctgagcaccaacaaggccgtggtttctctgagcaatggcgtgtccgtgctgacctctaaggtgctggacctgaagaactacatcgacaaacagctgctgcccatcgtcaacaagcagagctgccccatcagcaacatcgagacagtgatcgagttccagcagaagaacaaccggctgctggaaatcacccgcgagttttctgtgaatgccggcgtgaccacacctgtgtccacctacatgctgaccaacagcgagctgctgtccctgatcaacgacatgcccatcaccaacgaccagaaaaagctgatgagcagcaacgtgcagatcgtgcggcagcagagctactccatcatgagcattatcaaagaagaggtgctggcctacgtggtgcagctgcctctgtatggcgtgatcgataccccttgctggaagctgcacacaagccctctgtgcaccaccaacaccaaagagggctccaacatctgcctgaccagaaccgatagaggctggtactgcgataatgccggcagcgtcagcttcttcccacaagccgagacatgcaaggtgcagagcaacagagtgttctgcgataccatgaacagcctgacactgccctccgaagtgaatctgtgcaatatcgacatcttcaacccgaagtacgactgcaagatcatgaccagcaagaccgacgtgtcaagctccgtgatcacatctctgggcgccatcgtgtcctgctacggcaagacaaagtgcaccgccagcaacaagaaccggggcatcatcaagaccttcagcaacggctgcgactacgtgtccaacaaaggcgtggacaccgtgtctgtgggcaacaccctgtactacgtgaacaagcaagaaggcaagagcctgtacgtgaagggcgagcccatcatcaacttctacgaccctctggtgttccccagcgacgagtttgatgccagcatctcccaagtgaacgagaagatcaaccagagcctggccttcatcagaaagtccgatgagctgctgcacaacgtgaacgccggcaagtccaccaccaatatcatgatcaccacgatcatcatcgtgatcatcgtcatcctgctggctctgatcgctgtgggcctgctgctgtattgatga

SEQ ID NO: 160 - DNA, 1653 bp, synthetic construct
  source 1..1653: mol_type = other DNA
atggaactgctgattcacagaagcagcgccatctttctgaccctggccatcaatgccctgtacctgaccagcagccagaacatcaccgaagagttctaccagagcacctgtagcgccgtgtccagaggctacttttctgccctgagaaccggctggtataccagcgtgatcaccatcgagctgagcaacatcaaaatcacaaagtgcaacggcaccgacaccaaagtgaagctgatcaagcaagagctggacaagtacaagaacgccgtgaccgaactgcagctgctgatgcagaataccccttgcgccaacaaccgggccagaagagaagcccctcagtacatgaactacaccatcaacaccaccaagaacctgaacgtgtccatcagcaagaagcggaagcggagattcctgggctttctgctcggagtgggaagcgccattgcctctggatgcgccgtgtctaaggtgctgcacctggaaggcgaagtgaacaagatcaagaatgccctgctgagcaccaacaaggccgtggtgtctctgtctaatggcgtgtccgtgctgaccagcaaggtgctggacctgaagaactacatcaacaaccagctgctgcccatcgtgaaccagcagagctgccccatcagcaacatcgagacagtgatcgagttccagcagaagaacagcagactgctggaaatcacccgcgagttttccgtgaatgccggcgtgacaacacccctgagcacctacatgctgaccaacagcgagctgctgtccctgatcaacgacatgcccatcaccaacgaccagaaaaagctgatgagcagcaacgtgcagatcgtgcggcagcagtcctacagcatcatgagcattatcaaagaagaggtgctggcctacgtggtgcagctgcctatctacggcgtgatcgataccccttgctggaagctgcacacaagccctctgtgcaccaccaatatcaaagagggctccaacatctgcctgaccagaaccgatagaggctggtactgcgataatgccggcagcgtcagcttcttcccacaagccgatacctgcaaggtgcagagcaacagagtgttctgcgataccatgaacagcctgacactgcccagcgaggtgtccctgtgcaacaccgacatcttcaactctaagtacgactgcaagatcatgacctccaagaccgacatcagctcctccgtgatcacatctctgggcgccatcgtgtcctgctacggcaagacaaagtgtaccgccagcaacaagaaccggggcatcatcaagaccttcagcaacggctgcgactacgtgtccaacaaaggcgtggacaccgtgtctgtgggcaacaccctgtactacgtgaacaagctggaaggcaagaatctgtacgtgaagggcgagcccatcatcaactactacgaccctctggtgttccccagcgacgagtttgatgccagcatcagccaagtgaacgagaagatcaaccagagcctggccttcatccgcagatccgatgaactgctgcacaatgtgaacaccggcaagagcaccacaaacatcatgatcaccgccatcatcatcgtgatcatcgtcgtgctgctgagcctgatcgctatcggcctgctgctgtactgatga

SEQ ID NO: 161 - DNA, 1653 bp, synthetic construct
  source 1..1653: mol_type = other DNA
atggaactgcccatcctgaaaacaaacgccatcaccaccatcctggccgccgtgacactgtgttttgccagcagccagaacatcaccgaagagttctaccagagcacctgtagcgccgtgtctaagggctatctgtctgccctgagaaccggctggtataccagcgtgatcaccatcgagctgagcaacatcaaaatcaacaagtgcaacggcaccgacgccaaagtgaagctgatcaagcaagagctggacaagtacaagaacgccgtgaccgaactgcagctgctgatgcagtctacctgcgccgccaatagcagagccagacgggaactgcctagattcatgaactacaccctgaacaacaccaagaacaccaacgtgaccctgagcaagaagcggaagcggagattcctgggctttctgctcggagtgggaagcgccattgcctctggatgcgccgtgtccaaggtgctgcatctggaaggcgaagtgaacaagatcaagagcgccctgctgagcaccaacaaggccgtggtttctctgagcaatggcgtgtccgtgctgacctctaaggtgctggacctgaagaactacatcgacaaacagctgctgcccatcgtcaacaagcagagctgccccatcagcaacatcgagacagtgatcgagttccagcagaagaacaaccggctgctggaaatcacccgcgagttttctgtgaatgccggcgtgaccacacctgtgtccacctacatgctgaccaacagcgagctgctgtccctgatcaacgacatgcccatcaccaacgaccagaaaaagctgatgagcagcaacgtgcagatcgtgcggcagcagagctactccatcatgagcattatcaaagaagaggtgctggcctacgtggtgcagctgcctctgtatggcgtgatcgataccccttgctggaagctgcacacaagccctctgtgcaccaccaacaccaaagagggctccaacatctgcctgaccagaaccgatagaggctggtactgcgataatgccggcagcgtcagcttcttcccacaagccgagacatgcaaggtgcagagcaacagagtgttctgcgataccatgaacagcctgacactgccctccgaagtgaatctgtgcaatatcgacatcttcaacccgaagtacgactgcaagatcatgaccagcaagaccgacgtgtcaagctccgtgatcacatctctgggcgccatcgtgtcctgctacggcaagacaaagtgcaccgccagcaacaagaaccggggcatcatcaagaccttcagcaacggctgcgactacgtgtccaacaaaggcgtggacaccgtgtctgtgggcaacaccctgtactacgtgaacaagcaagaaggcaagagcctgtacgtgaagggcgagcccatcatcaacttctacgaccctctggtgttccccagcgacgagtttgatgccagcatctcccaagtgaacgagaagatcaaccagagcctggccttcatcagaaagtccgatgagctgctgcacaacgtgaacgccggcaagtccaccaccaatatcatgatcaccacgatcatcatcgtgatcatcgtcatcctgctggctctgatcgctgtgggcctgctgctgtattgatga

SEQ ID NO: 162 - DNA, 1653 bp, synthetic construct
  source 1..1653: mol_type = other DNA
atggaactgctgattcacagaagcagcgccatctttctgaccctggccatcaatgccctgtacctgaccagcagccagaacatcaccgaagagttctaccagagcacctgtagcgccgtgtccagaggctacttttctgccctgagaaccggctggtataccagcgtgatcaccatcgagctgagcaacatcaaaatcacaaagtgcaacggcaccgacaccaaagtgaagctgatcaagcaagagctggacaagtacaagaacgccgtgaccgaactgcagctgctgatgcagaatacctgcgccgccaacaaccgggccagaagagaagcccctcagtacatgaactacaccatcaacaccaccaagaacctgaacgtgtccatcagcaagaagcggaagcggagattcctgggctttctgctcggagtgggaagcgccattgcctctggatgcgccgtgtctaaggtgctgcacctggaaggcgaagtgaacaagatcaagaatgccctgctgagcaccaacaaggccgtggtgtctctgtctaatggcgtgtccgtgctgaccagcaaggtgctggacctgaagaactacatcaacaaccagctgctgcccatcgtgaaccagcagagctgccccatcagcaacatcgagacagtgatcgagttccagcagaagaacagcagactgctggaaatcacccgcgagttttccgtgaatgccggcgtgacaacacccctgagcacctacatgctgaccaacagcgagctgctgtccctgatcaacgacatgcccatcaccaacgaccagaaaaagctgatgagcagcaacgtgcagatcgtgcggcagcagtcctacagcatcatgagcattatcaaagaagaggtgctggcctacgtggtgcagctgcctatctacggcgtgatcgataccccttgctggaagctgcacacaagccctctgtgcaccaccaatatcaaagagggctccaacatctgcctgaccagaaccgatagaggctggtactgcgataatgccggcagcgtcagcttcttcccacaagccgatacctgcaaggtgcagagcaacagagtgttctgcgataccatgaacagcctgacactgcccagcgaggtgtccctgtgcaacaccgacatcttcaactctaagtacgactgcaagatcatgacctccaagaccgacatcagctcctccgtgatcacatctctgggcgccatcgtgtcctgctacggcaagacaaagtgtaccgccagcaacaagaaccggggcatcatcaagaccttcagcaacggctgcgactacgtgtccaacaaaggcgtggacaccgtgtctgtgggcaacaccctgtactacgtgaacaagctggaaggcaagaatctgtacgtgaagggcgagcccatcatcaactactacgaccctctggtgttccccagcgacgagtttgatgccagcatcagccaagtgaacgagaagatcaaccagagcctggccttcatccgcagatccgatgaactgctgcacaatgtgaacaccggcaagagcaccacaaacatcatgatcaccgccatcatcatcgtgatcatcgtcgtgctgctgagcctgatcgctatcggcctgctgctgtactgatga

SEQ ID NO: 163 - DNA, 1653 bp, synthetic construct
  source 1..1653: mol_type = other DNA
atggaactgcccatcctgaaaacaaacgccatcaccaccatcctggccgccgtgacactgtgttttgccagcagccagaacatcaccgaagagttctaccagagcacctgtagcgccgtgtctaagggctatctgtctgccctgagaaccggctggtataccagcgtgatcaccatcgagctgagcaacatcaaaatcaacaagtgcaacggcaccgacgccaaagtgaagctgatcaagcaagagctggacaagtacaagaacgccgtgaccgaactgcagctgctgatgcagtctacccctgccgccaatagcagagccagacgggaactgcctagattcatgaactacaccctgaacaacaccaagaacaccaacgtgaccctgagcaagaagcggaagcggagattcctgggctttctgctcggagtgggaagcgccattgcctctggaattgccgtgtccaaggtgctgcatctggaaggcgaagtgaacaagatcaagagcgccctgctgagcaccaacaaggccgtggtttctctgagcaatggcgtgtccgtgctgacctctaaggtgctggacctgaagaactacatcgacaaacagctgctgcccatcgtcaacaagcagagctgccccatcagcaacatcgagacagtgatcgagttccagcagaagaacaaccggctgctggaaatcacccgcgagttttctgtgaatgccggcgtgaccacacctgtgtccacctacatgctgaccaacagcgagctgctgtccctgatcaacgacatgcccatcaccaacgaccagaaaaagctgatgagcagcaacgtgcagatcgtgcggcagcagagctactccatcatgagcattatcaaagaagaggtgctggcctacgtggtgcagctgcctctgtatggcgtgatcgataccccttgctggaagctgcacacaagccctctgtgcaccaccaacaccaaagagggctccaacatctgcctgaccagaaccgatagaggctggtactgcgataatgccggcagcgtcagcttcttcccacaagccgagacatgcaaggtgcagagcaacagagtgttctgcgataccatgaacagcctgacactgccctccgaagtgaatctgtgcaatatcgacatcttcaacccgaagtacgactgcaagatcatgaccagcaagaccgacgtgtcaagctccgtgatcacatctctgggcgccatcgtgtcctgctacggcaagacaaagtgcaccgccagcaacaagaaccggggcatcatcaagaccttcagcaacggctgcgactacgtgtccaacaaaggcgtggacaccgtgtctgtgggcaacaccctgtactacgtgaacaagcaagaaggcaagagcctgtacgtgaagggcgagcccatcatcaacttctacgaccctctggtgttccccagcgacgagtttgatgccagcatctcccaagtgaacgagaagatcaaccagagcctggccttcatcagaaagtccgatgagctgctgcacaacgtgaacgccggcaagtccaccaccaatatcatgatcaccacgatcatcatcgtgatcatcgtcatcctgctggctctgatcgctgtgggcctgctgctgtattgatga

SEQ ID NO: 164 - DNA, 1653 bp, synthetic construct
  source 1..1653: mol_type = other DNA
atggaactgctgattcacagaagcagcgccatctttctgaccctggccatcaatgccctgtacctgaccagcagccagaacatcaccgaagagttctaccagagcacctgtagcgccgtgtccagaggctacttttctgccctgagaaccggctggtataccagcgtgatcaccatcgagctgagcaacatcaaaatcacaaagtgcaacggcaccgacaccaaagtgaagctgatcaagcaagagctggacaagtacaagaacgccgtgaccgaactgcagctgctgatgcagaatacccctgccgccaacaaccgggccagaagagaagcccctcagtacatgaactacaccatcaacaccaccaagaacctgaacgtgtccatcagcaagaagcggaagcggagattcctgggctttctgctcggagtgggaagcgccattgcctctggaattgccgtgtctaaggtgctgcacctggaaggcgaagtgaacaagatcaagaatgccctgctgagcaccaacaaggccgtggtgtctctgtctaatggcgtgtccgtgctgaccagcaaggtgctggacctgaagaactacatcaacaaccagctgctgcccatcgtgaaccagcagagctgccccatcagcaacatcgagacagtgatcgagttccagcagaagaacagcagactgctggaaatcacccgcgagttttccgtgaatgccggcgtgacaacacccctgagcacctacatgctgaccaacagcgagctgctgtccctgatcaacgacatgcccatcaccaacgaccagaaaaagctgatgagcagcaacgtgcagatcgtgcggcagcagtcctacagcatcatgagcattatcaaagaagaggtgctggcctacgtggtgcagctgcctatctacggcgtgatcgataccccttgctggaagctgcacacaagccctctgtgcaccaccaatatcaaagagggctccaacatctgcctgaccagaaccgatagaggctggtactgcgataatgccggcagcgtcagcttcttcccacaagccgatacctgcaaggtgcagagcaacagagtgttctgcgataccatgaacagcctgacactgcccagcgaggtgtccctgtgcaacaccgacatcttcaactctaagtacgactgcaagatcatgacctccaagaccgacatcagctcctccgtgatcacatctctgggcgccatcgtgtcctgctacggcaagacaaagtgtaccgccagcaacaagaaccggggcatcatcaagaccttcagcaacggctgcgactacgtgtccaacaaaggcgtggacaccgtgtctgtgggcaacaccctgtactacgtgaacaagctggaaggcaagaatctgtacgtgaagggcgagcccatcatcaactactacgaccctctggtgttccccagcgacgagtttgatgccagcatcagccaagtgaacgagaagatcaaccagagcctggccttcatccgcagatccgatgaactgctgcacaatgtgaacaccggcaagagcaccacaaacatcatgatcaccgccatcatcatcgtgatcatcgtcgtgctgctgagcctgatcgctatcggcctgctgctgtactgatga

SEQ ID NO: 165 - DNA, 1653 bp, synthetic construct
  source 1..1653: mol_type = other DNA
atggaactgcccatcctgaaaacaaacgccatcaccaccatcctggccgccgtgacactgtgttttgccagcagccagaacatcaccgaagagttctaccagagcacctgtagcgccgtgtctaagggctatctgtctgccctgagaaccggctggtatgtgagcgtgatcaccatcgagctgagcaacatcaaagaaaacaagtgcaacggcaccgacgccaaagtgaagctgatcaagcaagagctggacaagtacaagaacgccgtgaccgaactgcagctgctgatgcagtctaccccttgcgccaatagcagagccagacgggaactgcctagattcatgaactacaccctgaacaacaccaagaacaccaacgtgaccctgagcaagaagcggaagcggagattcctgggctttctgctcggagtgggaagcgccattgcctctggatgcgccgtgtccaaggtgctgcatctggaaggcgaagtgaacaagatcaagagcgccctgctgagcaccaacaaggccgtggtttctctgagcaatggcgtgtccgtgctgaccatgaaggtgctggacctgaagaactacatcgacaaacagctgctgcccatcgtcaacaagcagagctgcagcatcagcaacatcgagacagtgatcgagttccagcagaagaacaaccggctgctggaaatcacccgcgagttttctgtgaatgccggcgtgaccacacctgtgtccacctacatgctgaccaacagcgagctgctgtccctgatcaacgacatgcccatcaccaacgaccagaaaaagctgatgagcagcaacgtgcagatcgtgcggcagcagagctactccatcatgagcattatcaaagaagagctgctggcctacgtggtgcagctgcctctgtatggcgtgatcgataccccttgctggaagctgcacacaagccctctgtgcaccaccaacaccaaagagggctccaacatctgcctgaccagaaccgatagaggctggtactgcgataatgccggcagcgtcagcttcttcccacaagccgagacatgcaaggtgcagagcaacagagtgttctgcgataccatgaacagcctgacactgccctccgaagtgaatctgtgcaatatcgacatcttcaacccgaagtacgactgcaagatcatgaccagcaagaccgacgtgtcaagctccgtgatcacatctctgggcgccatcgtgtcctgctacggcaagacaaagtgcaccgccagcaacaagaaccggggcatcatcaagaccttcagcaacggctgcgactacgtgtccaacaaaggcgtggacaccgtgtctgtgggcaacaccctgtactacgtgaacaagcaagaaggcaagagcctgtacgtgaagggcgagcccatcatcaacttctacgaccctctggtgttccccagcgacgagtttgatgccagcatctcccaagtgaacgagaagatcaaccagagcctggccttcatcagaaagtccgatgagctgctgcacaacgtgaacgccggcaagtccaccaccaatatcatgatcaccacgatcatcatcgtgatcatcgtcatcctgctggctctgatcgctgtgggcctgctgctgtattgatga

SEQ ID NO: 166 - DNA, 1653 bp, synthetic construct
  source 1..1653: mol_type = other DNA
atggaactgctgattcacagaagcagcgccatctttctgaccctggccatcaatgccctgtacctgaccagcagccagaacatcaccgaagagttctaccagagcacctgtagcgccgtgtccagaggctacttttctgccctgagaaccggctggtatgtgagcgtgatcaccatcgagctgagcaacatcaaagaaacaaagtgcaacggcaccgacaccaaagtgaagctgatcaagcaagagctggacaagtacaagaacgccgtgaccgaactgcagctgctgatgcagaataccccttgcgccaacaaccgggccagaagagaagcccctcagtacatgaactacaccatcaacaccaccaagaacctgaacgtgtccatcagcaagaagcggaagcggagattcctgggctttctgctcggagtgggaagcgccattgcctctggatgcgccgtgtctaaggtgctgcacctggaaggcgaagtgaacaagatcaagaatgccctgctgagcaccaacaaggccgtggtgtctctgtctaatggcgtgtccgtgctgaccatgaaggtgctggacctgaagaactacatcaacaaccagctgctgcccatcgtgaaccagcagagctgccggatcagcaacatcgagacagtgatcgagttccagcagaagaacagcagactgctggaaatcacccgcgagttttccgtgaatgccggcgtgacaacacccctgagcacctacatgctgaccaacagcgagctgctgtccctgatcaacgacatgcccatcaccaacgaccagaaaaagctgatgagcagcaacgtgcagatcgtgcggcagcagtcctacagcatcatgagcattatcaaagaagagctgctggcctacgtggtgcagctgcctatctacggcgtgatcgataccccttgctggaagctgcacacaagccctctgtgcaccaccaatatcaaagagggctccaacatctgcctgaccagaaccgatagaggctggtactgcgataatgccggcagcgtcagcttcttcccacaagccgatacctgcaaggtgcagagcaacagagtgttctgcgataccatgaacagcctgacactgcccagcgaggtgtccctgtgcaacaccgacatcttcaactctaagtacgactgcaagatcatgacctccaagaccgacatcagctcctccgtgatcacatctctgggcgccatcgtgtcctgctacggcaagacaaagtgtaccgccagcaacaagaaccggggcatcatcaagaccttcagcaacggctgcgactacgtgtccaacaaaggcgtggacaccgtgtctgtgggcaacaccctgtactacgtgaacaagctggaaggcaagaatctgtacgtgaagggcgagcccatcatcaactactacgaccctctggtgttccccagcgacgagtttgatgccagcatcagccaagtgaacgagaagatcaaccagagcctggccttcatccgcagatccgatgaactgctgcacaatgtgaacaccggcaagagcaccacaaacatcatgatcaccgccatcatcatcgtgatcatcgtcgtgctgctgagcctgatcgctatcggcctgctgctgtactgatga

SEQ ID NO: 167 - DNA, 1653 bp, synthetic construct
  source 1..1653: mol_type = other DNA
atggaactgcccatcctgaaaacaaacgccatcaccaccatcctggccgccgtgacactgtgttttgccagcagccagaacatcaccgaagagttctaccagagcacctgtagcgccgtgtctaagggctatctgtctgccctgagaaccggctggtatttcagcgtgatcaccatcgagctgagcaacatcaaagaaaacaagtgcaacggcaccgacgccaaagtgaagctgatcaagcaagagctggacaagtacaagaacgccgtgaccgaactgcagctgctgatgcagtctaccccttgcgccaatagcagagccagacgggaactgcctagattcatgaactacaccctgaacaacaccaagaacaccaacgtgaccctgagcaagaagcggaagcggagattcctgggctttctgctcggagtgggaagcgccattgcctctggatgcgccgtgtccaaggtgctgcatctggaaggcgaagtgaacaagatcaagagcgccctgctgagcaccaacaaggccgtggtttctctgagcaatggcgtgtccgtgctgaccatgaaggtgctggacctgaagaactacatcgacaaacagctgctgcccatcgtcaacaagcagagctgcagcatcagcaacatcgagacagtgatcgagttccagcagaagaacaaccggctgctggaaatcacccgcgagttttctgtgaatgccggcgtgaccacacctgtgtccacctacatgctgaccaacagcgagctgctgtccctgatcaacgacatgcccatcaccaacgaccagaaaaagctgatgagcagcaacgtgcagatcgtgcggcagcagagctactccatcatgagcattatcaaagaagagctgctggcctacgtggtgcagctgcctctgtatggcgtgatcgataccccttgctggaagctgcacacaagccctctgtgcaccaccaacaccaaagagggctccaacatctgcctgaccagaaccgatagaggctggtactgcgataatgccggcagcgtcagcttcttcccacaagccgagacatgcaaggtgcagagcaacagagtgttctgcgataccatgaacagcctgacactgccctccgaagtgaatctgtgcaatatcgacatcttcaacccgaagtacgactgcaagatcatgaccagcaagaccgacgtgtcaagctccgtgatcacatctctgggcgccatcgtgtcctgctacggcaagacaaagtgcaccgccagcaacaagaaccggggcatcatcaagaccttcagcaacggctgcgactacgtgtccaacaaaggcgtggacaccgtgtctgtgggcaacaccctgtactacgtgaacaagcaagaaggcaagagcctgtacgtgaagggcgagcccatcatcaacttctacgaccctctggtgttccccagcgacgagtttgatgccagcatctcccaagtgaacgagaagatcaaccagagcctggccttcatcagaaagtccgatgagctgctgcacaacgtgaacgccggcaagtccaccaccaatatcatgatcaccacgatcatcatcgtgatcatcgtcatcctgctggctctgatcgctgtgggcctgctgctgtattgatga

SEQ ID NO: 168 - DNA, 1653 bp, synthetic construct
  source 1..1653: mol_type = other DNA
atggaactgctgattcacagaagcagcgccatctttctgaccctggccatcaatgccctgtacctgaccagcagccagaacatcaccgaagagttctaccagagcacctgtagcgccgtgtccagaggctacttttctgccctgagaaccggctggtatttcagcgtgatcaccatcgagctgagcaacatcaaagaaacaaagtgcaacggcaccgacaccaaagtgaagctgatcaagcaagagctggacaagtacaagaacgccgtgaccgaactgcagctgctgatgcagaataccccttgcgccaacaaccgggccagaagagaagcccctcagtacatgaactacaccatcaacaccaccaagaacctgaacgtgtccatcagcaagaagcggaagcggagattcctgggctttctgctcggagtgggaagcgccattgcctctggatgcgccgtgtctaaggtgctgcacctggaaggcgaagtgaacaagatcaagaatgccctgctgagcaccaacaaggccgtggtgtctctgtctaatggcgtgtccgtgctgaccatgaaggtgctggacctgaagaactacatcaacaaccagctgctgcccatcgtgaaccagcagagctgccggatcagcaacatcgagacagtgatcgagttccagcagaagaacagcagactgctggaaatcacccgcgagttttccgtgaatgccggcgtgacaacacccctgagcacctacatgctgaccaacagcgagctgctgtccctgatcaacgacatgcccatcaccaacgaccagaaaaagctgatgagcagcaacgtgcagatcgtgcggcagcagtcctacagcatcatgagcattatcaaagaagagctgctggcctacgtggtgcagctgcctatctacggcgtgatcgataccccttgctggaagctgcacacaagccctctgtgcaccaccaatatcaaagagggctccaacatctgcctgaccagaaccgatagaggctggtactgcgataatgccggcagcgtcagcttcttcccacaagccgatacctgcaaggtgcagagcaacagagtgttctgcgataccatgaacagcctgacactgcccagcgaggtgtccctgtgcaacaccgacatcttcaactctaagtacgactgcaagatcatgacctccaagaccgacatcagctcctccgtgatcacatctctgggcgccatcgtgtcctgctacggcaagacaaagtgtaccgccagcaacaagaaccggggcatcatcaagaccttcagcaacggctgcgactacgtgtccaacaaaggcgtggacaccgtgtctgtgggcaacaccctgtactacgtgaacaagctggaaggcaagaatctgtacgtgaagggcgagcccatcatcaactactacgaccctctggtgttccccagcgacgagtttgatgccagcatcagccaagtgaacgagaagatcaaccagagcctggccttcatccgcagatccgatgaactgctgcacaatgtgaacaccggcaagagcaccacaaacatcatgatcaccgccatcatcatcgtgatcatcgtcgtgctgctgagcctgatcgctatcggcctgctgctgtactgatga

SEQ ID NO: 169 - DNA, 1653 bp, synthetic construct
  source 1..1653: mol_type = other DNA
atggaactgcccatcctgaaaacaaacgccatcaccaccatcctggccgccgtgacactgtgttttgccagcagccagaacatcaccgaagagttctaccagagcacctgtagcgccgtgtctaagggctatctgtctgccctgagaaccggctggtattgcagcgtgatcaccatcgagctgagcaacatcaaagaaaacaagtgcaacggcaccgacgccaaagtgaagctgatcaagcaagagctggacaagtacaagaacgccgtgaccgaactgcagctgctgatgcagtctaccccttgcgccaatagcagagccagacgggaactgcctagattcatgaactacaccctgaacaacaccaagaacaccaacgtgaccctgagcaagaagcggaagcggagattcctgggctttctgctcggagtgggaagcgccattgcctctggatgcgccgtgtccaaggtgctgcatctggaaggcgaagtgaacaagatcaagagcgccctgctgagcaccaacaaggccgtggtttctctgagcaatggcgtgtccgtgctgaccatgaaggtgctggacctgaagaactacatcgacaaacagctgctgcccatcgtcaacaagcagagctgcagcatcagcaacatcgagacagtgatcgagttccagcagaagaacaaccggctgctggaaatcacccgcgagttttctgtgaatgccggcgtgaccacacctgtgtccacctacatgctgaccaacagcgagctgctgtccctgatcaacgacatgcccatcaccaacgaccagaaaaagctgatgagcagcaacgtgcagatcgtgcggcagcagagctactccatcatgagcattatcaaagaagagctgctggcctacgtggtgcagctgcctctgtatggcgtgatcgataccccttgctggaagctgcacacaagccctctgtgcaccaccaacaccaaagagggctccaacatctgcctgaccagaaccgatagaggctggtactgcgataatgccggcagcgtcagcttcttcccacaagccgagacatgcaaggtgcagagcaacagagtgttctgcgataccatgaacagcctgacactgccctccgaagtgaatctgtgcaatatcgacatcttcaacccgaagtacgactgcaagatcatgaccagcaagaccgacgtgtcaagctccgtgatcacatctctgggcgccatcgtgtcctgctacggcaagacaaagtgcaccgccagcaacaagaaccggggcatcatcaagaccttcagcaacggctgcgactacgtgtccaacaaaggcgtggacaccgtgtctgtgggcaacaccctgtactacgtgaacaagcaagaaggcaagagcctgtacgtgaagggcgagcccatcatcaacttctacgaccctctggtgttccccagcgacgagtttgatgccagcatctcccaagtgaacgagaagatcaaccagagcctggccttcatcagaaagtccgatgagctgctgcacaacgtgaacgccggcaagtccaccaccaatatcatgatcaccacgatcatcatcgtgatcatcgtcatcctgctggctctgatcgctgtgggcctgctgctgtattgatga

SEQ ID NO: 170 - DNA, 1653 bp, synthetic construct
  source 1..1653: mol_type = other DNA
atggaactgctgattcacagaagcagcgccatctttctgaccctggccatcaatgccctgtacctgaccagcagccagaacatcaccgaagagttctaccagagcacctgtagcgccgtgtccagaggctacttttctgccctgagaaccggctggtattgcagcgtgatcaccatcgagctgagcaacatcaaagaaacaaagtgcaacggcaccgacaccaaagtgaagctgatcaagcaagagctggacaagtacaagaacgccgtgaccgaactgcagctgctgatgcagaataccccttgcgccaacaaccgggccagaagagaagcccctcagtacatgaactacaccatcaacaccaccaagaacctgaacgtgtccatcagcaagaagcggaagcggagattcctgggctttctgctcggagtgggaagcgccattgcctctggatgcgccgtgtctaaggtgctgcacctggaaggcgaagtgaacaagatcaagaatgccctgctgagcaccaacaaggccgtggtgtctctgtctaatggcgtgtccgtgctgaccatgaaggtgctggacctgaagaactacatcaacaaccagctgctgcccatcgtgaaccagcagagctgccggatcagcaacatcgagacagtgatcgagttccagcagaagaacagcagactgctggaaatcacccgcgagttttccgtgaatgccggcgtgacaacacccctgagcacctacatgctgaccaacagcgagctgctgtccctgatcaacgacatgcccatcaccaacgaccagaaaaagctgatgagcagcaacgtgcagatcgtgcggcagcagtcctacagcatcatgagcattatcaaagaagagctgctggcctacgtggtgcagctgcctatctacggcgtgatcgataccccttgctggaagctgcacacaagccctctgtgcaccaccaatatcaaagagggctccaacatctgcctgaccagaaccgatagaggctggtactgcgataatgccggcagcgtcagcttcttcccacaagccgatacctgcaaggtgcagagcaacagagtgttctgcgataccatgaacagcctgacactgcccagcgaggtgtccctgtgcaacaccgacatcttcaactctaagtacgactgcaagatcatgacctccaagaccgacatcagctcctccgtgatcacatctctgggcgccatcgtgtcctgctacggcaagacaaagtgtaccgccagcaacaagaaccggggcatcatcaagaccttcagcaacggctgcgactacgtgtccaacaaaggcgtggacaccgtgtctgtgggcaacaccctgtactacgtgaacaagctggaaggcaagaatctgtacgtgaagggcgagcccatcatcaactactacgaccctctggtgttccccagcgacgagtttgatgccagcatcagccaagtgaacgagaagatcaaccagagcctggccttcatccgcagatccgatgaactgctgcacaatgtgaacaccggcaagagcaccacaaacatcatgatcaccgccatcatcatcgtgatcatcgtcgtgctgctgagcctgatcgctatcggcctgctgctgtactgatga

SEQ ID NO: 171 - DNA, 1653 bp, synthetic construct
  source 1..1653: mol_type = other DNA
atggaactgcccatcctgaaaacaaacgccatcaccaccatcctggccgccgtgacactgtgttttgccagcagccagaacatcaccgaagagttctaccagagcacctgtagcgccgtgtctaagggctatctgtctgccctgagaaccggctggtatgccagcgtgatcaccatcgagctgagcaacatcaaagaaaacaagtgcaacggcaccgacgccaaagtgaagctgatcaagcaagagctggacaagtacaagaacgccgtgaccgaactgcagctgctgatgcagtctaccccttgcgccaatagcagagccagacgggaactgcctagattcatgaactacaccctgaacaacaccaagaacaccaacgtgaccctgagcaagaagcggaagcggagattcctgggctttctgctcggagtgggaagcgccattgcctctggatgcgccgtgtccaaggtgctgcatctggaaggcgaagtgaacaagatcaagagcgccctgctgagcaccaacaaggccgtggtttctctgagcaatggcgtgtccgtgctgaccatgaaggtgctggacctgaagaactacatcgacaaacagctgctgcccatcgtcaacaagcagagctgcagcatcagcaacatcgagacagtgatcgagttccagcagaagaacaaccggctgctggaaatcacccgcgagttttctgtgaatgccggcgtgaccacacctgtgtccacctacatgctgaccaacagcgagctgctgtccctgatcaacgacatgcccatcaccaacgaccagaaaaagctgatgagcagcaacgtgcagatcgtgcggcagcagagctactccatcatgagcattatcaaagaagagctgctggcctacgtggtgcagctgcctctgtatggcgtgatcgataccccttgctggaagctgcacacaagccctctgtgcaccaccaacaccaaagagggctccaacatctgcctgaccagaaccgatagaggctggtactgcgataatgccggcagcgtcagcttcttcccacaagccgagacatgcaaggtgcagagcaacagagtgttctgcgataccatgaacagcctgacactgccctccgaagtgaatctgtgcaatatcgacatcttcaacccgaagtacgactgcaagatcatgaccagcaagaccgacgtgtcaagctccgtgatcacatctctgggcgccatcgtgtcctgctacggcaagacaaagtgcaccgccagcaacaagaaccggggcatcatcaagaccttcagcaacggctgcgactacgtgtccaacaaaggcgtggacaccgtgtctgtgggcaacaccctgtactacgtgaacaagcaagaaggcaagagcctgtacgtgaagggcgagcccatcatcaacttctacgaccctctggtgttccccagcgacgagtttgatgccagcatctcccaagtgaacgagaagatcaaccagagcctggccttcatcagaaagtccgatgagctgctgcacaacgtgaacgccggcaagtccaccaccaatatcatgatcaccacgatcatcatcgtgatcatcgtcatcctgctggctctgatcgctgtgggcctgctgctgtattgatga

SEQ ID NO: 172 - DNA, 1653 bp, synthetic construct
  source 1..1653: mol_type = other DNA
atggaactgctgattcacagaagcagcgccatctttctgaccctggccatcaatgccctgtacctgaccagcagccagaacatcaccgaagagttctaccagagcacctgtagcgccgtgtccagaggctacttttctgccctgagaaccggctggtatgccagcgtgatcaccatcgagctgagcaacatcaaagaaacaaagtgcaacggcaccgacaccaaagtgaagctgatcaagcaagagctggacaagtacaagaacgccgtgaccgaactgcagctgctgatgcagaataccccttgcgccaacaaccgggccagaagagaagcccctcagtacatgaactacaccatcaacaccaccaagaacctgaacgtgtccatcagcaagaagcggaagcggagattcctgggctttctgctcggagtgggaagcgccattgcctctggatgcgccgtgtctaaggtgctgcacctggaaggcgaagtgaacaagatcaagaatgccctgctgagcaccaacaaggccgtggtgtctctgtctaatggcgtgtccgtgctgaccatgaaggtgctggacctgaagaactacatcaacaaccagctgctgcccatcgtgaaccagcagagctgccggatcagcaacatcgagacagtgatcgagttccagcagaagaacagcagactgctggaaatcacccgcgagttttccgtgaatgccggcgtgacaacacccctgagcacctacatgctgaccaacagcgagctgctgtccctgatcaacgacatgcccatcaccaacgaccagaaaaagctgatgagcagcaacgtgcagatcgtgcggcagcagtcctacagcatcatgagcattatcaaagaagagctgctggcctacgtggtgcagctgcctatctacggcgtgatcgataccccttgctggaagctgcacacaagccctctgtgcaccaccaatatcaaagagggctccaacatctgcctgaccagaaccgatagaggctggtactgcgataatgccggcagcgtcagcttcttcccacaagccgatacctgcaaggtgcagagcaacagagtgttctgcgataccatgaacagcctgacactgcccagcgaggtgtccctgtgcaacaccgacatcttcaactctaagtacgactgcaagatcatgacctccaagaccgacatcagctcctccgtgatcacatctctgggcgccatcgtgtcctgctacggcaagacaaagtgtaccgccagcaacaagaaccggggcatcatcaagaccttcagcaacggctgcgactacgtgtccaacaaaggcgtggacaccgtgtctgtgggcaacaccctgtactacgtgaacaagctggaaggcaagaatctgtacgtgaagggcgagcccatcatcaactactacgaccctctggtgttccccagcgacgagtttgatgccagcatcagccaagtgaacgagaagatcaaccagagcctggccttcatccgcagatccgatgaactgctgcacaatgtgaacaccggcaagagcaccacaaacatcatgatcaccgccatcatcatcgtgatcatcgtcgtgctgctgagcctgatcgctatcggcctgctgctgtactgatga

SEQ ID NO: 173 - DNA, 1653 bp, synthetic construct
  source 1..1653: mol_type = other DNA
atggaactgcccatcctgaaaacaaacgccatcaccaccatcctggccgccgtgacactgtgttttgccagcagccagaacatcaccgaagagttctaccagagcacctgtagcgccgtgtctaagggctatctgtctgccctgagaaccggctggtatgtgagcgtgatcaccatcgagctgagcaacatcaaagaaaacaagtgcaacggcaccgacgccaaagtgaagctgatcaagcaagagctggacaagtacaagaacgccgtgaccgaactgcagctgctgatgcagtctaccccttgcgccaatagcagagccagacgggaactgcctagattcatgaactacaccctgaacaacaccaagaacaccaacgtgaccctgagcaagaagcggaagcggagattcctgggctttctgctcggagtgggaagcgccattgcctctggatgcgccgtgtccaaggtgctgcatctggaaggcgaagtgaacaagatcaagagcgccctgctgagcaccaacaaggccgtggtttctctgagcaatggcgtgtccgtgctgaccttcaaggtgctggacctgaagaactacatcgacaaacagctgctgcccatcgtcaacaagcagagctgcagcatcagcaacatcgagacagtgatcgagttccagcagaagaacaaccggctgctggaaatcacccgcgagttttctgtgaatgccggcgtgaccacacctgtgtccacctacatgctgaccaacagcgagctgctgtccctgatcaacgacatgcccatcaccaacgaccagaaaaagctgatgagcagcaacgtgcagatcgtgcggcagcagagctactccatcatgagcattatcaaagaagagctgctggcctacgtggtgcagctgcctctgtatggcgtgatcgataccccttgctggaagctgcacacaagccctctgtgcaccaccaacaccaaagagggctccaacatctgcctgaccagaaccgatagaggctggtactgcgataatgccggcagcgtcagcttcttcccacaagccgagacatgcaaggtgcagagcaacagagtgttctgcgataccatgaacagcctgacactgccctccgaagtgaatctgtgcaatatcgacatcttcaacccgaagtacgactgcaagatcatgaccagcaagaccgacgtgtcaagctccgtgatcacatctctgggcgccatcgtgtcctgctacggcaagacaaagtgcaccgccagcaacaagaaccggggcatcatcaagaccttcagcaacggctgcgactacgtgtccaacaaaggcgtggacaccgtgtctgtgggcaacaccctgtactacgtgaacaagcaagaaggcaagagcctgtacgtgaagggcgagcccatcatcaacttctacgaccctctggtgttccccagcgacgagtttgatgccagcatctcccaagtgaacgagaagatcaaccagagcctggccttcatcagaaagtccgatgagctgctgcacaacgtgaacgccggcaagtccaccaccaatatcatgatcaccacgatcatcatcgtgatcatcgtcatcctgctggctctgatcgctgtgggcctgctgctgtattgatga

SEQ ID NO: 174 - DNA, 1653 bp, synthetic construct
  source 1..1653: mol_type = other DNA
atggaactgctgattcacagaagcagcgccatctttctgaccctggccatcaatgccctgtacctgaccagcagccagaacatcaccgaagagttctaccagagcacctgtagcgccgtgtccagaggctacttttctgccctgagaaccggctggtatgtgagcgtgatcaccatcgagctgagcaacatcaaagaaacaaagtgcaacggcaccgacaccaaagtgaagctgatcaagcaagagctggacaagtacaagaacgccgtgaccgaactgcagctgctgatgcagaataccccttgcgccaacaaccgggccagaagagaagcccctcagtacatgaactacaccatcaacaccaccaagaacctgaacgtgtccatcagcaagaagcggaagcggagattcctgggctttctgctcggagtgggaagcgccattgcctctggatgcgccgtgtctaaggtgctgcacctggaaggcgaagtgaacaagatcaagaatgccctgctgagcaccaacaaggccgtggtgtctctgtctaatggcgtgtccgtgctgaccttcaaggtgctggacctgaagaactacatcaacaaccagctgctgcccatcgtgaaccagcagagctgccggatcagcaacatcgagacagtgatcgagttccagcagaagaacagcagactgctggaaatcacccgcgagttttccgtgaatgccggcgtgacaacacccctgagcacctacatgctgaccaacagcgagctgctgtccctgatcaacgacatgcccatcaccaacgaccagaaaaagctgatgagcagcaacgtgcagatcgtgcggcagcagtcctacagcatcatgagcattatcaaagaagagctgctggcctacgtggtgcagctgcctatctacggcgtgatcgataccccttgctggaagctgcacacaagccctctgtgcaccaccaatatcaaagagggctccaacatctgcctgaccagaaccgatagaggctggtactgcgataatgccggcagcgtcagcttcttcccacaagccgatacctgcaaggtgcagagcaacagagtgttctgcgataccatgaacagcctgacactgcccagcgaggtgtccctgtgcaacaccgacatcttcaactctaagtacgactgcaagatcatgacctccaagaccgacatcagctcctccgtgatcacatctctgggcgccatcgtgtcctgctacggcaagacaaagtgtaccgccagcaacaagaaccggggcatcatcaagaccttcagcaacggctgcgactacgtgtccaacaaaggcgtggacaccgtgtctgtgggcaacaccctgtactacgtgaacaagctggaaggcaagaatctgtacgtgaagggcgagcccatcatcaactactacgaccctctggtgttccccagcgacgagtttgatgccagcatcagccaagtgaacgagaagatcaaccagagcctggccttcatccgcagatccgatgaactgctgcacaatgtgaacaccggcaagagcaccacaaacatcatgatcaccgccatcatcatcgtgatcatcgtcgtgctgctgagcctgatcgctatcggcctgctgctgtactgatga

SEQ ID NO: 175 - DNA, 1653 bp, synthetic construct
  source 1..1653: mol_type = other DNA
atggaactgcccatcctgaaaacaaacgccatcaccaccatcctggccgccgtgacactgtgttttgccagcagccagaacatcaccgaagagttctaccagagcacctgtagcgccgtgtctaagggctatctgtctgccctgagaaccggctggtatttcagcgtgatcaccatcgagctgagcaacatcaaagaaaacaagtgcaacggcaccgacgccaaagtgaagctgatcaagcaagagctggacaagtacaagaacgccgtgaccgaactgcagctgctgatgcagtctaccccttgcgccaatagcagagccagacgggaactgcctagattcatgaactacaccctgaacaacaccaagaacaccaacgtgaccctgagcaagaagcggaagcggagattcctgggctttctgctcggagtgggaagcgccattgcctctggatgcgccgtgtccaaggtgctgcatctggaaggcgaagtgaacaagatcaagagcgccctgctgagcaccaacaaggccgtggtttctctgagcaatggcgtgtccgtgctgaccttcaaggtgctggacctgaagaactacatcgacaaacagctgctgcccatcgtcaacaagcagagctgcagcatcagcaacatcgagacagtgatcgagttccagcagaagaacaaccggctgctggaaatcacccgcgagttttctgtgaatgccggcgtgaccacacctgtgtccacctacatgctgaccaacagcgagctgctgtccctgatcaacgacatgcccatcaccaacgaccagaaaaagctgatgagcagcaacgtgcagatcgtgcggcagcagagctactccatcatgagcattatcaaagaagagctgctggcctacgtggtgcagctgcctctgtatggcgtgatcgataccccttgctggaagctgcacacaagccctctgtgcaccaccaacaccaaagagggctccaacatctgcctgaccagaaccgatagaggctggtactgcgataatgccggcagcgtcagcttcttcccacaagccgagacatgcaaggtgcagagcaacagagtgttctgcgataccatgaacagcctgacactgccctccgaagtgaatctgtgcaatatcgacatcttcaacccgaagtacgactgcaagatcatgaccagcaagaccgacgtgtcaagctccgtgatcacatctctgggcgccatcgtgtcctgctacggcaagacaaagtgcaccgccagcaacaagaaccggggcatcatcaagaccttcagcaacggctgcgactacgtgtccaacaaaggcgtggacaccgtgtctgtgggcaacaccctgtactacgtgaacaagcaagaaggcaagagcctgtacgtgaagggcgagcccatcatcaacttctacgaccctctggtgttccccagcgacgagtttgatgccagcatctcccaagtgaacgagaagatcaaccagagcctggccttcatcagaaagtccgatgagctgctgcacaacgtgaacgccggcaagtccaccaccaatatcatgatcaccacgatcatcatcgtgatcatcgtcatcctgctggctctgatcgctgtgggcctgctgctgtattgatga

SEQ ID NO: 176 - DNA, 1653 bp, synthetic construct
  source 1..1653: mol_type = other DNA
atggaactgctgattcacagaagcagcgccatctttctgaccctggccatcaatgccctgtacctgaccagcagccagaacatcaccgaagagttctaccagagcacctgtagcgccgtgtccagaggctacttttctgccctgagaaccggctggtatttcagcgtgatcaccatcgagctgagcaacatcaaagaaacaaagtgcaacggcaccgacaccaaagtgaagctgatcaagcaagagctggacaagtacaagaacgccgtgaccgaactgcagctgctgatgcagaataccccttgcgccaacaaccgggccagaagagaagcccctcagtacatgaactacaccatcaacaccaccaagaacctgaacgtgtccatcagcaagaagcggaagcggagattcctgggctttctgctcggagtgggaagcgccattgcctctggatgcgccgtgtctaaggtgctgcacctggaaggcgaagtgaacaagatcaagaatgccctgctgagcaccaacaaggccgtggtgtctctgtctaatggcgtgtccgtgctgaccttcaaggtgctggacctgaagaactacatcaacaaccagctgctgcccatcgtgaaccagcagagctgccggatcagcaacatcgagacagtgatcgagttccagcagaagaacagcagactgctggaaatcacccgcgagttttccgtgaatgccggcgtgacaacacccctgagcacctacatgctgaccaacagcgagctgctgtccctgatcaacgacatgcccatcaccaacgaccagaaaaagctgatgagcagcaacgtgcagatcgtgcggcagcagtcctacagcatcatgagcattatcaaagaagagctgctggcctacgtggtgcagctgcctatctacggcgtgatcgataccccttgctggaagctgcacacaagccctctgtgcaccaccaatatcaaagagggctccaacatctgcctgaccagaaccgatagaggctggtactgcgataatgccggcagcgtcagcttcttcccacaagccgatacctgcaaggtgcagagcaacagagtgttctgcgataccatgaacagcctgacactgcccagcgaggtgtccctgtgcaacaccgacatcttcaactctaagtacgactgcaagatcatgacctccaagaccgacatcagctcctccgtgatcacatctctgggcgccatcgtgtcctgctacggcaagacaaagtgtaccgccagcaacaagaaccggggcatcatcaagaccttcagcaacggctgcgactacgtgtccaacaaaggcgtggacaccgtgtctgtgggcaacaccctgtactacgtgaacaagctggaaggcaagaatctgtacgtgaagggcgagcccatcatcaactactacgaccctctggtgttccccagcgacgagtttgatgccagcatcagccaagtgaacgagaagatcaaccagagcctggccttcatccgcagatccgatgaactgctgcacaatgtgaacaccggcaagagcaccacaaacatcatgatcaccgccatcatcatcgtgatcatcgtcgtgctgctgagcctgatcgctatcggcctgctgctgtactgatga

SEQ ID NO: 177 - DNA, 1653 bp, synthetic construct
  source 1..1653: mol_type = other DNA
atggaactgcccatcctgaaaacaaacgccatcaccaccatcctggccgccgtgacactgtgttttgccagcagccagaacatcaccgaagagttctaccagagcacctgtagcgccgtgtctaagggctatctgtctgccctgagaaccggctggtattgcagcgtgatcaccatcgagctgagcaacatcaaagaaaacaagtgcaacggcaccgacgccaaagtgaagctgatcaagcaagagctggacaagtacaagaacgccgtgaccgaactgcagctgctgatgcagtctaccccttgcgccaatagcagagccagacgggaactgcctagattcatgaactacaccctgaacaacaccaagaacaccaacgtgaccctgagcaagaagcggaagcggagattcctgggctttctgctcggagtgggaagcgccattgcctctggatgcgccgtgtccaaggtgctgcatctggaaggcgaagtgaacaagatcaagagcgccctgctgagcaccaacaaggccgtggtttctctgagcaatggcgtgtccgtgctgaccttcaaggtgctggacctgaagaactacatcgacaaacagctgctgcccatcgtcaacaagcagagctgcagcatcagcaacatcgagacagtgatcgagttccagcagaagaacaaccggctgctggaaatcacccgcgagttttctgtgaatgccggcgtgaccacacctgtgtccacctacatgctgaccaacagcgagctgctgtccctgatcaacgacatgcccatcaccaacgaccagaaaaagctgatgagcagcaacgtgcagatcgtgcggcagcagagctactccatcatgagcattatcaaagaagagctgctggcctacgtggtgcagctgcctctgtatggcgtgatcgataccccttgctggaagctgcacacaagccctctgtgcaccaccaacaccaaagagggctccaacatctgcctgaccagaaccgatagaggctggtactgcgataatgccggcagcgtcagcttcttcccacaagccgagacatgcaaggtgcagagcaacagagtgttctgcgataccatgaacagcctgacactgccctccgaagtgaatctgtgcaatatcgacatcttcaacccgaagtacgactgcaagatcatgaccagcaagaccgacgtgtcaagctccgtgatcacatctctgggcgccatcgtgtcctgctacggcaagacaaagtgcaccgccagcaacaagaaccggggcatcatcaagaccttcagcaacggctgcgactacgtgtccaacaaaggcgtggacaccgtgtctgtgggcaacaccctgtactacgtgaacaagcaagaaggcaagagcctgtacgtgaagggcgagcccatcatcaacttctacgaccctctggtgttccccagcgacgagtttgatgccagcatctcccaagtgaacgagaagatcaaccagagcctggccttcatcagaaagtccgatgagctgctgcacaacgtgaacgccggcaagtccaccaccaatatcatgatcaccacgatcatcatcgtgatcatcgtcatcctgctggctctgatcgctgtgggcctgctgctgtattgatga

SEQ ID NO: 178 - DNA, 1653 bp, synthetic construct
  source 1..1653: mol_type = other DNA
atggaactgctgattcacagaagcagcgccatctttctgaccctggccatcaatgccctgtacctgaccagcagccagaacatcaccgaagagttctaccagagcacctgtagcgccgtgtccagaggctacttttctgccctgagaaccggctggtattgcagcgtgatcaccatcgagctgagcaacatcaaagaaacaaagtgcaacggcaccgacaccaaagtgaagctgatcaagcaagagctggacaagtacaagaacgccgtgaccgaactgcagctgctgatgcagaataccccttgcgccaacaaccgggccagaagagaagcccctcagtacatgaactacaccatcaacaccaccaagaacctgaacgtgtccatcagcaagaagcggaagcggagattcctgggctttctgctcggagtgggaagcgccattgcctctggatgcgccgtgtctaaggtgctgcacctggaaggcgaagtgaacaagatcaagaatgccctgctgagcaccaacaaggccgtggtgtctctgtctaatggcgtgtccgtgctgaccttcaaggtgctggacctgaagaactacatcaacaaccagctgctgcccatcgtgaaccagcagagctgccggatcagcaacatcgagacagtgatcgagttccagcagaagaacagcagactgctggaaatcacccgcgagttttccgtgaatgccggcgtgacaacacccctgagcacctacatgctgaccaacagcgagctgctgtccctgatcaacgacatgcccatcaccaacgaccagaaaaagctgatgagcagcaacgtgcagatcgtgcggcagcagtcctacagcatcatgagcattatcaaagaagagctgctggcctacgtggtgcagctgcctatctacggcgtgatcgataccccttgctggaagctgcacacaagccctctgtgcaccaccaatatcaaagagggctccaacatctgcctgaccagaaccgatagaggctggtactgcgataatgccggcagcgtcagcttcttcccacaagccgatacctgcaaggtgcagagcaacagagtgttctgcgataccatgaacagcctgacactgcccagcgaggtgtccctgtgcaacaccgacatcttcaactctaagtacgactgcaagatcatgacctccaagaccgacatcagctcctccgtgatcacatctctgggcgccatcgtgtcctgctacggcaagacaaagtgtaccgccagcaacaagaaccggggcatcatcaagaccttcagcaacggctgcgactacgtgtccaacaaaggcgtggacaccgtgtctgtgggcaacaccctgtactacgtgaacaagctggaaggcaagaatctgtacgtgaagggcgagcccatcatcaactactacgaccctctggtgttccccagcgacgagtttgatgccagcatcagccaagtgaacgagaagatcaaccagagcctggccttcatccgcagatccgatgaactgctgcacaatgtgaacaccggcaagagcaccacaaacatcatgatcaccgccatcatcatcgtgatcatcgtcgtgctgctgagcctgatcgctatcggcctgctgctgtactgatga

SEQ ID NO: 179 - DNA, 1653 bp, synthetic construct
  source 1..1653: mol_type = other DNA
atggaactgcccatcctgaaaacaaacgccatcaccaccatcctggccgccgtgacactgtgttttgccagcagccagaacatcaccgaagagttctaccagagcacctgtagcgccgtgtctaagggctatctgtctgccctgagaaccggctggtatgccagcgtgatcaccatcgagctgagcaacatcaaagaaaacaagtgcaacggcaccgacgccaaagtgaagctgatcaagcaagagctggacaagtacaagaacgccgtgaccgaactgcagctgctgatgcagtctaccccttgcgccaatagcagagccagacgggaactgcctagattcatgaactacaccctgaacaacaccaagaacaccaacgtgaccctgagcaagaagcggaagcggagattcctgggctttctgctcggagtgggaagcgccattgcctctggatgcgccgtgtccaaggtgctgcatctggaaggcgaagtgaacaagatcaagagcgccctgctgagcaccaacaaggccgtggtttctctgagcaatggcgtgtccgtgctgaccttcaaggtgctggacctgaagaactacatcgacaaacagctgctgcccatcgtcaacaagcagagctgcagcatcagcaacatcgagacagtgatcgagttccagcagaagaacaaccggctgctggaaatcacccgcgagttttctgtgaatgccggcgtgaccacacctgtgtccacctacatgctgaccaacagcgagctgctgtccctgatcaacgacatgcccatcaccaacgaccagaaaaagctgatgagcagcaacgtgcagatcgtgcggcagcagagctactccatcatgagcattatcaaagaagagctgctggcctacgtggtgcagctgcctctgtatggcgtgatcgataccccttgctggaagctgcacacaagccctctgtgcaccaccaacaccaaagagggctccaacatctgcctgaccagaaccgatagaggctggtactgcgataatgccggcagcgtcagcttcttcccacaagccgagacatgcaaggtgcagagcaacagagtgttctgcgataccatgaacagcctgacactgccctccgaagtgaatctgtgcaatatcgacatcttcaacccgaagtacgactgcaagatcatgaccagcaagaccgacgtgtcaagctccgtgatcacatctctgggcgccatcgtgtcctgctacggcaagacaaagtgcaccgccagcaacaagaaccggggcatcatcaagaccttcagcaacggctgcgactacgtgtccaacaaaggcgtggacaccgtgtctgtgggcaacaccctgtactacgtgaacaagcaagaaggcaagagcctgtacgtgaagggcgagcccatcatcaacttctacgaccctctggtgttccccagcgacgagtttgatgccagcatctcccaagtgaacgagaagatcaaccagagcctggccttcatcagaaagtccgatgagctgctgcacaacgtgaacgccggcaagtccaccaccaatatcatgatcaccacgatcatcatcgtgatcatcgtcatcctgctggctctgatcgctgtgggcctgctgctgtattgatga

SEQ ID NO: 180 - DNA, 1653 bp, synthetic construct
  source 1..1653: mol_type = other DNA
atggaactgctgattcacagaagcagcgccatctttctgaccctggccatcaatgccctgtacctgaccagcagccagaacatcaccgaagagttctaccagagcacctgtagcgccgtgtccagaggctacttttctgccctgagaaccggctggtatgccagcgtgatcaccatcgagctgagcaacatcaaagaaacaaagtgcaacggcaccgacaccaaagtgaagctgatcaagcaagagctggacaagtacaagaacgccgtgaccgaactgcagctgctgatgcagaataccccttgcgccaacaaccgggccagaagagaagcccctcagtacatgaactacaccatcaacaccaccaagaacctgaacgtgtccatcagcaagaagcggaagcggagattcctgggctttctgctcggagtgggaagcgccattgcctctggatgcgccgtgtctaaggtgctgcacctggaaggcgaagtgaacaagatcaagaatgccctgctgagcaccaacaaggccgtggtgtctctgtctaatggcgtgtccgtgctgaccttcaaggtgctggacctgaagaactacatcaacaaccagctgctgcccatcgtgaaccagcagagctgccggatcagcaacatcgagacagtgatcgagttccagcagaagaacagcagactgctggaaatcacccgcgagttttccgtgaatgccggcgtgacaacacccctgagcacctacatgctgaccaacagcgagctgctgtccctgatcaacgacatgcccatcaccaacgaccagaaaaagctgatgagcagcaacgtgcagatcgtgcggcagcagtcctacagcatcatgagcattatcaaagaagagctgctggcctacgtggtgcagctgcctatctacggcgtgatcgataccccttgctggaagctgcacacaagccctctgtgcaccaccaatatcaaagagggctccaacatctgcctgaccagaaccgatagaggctggtactgcgataatgccggcagcgtcagcttcttcccacaagccgatacctgcaaggtgcagagcaacagagtgttctgcgataccatgaacagcctgacactgcccagcgaggtgtccctgtgcaacaccgacatcttcaactctaagtacgactgcaagatcatgacctccaagaccgacatcagctcctccgtgatcacatctctgggcgccatcgtgtcctgctacggcaagacaaagtgtaccgccagcaacaagaaccggggcatcatcaagaccttcagcaacggctgcgactacgtgtccaacaaaggcgtggacaccgtgtctgtgggcaacaccctgtactacgtgaacaagctggaaggcaagaatctgtacgtgaagggcgagcccatcatcaactactacgaccctctggtgttccccagcgacgagtttgatgccagcatcagccaagtgaacgagaagatcaaccagagcctggccttcatccgcagatccgatgaactgctgcacaatgtgaacaccggcaagagcaccacaaacatcatgatcaccgccatcatcatcgtgatcatcgtcgtgctgctgagcctgatcgctatcggcctgctgctgtactgatga

SEQ ID NO: 181 - DNA, 1653 bp, synthetic construct
  source 1..1653: mol_type = other DNA
atggaactgcccatcctgaaaacaaacgccatcaccaccatcctggccgccgtgacactgtgttttgccagcagccagaacatcaccgaagagttctaccagagcacctgtagcgccgtgtctaagggctatctgtctgccctgagaaccggctggtatgtgagcgtgatcaccatcgagctgagcaacatcaaagaaaacaagtgcaacggcaccgacgccaaagtgaagctgatcaagcaagagctggacaagtacaagaacgccgtgaccgaactgcagctgctgatgcagtctacctgcgccgccaatagcagagccagacgggaactgcctagattcatgaactacaccctgaacaacaccaagaacaccaacgtgaccctgagcaagaagcggaagcggagattcctgggctttctgctcggagtgggaagcgccattgcctctggatgcgccgtgtccaaggtgctgcatctggaaggcgaagtgaacaagatcaagagcgccctgctgagcaccaacaaggccgtggtttctctgagcaatggcgtgtccgtgctgaccatgaaggtgctggacctgaagaactacatcgacaaacagctgctgcccatcgtcaacaagcagagctgcagcatcagcaacatcgagacagtgatcgagttccagcagaagaacaaccggctgctggaaatcacccgcgagttttctgtgaatgccggcgtgaccacacctgtgtccacctacatgctgaccaacagcgagctgctgtccctgatcaacgacatgcccatcaccaacgaccagaaaaagctgatgagcagcaacgtgcagatcgtgcggcagcagagctactccatcatgagcattatcaaagaagagctgctggcctacgtggtgcagctgcctctgtatggcgtgatcgataccccttgctggaagctgcacacaagccctctgtgcaccaccaacaccaaagagggctccaacatctgcctgaccagaaccgatagaggctggtactgcgataatgccggcagcgtcagcttcttcccacaagccgagacatgcaaggtgcagagcaacagagtgttctgcgataccatgaacagcctgacactgccctccgaagtgaatctgtgcaatatcgacatcttcaacccgaagtacgactgcaagatcatgaccagcaagaccgacgtgtcaagctccgtgatcacatctctgggcgccatcgtgtcctgctacggcaagacaaagtgcaccgccagcaacaagaaccggggcatcatcaagaccttcagcaacggctgcgactacgtgtccaacaaaggcgtggacaccgtgtctgtgggcaacaccctgtactacgtgaacaagcaagaaggcaagagcctgtacgtgaagggcgagcccatcatcaacttctacgaccctctggtgttccccagcgacgagtttgatgccagcatctcccaagtgaacgagaagatcaaccagagcctggccttcatcagaaagtccgatgagctgctgcacaacgtgaacgccggcaagtccaccaccaatatcatgatcaccacgatcatcatcgtgatcatcgtcatcctgctggctctgatcgctgtgggcctgctgctgtattgatga

SEQ ID NO: 182 - DNA, 1653 bp, synthetic construct
  source 1..1653: mol_type = other DNA
atggaactgctgattcacagaagcagcgccatctttctgaccctggccatcaatgccctgtacctgaccagcagccagaacatcaccgaagagttctaccagagcacctgtagcgccgtgtccagaggctacttttctgccctgagaaccggctggtatgtgagcgtgatcaccatcgagctgagcaacatcaaagaaacaaagtgcaacggcaccgacaccaaagtgaagctgatcaagcaagagctggacaagtacaagaacgccgtgaccgaactgcagctgctgatgcagaatacctgcgccgccaacaaccgggccagaagagaagcccctcagtacatgaactacaccatcaacaccaccaagaacctgaacgtgtccatcagcaagaagcggaagcggagattcctgggctttctgctcggagtgggaagcgccattgcctctggatgcgccgtgtctaaggtgctgcacctggaaggcgaagtgaacaagatcaagaatgccctgctgagcaccaacaaggccgtggtgtctctgtctaatggcgtgtccgtgctgaccatgaaggtgctggacctgaagaactacatcaacaaccagctgctgcccatcgtgaaccagcagagctgccggatcagcaacatcgagacagtgatcgagttccagcagaagaacagcagactgctggaaatcacccgcgagttttccgtgaatgccggcgtgacaacacccctgagcacctacatgctgaccaacagcgagctgctgtccctgatcaacgacatgcccatcaccaacgaccagaaaaagctgatgagcagcaacgtgcagatcgtgcggcagcagtcctacagcatcatgagcattatcaaagaagagctgctggcctacgtggtgcagctgcctatctacggcgtgatcgataccccttgctggaagctgcacacaagccctctgtgcaccaccaatatcaaagagggctccaacatctgcctgaccagaaccgatagaggctggtactgcgataatgccggcagcgtcagcttcttcccacaagccgatacctgcaaggtgcagagcaacagagtgttctgcgataccatgaacagcctgacactgcccagcgaggtgtccctgtgcaacaccgacatcttcaactctaagtacgactgcaagatcatgacctccaagaccgacatcagctcctccgtgatcacatctctgggcgccatcgtgtcctgctacggcaagacaaagtgtaccgccagcaacaagaaccggggcatcatcaagaccttcagcaacggctgcgactacgtgtccaacaaaggcgtggacaccgtgtctgtgggcaacaccctgtactacgtgaacaagctggaaggcaagaatctgtacgtgaagggcgagcccatcatcaactactacgaccctctggtgttccccagcgacgagtttgatgccagcatcagccaagtgaacgagaagatcaaccagagcctggccttcatccgcagatccgatgaactgctgcacaatgtgaacaccggcaagagcaccacaaacatcatgatcaccgccatcatcatcgtgatcatcgtcgtgctgctgagcctgatcgctatcggcctgctgctgtactgatga

SEQ ID NO: 183 - DNA, 1653 bp, synthetic construct
  source 1..1653: mol_type = other DNA
atggaactgcccatcctgaaaacaaacgccatcaccaccatcctggccgccgtgacactgtgttttgccagcagccagaacatcaccgaagagttctaccagagcacctgtagcgccgtgtctaagggctatctgtctgccctgagaaccggctggtatttcagcgtgatcaccatcgagctgagcaacatcaaagaaaacaagtgcaacggcaccgacgccaaagtgaagctgatcaagcaagagctggacaagtacaagaacgccgtgaccgaactgcagctgctgatgcagtctacctgcgccgccaatagcagagccagacgggaactgcctagattcatgaactacaccctgaacaacaccaagaacaccaacgtgaccctgagcaagaagcggaagcggagattcctgggctttctgctcggagtgggaagcgccattgcctctggatgcgccgtgtccaaggtgctgcatctggaaggcgaagtgaacaagatcaagagcgccctgctgagcaccaacaaggccgtggtttctctgagcaatggcgtgtccgtgctgaccatgaaggtgctggacctgaagaactacatcgacaaacagctgctgcccatcgtcaacaagcagagctgcagcatcagcaacatcgagacagtgatcgagttccagcagaagaacaaccggctgctggaaatcacccgcgagttttctgtgaatgccggcgtgaccacacctgtgtccacctacatgctgaccaacagcgagctgctgtccctgatcaacgacatgcccatcaccaacgaccagaaaaagctgatgagcagcaacgtgcagatcgtgcggcagcagagctactccatcatgagcattatcaaagaagagctgctggcctacgtggtgcagctgcctctgtatggcgtgatcgataccccttgctggaagctgcacacaagccctctgtgcaccaccaacaccaaagagggctccaacatctgcctgaccagaaccgatagaggctggtactgcgataatgccggcagcgtcagcttcttcccacaagccgagacatgcaaggtgcagagcaacagagtgttctgcgataccatgaacagcctgacactgccctccgaagtgaatctgtgcaatatcgacatcttcaacccgaagtacgactgcaagatcatgaccagcaagaccgacgtgtcaagctccgtgatcacatctctgggcgccatcgtgtcctgctacggcaagacaaagtgcaccgccagcaacaagaaccggggcatcatcaagaccttcagcaacggctgcgactacgtgtccaacaaaggcgtggacaccgtgtctgtgggcaacaccctgtactacgtgaacaagcaagaaggcaagagcctgtacgtgaagggcgagcccatcatcaacttctacgaccctctggtgttccccagcgacgagtttgatgccagcatctcccaagtgaacgagaagatcaaccagagcctggccttcatcagaaagtccgatgagctgctgcacaacgtgaacgccggcaagtccaccaccaatatcatgatcaccacgatcatcatcgtgatcatcgtcatcctgctggctctgatcgctgtgggcctgctgctgtattgatga

SEQ ID NO: 184 - DNA, 1653 bp, synthetic construct
  source 1..1653: mol_type = other DNA
atggaactgctgattcacagaagcagcgccatctttctgaccctggccatcaatgccctgtacctgaccagcagccagaacatcaccgaagagttctaccagagcacctgtagcgccgtgtccagaggctacttttctgccctgagaaccggctggtatttcagcgtgatcaccatcgagctgagcaacatcaaagaaacaaagtgcaacggcaccgacaccaaagtgaagctgatcaagcaagagctggacaagtacaagaacgccgtgaccgaactgcagctgctgatgcagaatacctgcgccgccaacaaccgggccagaagagaagcccctcagtacatgaactacaccatcaacaccaccaagaacctgaacgtgtccatcagcaagaagcggaagcggagattcctgggctttctgctcggagtgggaagcgccattgcctctggatgcgccgtgtctaaggtgctgcacctggaaggcgaagtgaacaagatcaagaatgccctgctgagcaccaacaaggccgtggtgtctctgtctaatggcgtgtccgtgctgaccatgaaggtgctggacctgaagaactacatcaacaaccagctgctgcccatcgtgaaccagcagagctgccggatcagcaacatcgagacagtgatcgagttccagcagaagaacagcagactgctggaaatcacccgcgagttttccgtgaatgccggcgtgacaacacccctgagcacctacatgctgaccaacagcgagctgctgtccctgatcaacgacatgcccatcaccaacgaccagaaaaagctgatgagcagcaacgtgcagatcgtgcggcagcagtcctacagcatcatgagcattatcaaagaagagctgctggcctacgtggtgcagctgcctatctacggcgtgatcgataccccttgctggaagctgcacacaagccctctgtgcaccaccaatatcaaagagggctccaacatctgcctgaccagaaccgatagaggctggtactgcgataatgccggcagcgtcagcttcttcccacaagccgatacctgcaaggtgcagagcaacagagtgttctgcgataccatgaacagcctgacactgcccagcgaggtgtccctgtgcaacaccgacatcttcaactctaagtacgactgcaagatcatgacctccaagaccgacatcagctcctccgtgatcacatctctgggcgccatcgtgtcctgctacggcaagacaaagtgtaccgccagcaacaagaaccggggcatcatcaagaccttcagcaacggctgcgactacgtgtccaacaaaggcgtggacaccgtgtctgtgggcaacaccctgtactacgtgaacaagctggaaggcaagaatctgtacgtgaagggcgagcccatcatcaactactacgaccctctggtgttccccagcgacgagtttgatgccagcatcagccaagtgaacgagaagatcaaccagagcctggccttcatccgcagatccgatgaactgctgcacaatgtgaacaccggcaagagcaccacaaacatcatgatcaccgccatcatcatcgtgatcatcgtcgtgctgctgagcctgatcgctatcggcctgctgctgtactgatga

SEQ ID NO: 185 - DNA, 1653 bp, synthetic construct
  source 1..1653: mol_type = other DNA
atggaactgcccatcctgaaaacaaacgccatcaccaccatcctggccgccgtgacactgtgttttgccagcagccagaacatcaccgaagagttctaccagagcacctgtagcgccgtgtctaagggctatctgtctgccctgagaaccggctggtattgcagcgtgatcaccatcgagctgagcaacatcaaagaaaacaagtgcaacggcaccgacgccaaagtgaagctgatcaagcaagagctggacaagtacaagaacgccgtgaccgaactgcagctgctgatgcagtctacctgcgccgccaatagcagagccagacgggaactgcctagattcatgaactacaccctgaacaacaccaagaacaccaacgtgaccctgagcaagaagcggaagcggagattcctgggctttctgctcggagtgggaagcgccattgcctctggatgcgccgtgtccaaggtgctgcatctggaaggcgaagtgaacaagatcaagagcgccctgctgagcaccaacaaggccgtggtttctctgagcaatggcgtgtccgtgctgaccatgaaggtgctggacctgaagaactacatcgacaaacagctgctgcccatcgtcaacaagcagagctgcagcatcagcaacatcgagacagtgatcgagttccagcagaagaacaaccggctgctggaaatcacccgcgagttttctgtgaatgccggcgtgaccacacctgtgtccacctacatgctgaccaacagcgagctgctgtccctgatcaacgacatgcccatcaccaacgaccagaaaaagctgatgagcagcaacgtgcagatcgtgcggcagcagagctactccatcatgagcattatcaaagaagagctgctggcctacgtggtgcagctgcctctgtatggcgtgatcgataccccttgctggaagctgcacacaagccctctgtgcaccaccaacaccaaagagggctccaacatctgcctgaccagaaccgatagaggctggtactgcgataatgccggcagcgtcagcttcttcccacaagccgagacatgcaaggtgcagagcaacagagtgttctgcgataccatgaacagcctgacactgccctccgaagtgaatctgtgcaatatcgacatcttcaacccgaagtacgactgcaagatcatgaccagcaagaccgacgtgtcaagctccgtgatcacatctctgggcgccatcgtgtcctgctacggcaagacaaagtgcaccgccagcaacaagaaccggggcatcatcaagaccttcagcaacggctgcgactacgtgtccaacaaaggcgtggacaccgtgtctgtgggcaacaccctgtactacgtgaacaagcaagaaggcaagagcctgtacgtgaagggcgagcccatcatcaacttctacgaccctctggtgttccccagcgacgagtttgatgccagcatctcccaagtgaacgagaagatcaaccagagcctggccttcatcagaaagtccgatgagctgctgcacaacgtgaacgccggcaagtccaccaccaatatcatgatcaccacgatcatcatcgtgatcatcgtcatcctgctggctctgatcgctgtgggcctgctgctgtattgatga

SEQ ID NO: 186 - DNA, 1653 bp, synthetic construct
  source 1..1653: mol_type = other DNA
atggaactgctgattcacagaagcagcgccatctttctgaccctggccatcaatgccctgtacctgaccagcagccagaacatcaccgaagagttctaccagagcacctgtagcgccgtgtccagaggctacttttctgccctgagaaccggctggtattgcagcgtgatcaccatcgagctgagcaacatcaaagaaacaaagtgcaacggcaccgacaccaaagtgaagctgatcaagcaagagctggacaagtacaagaacgccgtgaccgaactgcagctgctgatgcagaatacctgcgccgccaacaaccgggccagaagagaagcccctcagtacatgaactacaccatcaacaccaccaagaacctgaacgtgtccatcagcaagaagcggaagcggagattcctgggctttctgctcggagtgggaagcgccattgcctctggatgcgccgtgtctaaggtgctgcacctggaaggcgaagtgaacaagatcaagaatgccctgctgagcaccaacaaggccgtggtgtctctgtctaatggcgtgtccgtgctgaccatgaaggtgctggacctgaagaactacatcaacaaccagctgctgcccatcgtgaaccagcagagctgccggatcagcaacatcgagacagtgatcgagttccagcagaagaacagcagactgctggaaatcacccgcgagttttccgtgaatgccggcgtgacaacacccctgagcacctacatgctgaccaacagcgagctgctgtccctgatcaacgacatgcccatcaccaacgaccagaaaaagctgatgagcagcaacgtgcagatcgtgcggcagcagtcctacagcatcatgagcattatcaaagaagagctgctggcctacgtggtgcagctgcctatctacggcgtgatcgataccccttgctggaagctgcacacaagccctctgtgcaccaccaatatcaaagagggctccaacatctgcctgaccagaaccgatagaggctggtactgcgataatgccggcagcgtcagcttcttcccacaagccgatacctgcaaggtgcagagcaacagagtgttctgcgataccatgaacagcctgacactgcccagcgaggtgtccctgtgcaacaccgacatcttcaactctaagtacgactgcaagatcatgacctccaagaccgacatcagctcctccgtgatcacatctctgggcgccatcgtgtcctgctacggcaagacaaagtgtaccgccagcaacaagaaccggggcatcatcaagaccttcagcaacggctgcgactacgtgtccaacaaaggcgtggacaccgtgtctgtgggcaacaccctgtactacgtgaacaagctggaaggcaagaatctgtacgtgaagggcgagcccatcatcaactactacgaccctctggtgttccccagcgacgagtttgatgccagcatcagccaagtgaacgagaagatcaaccagagcctggccttcatccgcagatccgatgaactgctgcacaatgtgaacaccggcaagagcaccacaaacatcatgatcaccgccatcatcatcgtgatcatcgtcgtgctgctgagcctgatcgctatcggcctgctgctgtactgatga

SEQ ID NO: 187 - DNA, 1653 bp, synthetic construct
  source 1..1653: mol_type = other DNA
atggaactgcccatcctgaaaacaaacgccatcaccaccatcctggccgccgtgacactgtgttttgccagcagccagaacatcaccgaagagttctaccagagcacctgtagcgccgtgtctaagggctatctgtctgccctgagaaccggctggtatgccagcgtgatcaccatcgagctgagcaacatcaaagaaaacaagtgcaacggcaccgacgccaaagtgaagctgatcaagcaagagctggacaagtacaagaacgccgtgaccgaactgcagctgctgatgcagtctacctgcgccgccaatagcagagccagacgggaactgcctagattcatgaactacaccctgaacaacaccaagaacaccaacgtgaccctgagcaagaagcggaagcggagattcctgggctttctgctcggagtgggaagcgccattgcctctggatgcgccgtgtccaaggtgctgcatctggaaggcgaagtgaacaagatcaagagcgccctgctgagcaccaacaaggccgtggtttctctgagcaatggcgtgtccgtgctgaccatgaaggtgctggacctgaagaactacatcgacaaacagctgctgcccatcgtcaacaagcagagctgcagcatcagcaacatcgagacagtgatcgagttccagcagaagaacaaccggctgctggaaatcacccgcgagttttctgtgaatgccggcgtgaccacacctgtgtccacctacatgctgaccaacagcgagctgctgtccctgatcaacgacatgcccatcaccaacgaccagaaaaagctgatgagcagcaacgtgcagatcgtgcggcagcagagctactccatcatgagcattatcaaagaagagctgctggcctacgtggtgcagctgcctctgtatggcgtgatcgataccccttgctggaagctgcacacaagccctctgtgcaccaccaacaccaaagagggctccaacatctgcctgaccagaaccgatagaggctggtactgcgataatgccggcagcgtcagcttcttcccacaagccgagacatgcaaggtgcagagcaacagagtgttctgcgataccatgaacagcctgacactgccctccgaagtgaatctgtgcaatatcgacatcttcaacccgaagtacgactgcaagatcatgaccagcaagaccgacgtgtcaagctccgtgatcacatctctgggcgccatcgtgtcctgctacggcaagacaaagtgcaccgccagcaacaagaaccggggcatcatcaagaccttcagcaacggctgcgactacgtgtccaacaaaggcgtggacaccgtgtctgtgggcaacaccctgtactacgtgaacaagcaagaaggcaagagcctgtacgtgaagggcgagcccatcatcaacttctacgaccctctggtgttccccagcgacgagtttgatgccagcatctcccaagtgaacgagaagatcaaccagagcctggccttcatcagaaagtccgatgagctgctgcacaacgtgaacgccggcaagtccaccaccaatatcatgatcaccacgatcatcatcgtgatcatcgtcatcctgctggctctgatcgctgtgggcctgctgctgtattgatga

SEQ ID NO: 188 - DNA, 1653 bp, synthetic construct
  source 1..1653: mol_type = other DNA
atggaactgctgattcacagaagcagcgccatctttctgaccctggccatcaatgccctgtacctgaccagcagccagaacatcaccgaagagttctaccagagcacctgtagcgccgtgtccagaggctacttttctgccctgagaaccggctggtatgccagcgtgatcaccatcgagctgagcaacatcaaagaaacaaagtgcaacggcaccgacaccaaagtgaagctgatcaagcaagagctggacaagtacaagaacgccgtgaccgaactgcagctgctgatgcagaatacctgcgccgccaacaaccgggccagaagagaagcccctcagtacatgaactacaccatcaacaccaccaagaacctgaacgtgtccatcagcaagaagcggaagcggagattcctgggctttctgctcggagtgggaagcgccattgcctctggatgcgccgtgtctaaggtgctgcacctggaaggcgaagtgaacaagatcaagaatgccctgctgagcaccaacaaggccgtggtgtctctgtctaatggcgtgtccgtgctgaccatgaaggtgctggacctgaagaactacatcaacaaccagctgctgcccatcgtgaaccagcagagctgccggatcagcaacatcgagacagtgatcgagttccagcagaagaacagcagactgctggaaatcacccgcgagttttccgtgaatgccggcgtgacaacacccctgagcacctacatgctgaccaacagcgagctgctgtccctgatcaacgacatgcccatcaccaacgaccagaaaaagctgatgagcagcaacgtgcagatcgtgcggcagcagtcctacagcatcatgagcattatcaaagaagagctgctggcctacgtggtgcagctgcctatctacggcgtgatcgataccccttgctggaagctgcacacaagccctctgtgcaccaccaatatcaaagagggctccaacatctgcctgaccagaaccgatagaggctggtactgcgataatgccggcagcgtcagcttcttcccacaagccgatacctgcaaggtgcagagcaacagagtgttctgcgataccatgaacagcctgacactgcccagcgaggtgtccctgtgcaacaccgacatcttcaactctaagtacgactgcaagatcatgacctccaagaccgacatcagctcctccgtgatcacatctctgggcgccatcgtgtcctgctacggcaagacaaagtgtaccgccagcaacaagaaccggggcatcatcaagaccttcagcaacggctgcgactacgtgtccaacaaaggcgtggacaccgtgtctgtgggcaacaccctgtactacgtgaacaagctggaaggcaagaatctgtacgtgaagggcgagcccatcatcaactactacgaccctctggtgttccccagcgacgagtttgatgccagcatcagccaagtgaacgagaagatcaaccagagcctggccttcatccgcagatccgatgaactgctgcacaatgtgaacaccggcaagagcaccacaaacatcatgatcaccgccatcatcatcgtgatcatcgtcgtgctgctgagcctgatcgctatcggcctgctgctgtactgatga

SEQ ID NO: 189 - DNA, 1653 bp, synthetic construct
  source 1..1653: mol_type = other DNA
atggaactgcccatcctgaaaacaaacgccatcaccaccatcctggccgccgtgacactgtgttttgccagcagccagaacatcaccgaagagttctaccagagcacctgtagcgccgtgtctaagggctatctgtctgccctgagaaccggctggtatgtgagcgtgatcaccatcgagctgagcaacatcaaagaaaacaagtgcaacggcaccgacgccaaagtgaagctgatcaagcaagagctggacaagtacaagaacgccgtgaccgaactgcagctgctgatgcagtctacctgcgccgccaatagcagagccagacgggaactgcctagattcatgaactacaccctgaacaacaccaagaacaccaacgtgaccctgagcaagaagcggaagcggagattcctgggctttctgctcggagtgggaagcgccattgcctctggatgcgccgtgtccaaggtgctgcatctggaaggcgaagtgaacaagatcaagagcgccctgctgagcaccaacaaggccgtggtttctctgagcaatggcgtgtccgtgctgaccttcaaggtgctggacctgaagaactacatcgacaaacagctgctgcccatcgtcaacaagcagagctgcagcatcagcaacatcgagacagtgatcgagttccagcagaagaacaaccggctgctggaaatcacccgcgagttttctgtgaatgccggcgtgaccacacctgtgtccacctacatgctgaccaacagcgagctgctgtccctgatcaacgacatgcccatcaccaacgaccagaaaaagctgatgagcagcaacgtgcagatcgtgcggcagcagagctactccatcatgagcattatcaaagaagagctgctggcctacgtggtgcagctgcctctgtatggcgtgatcgataccccttgctggaagctgcacacaagccctctgtgcaccaccaacaccaaagagggctccaacatctgcctgaccagaaccgatagaggctggtactgcgataatgccggcagcgtcagcttcttcccacaagccgagacatgcaaggtgcagagcaacagagtgttctgcgataccatgaacagcctgacactgccctccgaagtgaatctgtgcaatatcgacatcttcaacccgaagtacgactgcaagatcatgaccagcaagaccgacgtgtcaagctccgtgatcacatctctgggcgccatcgtgtcctgctacggcaagacaaagtgcaccgccagcaacaagaaccggggcatcatcaagaccttcagcaacggctgcgactacgtgtccaacaaaggcgtggacaccgtgtctgtgggcaacaccctgtactacgtgaacaagcaagaaggcaagagcctgtacgtgaagggcgagcccatcatcaacttctacgaccctctggtgttccccagcgacgagtttgatgccagcatctcccaagtgaacgagaagatcaaccagagcctggccttcatcagaaagtccgatgagctgctgcacaacgtgaacgccggcaagtccaccaccaatatcatgatcaccacgatcatcatcgtgatcatcgtcatcctgctggctctgatcgctgtgggcctgctgctgtattgatga

SEQ ID NO: 190 - DNA, 1653 bp, synthetic construct
  source 1..1653: mol_type = other DNA
atggaactgctgattcacagaagcagcgccatctttctgaccctggccatcaatgccctgtacctgaccagcagccagaacatcaccgaagagttctaccagagcacctgtagcgccgtgtccagaggctacttttctgccctgagaaccggctggtatgtgagcgtgatcaccatcgagctgagcaacatcaaagaaacaaagtgcaacggcaccgacaccaaagtgaagctgatcaagcaagagctggacaagtacaagaacgccgtgaccgaactgcagctgctgatgcagaatacctgcgccgccaacaaccgggccagaagagaagcccctcagtacatgaactacaccatcaacaccaccaagaacctgaacgtgtccatcagcaagaagcggaagcggagattcctgggctttctgctcggagtgggaagcgccattgcctctggatgcgccgtgtctaaggtgctgcacctggaaggcgaagtgaacaagatcaagaatgccctgctgagcaccaacaaggccgtggtgtctctgtctaatggcgtgtccgtgctgaccttcaaggtgctggacctgaagaactacatcaacaaccagctgctgcccatcgtgaaccagcagagctgccggatcagcaacatcgagacagtgatcgagttccagcagaagaacagcagactgctggaaatcacccgcgagttttccgtgaatgccggcgtgacaacacccctgagcacctacatgctgaccaacagcgagctgctgtccctgatcaacgacatgcccatcaccaacgaccagaaaaagctgatgagcagcaacgtgcagatcgtgcggcagcagtcctacagcatcatgagcattatcaaagaagagctgctggcctacgtggtgcagctgcctatctacggcgtgatcgataccccttgctggaagctgcacacaagccctctgtgcaccaccaatatcaaagagggctccaacatctgcctgaccagaaccgatagaggctggtactgcgataatgccggcagcgtcagcttcttcccacaagccgatacctgcaaggtgcagagcaacagagtgttctgcgataccatgaacagcctgacactgcccagcgaggtgtccctgtgcaacaccgacatcttcaactctaagtacgactgcaagatcatgacctccaagaccgacatcagctcctccgtgatcacatctctgggcgccatcgtgtcctgctacggcaagacaaagtgtaccgccagcaacaagaaccggggcatcatcaagaccttcagcaacggctgcgactacgtgtccaacaaaggcgtggacaccgtgtctgtgggcaacaccctgtactacgtgaacaagctggaaggcaagaatctgtacgtgaagggcgagcccatcatcaactactacgaccctctggtgttccccagcgacgagtttgatgccagcatcagccaagtgaacgagaagatcaaccagagcctggccttcatccgcagatccgatgaactgctgcacaatgtgaacaccggcaagagcaccacaaacatcatgatcaccgccatcatcatcgtgatcatcgtcgtgctgctgagcctgatcgctatcggcctgctgctgtactgatga

SEQ ID NO: 191 - DNA, 1653 bp, synthetic construct
  source 1..1653: mol_type = other DNA
atggaactgcccatcctgaaaacaaacgccatcaccaccatcctggccgccgtgacactgtgttttgccagcagccagaacatcaccgaagagttctaccagagcacctgtagcgccgtgtctaagggctatctgtctgccctgagaaccggctggtatttcagcgtgatcaccatcgagctgagcaacatcaaagaaaacaagtgcaacggcaccgacgccaaagtgaagctgatcaagcaagagctggacaagtacaagaacgccgtgaccgaactgcagctgctgatgcagtctacctgcgccgccaatagcagagccagacgggaactgcctagattcatgaactacaccctgaacaacaccaagaacaccaacgtgaccctgagcaagaagcggaagcggagattcctgggctttctgctcggagtgggaagcgccattgcctctggatgcgccgtgtccaaggtgctgcatctggaaggcgaagtgaacaagatcaagagcgccctgctgagcaccaacaaggccgtggtttctctgagcaatggcgtgtccgtgctgaccttcaaggtgctggacctgaagaactacatcgacaaacagctgctgcccatcgtcaacaagcagagctgcagcatcagcaacatcgagacagtgatcgagttccagcagaagaacaaccggctgctggaaatcacccgcgagttttctgtgaatgccggcgtgaccacacctgtgtccacctacatgctgaccaacagcgagctgctgtccctgatcaacgacatgcccatcaccaacgaccagaaaaagctgatgagcagcaacgtgcagatcgtgcggcagcagagctactccatcatgagcattatcaaagaagagctgctggcctacgtggtgcagctgcctctgtatggcgtgatcgataccccttgctggaagctgcacacaagccctctgtgcaccaccaacaccaaagagggctccaacatctgcctgaccagaaccgatagaggctggtactgcgataatgccggcagcgtcagcttcttcccacaagccgagacatgcaaggtgcagagcaacagagtgttctgcgataccatgaacagcctgacactgccctccgaagtgaatctgtgcaatatcgacatcttcaacccgaagtacgactgcaagatcatgaccagcaagaccgacgtgtcaagctccgtgatcacatctctgggcgccatcgtgtcctgctacggcaagacaaagtgcaccgccagcaacaagaaccggggcatcatcaagaccttcagcaacggctgcgactacgtgtccaacaaaggcgtggacaccgtgtctgtgggcaacaccctgtactacgtgaacaagcaagaaggcaagagcctgtacgtgaagggcgagcccatcatcaacttctacgaccctctggtgttccccagcgacgagtttgatgccagcatctcccaagtgaacgagaagatcaaccagagcctggccttcatcagaaagtccgatgagctgctgcacaacgtgaacgccggcaagtccaccaccaatatcatgatcaccacgatcatcatcgtgatcatcgtcatcctgctggctctgatcgctgtgggcctgctgctgtattgatga

SEQ ID NO: 192 - DNA, 1653 bp, synthetic construct
  source 1..1653: mol_type = other DNA
atggaactgctgattcacagaagcagcgccatctttctgaccctggccatcaatgccctgtacctgaccagcagccagaacatcaccgaagagttctaccagagcacctgtagcgccgtgtccagaggctacttttctgccctgagaaccggctggtatttcagcgtgatcaccatcgagctgagcaacatcaaagaaacaaagtgcaacggcaccgacaccaaagtgaagctgatcaagcaagagctggacaagtacaagaacgccgtgaccgaactgcagctgctgatgcagaatacctgcgccgccaacaaccgggccagaagagaagcccctcagtacatgaactacaccatcaacaccaccaagaacctgaacgtgtccatcagcaagaagcggaagcggagattcctgggctttctgctcggagtgggaagcgccattgcctctggatgcgccgtgtctaaggtgctgcacctggaaggcgaagtgaacaagatcaagaatgccctgctgagcaccaacaaggccgtggtgtctctgtctaatggcgtgtccgtgctgaccttcaaggtgctggacctgaagaactacatcaacaaccagctgctgcccatcgtgaaccagcagagctgccggatcagcaacatcgagacagtgatcgagttccagcagaagaacagcagactgctggaaatcacccgcgagttttccgtgaatgccggcgtgacaacacccctgagcacctacatgctgaccaacagcgagctgctgtccctgatcaacgacatgcccatcaccaacgaccagaaaaagctgatgagcagcaacgtgcagatcgtgcggcagcagtcctacagcatcatgagcattatcaaagaagagctgctggcctacgtggtgcagctgcctatctacggcgtgatcgataccccttgctggaagctgcacacaagccctctgtgcaccaccaatatcaaagagggctccaacatctgcctgaccagaaccgatagaggctggtactgcgataatgccggcagcgtcagcttcttcccacaagccgatacctgcaaggtgcagagcaacagagtgttctgcgataccatgaacagcctgacactgcccagcgaggtgtccctgtgcaacaccgacatcttcaactctaagtacgactgcaagatcatgacctccaagaccgacatcagctcctccgtgatcacatctctgggcgccatcgtgtcctgctacggcaagacaaagtgtaccgccagcaacaagaaccggggcatcatcaagaccttcagcaacggctgcgactacgtgtccaacaaaggcgtggacaccgtgtctgtgggcaacaccctgtactacgtgaacaagctggaaggcaagaatctgtacgtgaagggcgagcccatcatcaactactacgaccctctggtgttccccagcgacgagtttgatgccagcatcagccaagtgaacgagaagatcaaccagagcctggccttcatccgcagatccgatgaactgctgcacaatgtgaacaccggcaagagcaccacaaacatcatgatcaccgccatcatcatcgtgatcatcgtcgtgctgctgagcctgatcgctatcggcctgctgctgtactgatga

SEQ ID NO: 193 - DNA, 1653 bp, synthetic construct
  source 1..1653: mol_type = other DNA
atggaactgcccatcctgaaaacaaacgccatcaccaccatcctggccgccgtgacactgtgttttgccagcagccagaacatcaccgaagagttctaccagagcacctgtagcgccgtgtctaagggctatctgtctgccctgagaaccggctggtattgcagcgtgatcaccatcgagctgagcaacatcaaagaaaacaagtgcaacggcaccgacgccaaagtgaagctgatcaagcaagagctggacaagtacaagaacgccgtgaccgaactgcagctgctgatgcagtctacctgcgccgccaatagcagagccagacgggaactgcctagattcatgaactacaccctgaacaacaccaagaacaccaacgtgaccctgagcaagaagcggaagcggagattcctgggctttctgctcggagtgggaagcgccattgcctctggatgcgccgtgtccaaggtgctgcatctggaaggcgaagtgaacaagatcaagagcgccctgctgagcaccaacaaggccgtggtttctctgagcaatggcgtgtccgtgctgaccttcaaggtgctggacctgaagaactacatcgacaaacagctgctgcccatcgtcaacaagcagagctgcagcatcagcaacatcgagacagtgatcgagttccagcagaagaacaaccggctgctggaaatcacccgcgagttttctgtgaatgccggcgtgaccacacctgtgtccacctacatgctgaccaacagcgagctgctgtccctgatcaacgacatgcccatcaccaacgaccagaaaaagctgatgagcagcaacgtgcagatcgtgcggcagcagagctactccatcatgagcattatcaaagaagagctgctggcctacgtggtgcagctgcctctgtatggcgtgatcgataccccttgctggaagctgcacacaagccctctgtgcaccaccaacaccaaagagggctccaacatctgcctgaccagaaccgatagaggctggtactgcgataatgccggcagcgtcagcttcttcccacaagccgagacatgcaaggtgcagagcaacagagtgttctgcgataccatgaacagcctgacactgccctccgaagtgaatctgtgcaatatcgacatcttcaacccgaagtacgactgcaagatcatgaccagcaagaccgacgtgtcaagctccgtgatcacatctctgggcgccatcgtgtcctgctacggcaagacaaagtgcaccgccagcaacaagaaccggggcatcatcaagaccttcagcaacggctgcgactacgtgtccaacaaaggcgtggacaccgtgtctgtgggcaacaccctgtactacgtgaacaagcaagaaggcaagagcctgtacgtgaagggcgagcccatcatcaacttctacgaccctctggtgttccccagcgacgagtttgatgccagcatctcccaagtgaacgagaagatcaaccagagcctggccttcatcagaaagtccgatgagctgctgcacaacgtgaacgccggcaagtccaccaccaatatcatgatcaccacgatcatcatcgtgatcatcgtcatcctgctggctctgatcgctgtgggcctgctgctgtattgatga

SEQ ID NO: 194 - DNA, 1653 bp, synthetic construct
  source 1..1653: mol_type = other DNA
atggaactgctgattcacagaagcagcgccatctttctgaccctggccatcaatgccctgtacctgaccagcagccagaacatcaccgaagagttctaccagagcacctgtagcgccgtgtccagaggctacttttctgccctgagaaccggctggtattgcagcgtgatcaccatcgagctgagcaacatcaaagaaacaaagtgcaacggcaccgacaccaaagtgaagctgatcaagcaagagctggacaagtacaagaacgccgtgaccgaactgcagctgctgatgcagaatacctgcgccgccaacaaccgggccagaagagaagcccctcagtacatgaactacaccatcaacaccaccaagaacctgaacgtgtccatcagcaagaagcggaagcggagattcctgggctttctgctcggagtgggaagcgccattgcctctggatgcgccgtgtctaaggtgctgcacctggaaggcgaagtgaacaagatcaagaatgccctgctgagcaccaacaaggccgtggtgtctctgtctaatggcgtgtccgtgctgaccttcaaggtgctggacctgaagaactacatcaacaaccagctgctgcccatcgtgaaccagcagagctgccggatcagcaacatcgagacagtgatcgagttccagcagaagaacagcagactgctggaaatcacccgcgagttttccgtgaatgccggcgtgacaacacccctgagcacctacatgctgaccaacagcgagctgctgtccctgatcaacgacatgcccatcaccaacgaccagaaaaagctgatgagcagcaacgtgcagatcgtgcggcagcagtcctacagcatcatgagcattatcaaagaagagctgctggcctacgtggtgcagctgcctatctacggcgtgatcgataccccttgctggaagctgcacacaagccctctgtgcaccaccaatatcaaagagggctccaacatctgcctgaccagaaccgatagaggctggtactgcgataatgccggcagcgtcagcttcttcccacaagccgatacctgcaaggtgcagagcaacagagtgttctgcgataccatgaacagcctgacactgcccagcgaggtgtccctgtgcaacaccgacatcttcaactctaagtacgactgcaagatcatgacctccaagaccgacatcagctcctccgtgatcacatctctgggcgccatcgtgtcctgctacggcaagacaaagtgtaccgccagcaacaagaaccggggcatcatcaagaccttcagcaacggctgcgactacgtgtccaacaaaggcgtggacaccgtgtctgtgggcaacaccctgtactacgtgaacaagctggaaggcaagaatctgtacgtgaagggcgagcccatcatcaactactacgaccctctggtgttccccagcgacgagtttgatgccagcatcagccaagtgaacgagaagatcaaccagagcctggccttcatccgcagatccgatgaactgctgcacaatgtgaacaccggcaagagcaccacaaacatcatgatcaccgccatcatcatcgtgatcatcgtcgtgctgctgagcctgatcgctatcggcctgctgctgtactgatga

SEQ ID NO: 195 - DNA, 1653 bp, synthetic construct
  source 1..1653: mol_type = other DNA
atggaactgcccatcctgaaaacaaacgccatcaccaccatcctggccgccgtgacactgtgttttgccagcagccagaacatcaccgaagagttctaccagagcacctgtagcgccgtgtctaagggctatctgtctgccctgagaaccggctggtatgccagcgtgatcaccatcgagctgagcaacatcaaagaaaacaagtgcaacggcaccgacgccaaagtgaagctgatcaagcaagagctggacaagtacaagaacgccgtgaccgaactgcagctgctgatgcagtctacctgcgccgccaatagcagagccagacgggaactgcctagattcatgaactacaccctgaacaacaccaagaacaccaacgtgaccctgagcaagaagcggaagcggagattcctgggctttctgctcggagtgggaagcgccattgcctctggatgcgccgtgtccaaggtgctgcatctggaaggcgaagtgaacaagatcaagagcgccctgctgagcaccaacaaggccgtggtttctctgagcaatggcgtgtccgtgctgaccttcaaggtgctggacctgaagaactacatcgacaaacagctgctgcccatcgtcaacaagcagagctgcagcatcagcaacatcgagacagtgatcgagttccagcagaagaacaaccggctgctggaaatcacccgcgagttttctgtgaatgccggcgtgaccacacctgtgtccacctacatgctgaccaacagcgagctgctgtccctgatcaacgacatgcccatcaccaacgaccagaaaaagctgatgagcagcaacgtgcagatcgtgcggcagcagagctactccatcatgagcattatcaaagaagagctgctggcctacgtggtgcagctgcctctgtatggcgtgatcgataccccttgctggaagctgcacacaagccctctgtgcaccaccaacaccaaagagggctccaacatctgcctgaccagaaccgatagaggctggtactgcgataatgccggcagcgtcagcttcttcccacaagccgagacatgcaaggtgcagagcaacagagtgttctgcgataccatgaacagcctgacactgccctccgaagtgaatctgtgcaatatcgacatcttcaacccgaagtacgactgcaagatcatgaccagcaagaccgacgtgtcaagctccgtgatcacatctctgggcgccatcgtgtcctgctacggcaagacaaagtgcaccgccagcaacaagaaccggggcatcatcaagaccttcagcaacggctgcgactacgtgtccaacaaaggcgtggacaccgtgtctgtgggcaacaccctgtactacgtgaacaagcaagaaggcaagagcctgtacgtgaagggcgagcccatcatcaacttctacgaccctctggtgttccccagcgacgagtttgatgccagcatctcccaagtgaacgagaagatcaaccagagcctggccttcatcagaaagtccgatgagctgctgcacaacgtgaacgccggcaagtccaccaccaatatcatgatcaccacgatcatcatcgtgatcatcgtcatcctgctggctctgatcgctgtgggcctgctgctgtattgatga

SEQ ID NO: 196 - DNA, 1653 bp, synthetic construct
  source 1..1653: mol_type = other DNA
atggaactgctgattcacagaagcagcgccatctttctgaccctggccatcaatgccctgtacctgaccagcagccagaacatcaccgaagagttctaccagagcacctgtagcgccgtgtccagaggctacttttctgccctgagaaccggctggtatgccagcgtgatcaccatcgagctgagcaacatcaaagaaacaaagtgcaacggcaccgacaccaaagtgaagctgatcaagcaagagctggacaagtacaagaacgccgtgaccgaactgcagctgctgatgcagaatacctgcgccgccaacaaccgggccagaagagaagcccctcagtacatgaactacaccatcaacaccaccaagaacctgaacgtgtccatcagcaagaagcggaagcggagattcctgggctttctgctcggagtgggaagcgccattgcctctggatgcgccgtgtctaaggtgctgcacctggaaggcgaagtgaacaagatcaagaatgccctgctgagcaccaacaaggccgtggtgtctctgtctaatggcgtgtccgtgctgaccttcaaggtgctggacctgaagaactacatcaacaaccagctgctgcccatcgtgaaccagcagagctgccggatcagcaacatcgagacagtgatcgagttccagcagaagaacagcagactgctggaaatcacccgcgagttttccgtgaatgccggcgtgacaacacccctgagcacctacatgctgaccaacagcgagctgctgtccctgatcaacgacatgcccatcaccaacgaccagaaaaagctgatgagcagcaacgtgcagatcgtgcggcagcagtcctacagcatcatgagcattatcaaagaagagctgctggcctacgtggtgcagctgcctatctacggcgtgatcgataccccttgctggaagctgcacacaagccctctgtgcaccaccaatatcaaagagggctccaacatctgcctgaccagaaccgatagaggctggtactgcgataatgccggcagcgtcagcttcttcccacaagccgatacctgcaaggtgcagagcaacagagtgttctgcgataccatgaacagcctgacactgcccagcgaggtgtccctgtgcaacaccgacatcttcaactctaagtacgactgcaagatcatgacctccaagaccgacatcagctcctccgtgatcacatctctgggcgccatcgtgtcctgctacggcaagacaaagtgtaccgccagcaacaagaaccggggcatcatcaagaccttcagcaacggctgcgactacgtgtccaacaaaggcgtggacaccgtgtctgtgggcaacaccctgtactacgtgaacaagctggaaggcaagaatctgtacgtgaagggcgagcccatcatcaactactacgaccctctggtgttccccagcgacgagtttgatgccagcatcagccaagtgaacgagaagatcaaccagagcctggccttcatccgcagatccgatgaactgctgcacaatgtgaacaccggcaagagcaccacaaacatcatgatcaccgccatcatcatcgtgatcatcgtcgtgctgctgagcctgatcgctatcggcctgctgctgtactgatga

SEQ ID NO: 197 - DNA, 1653 bp, synthetic construct
  source 1..1653: mol_type = other DNA
atggaactgcccatcctgaaaacaaacgccatcaccaccatcctggccgccgtgacactgtgttttgccagcagccagaacatcaccgaagagttctaccagagcacctgtagcgccgtgtctaagggctatctgtctgccctgagaaccggctggtatgtgagcgtgatcaccatcgagctgagcaacatcaaagaaaacaagtgcaacggcaccgacgccaaagtgaagctgatcaagcaagagctggacaagtacaagaacgccgtgaccgaactgcagctgctgatgcagtctaccccttgcgccaatagcagagccagacgggaactgcctagattcatgaactacaccctgaacaacaccaagaacaccaacgtgaccctgagcaagaagcggaagcggagattcctgggctttctgctcggagtgggaagcgccattgcctctggatgcgccgtgtccaaggtgctgcatctggaaggcgaagtgaacaagatcaagagcgccctgctgagcaccaacaaggccgtggtttctctgagcaatggcgtgtccgtgctgaccatcaaggtgctggacctgaagaactacatcgacaaacagctgctgcccatcgtcaacaagcagagctgcagcatcagcaacatcgagacagtgatcgagttccagcagaagaacaaccggctgctggaaatcacccgcgagttttctgtgaatgccggcgtgaccacacctgtgtccacctacatgctgaccaacagcgagctgctgtccctgatcaacgacatgcccatcaccaacgaccagaaaaagctgatgagcagcaacgtgcagatcgtgcggcagcagagctactccatcatgagcattatcaaagaagagctgctggcctacgtggtgcagctgcctctgtatggcgtgatcgataccccttgctggaagctgcacacaagccctctgtgcaccaccaacaccaaagagggctccaacatctgcctgaccagaaccgatagaggctggtactgcgataatgccggcagcgtcagcttcttcccacaagccgagacatgcaaggtgcagagcaacagagtgttctgcgataccatgaacagcctgacactgccctccgaagtgaatctgtgcaatatcgacatcttcaacccgaagtacgactgcaagatcatgaccagcaagaccgacgtgtcaagctccgtgatcacatctctgggcgccatcgtgtcctgctacggcaagacaaagtgcaccgccagcaacaagaaccggggcatcatcaagaccttcagcaacggctgcgactacgtgtccaacaaaggcgtggacaccgtgtctgtgggcaacaccctgtactacgtgaacaagcaagaaggcaagagcctgtacgtgaagggcgagcccatcatcaacttctacgaccctctggtgttccccagcgacgagtttgatgccagcatctcccaagtgaacgagaagatcaaccagagcctggccttcatcagaaagtccgatgagctgctgcacaacgtgaacgccggcaagtccaccaccaatatcatgatcaccacgatcatcatcgtgatcatcgtcatcctgctggctctgatcgctgtgggcctgctgctgtattgatga

SEQ ID NO: 198 - DNA, 1653 bp, synthetic construct
  source 1..1653: mol_type = other DNA
atggaactgctgattcacagaagcagcgccatctttctgaccctggccatcaatgccctgtacctgaccagcagccagaacatcaccgaagagttctaccagagcacctgtagcgccgtgtccagaggctacttttctgccctgagaaccggctggtatgtgagcgtgatcaccatcgagctgagcaacatcaaagaaacaaagtgcaacggcaccgacaccaaagtgaagctgatcaagcaagagctggacaagtacaagaacgccgtgaccgaactgcagctgctgatgcagaataccccttgcgccaacaaccgggccagaagagaagcccctcagtacatgaactacaccatcaacaccaccaagaacctgaacgtgtccatcagcaagaagcggaagcggagattcctgggctttctgctcggagtgggaagcgccattgcctctggatgcgccgtgtctaaggtgctgcacctggaaggcgaagtgaacaagatcaagaatgccctgctgagcaccaacaaggccgtggtgtctctgtctaatggcgtgtccgtgctgaccatcaaggtgctggacctgaagaactacatcaacaaccagctgctgcccatcgtgaaccagcagagctgccggatcagcaacatcgagacagtgatcgagttccagcagaagaacagcagactgctggaaatcacccgcgagttttccgtgaatgccggcgtgacaacacccctgagcacctacatgctgaccaacagcgagctgctgtccctgatcaacgacatgcccatcaccaacgaccagaaaaagctgatgagcagcaacgtgcagatcgtgcggcagcagtcctacagcatcatgagcattatcaaagaagagctgctggcctacgtggtgcagctgcctatctacggcgtgatcgataccccttgctggaagctgcacacaagccctctgtgcaccaccaatatcaaagagggctccaacatctgcctgaccagaaccgatagaggctggtactgcgataatgccggcagcgtcagcttcttcccacaagccgatacctgcaaggtgcagagcaacagagtgttctgcgataccatgaacagcctgacactgcccagcgaggtgtccctgtgcaacaccgacatcttcaactctaagtacgactgcaagatcatgacctccaagaccgacatcagctcctccgtgatcacatctctgggcgccatcgtgtcctgctacggcaagacaaagtgtaccgccagcaacaagaaccggggcatcatcaagaccttcagcaacggctgcgactacgtgtccaacaaaggcgtggacaccgtgtctgtgggcaacaccctgtactacgtgaacaagctggaaggcaagaatctgtacgtgaagggcgagcccatcatcaactactacgaccctctggtgttccccagcgacgagtttgatgccagcatcagccaagtgaacgagaagatcaaccagagcctggccttcatccgcagatccgatgaactgctgcacaatgtgaacaccggcaagagcaccacaaacatcatgatcaccgccatcatcatcgtgatcatcgtcgtgctgctgagcctgatcgctatcggcctgctgctgtactgatga

SEQ ID NO: 199 - DNA, 1653 bp, synthetic construct
  source 1..1653: mol_type = other DNA
atggaactgcccatcctgaaaacaaacgccatcaccaccatcctggccgccgtgacactgtgttttgccagcagccagaacatcaccgaagagttctaccagagcacctgtagcgccgtgtctaagggctatctgtctgccctgagaaccggctggtatttcagcgtgatcaccatcgagctgagcaacatcaaagaaaacaagtgcaacggcaccgacgccaaagtgaagctgatcaagcaagagctggacaagtacaagaacgccgtgaccgaactgcagctgctgatgcagtctaccccttgcgccaatagcagagccagacgggaactgcctagattcatgaactacaccctgaacaacaccaagaacaccaacgtgaccctgagcaagaagcggaagcggagattcctgggctttctgctcggagtgggaagcgccattgcctctggatgcgccgtgtccaaggtgctgcatctggaaggcgaagtgaacaagatcaagagcgccctgctgagcaccaacaaggccgtggtttctctgagcaatggcgtgtccgtgctgaccatcaaggtgctggacctgaagaactacatcgacaaacagctgctgcccatcgtcaacaagcagagctgcagcatcagcaacatcgagacagtgatcgagttccagcagaagaacaaccggctgctggaaatcacccgcgagttttctgtgaatgccggcgtgaccacacctgtgtccacctacatgctgaccaacagcgagctgctgtccctgatcaacgacatgcccatcaccaacgaccagaaaaagctgatgagcagcaacgtgcagatcgtgcggcagcagagctactccatcatgagcattatcaaagaagagctgctggcctacgtggtgcagctgcctctgtatggcgtgatcgataccccttgctggaagctgcacacaagccctctgtgcaccaccaacaccaaagagggctccaacatctgcctgaccagaaccgatagaggctggtactgcgataatgccggcagcgtcagcttcttcccacaagccgagacatgcaaggtgcagagcaacagagtgttctgcgataccatgaacagcctgacactgccctccgaagtgaatctgtgcaatatcgacatcttcaacccgaagtacgactgcaagatcatgaccagcaagaccgacgtgtcaagctccgtgatcacatctctgggcgccatcgtgtcctgctacggcaagacaaagtgcaccgccagcaacaagaaccggggcatcatcaagaccttcagcaacggctgcgactacgtgtccaacaaaggcgtggacaccgtgtctgtgggcaacaccctgtactacgtgaacaagcaagaaggcaagagcctgtacgtgaagggcgagcccatcatcaacttctacgaccctctggtgttccccagcgacgagtttgatgccagcatctcccaagtgaacgagaagatcaaccagagcctggccttcatcagaaagtccgatgagctgctgcacaacgtgaacgccggcaagtccaccaccaatatcatgatcaccacgatcatcatcgtgatcatcgtcatcctgctggctctgatcgctgtgggcctgctgctgtattgatga

SEQ ID NO: 200 - DNA, 1653 bp, synthetic construct
  source 1..1653: mol_type = other DNA
atggaactgctgattcacagaagcagcgccatctttctgaccctggccatcaatgccctgtacctgaccagcagccagaacatcaccgaagagttctaccagagcacctgtagcgccgtgtccagaggctacttttctgccctgagaaccggctggtatttcagcgtgatcaccatcgagctgagcaacatcaaagaaacaaagtgcaacggcaccgacaccaaagtgaagctgatcaagcaagagctggacaagtacaagaacgccgtgaccgaactgcagctgctgatgcagaataccccttgcgccaacaaccgggccagaagagaagcccctcagtacatgaactacaccatcaacaccaccaagaacctgaacgtgtccatcagcaagaagcggaagcggagattcctgggctttctgctcggagtgggaagcgccattgcctctggatgcgccgtgtctaaggtgctgcacctggaaggcgaagtgaacaagatcaagaatgccctgctgagcaccaacaaggccgtggtgtctctgtctaatggcgtgtccgtgctgaccatcaaggtgctggacctgaagaactacatcaacaaccagctgctgcccatcgtgaaccagcagagctgccggatcagcaacatcgagacagtgatcgagttccagcagaagaacagcagactgctggaaatcacccgcgagttttccgtgaatgccggcgtgacaacacccctgagcacctacatgctgaccaacagcgagctgctgtccctgatcaacgacatgcccatcaccaacgaccagaaaaagctgatgagcagcaacgtgcagatcgtgcggcagcagtcctacagcatcatgagcattatcaaagaagagctgctggcctacgtggtgcagctgcctatctacggcgtgatcgataccccttgctggaagctgcacacaagccctctgtgcaccaccaatatcaaagagggctccaacatctgcctgaccagaaccgatagaggctggtactgcgataatgccggcagcgtcagcttcttcccacaagccgatacctgcaaggtgcagagcaacagagtgttctgcgataccatgaacagcctgacactgcccagcgaggtgtccctgtgcaacaccgacatcttcaactctaagtacgactgcaagatcatgacctccaagaccgacatcagctcctccgtgatcacatctctgggcgccatcgtgtcctgctacggcaagacaaagtgtaccgccagcaacaagaaccggggcatcatcaagaccttcagcaacggctgcgactacgtgtccaacaaaggcgtggacaccgtgtctgtgggcaacaccctgtactacgtgaacaagctggaaggcaagaatctgtacgtgaagggcgagcccatcatcaactactacgaccctctggtgttccccagcgacgagtttgatgccagcatcagccaagtgaacgagaagatcaaccagagcctggccttcatccgcagatccgatgaactgctgcacaatgtgaacaccggcaagagcaccacaaacatcatgatcaccgccatcatcatcgtgatcatcgtcgtgctgctgagcctgatcgctatcggcctgctgctgtactgatga

SEQ ID NO: 201 - DNA, 1653 bp, synthetic construct
  source 1..1653: mol_type = other DNA
atggaactgcccatcctgaaaacaaacgccatcaccaccatcctggccgccgtgacactgtgttttgccagcagccagaacatcaccgaagagttctaccagagcacctgtagcgccgtgtctaagggctatctgtctgccctgagaaccggctggtattgcagcgtgatcaccatcgagctgagcaacatcaaagaaaacaagtgcaacggcaccgacgccaaagtgaagctgatcaagcaagagctggacaagtacaagaacgccgtgaccgaactgcagctgctgatgcagtctaccccttgcgccaatagcagagccagacgggaactgcctagattcatgaactacaccctgaacaacaccaagaacaccaacgtgaccctgagcaagaagcggaagcggagattcctgggctttctgctcggagtgggaagcgccattgcctctggatgcgccgtgtccaaggtgctgcatctggaaggcgaagtgaacaagatcaagagcgccctgctgagcaccaacaaggccgtggtttctctgagcaatggcgtgtccgtgctgaccatcaaggtgctggacctgaagaactacatcgacaaacagctgctgcccatcgtcaacaagcagagctgcagcatcagcaacatcgagacagtgatcgagttccagcagaagaacaaccggctgctggaaatcacccgcgagttttctgtgaatgccggcgtgaccacacctgtgtccacctacatgctgaccaacagcgagctgctgtccctgatcaacgacatgcccatcaccaacgaccagaaaaagctgatgagcagcaacgtgcagatcgtgcggcagcagagctactccatcatgagcattatcaaagaagagctgctggcctacgtggtgcagctgcctctgtatggcgtgatcgataccccttgctggaagctgcacacaagccctctgtgcaccaccaacaccaaagagggctccaacatctgcctgaccagaaccgatagaggctggtactgcgataatgccggcagcgtcagcttcttcccacaagccgagacatgcaaggtgcagagcaacagagtgttctgcgataccatgaacagcctgacactgccctccgaagtgaatctgtgcaatatcgacatcttcaacccgaagtacgactgcaagatcatgaccagcaagaccgacgtgtcaagctccgtgatcacatctctgggcgccatcgtgtcctgctacggcaagacaaagtgcaccgccagcaacaagaaccggggcatcatcaagaccttcagcaacggctgcgactacgtgtccaacaaaggcgtggacaccgtgtctgtgggcaacaccctgtactacgtgaacaagcaagaaggcaagagcctgtacgtgaagggcgagcccatcatcaacttctacgaccctctggtgttccccagcgacgagtttgatgccagcatctcccaagtgaacgagaagatcaaccagagcctggccttcatcagaaagtccgatgagctgctgcacaacgtgaacgccggcaagtccaccaccaatatcatgatcaccacgatcatcatcgtgatcatcgtcatcctgctggctctgatcgctgtgggcctgctgctgtattgatga

SEQ ID NO: 202 - DNA, 1653 bp, synthetic construct
  source 1..1653: mol_type = other DNA
atggaactgctgattcacagaagcagcgccatctttctgaccctggccatcaatgccctgtacctgaccagcagccagaacatcaccgaagagttctaccagagcacctgtagcgccgtgtccagaggctacttttctgccctgagaaccggctggtattgcagcgtgatcaccatcgagctgagcaacatcaaagaaacaaagtgcaacggcaccgacaccaaagtgaagctgatcaagcaagagctggacaagtacaagaacgccgtgaccgaactgcagctgctgatgcagaataccccttgcgccaacaaccgggccagaagagaagcccctcagtacatgaactacaccatcaacaccaccaagaacctgaacgtgtccatcagcaagaagcggaagcggagattcctgggctttctgctcggagtgggaagcgccattgcctctggatgcgccgtgtctaaggtgctgcacctggaaggcgaagtgaacaagatcaagaatgccctgctgagcaccaacaaggccgtggtgtctctgtctaatggcgtgtccgtgctgaccatcaaggtgctggacctgaagaactacatcaacaaccagctgctgcccatcgtgaaccagcagagctgccggatcagcaacatcgagacagtgatcgagttccagcagaagaacagcagactgctggaaatcacccgcgagttttccgtgaatgccggcgtgacaacacccctgagcacctacatgctgaccaacagcgagctgctgtccctgatcaacgacatgcccatcaccaacgaccagaaaaagctgatgagcagcaacgtgcagatcgtgcggcagcagtcctacagcatcatgagcattatcaaagaagagctgctggcctacgtggtgcagctgcctatctacggcgtgatcgataccccttgctggaagctgcacacaagccctctgtgcaccaccaatatcaaagagggctccaacatctgcctgaccagaaccgatagaggctggtactgcgataatgccggcagcgtcagcttcttcccacaagccgatacctgcaaggtgcagagcaacagagtgttctgcgataccatgaacagcctgacactgcccagcgaggtgtccctgtgcaacaccgacatcttcaactctaagtacgactgcaagatcatgacctccaagaccgacatcagctcctccgtgatcacatctctgggcgccatcgtgtcctgctacggcaagacaaagtgtaccgccagcaacaagaaccggggcatcatcaagaccttcagcaacggctgcgactacgtgtccaacaaaggcgtggacaccgtgtctgtgggcaacaccctgtactacgtgaacaagctggaaggcaagaatctgtacgtgaagggcgagcccatcatcaactactacgaccctctggtgttccccagcgacgagtttgatgccagcatcagccaagtgaacgagaagatcaaccagagcctggccttcatccgcagatccgatgaactgctgcacaatgtgaacaccggcaagagcaccacaaacatcatgatcaccgccatcatcatcgtgatcatcgtcgtgctgctgagcctgatcgctatcggcctgctgctgtactgatga

SEQ ID NO: 203 - DNA, 1653 bp, synthetic construct
  source 1..1653: mol_type = other DNA
atggaactgcccatcctgaaaacaaacgccatcaccaccatcctggccgccgtgacactgtgttttgccagcagccagaacatcaccgaagagttctaccagagcacctgtagcgccgtgtctaagggctatctgtctgccctgagaaccggctggtatgccagcgtgatcaccatcgagctgagcaacatcaaagaaaacaagtgcaacggcaccgacgccaaagtgaagctgatcaagcaagagctggacaagtacaagaacgccgtgaccgaactgcagctgctgatgcagtctaccccttgcgccaatagcagagccagacgggaactgcctagattcatgaactacaccctgaacaacaccaagaacaccaacgtgaccctgagcaagaagcggaagcggagattcctgggctttctgctcggagtgggaagcgccattgcctctggatgcgccgtgtccaaggtgctgcatctggaaggcgaagtgaacaagatcaagagcgccctgctgagcaccaacaaggccgtggtttctctgagcaatggcgtgtccgtgctgaccatcaaggtgctggacctgaagaactacatcgacaaacagctgctgcccatcgtcaacaagcagagctgcagcatcagcaacatcgagacagtgatcgagttccagcagaagaacaaccggctgctggaaatcacccgcgagttttctgtgaatgccggcgtgaccacacctgtgtccacctacatgctgaccaacagcgagctgctgtccctgatcaacgacatgcccatcaccaacgaccagaaaaagctgatgagcagcaacgtgcagatcgtgcggcagcagagctactccatcatgagcattatcaaagaagagctgctggcctacgtggtgcagctgcctctgtatggcgtgatcgataccccttgctggaagctgcacacaagccctctgtgcaccaccaacaccaaagagggctccaacatctgcctgaccagaaccgatagaggctggtactgcgataatgccggcagcgtcagcttcttcccacaagccgagacatgcaaggtgcagagcaacagagtgttctgcgataccatgaacagcctgacactgccctccgaagtgaatctgtgcaatatcgacatcttcaacccgaagtacgactgcaagatcatgaccagcaagaccgacgtgtcaagctccgtgatcacatctctgggcgccatcgtgtcctgctacggcaagacaaagtgcaccgccagcaacaagaaccggggcatcatcaagaccttcagcaacggctgcgactacgtgtccaacaaaggcgtggacaccgtgtctgtgggcaacaccctgtactacgtgaacaagcaagaaggcaagagcctgtacgtgaagggcgagcccatcatcaacttctacgaccctctggtgttccccagcgacgagtttgatgccagcatctcccaagtgaacgagaagatcaaccagagcctggccttcatcagaaagtccgatgagctgctgcacaacgtgaacgccggcaagtccaccaccaatatcatgatcaccacgatcatcatcgtgatcatcgtcatcctgctggctctgatcgctgtgggcctgctgctgtattgatga

SEQ ID NO: 204 - DNA, 1653 bp, synthetic construct
  source 1..1653: mol_type = other DNA
atggaactgctgattcacagaagcagcgccatctttctgaccctggccatcaatgccctgtacctgaccagcagccagaacatcaccgaagagttctaccagagcacctgtagcgccgtgtccagaggctacttttctgccctgagaaccggctggtatgccagcgtgatcaccatcgagctgagcaacatcaaagaaacaaagtgcaacggcaccgacaccaaagtgaagctgatcaagcaagagctggacaagtacaagaacgccgtgaccgaactgcagctgctgatgcagaataccccttgcgccaacaaccgggccagaagagaagcccctcagtacatgaactacaccatcaacaccaccaagaacctgaacgtgtccatcagcaagaagcggaagcggagattcctgggctttctgctcggagtgggaagcgccattgcctctggatgcgccgtgtctaaggtgctgcacctggaaggcgaagtgaacaagatcaagaatgccctgctgagcaccaacaaggccgtggtgtctctgtctaatggcgtgtccgtgctgaccatcaaggtgctggacctgaagaactacatcaacaaccagctgctgcccatcgtgaaccagcagagctgccggatcagcaacatcgagacagtgatcgagttccagcagaagaacagcagactgctggaaatcacccgcgagttttccgtgaatgccggcgtgacaacacccctgagcacctacatgctgaccaacagcgagctgctgtccctgatcaacgacatgcccatcaccaacgaccagaaaaagctgatgagcagcaacgtgcagatcgtgcggcagcagtcctacagcatcatgagcattatcaaagaagagctgctggcctacgtggtgcagctgcctatctacggcgtgatcgataccccttgctggaagctgcacacaagccctctgtgcaccaccaatatcaaagagggctccaacatctgcctgaccagaaccgatagaggctggtactgcgataatgccggcagcgtcagcttcttcccacaagccgatacctgcaaggtgcagagcaacagagtgttctgcgataccatgaacagcctgacactgcccagcgaggtgtccctgtgcaacaccgacatcttcaactctaagtacgactgcaagatcatgacctccaagaccgacatcagctcctccgtgatcacatctctgggcgccatcgtgtcctgctacggcaagacaaagtgtaccgccagcaacaagaaccggggcatcatcaagaccttcagcaacggctgcgactacgtgtccaacaaaggcgtggacaccgtgtctgtgggcaacaccctgtactacgtgaacaagctggaaggcaagaatctgtacgtgaagggcgagcccatcatcaactactacgaccctctggtgttccccagcgacgagtttgatgccagcatcagccaagtgaacgagaagatcaaccagagcctggccttcatccgcagatccgatgaactgctgcacaatgtgaacaccggcaagagcaccacaaacatcatgatcaccgccatcatcatcgtgatcatcgtcgtgctgctgagcctgatcgctatcggcctgctgctgtactgatga

SEQ ID NO: 205 - DNA, 1638 bp, synthetic construct
  source 1..1638: mol_type = other DNA
atggaactgcccatcctgaaaacaaacgccatcaccaccatcctggccgccgtgacactgtgttttgccagcagccagaacatcaccgaagagttctaccagagcacctgtagcgccgtgtctaagggctatctgtctgccctgagaaccggctggtatcacagcgtgatcaccatcgagctgagcaacatcaaagaaaacaagtgcaacggcaccgacgccaaagtgaagctgatcaagcaagagctggacaagtacaagaacgccgtgaccgaactgcagctgctgatgcagtctacccctgcctgcaatagcagagccagacgggaactgcctagattcatgaactacaccctgaacaacaccaagaacaccaacgtgaccctgagcaagaagcggaagcggagattcctgggctttctgctcggagtgggaagcgcctgcgcctctggaattgccgtgtccaaggtgctgcatctggaaggcgaagtgaacaagatcaagagcgccctgctgagcaccaacaaggccgtggtttctctgagcaatggcgtgtccgtgctgaccatcaaggtgctggacctgaagaactacatcgacaaacagctgctgcccatcgtcaacaagcagagctgcagcatcagcaacatcgagacagtgatcgagttccagcagaagaacaaccggctgctggaaatcacccgcgagttttctgtgaatgccggcgtgaccacacctgtgtccacctacatgctgaccaacagcgagctgctgtccctgatcaacgacatgcccatcaccaacgaccagaaaaagctgatgagcagcaacgtgcagatcgtgcggcagcagagctactccatcatgagcattatcaaagaagagatcctggcctacgtggtgcagctgcctctgtatggcgtgatcgataccccttgctggaagctgcacacaagccctctgtgcaccaccaacaccaaagagggctccaacatctgcctgaccagaaccgatagaggctggtactgcgataatgccggcagcgtcagcttcttcccacaagccgagacatgcaaggtgcagagcaacagagtgttctgcgataccatgaacagcctgacactgccctccgaagtgaatctgtgcaatatcgacatcttcaacccgaagtacgactgcaagatcatgaccagcaagaccgacgtgtcaagctccgtgatcacatctctgggcgccatcgtgtcctgctacggcaagacaaagtgcaccgccagcaacaagaaccggggcatcatcaagaccttcagcaacggctgcgactacgtgtccaacaaaggcgtggacaccgtgtctgtgggcaacaccctgtactacgtgaacaagcaagaaggcaagagcctgtacgtgaagggcgagcccatcatcaacttctacgaccctctggtgttccccagcagcgagtttgatgccagcatctcccaagtgaacgagaagatcaaccagagcctggccttcatcagaaagtccgatgagctgctgagcgccatcggcggctatatccctgaagctcctagagatggacaggcctatgtgcggaaggatggcgaatgggtgctgctgtctaccttcctgtgatga

SEQ ID NO: 206 - DNA, 1638 bp, synthetic construct
  source 1..1638: mol_type = other DNA
atggaactgctgattcacagaagcagcgccatctttctgaccctggccatcaatgccctgtacctgaccagcagccagaacatcaccgaagagttctaccagagcacctgtagcgccgtgtccagaggctacttttctgccctgagaaccggctggtatcacagcgtgatcaccatcgagctgagcaacatcaaagaaacaaagtgcaacggcaccgacaccaaagtgaagctgatcaagcaagagctggacaagtacaagaacgccgtgaccgaactgcagctgctgatgcagaatacccctgcctgcaacaaccgggccagaagagaagcccctcagtacatgaactacaccatcaacaccaccaagaacctgaacgtgtccatcagcaagaagcggaagcggagattcctgggctttctgctcggagtgggaagcgcctgcgcctctggaattgccgtgtctaaggtgctgcacctggaaggcgaagtgaacaagatcaagaatgccctgctgagcaccaacaaggccgtggtgtctctgtctaatggcgtgtccgtgctgaccatcaaggtgctggacctgaagaactacatcaacaaccagctgctgcccatcgtgaaccagcagagctgccggatcagcaacatcgagacagtgatcgagttccagcagaagaacagcagactgctggaaatcacccgcgagttttccgtgaatgccggcgtgacaacacccctgagcacctacatgctgaccaacagcgagctgctgtccctgatcaacgacatgcccatcaccaacgaccagaaaaagctgatgagcagcaacgtgcagatcgtgcggcagcagtcctacagcatcatgagcattatcaaagaagagatcctggcctacgtggtgcagctgcctatctacggcgtgatcgataccccttgctggaagctgcacacaagccctctgtgcaccaccaatatcaaagagggctccaacatctgcctgaccagaaccgatagaggctggtactgcgataatgccggcagcgtcagcttcttcccacaagccgatacctgcaaggtgcagagcaacagagtgttctgcgataccatgaacagcctgacactgcccagcgaggtgtccctgtgcaacaccgacatcttcaactctaagtacgactgcaagatcatgacctccaagaccgacatcagctcctccgtgatcacatctctgggcgccatcgtgtcctgctacggcaagacaaagtgtaccgccagcaacaagaaccggggcatcatcaagaccttcagcaacggctgcgactacgtgtccaacaaaggcgtggacaccgtgtctgtgggcaacaccctgtactacgtgaacaagctggaaggcaagaatctgtacgtgaagggcgagcccatcatcaactactacgaccctctggtgttccccagcagcgagtttgatgccagcatcagccaagtgaacgagaagatcaaccagagcctggccttcatccgcagatccgatgaactgctgtctgccatcggcggctatatccccgaagctcctagagatggacaggcctatgtgcggaaggatggcgaatgggtgctgctgtctaccttcctgtgatga

SEQ ID NO: 207 - DNA, 1653 bp, synthetic construct
  source 1..1653: mol_type = other DNA
atggaactgcccatcctgaaaacaaacgccatcaccaccatcctggccgccgtgacactgtgttttgccagcagccagaacatcaccgaagagttctaccagagcacctgtagcgccgtgtctaagggctatctgtctgccctgagaaccggctggtatcacagcgtgatcaccatcgagctgagcaacatcaaagaaaacaagtgcaacggcaccgacgccaaagtgaagctgatcaagcaagagctggacaagtacaagaacgccgtgaccgaactgcagctgctgatgcagtctacccctgcctgcaatagcagagccagacgggaactgcctagattcatgaactacaccctgaacaacaccaagaacaccaacgtgaccctgagcaagaagcggaagcggagattcctgggctttctgctcggagtgggaagcgcctgcgcctctggaattgccgtgtccaaggtgctgcatctggaaggcgaagtgaacaagatcaagagcgccctgctgagcaccaacaaggccgtggtttctctgagcaatggcgtgtccgtgctgaccatcaaggtgctggacctgaagaactacatcgacaaacagctgctgcccatcgtcaacaagcagagctgcagcatcagcaacatcgagacagtgatcgagttccagcagaagaacaaccggctgctggaaatcacccgcgagttttctgtgaatgccggcgtgaccacacctgtgtccacctacatgctgaccaacagcgagctgctgtccctgatcaacgacatgcccatcaccaacgaccagaaaaagctgatgagcagcaacgtgcagatcgtgcggcagcagagctactccatcatgagcattatcaaagaagagatcctggcctacgtggtgcagctgcctctgtatggcgtgatcgataccccttgctggaagctgcacacaagccctctgtgcaccaccaacaccaaagagggctccaacatctgcctgaccagaaccgatagaggctggtactgcgataatgccggcagcgtcagcttcttcccacaagccgagacatgcaaggtgcagagcaacagagtgttctgcgataccatgaacagcctgacactgccctccgaagtgaatctgtgcaatatcgacatcttcaacccgaagtacgactgcaagatcatgaccagcaagaccgacgtgtcaagctccgtgatcacatctctgggcgccatcgtgtcctgctacggcaagacaaagtgcaccgccagcaacaagaaccggggcatcatcaagaccttcagcaacggctgcgactacgtgtccaacaaaggcgtggacaccgtgtctgtgggcaacaccctgtactacgtgaacaagcaagaaggcaagagcctgtacgtgaagggcgagcccatcatcaacttctacgaccctctggtgttccccagcagcgagtttgatgccagcatctcccaagtgaacgagaagatcaaccagagcctggccttcatcagaaagtccgatgagctgctgcacaacgtgaacgccggcaagtccaccaccaatatcatgatcaccacgatcatcatcgtgatcatcgtcatcctgctggctctgatcgctgtgggcctgctgctgtattgatga

SEQ ID NO: 208 - DNA, 1653 bp, synthetic construct
  source 1..1653: mol_type = other DNA
atggaactgctgattcacagaagcagcgccatctttctgaccctggccatcaatgccctgtacctgaccagcagccagaacatcaccgaagagttctaccagagcacctgtagcgccgtgtccagaggctacttttctgccctgagaaccggctggtatcacagcgtgatcaccatcgagctgagcaacatcaaagaaacaaagtgcaacggcaccgacaccaaagtgaagctgatcaagcaagagctggacaagtacaagaacgccgtgaccgaactgcagctgctgatgcagaatacccctgcctgcaacaaccgggccagaagagaagcccctcagtacatgaactacaccatcaacaccaccaagaacctgaacgtgtccatcagcaagaagcggaagcggagattcctgggctttctgctcggagtgggaagcgcctgcgcctctggaattgccgtgtctaaggtgctgcacctggaaggcgaagtgaacaagatcaagaatgccctgctgagcaccaacaaggccgtggtgtctctgtctaatggcgtgtccgtgctgaccatcaaggtgctggacctgaagaactacatcaacaaccagctgctgcccatcgtgaaccagcagagctgccggatcagcaacatcgagacagtgatcgagttccagcagaagaacagcagactgctggaaatcacccgcgagttttccgtgaatgccggcgtgacaacacccctgagcacctacatgctgaccaacagcgagctgctgtccctgatcaacgacatgcccatcaccaacgaccagaaaaagctgatgagcagcaacgtgcagatcgtgcggcagcagtcctacagcatcatgagcattatcaaagaagagatcctggcctacgtggtgcagctgcctatctacggcgtgatcgataccccttgctggaagctgcacacaagccctctgtgcaccaccaatatcaaagagggctccaacatctgcctgaccagaaccgatagaggctggtactgcgataatgccggcagcgtcagcttcttcccacaagccgatacctgcaaggtgcagagcaacagagtgttctgcgataccatgaacagcctgacactgcccagcgaggtgtccctgtgcaacaccgacatcttcaactctaagtacgactgcaagatcatgacctccaagaccgacatcagctcctccgtgatcacatctctgggcgccatcgtgtcctgctacggcaagacaaagtgtaccgccagcaacaagaaccggggcatcatcaagaccttcagcaacggctgcgactacgtgtccaacaaaggcgtggacaccgtgtctgtgggcaacaccctgtactacgtgaacaagctggaaggcaagaatctgtacgtgaagggcgagcccatcatcaactactacgaccctctggtgttccccagcagcgagtttgatgccagcatcagccaagtgaacgagaagatcaaccagagcctggccttcatccgcagatccgatgaactgctgcacaatgtgaacaccggcaagagcaccacaaacatcatgatcaccgccatcatcatcgtgatcatcgtcgtgctgctgagcctgatcgctatcggcctgctgctgtactgatga

SEQ ID NO: 209 - DNA, 170 bp, synthetic construct
  source 1..170: mol_type = other DNA
taatacgactcactataggacagatcgcctggagacgccatccacgctgttttgacctccatagaagacaccgggaccgatccagcctccgcggccgggaacggtgcattggaacgcggattccccgtgccaagagtgacgtaagtaccgcagtcaccgtccttgacacg

SEQ ID NO: 210 - DNA, 74 bp, synthetic construct
  source 1..74: mol_type = other DNA
tcttcacccagtctgtctcttagaatttatttcccactgacacaaacaagccattttgtctgcttgtataaccc

SEQ ID NO: 211 - DNA, 106 bp, synthetic construct
  source 1..106: mol_type = other DNA
aaaaaaaaaaaagaaaaaaaaaaaaaaaaaagaaagaaaaaaaaaaaaaaaaaaaaaaaaaaaaaaaaaaaaaaaaaaaaaaaaaaaaaaaaaaaaaaaaaaaaaa

SEQ ID NO: 212 - protein, 27 aa, synthetic construct
GYIPEAPRDGQAYVRKDGEWVLLSTFL

SEQ ID NO: 213 - protein, 6 aa, synthetic construct
LVPRGS

SEQ ID NO: 214 - protein, 6 aa, synthetic construct
HHHHHH

SEQ ID NO: 215 - protein, 8 aa, synthetic construct
WSHPGFEK

SEQ ID NO: 216 - protein, 574 aa, synthetic construct
MELPILKTNAITTILAAVTLCFASSQNITEEFYQSTCSAVSKGYLSALRTGWYTSVITIELSNIKENKCNGTDAKVKLIKQELDKYKNAVTELQLLMQSTPAANSRARRELPRFMNYTLNNTKNTNVTLSKKRKRRFLGFLLGVGSAIASGIAVSKVLHLEGEVNKIKSALLSTNKAVVSLSNGVSVLTSKVLDLKNYIDKQLLPIVNKQSCSISNIETVIEFQQKNNRLLEITREFSVNAGVTTPVSTYMLTNSELLSLINDMPITNDQKKLMSSNVQIVRQQSYSIMSIIKEEVLAYVVQLPLYGVIDTPCWKLHTSPLCTTNTKEGSNICLTRTDRGWYCDNAGSVSFFPQAETCKVQSNRVFCDTMNSLTLPSEVNLCNIDIFNPKYDCKIMTSKTDVSSSVITSLGAIVSCYGKTKCTASNKNRGIIKTFSNGCDYVSNKGVDTVSVGNTLYYVNKQEGKSLYVKGEPIINFYDPLVFPSDEFDASISQVNEKINQSLAFIRKSDELLHNVNAGKSTTNIMITTIIIVIIVILLALIAVGLLLYCKARSTPVTLSKDQLSGINNIAFSN

SEQ ID NO: 217 - protein, 574 aa, synthetic construct
MELLIHRSSAIFLTLAINALYLTSSQNITEEFYQSTCSAVSRGYFSALRTGWYTSVITIELSNIKETKCNGTDTKVKLIKQELDKYKNAVTELQLLMQNTPAANNRARREAPQYMNYTINTTKNLNVSISKKRKRRFLGFLLGVGSAIASGIAVSKVLHLEGEVNKIKNALLSTNKAVVSLSNGVSVLTSKVLDLKNYINNQLLPIVNQQSCRISNIETVIEFQQKNSRLLEITREFSVNAGVTTPLSTYMLTNSELLSLINDMPITNDQKKLMSSNVQIVRQQSYSIMSIIKEEVLAYVVQLPIYGVIDTPCWKLHTSPLCTTNIKEGSNICLTRTDRGWYCDNAGSVSFFPQADTCKVQSNRVFCDTMNSLTLPSEVSLCNTDIFNSKYDCKIMTSKTDISSSVITSLGAIVSCYGKTKCTASNKNRGIIKTFSNGCDYVSNKGVDTVSVGNTLYYVNKLEGKNLYVKGEPIINYYDPLVFPSDEFDASISQVNEKINQSLAFIRRSDELLHNVNTGKSTTNIMITAIIIVIIVVLLSLIAIGLLLYCKAKNTPVTLSKDQLSGINNIAFSK

SEQ ID NO: 218 - protein, 510 aa, synthetic construct
MELLILKANAITTILTAVTFCFASGQNITEEFYQSTCSAVSKGYLSALRTGWYTSVITIELSNIKENKCNGTDAKVKLIKQELDKYKNAVTELQLLMQSTPATGSGSAICSGVAVCKVLHLEGEVNKIKSALLSTNKAVVSLSNGVSVLTFKVLDLKNYIDKQLLPILNKQSCSISNIETVIEFQQKNNRLLEITREFSVNAGVTTPVSTYMLTNSELLSLINDMPITNDQKKLMSNNVQIVRQQSYSIMCIIKEEVLAYVVQLPLYGVIDTPCWKLHTSPLCTTNTKEGSNICLTRTDRGWYCDNAGSVSFFPQAETCKVQSNRVFCDTMNSRTLPSEVNLCNVDIFNPKYDCKIMTSKTDVSSSVITSLGAIVSCYGKTKCTASNKNRGIIKTFSNGCDYVSNKGVDTVSVGNTLYCVNKQEGKSLYVKGEPIINFYDPLVFPSDEFDASISQVNEKINQSLAFIRKSDELLHNVNAGKSTTNIMITTIIIVIIVILLSLIAVGLLLY

SEQ ID NO: 219 - protein, 549 aa, synthetic construct
MELPILKTNAITTILAAVTLCFASSQNITEEFYQSTCSAVSKGYLSALRTGWYTSVITIELSNIKENKCNGTDAKVKLIKQELDKYKNAVTELQLLMQSTPACNSRARRELPRFMNYTLNNTKNTNVTLSKKRKRRFLGFLLGVGSACASGIAVSKVLHLEGEVNKIKSALLSTNKAVVSLSNGVSVLTIKVLDLKNYIDKQLLPIVNKQSCSISNIETVIEFQQKNNRLLEITREFSVNAGVTTPVSTYMLTNSELLSLINDMPITNDQKKLMSSNVQIVRQQSYSIMSIIKEEILAYVVQLPLYGVIDTPCWKLHTSPLCTTNTKEGSNICLTRTDRGWYCDNAGSVSFFPQAETCKVQSNRVFCDTMNSLTLPSEVNLCNIDIFNPKYDCKIMTSKTDVSSSVITSLGAIVSCYGKTKCTASNKNRGIIKTFSNGCDYVSNKGVDTVSVGNTLYYVNKQEGKSLYVKGEPIINFYDPLVFPSSEFDASISQVNEKINQSLAFIRKSDELLHNVNAGKSTTNIMITTIIIVIIVILLALIAVGLLLY

SEQ ID NO: 220 - protein, 549 aa, synthetic construct
MELLIHRSSAIFLTLAINALYLTSSQNITEEFYQSTCSAVSRGYFSALRTGWYTSVITIELSNIKETKCNGTDTKVKLIKQELDKYKNAVTELQLLMQNTPACNNRARREAPQYMNYTINTTKNLNVSISKKRKRRFLGFLLGVGSACASGIAVSKVLHLEGEVNKIKNALLSTNKAVVSLSNGVSVLTIKVLDLKNYINNQLLPIVNQQSCRISNIETVIEFQQKNSRLLEITREFSVNAGVTTPLSTYMLTNSELLSLINDMPITNDQKKLMSSNVQIVRQQSYSIMSIIKEEILAYVVQLPIYGVIDTPCWKLHTSPLCTTNIKEGSNICLTRTDRGWYCDNAGSVSFFPQADTCKVQSNRVFCDTMNSLTLPSEVSLCNTDIFNSKYDCKIMTSKTDISSSVITSLGAIVSCYGKTKCTASNKNRGIIKTFSNGCDYVSNKGVDTVSVGNTLYYVNKLEGKNLYVKGEPIINYYDPLVFPSSEFDASISQVNEKINQSLAFIRRSDELLHNVNTGKSTTNIMITAIIIVIIVVLLSLIAIGLLLY

SEQ ID NO: 221 - DNA, 1533 bp, synthetic construct
  source 1..1533: mol_type = other DNA
atggagctgctgatcctgaaggccaacgccatcacgaccatcctgaccgccgtgaccttctgcttcgccagcgggcagaacatcaccgaggagttctaccagtccacctgctccgccgtgagcaagggctacctgtctgccctgagaaccggctggtacaccagcgtgatcaccatcgagctgtccaacatcaaggagaacaagtgcaacggcaccgacgccaaggtgaagctgatcaagcaggagctggacaagtacaagaacgcagtgaccgagctgcagctgctgatgcagagcacaccagccaccggtagcgggtccgccatttgctccggcgtggccgtgtgcaaggtgctgcacctggagggcgaggtgaacaagatcaagagcgccctgctctccaccaacaaggccgtggtgagcctgagcaacggggtgagcgtgctgaccttcaaggtgctggacctgaagaactacatcgacaagcagctgctgcctatcctgaacaagcagagctgcagcatcagcaacatcgagacagtgatcgagttccagcagaagaacaaccggctgctggagatcaccagggagttcagcgtgaacgcaggggtgaccacacccgtgtccacctacatgctgaccaactccgagctgctgagcctgatcaacgatatgcccatcaccaacgaccagaagaagctgatgagcaacaacgtgcagatcgtgcggcagcagtcctactccatcatgtgcatcatcaaggaggaggtgctggcctacgtggtgcagctgcccctgtacggcgtgatcgacaccccttgctggaagctgcacaccagccctctgtgcaccaccaacacgaaggagggcagcaatatctgcctgacccggaccgacaggggctggtactgcgacaacgccggcagcgtgtccttctttccccaggccgagacatgcaaggtgcagtccaacagggtgttctgcgacaccatgaactctcgcaccctgcccagcgaggtgaacctgtgcaacgtggacatcttcaaccccaagtacgactgcaagatcatgacctccaagaccgacgtgtcctctagcgttatcacctccctgggcgccatcgtgagctgctacggcaagaccaagtgcaccgccagcaacaagaacaggggcatcatcaagaccttcagcaacgggtgcgactacgtgtccaacaagggcgtggacaccgtgtccgtgggcaacaccctgtactgcgtgaacaagcaggagggcaagagcctgtacgtgaagggcgagcccatcatcaacttctacgaccctctggtgttccccagcgacgagttcgacgccagcatctcccaggtgaacgagaagatcaaccagagcctggccttcatccgcaagagcgacgagctgctgcacaacgtgaacgccggcaagagcaccacaaacatcatgatcaccaccatcatcatcgtgataatcgtgatcctgctgtccctgatcgctgtgggcctgctgctgtactga

SEQ ID NO: 222 - DNA, 1650 bp, synthetic construct
  source 1..1650: mol_type = other DNA
atggaactgcccatcctgaaaacaaacgccatcaccaccatcctggccgccgtgacactgtgttttgccagcagccagaacatcaccgaagagttctaccagagcacctgtagcgccgtgtctaagggctatctgtctgccctgagaaccggctggtataccagcgtgatcaccatcgagctgagcaacatcaaagaaaacaagtgcaacggcaccgacgccaaagtgaagctgatcaagcaagagctggacaagtacaagaacgccgtgaccgaactgcagctgctgatgcagtctacccctgcctgcaatagcagagccagacgggaactgcctagattcatgaactacaccctgaacaacaccaagaacaccaacgtgaccctgagcaagaagcggaagcggagattcctgggctttctgctcggagtgggaagcgcctgcgcctctggaattgccgtgtccaaggtgctgcatctggaaggcgaagtgaacaagatcaagagcgccctgctgagcaccaacaaggccgtggtttctctgagcaatggcgtgtccgtgctgaccatcaaggtgctggacctgaagaactacatcgacaaacagctgctgcccatcgtcaacaagcagagctgcagcatcagcaacatcgagacagtgatcgagttccagcagaagaacaaccggctgctggaaatcacccgcgagttttctgtgaatgccggcgtgaccacacctgtgtccacctacatgctgaccaacagcgagctgctgtccctgatcaacgacatgcccatcaccaacgaccagaaaaagctgatgagcagcaacgtgcagatcgtgcggcagcagagctactccatcatgagcattatcaaagaagagatcctggcctacgtggtgcagctgcctctgtatggcgtgatcgataccccttgctggaagctgcacacaagccctctgtgcaccaccaacaccaaagagggctccaacatctgcctgaccagaaccgatagaggctggtactgcgataatgccggcagcgtcagcttcttcccacaagccgagacatgcaaggtgcagagcaacagagtgttctgcgataccatgaacagcctgacactgccctccgaagtgaatctgtgcaatatcgacatcttcaacccgaagtacgactgcaagatcatgaccagcaagaccgacgtgtcaagctccgtgatcacatctctgggcgccatcgtgtcctgctacggcaagacaaagtgcaccgccagcaacaagaaccggggcatcatcaagaccttcagcaacggctgcgactacgtgtccaacaaaggcgtggacaccgtgtctgtgggcaacaccctgtactacgtgaacaagcaagaaggcaagagcctgtacgtgaagggcgagcccatcatcaacttctacgaccctctggtgttccccagcagcgagtttgatgccagcatctcccaagtgaacgagaagatcaaccagagcctggccttcatcagaaagtccgatgagctgctgcacaacgtgaacgccggcaagtccaccaccaatatcatgatcaccacgatcatcatcgtgatcatcgtcatcctgctggctctgatcgctgtgggcctgctgctgtattga

SEQ ID NO: 223 - DNA, 1650 bp, synthetic construct
  source 1..1650: mol_type = other DNA
atggaactgctgattcacagaagcagcgccatctttctgaccctggccatcaatgccctgtacctgaccagcagccagaacatcaccgaagagttctaccagagcacctgtagcgccgtgtccagaggctacttttctgccctgagaaccggctggtataccagcgtgatcaccatcgagctgagcaacatcaaagaaacaaagtgcaacggcaccgacaccaaagtgaagctgatcaagcaagagctggacaagtacaagaacgccgtgaccgaactgcagctgctgatgcagaatacccctgcctgcaacaaccgggccagaagagaagcccctcagtacatgaactacaccatcaacaccaccaagaacctgaacgtgtccatcagcaagaagcggaagcggagattcctgggctttctgctcggagtgggaagcgcctgcgcctctggaattgccgtgtctaaggtgctgcacctggaaggcgaagtgaacaagatcaagaatgccctgctgagcaccaacaaggccgtggtgtctctgtctaatggcgtgtccgtgctgaccatcaaggtgctggacctgaagaactacatcaacaaccagctgctgcccatcgtgaaccagcagagctgccggatcagcaacatcgagacagtgatcgagttccagcagaagaacagcagactgctggaaatcacccgcgagttttccgtgaatgccggcgtgacaacacccctgagcacctacatgctgaccaacagcgagctgctgtccctgatcaacgacatgcccatcaccaacgaccagaaaaagctgatgagcagcaacgtgcagatcgtgcggcagcagtcctacagcatcatgagcattatcaaagaagagatcctggcctacgtggtgcagctgcctatctacggcgtgatcgataccccttgctggaagctgcacacaagccctctgtgcaccaccaatatcaaagagggctccaacatctgcctgaccagaaccgatagaggctggtactgcgataatgccggcagcgtcagcttcttcccacaagccgatacctgcaaggtgcagagcaacagagtgttctgcgataccatgaacagcctgacactgcccagcgaggtgtccctgtgcaacaccgacatcttcaactctaagtacgactgcaagatcatgacctccaagaccgacatcagctcctccgtgatcacatctctgggcgccatcgtgtcctgctacggcaagacaaagtgtaccgccagcaacaagaaccggggcatcatcaagaccttcagcaacggctgcgactacgtgtccaacaaaggcgtggacaccgtgtctgtgggcaacaccctgtactacgtgaacaagctggaaggcaagaatctgtacgtgaagggcgagcccatcatcaactactacgaccctctggtgttccccagcagcgagtttgatgccagcatcagccaagtgaacgagaagatcaaccagagcctggccttcatccgcagatccgatgaactgctgcacaatgtgaacaccggcaagagcaccacaaacatcatgatcaccgccatcatcatcgtgatcatcgtcgtgctgctgagcctgatcgctatcggcctgctgctgtactga

SEQ ID NO: 224 - protein, 549 aa, synthetic construct
MELPILKTNAITTILAAVTLCFASSQNITEEFYQSTCSAVSKGYLSALRTGWYHSVITIELSNIKENKCNGTDAKVKLIKQELDKYKNAVTELQLLMQSTPCANSRARRELPRFMNYTLNNTKNTNVTLSKKRKRRFLGFLLGVGSACASGIAVSKVLHLEGEVNKIKSALLSTNKAVVSLSNGVSVLTIKVLDLKNYIDKQLLPIVNKQSCSISNIETVIEFQQKNNRLLEITREFSVNAGVTTPVSTYMLTNSELLSLINDMPITNDQKKLMSSNVQIVRQQSYSIMSIIKEEILAYVVQLPLYGVIDTPCWKLHTSPLCTTNTKEGSNICLTRTDRGWYCDNAGSVSFFPQAETCKVQSNRVFCDTMNSLTLPSEVNLCNIDIFNPKYDCKIMTSKTDVSSSVITSLGAIVSCYGKTKCTASNKNRGIIKTFSNGCDYVSNKGVDTVSVGNTLYYVNKQEGKSLYVKGEPIINFYDPLVFPSSEFDASISQVNEKINQSLAFIRKSDELLHNVNAGKSTTNIMITTIIIVIIVILLALIAVGLLLY

SEQ ID NO: 225 - protein, 549 aa, synthetic construct
MELLIHRSSAIFLTLAINALYLTSSQNITEEFYQSTCSAVSRGYFSALRTGWYHSVITIELSNIKETKCNGTDTKVKLIKQELDKYKNAVTELQLLMQNTPCANNRARREAPQYMNYTINTTKNLNVSISKKRKRRFLGFLLGVGSACASGIAVSKVLHLEGEVNKIKNALLSTNKAVVSLSNGVSVLTIKVLDLKNYINNQLLPIVNQQSCRISNIETVIEFQQKNSRLLEITREFSVNAGVTTPLSTYMLTNSELLSLINDMPITNDQKKLMSSNVQIVRQQSYSIMSIIKEEILAYVVQLPIYGVIDTPCWKLHTSPLCTTNIKEGSNICLTRTDRGWYCDNAGSVSFFPQADTCKVQSNRVFCDTMNSLTLPSEVSLCNTDIFNSKYDCKIMTSKTDISSSVITSLGAIVSCYGKTKCTASNKNRGIIKTFSNGCDYVSNKGVDTVSVGNTLYYVNKLEGKNLYVKGEPIINYYDPLVFPSSEFDASISQVNEKINQSLAFIRRSDELLHNVNTGKSTTNIMITAIIIVIIVVLLSLIAIGLLLY

SEQ ID NO: 226 - protein, 549 aa, synthetic construct
MELPILKTNAITTILAAVTLCFASSQNITEEFYQSTCSAVSKGYLSALRTGWYHSVITIELSNIKENKCNGTDAKVKLIKQELDKYKNAVTELQLLMQSTPCANSRARRELPRFMNYTLNNTKNTNVTLSKKRKRRFLGFLLGVGSAIASGCAVSKVLHLEGEVNKIKSALLSTNKAVVSLSNGVSVLTIKVLDLKNYIDKQLLPIVNKQSCSISNIETVIEFQQKNNRLLEITREFSVNAGVTTPVSTYMLTNSELLSLINDMPITNDQKKLMSSNVQIVRQQSYSIMSIIKEEILAYVVQLPLYGVIDTPCWKLHTSPLCTTNTKEGSNICLTRTDRGWYCDNAGSVSFFPQAETCKVQSNRVFCDTMNSLTLPSEVNLCNIDIFNPKYDCKIMTSKTDVSSSVITSLGAIVSCYGKTKCTASNKNRGIIKTFSNGCDYVSNKGVDTVSVGNTLYYVNKQEGKSLYVKGEPIINFYDPLVFPSSEFDASISQVNEKINQSLAFIRKSDELLHNVNAGKSTTNIMITTIIIVIIVILLALIAVGLLLY

SEQ ID NO: 227 - protein, 549 aa, synthetic construct
MELLIHRSSAIFLTLAINALYLTSSQNITEEFYQSTCSAVSRGYFSALRTGWYHSVITIELSNIKETKCNGTDTKVKLIKQELDKYKNAVTELQLLMQNTPCANNRARREAPQYMNYTINTTKNLNVSISKKRKRRFLGFLLGVGSAIASGCAVSKVLHLEGEVNKIKNALLSTNKAVVSLSNGVSVLTIKVLDLKNYINNQLLPIVNQQSCRISNIETVIEFQQKNSRLLEITREFSVNAGVTTPLSTYMLTNSELLSLINDMPITNDQKKLMSSNVQIVRQQSYSIMSIIKEEILAYVVQLPIYGVIDTPCWKLHTSPLCTTNIKEGSNICLTRTDRGWYCDNAGSVSFFPQADTCKVQSNRVFCDTMNSLTLPSEVSLCNTDIFNSKYDCKIMTSKTDISSSVITSLGAIVSCYGKTKCTASNKNRGIIKTFSNGCDYVSNKGVDTVSVGNTLYYVNKLEGKNLYVKGEPIINYYDPLVFPSSEFDASISQVNEKINQSLAFIRRSDELLHNVNTGKSTTNIMITAIIIVIIVVLLSLIAIGLLLY

SEQ ID NO: 228 - protein, 549 aa, synthetic construct
MELPILKTNAITTILAAVTLCFASSQNITEEFYQSTCSAVSKGYLSALRTGWYHSVITIELSNIKENKCNGTDAKVKLIKQELDKYKNAVTELQLLMQSTPAACSRARRELPRFMNYTLNNTKNTNVTLSKKRKRRFLGFLLGVCSAIASGIAVSKVLHLEGEVNKIKSALLSTNKAVVSLSNGVSVLTIKVLDLKNYIDKQLLPIVNKQSCSISNIETVIEFQQKNNRLLEITREFSVNAGVTTPVSTYMLTNSELLSLINDMPITNDQKKLMSSNVQIVRQQSYSIMSIIKEEILAYVVQLPLYGVIDTPCWKLHTSPLCTTNTKEGSNICLTRTDRGWYCDNAGSVSFFPQAETCKVQSNRVFCDTMNSLTLPSEVNLCNIDIFNPKYDCKIMTSKTDVSSSVITSLGAIVSCYGKTKCTASNKNRGIIKTFSNGCDYVSNKGVDTVSVGNTLYYVNKQEGKSLYVKGEPIINFYDPLVFPSSEFDASISQVNEKINQSLAFIRKSDELLHNVNAGKSTTNIMITTIIIVIIVILLALIAVGLLLY

SEQ ID NO: 229 - protein, 549 aa, synthetic construct
MELLIHRSSAIFLTLAINALYLTSSQNITEEFYQSTCSAVSRGYFSALRTGWYHSVITIELSNIKETKCNGTDTKVKLIKQELDKYKNAVTELQLLMQNTPAACNRARREAPQYMNYTINTTKNLNVSISKKRKRRFLGFLLGVCSAIASGIAVSKVLHLEGEVNKIKNALLSTNKAVVSLSNGVSVLTIKVLDLKNYINNQLLPIVNQQSCRISNIETVIEFQQKNSRLLEITREFSVNAGVTTPLSTYMLTNSELLSLINDMPITNDQKKLMSSNVQIVRQQSYSIMSIIKEEILAYVVQLPIYGVIDTPCWKLHTSPLCTTNIKEGSNICLTRTDRGWYCDNAGSVSFFPQADTCKVQSNRVFCDTMNSLTLPSEVSLCNTDIFNSKYDCKIMTSKTDISSSVITSLGAIVSCYGKTKCTASNKNRGIIKTFSNGCDYVSNKGVDTVSVGNTLYYVNKLEGKNLYVKGEPIINYYDPLVFPSSEFDASISQVNEKINQSLAFIRRSDELLHNVNTGKSTTNIMITAIIIVIIVVLLSLIAIGLLLY

SEQ ID NO: 230 - protein, 549 aa, synthetic construct
MELPILKTNAITTILAAVTLCFASSQNITEEFYQSTCSAVSKGYLSALRTGWYHSVITIELSNIKENKCNGTDAKVKLIKQELDKYKNAVTELQLLMQSTPAACSRARRELPRFMNYTLNNTKNTNVTLSKKRKRRFLGFLLGVGCAIASGIAVSKVLHLEGEVNKIKSALLSTNKAVVSLSNGVSVLTIKVLDLKNYIDKQLLPIVNKQSCSISNIETVIEFQQKNNRLLEITREFSVNAGVTTPVSTYMLTNSELLSLINDMPITNDQKKLMSSNVQIVRQQSYSIMSIIKEEILAYVVQLPLYGVIDTPCWKLHTSPLCTTNTKEGSNICLTRTDRGWYCDNAGSVSFFPQAETCKVQSNRVFCDTMNSLTLPSEVNLCNIDIFNPKYDCKIMTSKTDVSSSVITSLGAIVSCYGKTKCTASNKNRGIIKTFSNGCDYVSNKGVDTVSVGNTLYYVNKQEGKSLYVKGEPIINFYDPLVFPSSEFDASISQVNEKINQSLAFIRKSDELLHNVNAGKSTTNIMITTIIIVIIVILLALIAVGLLLY

SEQ ID NO: 231 - protein, 549 aa, synthetic construct
MELLIHRSSAIFLTLAINALYLTSSQNITEEFYQSTCSAVSRGYFSALRTGWYHSVITIELSNIKETKCNGTDTKVKLIKQELDKYKNAVTELQLLMQNTPAACNRARREAPQYMNYTINTTKNLNVSISKKRKRRFLGFLLGVGCAIASGIAVSKVLHLEGEVNKIKNALLSTNKAVVSLSNGVSVLTIKVLDLKNYINNQLLPIVNQQSCRISNIETVIEFQQKNSRLLEITREFSVNAGVTTPLSTYMLTNSELLSLINDMPITNDQKKLMSSNVQIVRQQSYSIMSIIKEEILAYVVQLPIYGVIDTPCWKLHTSPLCTTNIKEGSNICLTRTDRGWYCDNAGSVSFFPQADTCKVQSNRVFCDTMNSLTLPSEVSLCNTDIFNSKYDCKIMTSKTDISSSVITSLGAIVSCYGKTKCTASNKNRGIIKTFSNGCDYVSNKGVDTVSVGNTLYYVNKLEGKNLYVKGEPIINYYDPLVFPSSEFDASISQVNEKINQSLAFIRRSDELLHNVNTGKSTTNIMITAIIIVIIVVLLSLIAIGLLLY

SEQ ID NO: 232 - protein, 549 aa, synthetic construct
MELPILKTNAITTILAAVTLCFASSQNITEEFYQSTCSAVSKGYLSALRTGWYHSVITIELSNIKENKCNGTDAKVKLIKQELDKYKNAVTELQLLMQSTPAANCRARRELPRFMNYTLNNTKNTNVTLSKKRKRRFLGFLLGVGSCIASGIAVSKVLHLEGEVNKIKSALLSTNKAVVSLSNGVSVLTIKVLDLKNYIDKQLLPIVNKQSCSISNIETVIEFQQKNNRLLEITREFSVNAGVTTPVSTYMLTNSELLSLINDMPITNDQKKLMSSNVQIVRQQSYSIMSIIKEEILAYVVQLPLYGVIDTPCWKLHTSPLCTTNTKEGSNICLTRTDRGWYCDNAGSVSFFPQAETCKVQSNRVFCDTMNSLTLPSEVNLCNIDIFNPKYDCKIMTSKTDVSSSVITSLGAIVSCYGKTKCTASNKNRGIIKTFSNGCDYVSNKGVDTVSVGNTLYYVNKQEGKSLYVKGEPIINFYDPLVFPSSEFDASISQVNEKINQSLAFIRKSDELLHNVNAGKSTTNIMITTIIIVIIVILLALIAVGLLLY

SEQ ID NO: 233 - protein, 549 aa, synthetic construct
MELLIHRSSAIFLTLAINALYLTSSQNITEEFYQSTCSAVSRGYFSALRTGWYHSVITIELSNIKETKCNGTDTKVKLIKQELDKYKNAVTELQLLMQNTPAANCRARREAPQYMNYTINTTKNLNVSISKKRKRRFLGFLLGVGSCIASGIAVSKVLHLEGEVNKIKNALLSTNKAVVSLSNGVSVLTIKVLDLKNYINNQLLPIVNQQSCRISNIETVIEFQQKNSRLLEITREFSVNAGVTTPLSTYMLTNSELLSLINDMPITNDQKKLMSSNVQIVRQQSYSIMSIIKEEILAYVVQLPIYGVIDTPCWKLHTSPLCTTNIKEGSNICLTRTDRGWYCDNAGSVSFFPQADTCKVQSNRVFCDTMNSLTLPSEVSLCNTDIFNSKYDCKIMTSKTDISSSVITSLGAIVSCYGKTKCTASNKNRGIIKTFSNGCDYVSNKGVDTVSVGNTLYYVNKLEGKNLYVKGEPIINYYDPLVFPSSEFDASISQVNEKINQSLAFIRRSDELLHNVNTGKSTTNIMITAIIIVIIVVLLSLIAIGLLLY

SEQ ID NO: 234 - protein, 549 aa, synthetic construct
MELPILKTNAITTILAAVTLCFASSQNITEEFYQSTCSAVSKGYLSALRTGWYHSVITIELSNIKENKCNGTDAKVKLIKQELDKYKNAVTELQLLMQSTPAANCRARRELPRFMNYTLNNTKNTNVTLSKKRKRRFLGFLLGVCSAIASGIAVSKVLHLEGEVNKIKSALLSTNKAVVSLSNGVSVLTIKVLDLKNYIDKQLLPIVNKQSCSISNIETVIEFQQKNNRLLEITREFSVNAGVTTPVSTYMLTNSELLSLINDMPITNDQKKLMSSNVQIVRQQSYSIMSIIKEEILAYVVQLPLYGVIDTPCWKLHTSPLCTTNTKEGSNICLTRTDRGWYCDNAGSVSFFPQAETCKVQSNRVFCDTMNSLTLPSEVNLCNIDIFNPKYDCKIMTSKTDVSSSVITSLGAIVSCYGKTKCTASNKNRGIIKTFSNGCDYVSNKGVDTVSVGNTLYYVNKQEGKSLYVKGEPIINFYDPLVFPSSEFDASISQVNEKINQSLAFIRKSDELLHNVNAGKSTTNIMITTIIIVIIVILLALIAVGLLLY

SEQ ID NO: 235 - protein, 549 aa, synthetic construct
MELLIHRSSAIFLTLAINALYLTSSQNITEEFYQSTCSAVSRGYFSALRTGWYHSVITIELSNIKETKCNGTDTKVKLIKQELDKYKNAVTELQLLMQNTPAANCRARREAPQYMNYTINTTKNLNVSISKKRKRRFLGFLLGVCSAIASGIAVSKVLHLEGEVNKIKNALLSTNKAVVSLSNGVSVLTIKVLDLKNYINNQLLPIVNQQSCRISNIETVIEFQQKNSRLLEITREFSVNAGVTTPLSTYMLTNSELLSLINDMPITNDQKKLMSSNVQIVRQQSYSIMSIIKEEILAYVVQLPIYGVIDTPCWKLHTSPLCTTNIKEGSNICLTRTDRGWYCDNAGSVSFFPQADTCKVQSNRVFCDTMNSLTLPSEVSLCNTDIFNSKYDCKIMTSKTDISSSVITSLGAIVSCYGKTKCTASNKNRGIIKTFSNGCDYVSNKGVDTVSVGNTLYYVNKLEGKNLYVKGEPIINYYDPLVFPSSEFDASISQVNEKINQSLAFIRRSDELLHNVNTGKSTTNIMITAIIIVIIVVLLSLIAIGLLLY

SEQ ID NO: 236 - protein, 549 aa, synthetic construct
MELPILKTNAITTILAAVTLCFASSQNITEEFYQSTCSAVSKGYLSALRTGWYHSVITIELSNIKENKCNGTDAKVKLIKQELDKYKNAVTELQLLMQSTPAANCRARRELPRFMNYTLNNTKNTNVTLSKKRKRRFLGFLLGVGCAIASGIAVSKVLHLEGEVNKIKSALLSTNKAVVSLSNGVSVLTIKVLDLKNYIDKQLLPIVNKQSCSISNIETVIEFQQKNNRLLEITREFSVNAGVTTPVSTYMLTNSELLSLINDMPITNDQKKLMSSNVQIVRQQSYSIMSIIKEEILAYVVQLPLYGVIDTPCWKLHTSPLCTTNTKEGSNICLTRTDRGWYCDNAGSVSFFPQAETCKVQSNRVFCDTMNSLTLPSEVNLCNIDIFNPKYDCKIMTSKTDVSSSVITSLGAIVSCYGKTKCTASNKNRGIIKTFSNGCDYVSNKGVDTVSVGNTLYYVNKQEGKSLYVKGEPIINFYDPLVFPSSEFDASISQVNEKINQSLAFIRKSDELLHNVNAGKSTTNIMITTIIIVIIVILLALIAVGLLLY

SEQ ID NO: 237 - protein, 549 aa, synthetic construct
MELLIHRSSAIFLTLAINALYLTSSQNITEEFYQSTCSAVSRGYFSALRTGWYHSVITIELSNIKETKCNGTDTKVKLIKQELDKYKNAVTELQLLMQNTPAANCRARREAPQYMNYTINTTKNLNVSISKKRKRRFLGFLLGVGCAIASGIAVSKVLHLEGEVNKIKNALLSTNKAVVSLSNGVSVLTIKVLDLKNYINNQLLPIVNQQSCRISNIETVIEFQQKNSRLLEITREFSVNAGVTTPLSTYMLTNSELLSLINDMPITNDQKKLMSSNVQIVRQQSYSIMSIIKEEILAYVVQLPIYGVIDTPCWKLHTSPLCTTNIKEGSNICLTRTDRGWYCDNAGSVSFFPQADTCKVQSNRVFCDTMNSLTLPSEVSLCNTDIFNSKYDCKIMTSKTDISSSVITSLGAIVSCYGKTKCTASNKNRGIIKTFSNGCDYVSNKGVDTVSVGNTLYYVNKLEGKNLYVKGEPIINYYDPLVFPSSEFDASISQVNEKINQSLAFIRRSDELLHNVNTGKSTTNIMITAIIIVIIVVLLSLIAIGLLLY

SEQ ID NO: 238 - protein, 549 aa, synthetic construct
MELPILKTNAITTILAAVTLCFASSQNITEEFYQSTCSAVSKGYLSALRTGWYHSVITIELSNIKENKCNGTDAKVKLIKQELDKYKNAVTELQLLMQSTCAANSRARRELPRFMNYTLNNTKNTNVTLSKKRKRRFLGFLLGVGSAIASGCAVSKVLHLEGEVNKIKSALLSTNKAVVSLSNGVSVLTIKVLDLKNYIDKQLLPIVNKQSCSISNIETVIEFQQKNNRLLEITREFSVNAGVTTPVSTYMLTNSELLSLINDMPITNDQKKLMSSNVQIVRQQSYSIMSIIKEEILAYVVQLPLYGVIDTPCWKLHTSPLCTTNTKEGSNICLTRTDRGWYCDNAGSVSFFPQAETCKVQSNRVFCDTMNSLTLPSEVNLCNIDIFNPKYDCKIMTSKTDVSSSVITSLGAIVSCYGKTKCTASNKNRGIIKTFSNGCDYVSNKGVDTVSVGNTLYYVNKQEGKSLYVKGEPIINFYDPLVFPSSEFDASISQVNEKINQSLAFIRKSDELLHNVNAGKSTTNIMITTIIIVIIVILLALIAVGLLLY

SEQ ID NO: 239 - protein, 549 aa, synthetic construct
MELLIHRSSAIFLTLAINALYLTSSQNITEEFYQSTCSAVSRGYFSALRTGWYHSVITIELSNIKETKCNGTDTKVKLIKQELDKYKNAVTELQLLMQNTCAANNRARREAPQYMNYTINTTKNLNVSISKKRKRRFLGFLLGVGSAIASGCAVSKVLHLEGEVNKIKNALLSTNKAVVSLSNGVSVLTIKVLDLKNYINNQLLPIVNQQSCRISNIETVIEFQQKNSRLLEITREFSVNAGVTTPLSTYMLTNSELLSLINDMPITNDQKKLMSSNVQIVRQQSYSIMSIIKEEILAYVVQLPIYGVIDTPCWKLHTSPLCTTNIKEGSNICLTRTDRGWYCDNAGSVSFFPQADTCKVQSNRVFCDTMNSLTLPSEVSLCNTDIFNSKYDCKIMTSKTDISSSVITSLGAIVSCYGKTKCTASNKNRGIIKTFSNGCDYVSNKGVDTVSVGNTLYYVNKLEGKNLYVKGEPIINYYDPLVFPSSEFDASISQVNEKINQSLAFIRRSDELLHNVNTGKSTTNIMITAIIIVIIVVLLSLIAIGLLLY

SEQ ID NO: 240 - protein, 549 aa, synthetic construct
MELLIHRSSAIFLTLAINALYLTSSQNITEEFYQSTCSAVSRGYFSALRTGWYHSVITIELSNIKETKCNGTDTKVKLIKQELDKYKNAVTELQLLMQNTPACNNRARREAPQYMNYTINTTKNLNVSISKKRKRRFLGFLLGVGCAIASGIAVSKVLHLEGEVNKIKNALLSTNKAVVSLSNGVSVLTIKVLDLKNYINNQLLPIVNQQSCRISNIETVIEFQQKNSRLLEITREFSVNAGVTTPLSTYMLTNSELLSLINDMPITNDQKKLMSSNVQIVRQQSYSIMSIIKEEILAYVVQLPIYGVIDTPCWKLHTSPLCTTNIKEGSNICLTRTDRGWYCDNAGSVSFFPQADTCKVQSNRVFCDTMNSLTLPSEVSLCNTDIFNSKYDCKIMTSKTDISSSVITSLGAIVSCYGKTKCTASNKNRGIIKTFSNGCDYVSNKGVDTVSVGNTLYYVNKLEGKNLYVKGEPIINYYDPLVFPSSEFDASISQVNEKINQSLAFIRRSDELLHNVNTGKSTTNIMITAIIIVIIVVLLSLIAIGLLLY

SEQ ID NO: 241 - protein, 549 aa, synthetic construct
MELPILKTNAITTILAAVTLCFASSQNITEEFYQSTCSAVSKGYLSALRTGWYHSVITIELSNIKENKCNGTDAKVKLIKQELDKYKNAVTELQLLMQSTPACNSRARRELPRFMNYTLNNTKNTNVTLSKKRKRRFLGFLLGVGCAIASGIAVSKVLHLEGEVNKIKSALLSTNKAVVSLSNGVSVLTIKVLDLKNYIDKQLLPIVNKQSCSISNIETVIEFQQKNNRLLEITREFSVNAGVTTPVSTYMLTNSELLSLINDMPITNDQKKLMSSNVQIVRQQSYSIMSIIKEEILAYVVQLPLYGVIDTPCWKLHTSPLCTTNTKEGSNICLTRTDRGWYCDNAGSVSFFPQAETCKVQSNRVFCDTMNSLTLPSEVNLCNIDIFNPKYDCKIMTSKTDVSSSVITSLGAIVSCYGKTKCTASNKNRGIIKTFSNGCDYVSNKGVDTVSVGNTLYYVNKQEGKSLYVKGEPIINFYDPLVFPSSEFDASISQVNEKINQSLAFIRKSDELLHNVNAGKSTTNIMITTIIIVIIVILLALIAVGLLLY

SEQ ID NO: 242 - protein, 549 aa, synthetic construct
MELLIHRSSAIFLTLAINALYLTSSQNITEEFYQSTCSAVSRGYFSALRTGWYHSVITIELSNIKETKCNGTDTKVKLIKQELDKYKNAVTELQLLMQNTPCANNRARREAPQYMNYTINTTKNLNVSISKKRKRRFLGFLLGVGSAIASGICVSKVLHLEGEVNKIKNALLSTNKAVVSLSNGVSVLTIKVLDLKNYINNQLLPIVNQQSCRISNIETVIEFQQKNSRLLEITREFSVNAGVTTPLSTYMLTNSELLSLINDMPITNDQKKLMSSNVQIVRQQSYSIMSIIKEEILAYVVQLPIYGVIDTPCWKLHTSPLCTTNIKEGSNICLTRTDRGWYCDNAGSVSFFPQADTCKVQSNRVFCDTMNSLTLPSEVSLCNTDIFNSKYDCKIMTSKTDISSSVITSLGAIVSCYGKTKCTASNKNRGIIKTFSNGCDYVSNKGVDTVSVGNTLYYVNKLEGKNLYVKGEPIINYYDPLVFPSSEFDASISQVNEKINQSLAFIRRSDELLHNVNTGKSTTNIMITAIIIVIIVVLLSLIAIGLLLY

SEQ ID NO: 243 - protein, 549 aa, synthetic construct
MELLIHRSSAIFLTLAINALYLTSSQNITEEFYQSTCSAVSRGYFSALRTGWYHSVITIELSNIKETKCNGTDTKVKLIKQELDKYKNAVTELQLLMQNTPCANNRARREAPQYMNYTINTTKNLNVSISKKRKRRFLGFLLGVGSAIACGIAVSKVLHLEGEVNKIKNALLSTNKAVVSLSNGVSVLTIKVLDLKNYINNQLLPIVNQQSCRISNIETVIEFQQKNSRLLEITREFSVNAGVTTPLSTYMLTNSELLSLINDMPITNDQKKLMSSNVQIVRQQSYSIMSIIKEEILAYVVQLPIYGVIDTPCWKLHTSPLCTTNIKEGSNICLTRTDRGWYCDNAGSVSFFPQADTCKVQSNRVFCDTMNSLTLPSEVSLCNTDIFNSKYDCKIMTSKTDISSSVITSLGAIVSCYGKTKCTASNKNRGIIKTFSNGCDYVSNKGVDTVSVGNTLYYVNKLEGKNLYVKGEPIINYYDPLVFPSSEFDASISQVNEKINQSLAFIRRSDELLHNVNTGKSTTNIMITAIIIVIIVVLLSLIAIGLLLY

SEQ ID NO: 244 - protein, 549 aa, synthetic construct
MELPILKTNAITTILAAVTLCFASSQNITEEFYQSTCSAVSKGYLSALRTGWYHSVITIELSNIKENKCNGTDAKVKLIKQELDKYKNAVTELQLLMQSTPCANSRARRELPRFMNYTLNNTKNTNVTLSKKRKRRFLGFLLGVGSAIASGICVSKVLHLEGEVNKIKSALLSTNKAVVSLSNGVSVLTIKVLDLKNYIDKQLLPIVNKQSCSISNIETVIEFQQKNNRLLEITREFSVNAGVTTPVSTYMLTNSELLSLINDMPITNDQKKLMSSNVQIVRQQSYSIMSIIKEEILAYVVQLPLYGVIDTPCWKLHTSPLCTTNTKEGSNICLTRTDRGWYCDNAGSVSFFPQAETCKVQSNRVFCDTMNSLTLPSEVNLCNIDIFNPKYDCKIMTSKTDVSSSVITSLGAIVSCYGKTKCTASNKNRGIIKTFSNGCDYVSNKGVDTVSVGNTLYYVNKQEGKSLYVKGEPIINFYDPLVFPSSEFDASISQVNEKINQSLAFIRKSDELLHNVNAGKSTTNIMITTIIIVIIVILLALIAVGLLLY

SEQ ID NO: 245 - protein, 549 aa, synthetic construct
MELPILKTNAITTILAAVTLCFASSQNITEEFYQSTCSAVSKGYLSALRTGWYHSVITIELSNIKENKCNGTDAKVKLIKQELDKYKNAVTELQLLMQSTPCANSRARRELPRFMNYTLNNTKNTNVTLSKKRKRRFLGFLLGVGSAIACGIAVSKVLHLEGEVNKIKSALLSTNKAVVSLSNGVSVLTIKVLDLKNYIDKQLLPIVNKQSCSISNIETVIEFQQKNNRLLEITREFSVNAGVTTPVSTYMLTNSELLSLINDMPITNDQKKLMSSNVQIVRQQSYSIMSIIKEEILAYVVQLPLYGVIDTPCWKLHTSPLCTTNTKEGSNICLTRTDRGWYCDNAGSVSFFPQAETCKVQSNRVFCDTMNSLTLPSEVNLCNIDIFNPKYDCKIMTSKTDVSSSVITSLGAIVSCYGKTKCTASNKNRGIIKTFSNGCDYVSNKGVDTVSVGNTLYYVNKQEGKSLYVKGEPIINFYDPLVFPSSEFDASISQVNEKINQSLAFIRKSDELLHNVNAGKSTTNIMITTIIIVIIVILLALIAVGLLLY

SEQ ID NO: 246 - protein, 549 aa, synthetic construct
MELPILKTNAITTILAAVTLCFASSQNITEEFYQSTCSAVSKGYLSALRTGWYASVITIELSNIKENKCNGTDAKVKLIKQELDKYKNAVTELQLLMQSTPAANSRARRELPRFMNYTLNNTKNTNVTLSKKRKRRFLGFLLGVGSAIASGIAVSKVLHLEGEVNKIKSALLSTNKAVVSLSNGVSVLTSKVLDLKNYIDKQLLPIVNKQSCSISNIETVIEFQQKNNRLLEITREFSVNAGVTTPVSTYMLTNSELLSLINDMPITNDQKKLMSSNVQIVRQQSYSIMSIIKEEVLAYVVQLPLYGVIDTPCWKLHTSPLCTTNTKEGSNICLTRTDRGWYCDNAGSVSFFPQAETCKVQSNRVFCDTMNSLTLPSEVNLCNIDIFNPKYDCKIMTSKTDVSSSVITSLGAIVSCYGKTKCTASNKNRGIIKTFSNGCDYVSNKGVDTVSVGNTLYYVNKQEGKSLYVKGEPIINFYDPLVFPSDEFDASISQVNEKINQSLAFIRKSDELLHNVNAGKSTTNIMITTIIIVIIVILLALIAVGLLLY

SEQ ID NO: 247 - protein, 549 aa, synthetic construct
MELPILKTNAITTILAAVTLCFASSQNITEEFYQSTCSAVSKGYLSALRTGWYTSVITIELSNIKENKCNGTDAKVKLIKQELDKYKNAVTELQLLMQSTCAANSRARRELPRFMNYTLNNTKNTNVTLSKKRKRRFLGFLLGVGSAIASGCAVSKVLHLEGEVNKIKSALLSTNKAVVSLSNGVSVLTSKVLDLKNYIDKQLLPIVNKQSCSISNIETVIEFQQKNNRLLEITREFSVNAGVTTPVSTYMLTNSELLSLINDMPITNDQKKLMSSNVQIVRQQSYSIMSIIKEEVLAYVVQLPLYGVIDTPCWKLHTSPLCTTNTKEGSNICLTRTDRGWYCDNAGSVSFFPQAETCKVQSNRVFCDTMNSLTLPSEVNLCNIDIFNPKYDCKIMTSKTDVSSSVITSLGAIVSCYGKTKCTASNKNRGIIKTFSNGCDYVSNKGVDTVSVGNTLYYVNKQEGKSLYVKGEPIINFYDPLVFPSDEFDASISQVNEKINQSLAFIRKSDELLHNVNAGKSTTNIMITTIIIVIIVILLALIAVGLLLY

SEQ ID NO: 248 - protein, 549 aa, synthetic construct
MELPILKTNAITTILAAVTLCFASSQNITEEFYQSTCSAVSKGYLSALRTGWYTSVITIELSNIKENKCNGTDAKVKLIKQELDKYKNAVTELQLLMQSTPACNSRARRELPRFMNYTLNNTKNTNVTLSKKRKRRFLGFLLGVGSACASGIAVSKVLHLEGEVNKIKSALLSTNKAVVSLSNGVSVLTSKVLDLKNYIDKQLLPIVNKQSCSISNIETVIEFQQKNNRLLEITREFSVNAGVTTPVSTYMLTNSELLSLINDMPITNDQKKLMSSNVQIVRQQSYSIMSIIKEEVLAYVVQLPLYGVIDTPCWKLHTSPLCTTNTKEGSNICLTRTDRGWYCDNAGSVSFFPQAETCKVQSNRVFCDTMNSLTLPSEVNLCNIDIFNPKYDCKIMTSKTDVSSSVITSLGAIVSCYGKTKCTASNKNRGIIKTFSNGCDYVSNKGVDTVSVGNTLYYVNKQEGKSLYVKGEPIINFYDPLVFPSDEFDASISQVNEKINQSLAFIRKSDELLHNVNAGKSTTNIMITTIIIVIIVILLALIAVGLLLY

SEQ ID NO: 249 - protein, 549 aa, synthetic construct
MELPILKTNAITTILAAVTLCFASSQNITEEFYQSTCSAVSKGYLSALRTGWYTSVITIELSNIKENKCNGTDAKVKLIKQELDKYKNAVTELQLLMQSTPAANSRARRELPRFMNYTLNNTKNTNVTLSKKRKRRFLGFLLGVGSAIASGIAVSKVLHLEGEVNKIKSALLSTNKAVVSLSNGVSVLTMKVLDLKNYIDKQLLPIVNKQSCSISNIETVIEFQQKNNRLLEITREFSVNAGVTTPVSTYMLTNSELLSLINDMPITNDQKKLMSSNVQIVRQQSYSIMSIIKEEVLAYVVQLPLYGVIDTPCWKLHTSPLCTTNTKEGSNICLTRTDRGWYCDNAGSVSFFPQAETCKVQSNRVFCDTMNSLTLPSEVNLCNIDIFNPKYDCKIMTSKTDVSSSVITSLGAIVSCYGKTKCTASNKNRGIIKTFSNGCDYVSNKGVDTVSVGNTLYYVNKQEGKSLYVKGEPIINFYDPLVFPSDEFDASISQVNEKINQSLAFIRKSDELLHNVNAGKSTTNIMITTIIIVIIVILLALIAVGLLLY

SEQ ID NO: 250 - protein, 549 aa, synthetic construct
MELPILKTNAITTILAAVTLCFASSQNITEEFYQSTCSAVSKGYLSALRTGWYTSVITIELSNIKENKCNGTDAKVKLIKQELDKYKNAVTELQLLMQSTPAANSRARRELPRFMNYTLNNTKNTNVTLSKKRKRRFLGFLLGVGSAIASGIAVSKVLHLEGEVNKIKSALLSTNKAVVSLSNGVSVLTIKVLDLKNYIDKQLLPIVNKQSCSISNIETVIEFQQKNNRLLEITREFSVNAGVTTPVSTYMLTNSELLSLINDMPITNDQKKLMSSNVQIVRQQSYSIMSIIKEEVLAYVVQLPLYGVIDTPCWKLHTSPLCTTNTKEGSNICLTRTDRGWYCDNAGSVSFFPQAETCKVQSNRVFCDTMNSLTLPSEVNLCNIDIFNPKYDCKIMTSKTDVSSSVITSLGAIVSCYGKTKCTASNKNRGIIKTFSNGCDYVSNKGVDTVSVGNTLYYVNKQEGKSLYVKGEPIINFYDPLVFPSDEFDASISQVNEKINQSLAFIRKSDELLHNVNAGKSTTNIMITTIIIVIIVILLALIAVGLLLY

SEQ ID NO: 251 - protein, 549 aa, synthetic construct
MELPILKTNAITTILAAVTLCFASSQNITEEFYQSTCSAVSKGYLSALRTGWYTSVITIELSNIKENKCNGTDAKVKLIKQELDKYKNAVTELQLLMQSTPAANSRARRELPRFMNYTLNNTKNTNVTLSKKRKRRFLGFLLGVGSAIASGIAVSKVLHLEGEVNKIKSALLSTNKAVVSLSNGVSVLTSKVLDLKNYIDKQLLPIVNKQSCSISNIETVIEFQQKNNRLLEITREFSVNAGVTTPVSTYMLTNSELLSLINDMPITNDQKKLMSSNVQIVRQQSYSIMSIIKEELLAYVVQLPLYGVIDTPCWKLHTSPLCTTNTKEGSNICLTRTDRGWYCDNAGSVSFFPQAETCKVQSNRVFCDTMNSLTLPSEVNLCNIDIFNPKYDCKIMTSKTDVSSSVITSLGAIVSCYGKTKCTASNKNRGIIKTFSNGCDYVSNKGVDTVSVGNTLYYVNKQEGKSLYVKGEPIINFYDPLVFPSDEFDASISQVNEKINQSLAFIRKSDELLHNVNAGKSTTNIMITTIIIVIIVILLALIAVGLLLY

SEQ ID NO: 252 - protein, 549 aa, synthetic construct
MELPILKTNAITTILAAVTLCFASSQNITEEFYQSTCSAVSKGYLSALRTGWYASVITIELSNIKENKCNGTDAKVKLIKQELDKYKNAVTELQLLMQSTPAANSRARRELPRFMNYTLNNTKNTNVTLSKKRKRRFLGFLLGVGSAIASGIAVSKVLHLEGEVNKIKSALLSTNKAVVSLSNGVSVLTMKVLDLKNYIDKQLLPIVNKQSCSISNIETVIEFQQKNNRLLEITREFSVNAGVTTPVSTYMLTNSELLSLINDMPITNDQKKLMSSNVQIVRQQSYSIMSIIKEEVLAYVVQLPLYGVIDTPCWKLHTSPLCTTNTKEGSNICLTRTDRGWYCDNAGSVSFFPQAETCKVQSNRVFCDTMNSLTLPSEVNLCNIDIFNPKYDCKIMTSKTDVSSSVITSLGAIVSCYGKTKCTASNKNRGIIKTFSNGCDYVSNKGVDTVSVGNTLYYVNKQEGKSLYVKGEPIINFYDPLVFPSDEFDASISQVNEKINQSLAFIRKSDELLHNVNAGKSTTNIMITTIIIVIIVILLALIAVGLLLY

SEQ ID NO: 253 - protein, 549 aa, synthetic construct
MELPILKTNAITTILAAVTLCFASSQNITEEFYQSTCSAVSKGYLSALRTGWYASVITIELSNIKENKCNGTDAKVKLIKQELDKYKNAVTELQLLMQSTPAANSRARRELPRFMNYTLNNTKNTNVTLSKKRKRRFLGFLLGVGSAIASGIAVSKVLHLEGEVNKIKSALLSTNKAVVSLSNGVSVLTSKVLDLKNYIDKQLLPIVNKQSCSISNIETVIEFQQKNNRLLEITREFSVNAGVTTPVSTYMLTNSELLSLINDMPITNDQKKLMSSNVQIVRQQSYSIMSIIKEELLAYVVQLPLYGVIDTPCWKLHTSPLCTTNTKEGSNICLTRTDRGWYCDNAGSVSFFPQAETCKVQSNRVFCDTMNSLTLPSEVNLCNIDIFNPKYDCKIMTSKTDVSSSVITSLGAIVSCYGKTKCTASNKNRGIIKTFSNGCDYVSNKGVDTVSVGNTLYYVNKQEGKSLYVKGEPIINFYDPLVFPSDEFDASISQVNEKINQSLAFIRKSDELLHNVNAGKSTTNIMITTIIIVIIVILLALIAVGLLLY

SEQ ID NO: 254 - protein, 549 aa, synthetic construct
MELPILKTNAITTILAAVTLCFASSQNITEEFYQSTCSAVSKGYLSALRTGWYTSVITIELSNIKENKCNGTDAKVKLIKQELDKYKNAVTELQLLMQSTPAANSRARRELPRFMNYTLNNTKNTNVTLSKKRKRRFLGFLLGVGSAIASGIAVSKVLHLEGEVNKIKSALLSTNKAVVSLSNGVSVLTMKVLDLKNYIDKQLLPIVNKQSCSISNIETVIEFQQKNNRLLEITREFSVNAGVTTPVSTYMLTNSELLSLINDMPITNDQKKLMSSNVQIVRQQSYSIMSIIKEELLAYVVQLPLYGVIDTPCWKLHTSPLCTTNTKEGSNICLTRTDRGWYCDNAGSVSFFPQAETCKVQSNRVFCDTMNSLTLPSEVNLCNIDIFNPKYDCKIMTSKTDVSSSVITSLGAIVSCYGKTKCTASNKNRGIIKTFSNGCDYVSNKGVDTVSVGNTLYYVNKQEGKSLYVKGEPIINFYDPLVFPSDEFDASISQVNEKINQSLAFIRKSDELLHNVNAGKSTTNIMITTIIIVIIVILLALIAVGLLLY

SEQ ID NO: 255 - protein, 549 aa, synthetic construct
MELPILKTNAITTILAAVTLCFASSQNITEEFYQSTCSAVSKGYLSALRTGWYASVITIELSNIKENKCNGTDAKVKLIKQELDKYKNAVTELQLLMQSTPAANSRARRELPRFMNYTLNNTKNTNVTLSKKRKRRFLGFLLGVGSAIASGIAVSKVLHLEGEVNKIKSALLSTNKAVVSLSNGVSVLTMKVLDLKNYIDKQLLPIVNKQSCSISNIETVIEFQQKNNRLLEITREFSVNAGVTTPVSTYMLTNSELLSLINDMPITNDQKKLMSSNVQIVRQQSYSIMSIIKEELLAYVVQLPLYGVIDTPCWKLHTSPLCTTNTKEGSNICLTRTDRGWYCDNAGSVSFFPQAETCKVQSNRVFCDTMNSLTLPSEVNLCNIDIFNPKYDCKIMTSKTDVSSSVITSLGAIVSCYGKTKCTASNKNRGIIKTFSNGCDYVSNKGVDTVSVGNTLYYVNKQEGKSLYVKGEPIINFYDPLVFPSDEFDASISQVNEKINQSLAFIRKSDELLHNVNAGKSTTNIMITTIIIVIIVILLALIAVGLLLY

SEQ ID NO: 256 - protein, 549 aa, synthetic construct
MELPILKTNAITTILAAVTLCFASSQNITEEFYQSTCSAVSKGYLSALRTGWYTSVITIELSNIKENKCNGTDAKVKLIKQELDKYKNAVTELQLLMQSTPCANSRARRELPRFMNYTLNNTKNTNVTLSKKRKRRFLGFLLGVGSAIASGCAVSKVLHLEGEVNKIKSALLSTNKAVVSLSNGVSVLTSKVLDLKNYIDKQLLPIVNKQSCSISNIETVIEFQQKNNRLLEITREFSVNAGVTTPVSTYMLTNSELLSLINDMPITNDQKKLMSSNVQIVRQQSYSIMSIIKEEVLAYVVQLPLYGVIDTPCWKLHTSPLCTTNTKEGSNICLTRTDRGWYCDNAGSVSFFPQAETCKVQSNRVFCDTMNSLTLPSEVNLCNIDIFNPKYDCKIMTSKTDVSSSVITSLGAIVSCYGKTKCTASNKNRGIIKTFSNGCDYVSNKGVDTVSVGNTLYYVNKQEGKSLYVKGEPIINFYDPLVFPSDEFDASISQVNEKINQSLAFIRKSDELLHNVNAGKSTTNIMITTIIIVIIVILLALIAVGLLLY

SEQ ID NO: 257 - protein, 549 aa, synthetic construct
MELPILKTNAITTILAAVTLCFASSQNITEEFYQSTCSAVSKGYLSALRTGWYTSVITIELSNIKENKCNGTDAKVKLIKQELDKYKNAVTELQLLMQSTPCANSRARRELPRFMNYTLNNTKNTNVTLSKKRKRRFLGFLLGVGSAIASGICVSKVLHLEGEVNKIKSALLSTNKAVVSLSNGVSVLTSKVLDLKNYIDKQLLPIVNKQSCSISNIETVIEFQQKNNRLLEITREFSVNAGVTTPVSTYMLTNSELLSLINDMPITNDQKKLMSSNVQIVRQQSYSIMSIIKEEVLAYVVQLPLYGVIDTPCWKLHTSPLCTTNTKEGSNICLTRTDRGWYCDNAGSVSFFPQAETCKVQSNRVFCDTMNSLTLPSEVNLCNIDIFNPKYDCKIMTSKTDVSSSVITSLGAIVSCYGKTKCTASNKNRGIIKTFSNGCDYVSNKGVDTVSVGNTLYYVNKQEGKSLYVKGEPIINFYDPLVFPSDEFDASISQVNEKINQSLAFIRKSDELLHNVNAGKSTTNIMITTIIIVIIVILLALIAVGLLLY

SEQ ID NO: 258 - protein, 549 aa, synthetic construct
MELPILKTNAITTILAAVTLCFASSQNITEEFYQSTCSAVSKGYLSALRTGWYTSVITIELSNIKENKCNGTDAKVKLIKQELDKYKNAVTELQLLMQSTPCANSRARRELPRFMNYTLNNTKNTNVTLSKKRKRRFLGFLLGVGSAIACGIAVSKVLHLEGEVNKIKSALLSTNKAVVSLSNGVSVLTSKVLDLKNYIDKQLLPIVNKQSCSISNIETVIEFQQKNNRLLEITREFSVNAGVTTPVSTYMLTNSELLSLINDMPITNDQKKLMSSNVQIVRQQSYSIMSIIKEEVLAYVVQLPLYGVIDTPCWKLHTSPLCTTNTKEGSNICLTRTDRGWYCDNAGSVSFFPQAETCKVQSNRVFCDTMNSLTLPSEVNLCNIDIFNPKYDCKIMTSKTDVSSSVITSLGAIVSCYGKTKCTASNKNRGIIKTFSNGCDYVSNKGVDTVSVGNTLYYVNKQEGKSLYVKGEPIINFYDPLVFPSDEFDASISQVNEKINQSLAFIRKSDELLHNVNAGKSTTNIMITTIIIVIIVILLALIAVGLLLY

SEQ ID NO: 259 - DNA, 1653 bp, synthetic construct
  source 1..1653: mol_type = other DNA
atggaactgcccatcctgaaaacaaacgccatcaccaccatcctggccgccgtgacactgtgttttgccagcagccagaacatcaccgaagagttctaccagagcacctgtagcgccgtgtctaagggctatctgtctgccctgagaaccggctggtatcacagcgtgatcaccatcgagctgagcaacatcaaagaaaacaagtgcaacggcaccgacgccaaagtgaagctgatcaagcaagagctggacaagtacaagaacgccgtgaccgaactgcagctgctgatgcagtctaccccttgcgccaatagcagagccagacgggaactgcctagattcatgaactacaccctgaacaacaccaagaacaccaacgtgaccctgagcaagaagcggaagcggagattcctgggctttctgctcggagtgggaagcgcctgcgcctctggaattgccgtgtccaaggtgctgcatctggaaggcgaagtgaacaagatcaagagcgccctgctgagcaccaacaaggccgtggtttctctgagcaatggcgtgtccgtgctgaccatcaaggtgctggacctgaagaactacatcgacaaacagctgctgcccatcgtcaacaagcagagctgcagcatcagcaacatcgagacagtgatcgagttccagcagaagaacaaccggctgctggaaatcacccgcgagttttctgtgaatgccggcgtgaccacacctgtgtccacctacatgctgaccaacagcgagctgctgtccctgatcaacgacatgcccatcaccaacgaccagaaaaagctgatgagcagcaacgtgcagatcgtgcggcagcagagctactccatcatgagcattatcaaagaagagatcctggcctacgtggtgcagctgcctctgtatggcgtgatcgataccccttgctggaagctgcacacaagccctctgtgcaccaccaacaccaaagagggctccaacatctgcctgaccagaaccgatagaggctggtactgcgataatgccggcagcgtcagcttcttcccacaagccgagacatgcaaggtgcagagcaacagagtgttctgcgataccatgaacagcctgacactgccctccgaagtgaatctgtgcaatatcgacatcttcaacccgaagtacgactgcaagatcatgaccagcaagaccgacgtgtcaagctccgtgatcacatctctgggcgccatcgtgtcctgctacggcaagacaaagtgcaccgccagcaacaagaaccggggcatcatcaagaccttcagcaacggctgcgactacgtgtccaacaaaggcgtggacaccgtgtctgtgggcaacaccctgtactacgtgaacaagcaagaaggcaagagcctgtacgtgaagggcgagcccatcatcaacttctacgaccctctggtgttccccagcagcgagtttgatgccagcatctcccaagtgaacgagaagatcaaccagagcctggccttcatcagaaagtccgatgagctgctgcacaacgtgaacgccggcaagtccaccaccaatatcatgatcaccacgatcatcatcgtgatcatcgtcatcctgctggctctgatcgctgtgggcctgctgctgtattgatga

SEQ ID NO: 260 - DNA, 1653 bp, synthetic construct
  source 1..1653: mol_type = other DNA
atggaactgctgattcacagaagcagcgccatctttctgaccctggccatcaatgccctgtacctgaccagcagccagaacatcaccgaagagttctaccagagcacctgtagcgccgtgtccagaggctacttttctgccctgagaaccggctggtatcacagcgtgatcaccatcgagctgagcaacatcaaagaaacaaagtgcaacggcaccgacaccaaagtgaagctgatcaagcaagagctggacaagtacaagaacgccgtgaccgaactgcagctgctgatgcagaataccccttgcgccaacaaccgggccagaagagaagcccctcagtacatgaactacaccatcaacaccaccaagaacctgaacgtgtccatcagcaagaagcggaagcggagattcctgggctttctgctcggagtgggaagcgcctgcgcctctggaattgccgtgtctaaggtgctgcacctggaaggcgaagtgaacaagatcaagaatgccctgctgagcaccaacaaggccgtggtgtctctgtctaatggcgtgtccgtgctgaccatcaaggtgctggacctgaagaactacatcaacaaccagctgctgcccatcgtgaaccagcagagctgccggatcagcaacatcgagacagtgatcgagttccagcagaagaacagcagactgctggaaatcacccgcgagttttccgtgaatgccggcgtgacaacacccctgagcacctacatgctgaccaacagcgagctgctgtccctgatcaacgacatgcccatcaccaacgaccagaaaaagctgatgagcagcaacgtgcagatcgtgcggcagcagtcctacagcatcatgagcattatcaaagaagagatcctggcctacgtggtgcagctgcctatctacggcgtgatcgataccccttgctggaagctgcacacaagccctctgtgcaccaccaatatcaaagagggctccaacatctgcctgaccagaaccgatagaggctggtactgcgataatgccggcagcgtcagcttcttcccacaagccgatacctgcaaggtgcagagcaacagagtgttctgcgataccatgaacagcctgacactgcccagcgaggtgtccctgtgcaacaccgacatcttcaactctaagtacgactgcaagatcatgacctccaagaccgacatcagctcctccgtgatcacatctctgggcgccatcgtgtcctgctacggcaagacaaagtgtaccgccagcaacaagaaccggggcatcatcaagaccttcagcaacggctgcgactacgtgtccaacaaaggcgtggacaccgtgtctgtgggcaacaccctgtactacgtgaacaagctggaaggcaagaatctgtacgtgaagggcgagcccatcatcaactactacgaccctctggtgttccccagcagcgagtttgatgccagcatcagccaagtgaacgagaagatcaaccagagcctggccttcatccgcagatccgatgaactgctgcacaatgtgaacaccggcaagagcaccacaaacatcatgatcaccgccatcatcatcgtgatcatcgtcgtgctgctgagcctgatcgctatcggcctgctgctgtactgatga

SEQ ID NO: 261 - DNA, 1653 bp, synthetic construct
  source 1..1653: mol_type = other DNA
atggaactgcccatcctgaaaacaaacgccatcaccaccatcctggccgccgtgacactgtgttttgccagcagccagaacatcaccgaagagttctaccagagcacctgtagcgccgtgtctaagggctatctgtctgccctgagaaccggctggtatcacagcgtgatcaccatcgagctgagcaacatcaaagaaaacaagtgcaacggcaccgacgccaaagtgaagctgatcaagcaagagctggacaagtacaagaacgccgtgaccgaactgcagctgctgatgcagtctaccccttgcgccaatagcagagccagacgggaactgcctagattcatgaactacaccctgaacaacaccaagaacaccaacgtgaccctgagcaagaagcggaagcggagattcctgggctttctgctcggagtgggaagcgccattgcctctggatgcgccgtgtccaaggtgctgcatctggaaggcgaagtgaacaagatcaagagcgccctgctgagcaccaacaaggccgtggtttctctgagcaatggcgtgtccgtgctgaccatcaaggtgctggacctgaagaactacatcgacaaacagctgctgcccatcgtcaacaagcagagctgcagcatcagcaacatcgagacagtgatcgagttccagcagaagaacaaccggctgctggaaatcacccgcgagttttctgtgaatgccggcgtgaccacacctgtgtccacctacatgctgaccaacagcgagctgctgtccctgatcaacgacatgcccatcaccaacgaccagaaaaagctgatgagcagcaacgtgcagatcgtgcggcagcagagctactccatcatgagcattatcaaagaagagatcctggcctacgtggtgcagctgcctctgtatggcgtgatcgataccccttgctggaagctgcacacaagccctctgtgcaccaccaacaccaaagagggctccaacatctgcctgaccagaaccgatagaggctggtactgcgataatgccggcagcgtcagcttcttcccacaagccgagacatgcaaggtgcagagcaacagagtgttctgcgataccatgaacagcctgacactgccctccgaagtgaatctgtgcaatatcgacatcttcaacccgaagtacgactgcaagatcatgaccagcaagaccgacgtgtcaagctccgtgatcacatctctgggcgccatcgtgtcctgctacggcaagacaaagtgcaccgccagcaacaagaaccggggcatcatcaagaccttcagcaacggctgcgactacgtgtccaacaaaggcgtggacaccgtgtctgtgggcaacaccctgtactacgtgaacaagcaagaaggcaagagcctgtacgtgaagggcgagcccatcatcaacttctacgaccctctggtgttccccagcagcgagtttgatgccagcatctcccaagtgaacgagaagatcaaccagagcctggccttcatcagaaagtccgatgagctgctgcacaacgtgaacgccggcaagtccaccaccaatatcatgatcaccacgatcatcatcgtgatcatcgtcatcctgctggctctgatcgctgtgggcctgctgctgtattgatga

SEQ ID NO: 262 - DNA, 1653 bp, synthetic construct
  source 1..1653: mol_type = other DNA
atggaactgctgattcacagaagcagcgccatctttctgaccctggccatcaatgccctgtacctgaccagcagccagaacatcaccgaagagttctaccagagcacctgtagcgccgtgtccagaggctacttttctgccctgagaaccggctggtatcacagcgtgatcaccatcgagctgagcaacatcaaagaaacaaagtgcaacggcaccgacaccaaagtgaagctgatcaagcaagagctggacaagtacaagaacgccgtgaccgaactgcagctgctgatgcagaataccccttgcgccaacaaccgggccagaagagaagcccctcagtacatgaactacaccatcaacaccaccaagaacctgaacgtgtccatcagcaagaagcggaagcggagattcctgggctttctgctcggagtgggaagcgccattgcctctggatgcgccgtgtctaaggtgctgcacctggaaggcgaagtgaacaagatcaagaatgccctgctgagcaccaacaaggccgtggtgtctctgtctaatggcgtgtccgtgctgaccatcaaggtgctggacctgaagaactacatcaacaaccagctgctgcccatcgtgaaccagcagagctgccggatcagcaacatcgagacagtgatcgagttccagcagaagaacagcagactgctggaaatcacccgcgagttttccgtgaatgccggcgtgacaacacccctgagcacctacatgctgaccaacagcgagctgctgtccctgatcaacgacatgcccatcaccaacgaccagaaaaagctgatgagcagcaacgtgcagatcgtgcggcagcagtcctacagcatcatgagcattatcaaagaagagatcctggcctacgtggtgcagctgcctatctacggcgtgatcgataccccttgctggaagctgcacacaagccctctgtgcaccaccaatatcaaagagggctccaacatctgcctgaccagaaccgatagaggctggtactgcgataatgccggcagcgtcagcttcttcccacaagccgatacctgcaaggtgcagagcaacagagtgttctgcgataccatgaacagcctgacactgcccagcgaggtgtccctgtgcaacaccgacatcttcaactctaagtacgactgcaagatcatgacctccaagaccgacatcagctcctccgtgatcacatctctgggcgccatcgtgtcctgctacggcaagacaaagtgtaccgccagcaacaagaaccggggcatcatcaagaccttcagcaacggctgcgactacgtgtccaacaaaggcgtggacaccgtgtctgtgggcaacaccctgtactacgtgaacaagctggaaggcaagaatctgtacgtgaagggcgagcccatcatcaactactacgaccctctggtgttccccagcagcgagtttgatgccagcatcagccaagtgaacgagaagatcaaccagagcctggccttcatccgcagatccgatgaactgctgcacaatgtgaacaccggcaagagcaccacaaacatcatgatcaccgccatcatcatcgtgatcatcgtcgtgctgctgagcctgatcgctatcggcctgctgctgtactgatga

SEQ ID NO: 263 - DNA, 1653 bp, synthetic construct
  source 1..1653: mol_type = other DNA
atggaactgcccatcctgaaaacaaacgccatcaccaccatcctggccgccgtgacactgtgttttgccagcagccagaacatcaccgaagagttctaccagagcacctgtagcgccgtgtctaagggctatctgtctgccctgagaaccggctggtatcacagcgtgatcaccatcgagctgagcaacatcaaagaaaacaagtgcaacggcaccgacgccaaagtgaagctgatcaagcaagagctggacaagtacaagaacgccgtgaccgaactgcagctgctgatgcagtctacccctgccgcctgcagcagagccagacgggaactgcctagattcatgaactacaccctgaacaacaccaagaacaccaacgtgaccctgagcaagaagcggaagcggagattcctgggctttctgctcggagtgtgcagcgccattgcctctggaattgccgtgtccaaggtgctgcatctggaaggcgaagtgaacaagatcaagagcgccctgctgagcaccaacaaggccgtggtttctctgagcaatggcgtgtccgtgctgaccatcaaggtgctggacctgaagaactacatcgacaaacagctgctgcccatcgtcaacaagcagagctgcagcatcagcaacatcgagacagtgatcgagttccagcagaagaacaaccggctgctggaaatcacccgcgagttttctgtgaatgccggcgtgaccacacctgtgtccacctacatgctgaccaacagcgagctgctgtccctgatcaacgacatgcccatcaccaacgaccagaaaaagctgatgagcagcaacgtgcagatcgtgcggcagcagagctactccatcatgagcattatcaaagaagagatcctggcctacgtggtgcagctgcctctgtatggcgtgatcgataccccttgctggaagctgcacacaagccctctgtgcaccaccaacaccaaagagggctccaacatctgcctgaccagaaccgatagaggctggtactgcgataatgccggcagcgtcagcttcttcccacaagccgagacatgcaaggtgcagagcaacagagtgttctgcgataccatgaacagcctgacactgccctccgaagtgaatctgtgcaatatcgacatcttcaacccgaagtacgactgcaagatcatgaccagcaagaccgacgtgtcaagctccgtgatcacatctctgggcgccatcgtgtcctgctacggcaagacaaagtgcaccgccagcaacaagaaccggggcatcatcaagaccttcagcaacggctgcgactacgtgtccaacaaaggcgtggacaccgtgtctgtgggcaacaccctgtactacgtgaacaagcaagaaggcaagagcctgtacgtgaagggcgagcccatcatcaacttctacgaccctctggtgttccccagcagcgagtttgatgccagcatctcccaagtgaacgagaagatcaaccagagcctggccttcatcagaaagtccgatgagctgctgcacaacgtgaacgccggcaagtccaccaccaatatcatgatcaccacgatcatcatcgtgatcatcgtcatcctgctggctctgatcgctgtgggcctgctgctgtattgatga

SEQ ID NO: 264 - DNA, 1653 bp, synthetic construct
  source 1..1653: mol_type = other DNA
atggaactgctgattcacagaagcagcgccatctttctgaccctggccatcaatgccctgtacctgaccagcagccagaacatcaccgaagagttctaccagagcacctgtagcgccgtgtccagaggctacttttctgccctgagaaccggctggtatcacagcgtgatcaccatcgagctgagcaacatcaaagaaacaaagtgcaacggcaccgacaccaaagtgaagctgatcaagcaagagctggacaagtacaagaacgccgtgaccgaactgcagctgctgatgcagaatacccctgccgcctgcaaccgggccagaagagaagcccctcagtacatgaactacaccatcaacaccaccaagaacctgaacgtgtccatcagcaagaagcggaagcggagattcctgggctttctgctcggagtgtgcagcgccattgcctctggaattgccgtgtctaaggtgctgcacctggaaggcgaagtgaacaagatcaagaatgccctgctgagcaccaacaaggccgtggtgtctctgtctaatggcgtgtccgtgctgaccatcaaggtgctggacctgaagaactacatcaacaaccagctgctgcccatcgtgaaccagcagagctgccggatcagcaacatcgagacagtgatcgagttccagcagaagaacagcagactgctggaaatcacccgcgagttttccgtgaatgccggcgtgacaacacccctgagcacctacatgctgaccaacagcgagctgctgtccctgatcaacgacatgcccatcaccaacgaccagaaaaagctgatgagcagcaacgtgcagatcgtgcggcagcagtcctacagcatcatgagcattatcaaagaagagatcctggcctacgtggtgcagctgcctatctacggcgtgatcgataccccttgctggaagctgcacacaagccctctgtgcaccaccaatatcaaagagggctccaacatctgcctgaccagaaccgatagaggctggtactgcgataatgccggcagcgtcagcttcttcccacaagccgatacctgcaaggtgcagagcaacagagtgttctgcgataccatgaacagcctgacactgcccagcgaggtgtccctgtgcaacaccgacatcttcaactctaagtacgactgcaagatcatgacctccaagaccgacatcagctcctccgtgatcacatctctgggcgccatcgtgtcctgctacggcaagacaaagtgtaccgccagcaacaagaaccggggcatcatcaagaccttcagcaacggctgcgactacgtgtccaacaaaggcgtggacaccgtgtctgtgggcaacaccctgtactacgtgaacaagctggaaggcaagaatctgtacgtgaagggcgagcccatcatcaactactacgaccctctggtgttccccagcagcgagtttgatgccagcatcagccaagtgaacgagaagatcaaccagagcctggccttcatccgcagatccgatgaactgctgcacaatgtgaacaccggcaagagcaccacaaacatcatgatcaccgccatcatcatcgtgatcatcgtcgtgctgctgagcctgatcgctatcggcctgctgctgtactgatga

SEQ ID NO: 265 - DNA, 1653 bp, synthetic construct
  source 1..1653: mol_type = other DNA
atggaactgcccatcctgaaaacaaacgccatcaccaccatcctggccgccgtgacactgtgttttgccagcagccagaacatcaccgaagagttctaccagagcacctgtagcgccgtgtctaagggctatctgtctgccctgagaaccggctggtatcacagcgtgatcaccatcgagctgagcaacatcaaagaaaacaagtgcaacggcaccgacgccaaagtgaagctgatcaagcaagagctggacaagtacaagaacgccgtgaccgaactgcagctgctgatgcagtctacccctgccgcctgcagcagagccagacgggaactgcctagattcatgaactacaccctgaacaacaccaagaacaccaacgtgaccctgagcaagaagcggaagcggagattcctgggctttctgctcggagtgggatgcgccattgcctctggaattgccgtgtccaaggtgctgcatctggaaggcgaagtgaacaagatcaagagcgccctgctgagcaccaacaaggccgtggtttctctgagcaatggcgtgtccgtgctgaccatcaaggtgctggacctgaagaactacatcgacaaacagctgctgcccatcgtcaacaagcagagctgcagcatcagcaacatcgagacagtgatcgagttccagcagaagaacaaccggctgctggaaatcacccgcgagttttctgtgaatgccggcgtgaccacacctgtgtccacctacatgctgaccaacagcgagctgctgtccctgatcaacgacatgcccatcaccaacgaccagaaaaagctgatgagcagcaacgtgcagatcgtgcggcagcagagctactccatcatgagcattatcaaagaagagatcctggcctacgtggtgcagctgcctctgtatggcgtgatcgataccccttgctggaagctgcacacaagccctctgtgcaccaccaacaccaaagagggctccaacatctgcctgaccagaaccgatagaggctggtactgcgataatgccggcagcgtcagcttcttcccacaagccgagacatgcaaggtgcagagcaacagagtgttctgcgataccatgaacagcctgacactgccctccgaagtgaatctgtgcaatatcgacatcttcaacccgaagtacgactgcaagatcatgaccagcaagaccgacgtgtcaagctccgtgatcacatctctgggcgccatcgtgtcctgctacggcaagacaaagtgcaccgccagcaacaagaaccggggcatcatcaagaccttcagcaacggctgcgactacgtgtccaacaaaggcgtggacaccgtgtctgtgggcaacaccctgtactacgtgaacaagcaagaaggcaagagcctgtacgtgaagggcgagcccatcatcaacttctacgaccctctggtgttccccagcagcgagtttgatgccagcatctcccaagtgaacgagaagatcaaccagagcctggccttcatcagaaagtccgatgagctgctgcacaacgtgaacgccggcaagtccaccaccaatatcatgatcaccacgatcatcatcgtgatcatcgtcatcctgctggctctgatcgctgtgggcctgctgctgtattgatga

SEQ ID NO: 266 - DNA, 1653 bp, synthetic construct
  source 1..1653: mol_type = other DNA
atggaactgctgattcacagaagcagcgccatctttctgaccctggccatcaatgccctgtacctgaccagcagccagaacatcaccgaagagttctaccagagcacctgtagcgccgtgtccagaggctacttttctgccctgagaaccggctggtatcacagcgtgatcaccatcgagctgagcaacatcaaagaaacaaagtgcaacggcaccgacaccaaagtgaagctgatcaagcaagagctggacaagtacaagaacgccgtgaccgaactgcagctgctgatgcagaatacccctgccgcctgcaaccgggccagaagagaagcccctcagtacatgaactacaccatcaacaccaccaagaacctgaacgtgtccatcagcaagaagcggaagcggagattcctgggctttctgctcggagtgggatgcgccattgcctctggaattgccgtgtctaaggtgctgcacctggaaggcgaagtgaacaagatcaagaatgccctgctgagcaccaacaaggccgtggtgtctctgtctaatggcgtgtccgtgctgaccatcaaggtgctggacctgaagaactacatcaacaaccagctgctgcccatcgtgaaccagcagagctgccggatcagcaacatcgagacagtgatcgagttccagcagaagaacagcagactgctggaaatcacccgcgagttttccgtgaatgccggcgtgacaacacccctgagcacctacatgctgaccaacagcgagctgctgtccctgatcaacgacatgcccatcaccaacgaccagaaaaagctgatgagcagcaacgtgcagatcgtgcggcagcagtcctacagcatcatgagcattatcaaagaagagatcctggcctacgtggtgcagctgcctatctacggcgtgatcgataccccttgctggaagctgcacacaagccctctgtgcaccaccaatatcaaagagggctccaacatctgcctgaccagaaccgatagaggctggtactgcgataatgccggcagcgtcagcttcttcccacaagccgatacctgcaaggtgcagagcaacagagtgttctgcgataccatgaacagcctgacactgcccagcgaggtgtccctgtgcaacaccgacatcttcaactctaagtacgactgcaagatcatgacctccaagaccgacatcagctcctccgtgatcacatctctgggcgccatcgtgtcctgctacggcaagacaaagtgtaccgccagcaacaagaaccggggcatcatcaagaccttcagcaacggctgcgactacgtgtccaacaaaggcgtggacaccgtgtctgtgggcaacaccctgtactacgtgaacaagctggaaggcaagaatctgtacgtgaagggcgagcccatcatcaactactacgaccctctggtgttccccagcagcgagtttgatgccagcatcagccaagtgaacgagaagatcaaccagagcctggccttcatccgcagatccgatgaactgctgcacaatgtgaacaccggcaagagcaccacaaacatcatgatcaccgccatcatcatcgtgatcatcgtcgtgctgctgagcctgatcgctatcggcctgctgctgtactgatga

SEQ ID NO: 267 - DNA, 1653 bp, synthetic construct
  source 1..1653: mol_type = other DNA
atggaactgcccatcctgaaaacaaacgccatcaccaccatcctggccgccgtgacactgtgttttgccagcagccagaacatcaccgaagagttctaccagagcacctgtagcgccgtgtctaagggctatctgtctgccctgagaaccggctggtatcacagcgtgatcaccatcgagctgagcaacatcaaagaaaacaagtgcaacggcaccgacgccaaagtgaagctgatcaagcaagagctggacaagtacaagaacgccgtgaccgaactgcagctgctgatgcagtctacccctgccgccaattgcagagccagacgggaactgcctagattcatgaactacaccctgaacaacaccaagaacaccaacgtgaccctgagcaagaagcggaagcggagattcctgggctttctgctcggagtgggaagctgcattgcctctggaattgccgtgtccaaggtgctgcatctggaaggcgaagtgaacaagatcaagagcgccctgctgagcaccaacaaggccgtggtttctctgagcaatggcgtgtccgtgctgaccatcaaggtgctggacctgaagaactacatcgacaaacagctgctgcccatcgtcaacaagcagagctgcagcatcagcaacatcgagacagtgatcgagttccagcagaagaacaaccggctgctggaaatcacccgcgagttttctgtgaatgccggcgtgaccacacctgtgtccacctacatgctgaccaacagcgagctgctgtccctgatcaacgacatgcccatcaccaacgaccagaaaaagctgatgagcagcaacgtgcagatcgtgcggcagcagagctactccatcatgagcattatcaaagaagagatcctggcctacgtggtgcagctgcctctgtatggcgtgatcgataccccttgctggaagctgcacacaagccctctgtgcaccaccaacaccaaagagggctccaacatctgcctgaccagaaccgatagaggctggtactgcgataatgccggcagcgtcagcttcttcccacaagccgagacatgcaaggtgcagagcaacagagtgttctgcgataccatgaacagcctgacactgccctccgaagtgaatctgtgcaatatcgacatcttcaacccgaagtacgactgcaagatcatgaccagcaagaccgacgtgtcaagctccgtgatcacatctctgggcgccatcgtgtcctgctacggcaagacaaagtgcaccgccagcaacaagaaccggggcatcatcaagaccttcagcaacggctgcgactacgtgtccaacaaaggcgtggacaccgtgtctgtgggcaacaccctgtactacgtgaacaagcaagaaggcaagagcctgtacgtgaagggcgagcccatcatcaacttctacgaccctctggtgttccccagcagcgagtttgatgccagcatctcccaagtgaacgagaagatcaaccagagcctggccttcatcagaaagtccgatgagctgctgcacaacgtgaacgccggcaagtccaccaccaatatcatgatcaccacgatcatcatcgtgatcatcgtcatcctgctggctctgatcgctgtgggcctgctgctgtattgatga

SEQ ID NO: 268 - DNA, 1653 bp, synthetic construct
  source 1..1653: mol_type = other DNA
atggaactgctgattcacagaagcagcgccatctttctgaccctggccatcaatgccctgtacctgaccagcagccagaacatcaccgaagagttctaccagagcacctgtagcgccgtgtccagaggctacttttctgccctgagaaccggctggtatcacagcgtgatcaccatcgagctgagcaacatcaaagaaacaaagtgcaacggcaccgacaccaaagtgaagctgatcaagcaagagctggacaagtacaagaacgccgtgaccgaactgcagctgctgatgcagaatacccctgccgccaactgccgggccagaagagaagcccctcagtacatgaactacaccatcaacaccaccaagaacctgaacgtgtccatcagcaagaagcggaagcggagattcctgggctttctgctcggagtgggaagctgcattgcctctggaattgccgtgtctaaggtgctgcacctggaaggcgaagtgaacaagatcaagaatgccctgctgagcaccaacaaggccgtggtgtctctgtctaatggcgtgtccgtgctgaccatcaaggtgctggacctgaagaactacatcaacaaccagctgctgcccatcgtgaaccagcagagctgccggatcagcaacatcgagacagtgatcgagttccagcagaagaacagcagactgctggaaatcacccgcgagttttccgtgaatgccggcgtgacaacacccctgagcacctacatgctgaccaacagcgagctgctgtccctgatcaacgacatgcccatcaccaacgaccagaaaaagctgatgagcagcaacgtgcagatcgtgcggcagcagtcctacagcatcatgagcattatcaaagaagagatcctggcctacgtggtgcagctgcctatctacggcgtgatcgataccccttgctggaagctgcacacaagccctctgtgcaccaccaatatcaaagagggctccaacatctgcctgaccagaaccgatagaggctggtactgcgataatgccggcagcgtcagcttcttcccacaagccgatacctgcaaggtgcagagcaacagagtgttctgcgataccatgaacagcctgacactgcccagcgaggtgtccctgtgcaacaccgacatcttcaactctaagtacgactgcaagatcatgacctccaagaccgacatcagctcctccgtgatcacatctctgggcgccatcgtgtcctgctacggcaagacaaagtgtaccgccagcaacaagaaccggggcatcatcaagaccttcagcaacggctgcgactacgtgtccaacaaaggcgtggacaccgtgtctgtgggcaacaccctgtactacgtgaacaagctggaaggcaagaatctgtacgtgaagggcgagcccatcatcaactactacgaccctctggtgttccccagcagcgagtttgatgccagcatcagccaagtgaacgagaagatcaaccagagcctggccttcatccgcagatccgatgaactgctgcacaatgtgaacaccggcaagagcaccacaaacatcatgatcaccgccatcatcatcgtgatcatcgtcgtgctgctgagcctgatcgctatcggcctgctgctgtactgatga

SEQ ID NO: 269 - DNA, 1653 bp, synthetic construct
  source 1..1653: mol_type = other DNA
atggaactgcccatcctgaaaacaaacgccatcaccaccatcctggccgccgtgacactgtgttttgccagcagccagaacatcaccgaagagttctaccagagcacctgtagcgccgtgtctaagggctatctgtctgccctgagaaccggctggtatcacagcgtgatcaccatcgagctgagcaacatcaaagaaaacaagtgcaacggcaccgacgccaaagtgaagctgatcaagcaagagctggacaagtacaagaacgccgtgaccgaactgcagctgctgatgcagtctacccctgccgccaattgcagagccagacgggaactgcctagattcatgaactacaccctgaacaacaccaagaacaccaacgtgaccctgagcaagaagcggaagcggagattcctgggctttctgctcggagtgtgcagcgccattgcctctggaattgccgtgtccaaggtgctgcatctggaaggcgaagtgaacaagatcaagagcgccctgctgagcaccaacaaggccgtggtttctctgagcaatggcgtgtccgtgctgaccatcaaggtgctggacctgaagaactacatcgacaaacagctgctgcccatcgtcaacaagcagagctgcagcatcagcaacatcgagacagtgatcgagttccagcagaagaacaaccggctgctggaaatcacccgcgagttttctgtgaatgccggcgtgaccacacctgtgtccacctacatgctgaccaacagcgagctgctgtccctgatcaacgacatgcccatcaccaacgaccagaaaaagctgatgagcagcaacgtgcagatcgtgcggcagcagagctactccatcatgagcattatcaaagaagagatcctggcctacgtggtgcagctgcctctgtatggcgtgatcgataccccttgctggaagctgcacacaagccctctgtgcaccaccaacaccaaagagggctccaacatctgcctgaccagaaccgatagaggctggtactgcgataatgccggcagcgtcagcttcttcccacaagccgagacatgcaaggtgcagagcaacagagtgttctgcgataccatgaacagcctgacactgccctccgaagtgaatctgtgcaatatcgacatcttcaacccgaagtacgactgcaagatcatgaccagcaagaccgacgtgtcaagctccgtgatcacatctctgggcgccatcgtgtcctgctacggcaagacaaagtgcaccgccagcaacaagaaccggggcatcatcaagaccttcagcaacggctgcgactacgtgtccaacaaaggcgtggacaccgtgtctgtgggcaacaccctgtactacgtgaacaagcaagaaggcaagagcctgtacgtgaagggcgagcccatcatcaacttctacgaccctctggtgttccccagcagcgagtttgatgccagcatctcccaagtgaacgagaagatcaaccagagcctggccttcatcagaaagtccgatgagctgctgcacaacgtgaacgccggcaagtccaccaccaatatcatgatcaccacgatcatcatcgtgatcatcgtcatcctgctggctctgatcgctgtgggcctgctgctgtattgatga

SEQ ID NO: 270 - DNA, 1653 bp, synthetic construct
  source 1..1653: mol_type = other DNA
atggaactgctgattcacagaagcagcgccatctttctgaccctggccatcaatgccctgtacctgaccagcagccagaacatcaccgaagagttctaccagagcacctgtagcgccgtgtccagaggctacttttctgccctgagaaccggctggtatcacagcgtgatcaccatcgagctgagcaacatcaaagaaacaaagtgcaacggcaccgacaccaaagtgaagctgatcaagcaagagctggacaagtacaagaacgccgtgaccgaactgcagctgctgatgcagaatacccctgccgccaactgccgggccagaagagaagcccctcagtacatgaactacaccatcaacaccaccaagaacctgaacgtgtccatcagcaagaagcggaagcggagattcctgggctttctgctcggagtgtgcagcgccattgcctctggaattgccgtgtctaaggtgctgcacctggaaggcgaagtgaacaagatcaagaatgccctgctgagcaccaacaaggccgtggtgtctctgtctaatggcgtgtccgtgctgaccatcaaggtgctggacctgaagaactacatcaacaaccagctgctgcccatcgtgaaccagcagagctgccggatcagcaacatcgagacagtgatcgagttccagcagaagaacagcagactgctggaaatcacccgcgagttttccgtgaatgccggcgtgacaacacccctgagcacctacatgctgaccaacagcgagctgctgtccctgatcaacgacatgcccatcaccaacgaccagaaaaagctgatgagcagcaacgtgcagatcgtgcggcagcagtcctacagcatcatgagcattatcaaagaagagatcctggcctacgtggtgcagctgcctatctacggcgtgatcgataccccttgctggaagctgcacacaagccctctgtgcaccaccaatatcaaagagggctccaacatctgcctgaccagaaccgatagaggctggtactgcgataatgccggcagcgtcagcttcttcccacaagccgatacctgcaaggtgcagagcaacagagtgttctgcgataccatgaacagcctgacactgcccagcgaggtgtccctgtgcaacaccgacatcttcaactctaagtacgactgcaagatcatgacctccaagaccgacatcagctcctccgtgatcacatctctgggcgccatcgtgtcctgctacggcaagacaaagtgtaccgccagcaacaagaaccggggcatcatcaagaccttcagcaacggctgcgactacgtgtccaacaaaggcgtggacaccgtgtctgtgggcaacaccctgtactacgtgaacaagctggaaggcaagaatctgtacgtgaagggcgagcccatcatcaactactacgaccctctggtgttccccagcagcgagtttgatgccagcatcagccaagtgaacgagaagatcaaccagagcctggccttcatccgcagatccgatgaactgctgcacaatgtgaacaccggcaagagcaccacaaacatcatgatcaccgccatcatcatcgtgatcatcgtcgtgctgctgagcctgatcgctatcggcctgctgctgtactgatga

SEQ ID NO: 271 - DNA, 1653 bp, synthetic construct
  source 1..1653: mol_type = other DNA
atggaactgcccatcctgaaaacaaacgccatcaccaccatcctggccgccgtgacactgtgttttgccagcagccagaacatcaccgaagagttctaccagagcacctgtagcgccgtgtctaagggctatctgtctgccctgagaaccggctggtatcacagcgtgatcaccatcgagctgagcaacatcaaagaaaacaagtgcaacggcaccgacgccaaagtgaagctgatcaagcaagagctggacaagtacaagaacgccgtgaccgaactgcagctgctgatgcagtctacccctgccgccaattgcagagccagacgggaactgcctagattcatgaactacaccctgaacaacaccaagaacaccaacgtgaccctgagcaagaagcggaagcggagattcctgggctttctgctcggagtgggatgcgccattgcctctggaattgccgtgtccaaggtgctgcatctggaaggcgaagtgaacaagatcaagagcgccctgctgagcaccaacaaggccgtggtttctctgagcaatggcgtgtccgtgctgaccatcaaggtgctggacctgaagaactacatcgacaaacagctgctgcccatcgtcaacaagcagagctgcagcatcagcaacatcgagacagtgatcgagttccagcagaagaacaaccggctgctggaaatcacccgcgagttttctgtgaatgccggcgtgaccacacctgtgtccacctacatgctgaccaacagcgagctgctgtccctgatcaacgacatgcccatcaccaacgaccagaaaaagctgatgagcagcaacgtgcagatcgtgcggcagcagagctactccatcatgagcattatcaaagaagagatcctggcctacgtggtgcagctgcctctgtatggcgtgatcgataccccttgctggaagctgcacacaagccctctgtgcaccaccaacaccaaagagggctccaacatctgcctgaccagaaccgatagaggctggtactgcgataatgccggcagcgtcagcttcttcccacaagccgagacatgcaaggtgcagagcaacagagtgttctgcgataccatgaacagcctgacactgccctccgaagtgaatctgtgcaatatcgacatcttcaacccgaagtacgactgcaagatcatgaccagcaagaccgacgtgtcaagctccgtgatcacatctctgggcgccatcgtgtcctgctacggcaagacaaagtgcaccgccagcaacaagaaccggggcatcatcaagaccttcagcaacggctgcgactacgtgtccaacaaaggcgtggacaccgtgtctgtgggcaacaccctgtactacgtgaacaagcaagaaggcaagagcctgtacgtgaagggcgagcccatcatcaacttctacgaccctctggtgttccccagcagcgagtttgatgccagcatctcccaagtgaacgagaagatcaaccagagcctggccttcatcagaaagtccgatgagctgctgcacaacgtgaacgccggcaagtccaccaccaatatcatgatcaccacgatcatcatcgtgatcatcgtcatcctgctggctctgatcgctgtgggcctgctgctgtattgatga

SEQ ID NO: 272 - DNA, 1653 bp, synthetic construct
  source 1..1653: mol_type = other DNA
atggaactgctgattcacagaagcagcgccatctttctgaccctggccatcaatgccctgtacctgaccagcagccagaacatcaccgaagagttctaccagagcacctgtagcgccgtgtccagaggctacttttctgccctgagaaccggctggtatcacagcgtgatcaccatcgagctgagcaacatcaaagaaacaaagtgcaacggcaccgacaccaaagtgaagctgatcaagcaagagctggacaagtacaagaacgccgtgaccgaactgcagctgctgatgcagaatacccctgccgccaactgccgggccagaagagaagcccctcagtacatgaactacaccatcaacaccaccaagaacctgaacgtgtccatcagcaagaagcggaagcggagattcctgggctttctgctcggagtgggatgcgccattgcctctggaattgccgtgtctaaggtgctgcacctggaaggcgaagtgaacaagatcaagaatgccctgctgagcaccaacaaggccgtggtgtctctgtctaatggcgtgtccgtgctgaccatcaaggtgctggacctgaagaactacatcaacaaccagctgctgcccatcgtgaaccagcagagctgccggatcagcaacatcgagacagtgatcgagttccagcagaagaacagcagactgctggaaatcacccgcgagttttccgtgaatgccggcgtgacaacacccctgagcacctacatgctgaccaacagcgagctgctgtccctgatcaacgacatgcccatcaccaacgaccagaaaaagctgatgagcagcaacgtgcagatcgtgcggcagcagtcctacagcatcatgagcattatcaaagaagagatcctggcctacgtggtgcagctgcctatctacggcgtgatcgataccccttgctggaagctgcacacaagccctctgtgcaccaccaatatcaaagagggctccaacatctgcctgaccagaaccgatagaggctggtactgcgataatgccggcagcgtcagcttcttcccacaagccgatacctgcaaggtgcagagcaacagagtgttctgcgataccatgaacagcctgacactgcccagcgaggtgtccctgtgcaacaccgacatcttcaactctaagtacgactgcaagatcatgacctccaagaccgacatcagctcctccgtgatcacatctctgggcgccatcgtgtcctgctacggcaagacaaagtgtaccgccagcaacaagaaccggggcatcatcaagaccttcagcaacggctgcgactacgtgtccaacaaaggcgtggacaccgtgtctgtgggcaacaccctgtactacgtgaacaagctggaaggcaagaatctgtacgtgaagggcgagcccatcatcaactactacgaccctctggtgttccccagcagcgagtttgatgccagcatcagccaagtgaacgagaagatcaaccagagcctggccttcatccgcagatccgatgaactgctgcacaatgtgaacaccggcaagagcaccacaaacatcatgatcaccgccatcatcatcgtgatcatcgtcgtgctgctgagcctgatcgctatcggcctgctgctgtactgatga

SEQ ID NO: 273 - DNA, 1653 bp, synthetic construct
  source 1..1653: mol_type = other DNA
atggaactgcccatcctgaaaacaaacgccatcaccaccatcctggccgccgtgacactgtgttttgccagcagccagaacatcaccgaagagttctaccagagcacctgtagcgccgtgtctaagggctatctgtctgccctgagaaccggctggtatcacagcgtgatcaccatcgagctgagcaacatcaaagaaaacaagtgcaacggcaccgacgccaaagtgaagctgatcaagcaagagctggacaagtacaagaacgccgtgaccgaactgcagctgctgatgcagtctacctgcgccgccaatagcagagccagacgggaactgcctagattcatgaactacaccctgaacaacaccaagaacaccaacgtgaccctgagcaagaagcggaagcggagattcctgggctttctgctcggagtgggaagcgccattgcctctggatgcgccgtgtccaaggtgctgcatctggaaggcgaagtgaacaagatcaagagcgccctgctgagcaccaacaaggccgtggtttctctgagcaatggcgtgtccgtgctgaccatcaaggtgctggacctgaagaactacatcgacaaacagctgctgcccatcgtcaacaagcagagctgcagcatcagcaacatcgagacagtgatcgagttccagcagaagaacaaccggctgctggaaatcacccgcgagttttctgtgaatgccggcgtgaccacacctgtgtccacctacatgctgaccaacagcgagctgctgtccctgatcaacgacatgcccatcaccaacgaccagaaaaagctgatgagcagcaacgtgcagatcgtgcggcagcagagctactccatcatgagcattatcaaagaagagatcctggcctacgtggtgcagctgcctctgtatggcgtgatcgataccccttgctggaagctgcacacaagccctctgtgcaccaccaacaccaaagagggctccaacatctgcctgaccagaaccgatagaggctggtactgcgataatgccggcagcgtcagcttcttcccacaagccgagacatgcaaggtgcagagcaacagagtgttctgcgataccatgaacagcctgacactgccctccgaagtgaatctgtgcaatatcgacatcttcaacccgaagtacgactgcaagatcatgaccagcaagaccgacgtgtcaagctccgtgatcacatctctgggcgccatcgtgtcctgctacggcaagacaaagtgcaccgccagcaacaagaaccggggcatcatcaagaccttcagcaacggctgcgactacgtgtccaacaaaggcgtggacaccgtgtctgtgggcaacaccctgtactacgtgaacaagcaagaaggcaagagcctgtacgtgaagggcgagcccatcatcaacttctacgaccctctggtgttccccagcagcgagtttgatgccagcatctcccaagtgaacgagaagatcaaccagagcctggccttcatcagaaagtccgatgagctgctgcacaacgtgaacgccggcaagtccaccaccaatatcatgatcaccacgatcatcatcgtgatcatcgtcatcctgctggctctgatcgctgtgggcctgctgctgtattgatga

SEQ ID NO: 274 - DNA, 1653 bp, synthetic construct
  source 1..1653: mol_type = other DNA
atggaactgctgattcacagaagcagcgccatctttctgaccctggccatcaatgccctgtacctgaccagcagccagaacatcaccgaagagttctaccagagcacctgtagcgccgtgtccagaggctacttttctgccctgagaaccggctggtatcacagcgtgatcaccatcgagctgagcaacatcaaagaaacaaagtgcaacggcaccgacaccaaagtgaagctgatcaagcaagagctggacaagtacaagaacgccgtgaccgaactgcagctgctgatgcagaatacctgcgccgccaacaaccgggccagaagagaagcccctcagtacatgaactacaccatcaacaccaccaagaacctgaacgtgtccatcagcaagaagcggaagcggagattcctgggctttctgctcggagtgggaagcgccattgcctctggatgcgccgtgtctaaggtgctgcacctggaaggcgaagtgaacaagatcaagaatgccctgctgagcaccaacaaggccgtggtgtctctgtctaatggcgtgtccgtgctgaccatcaaggtgctggacctgaagaactacatcaacaaccagctgctgcccatcgtgaaccagcagagctgccggatcagcaacatcgagacagtgatcgagttccagcagaagaacagcagactgctggaaatcacccgcgagttttccgtgaatgccggcgtgacaacacccctgagcacctacatgctgaccaacagcgagctgctgtccctgatcaacgacatgcccatcaccaacgaccagaaaaagctgatgagcagcaacgtgcagatcgtgcggcagcagtcctacagcatcatgagcattatcaaagaagagatcctggcctacgtggtgcagctgcctatctacggcgtgatcgataccccttgctggaagctgcacacaagccctctgtgcaccaccaatatcaaagagggctccaacatctgcctgaccagaaccgatagaggctggtactgcgataatgccggcagcgtcagcttcttcccacaagccgatacctgcaaggtgcagagcaacagagtgttctgcgataccatgaacagcctgacactgcccagcgaggtgtccctgtgcaacaccgacatcttcaactctaagtacgactgcaagatcatgacctccaagaccgacatcagctcctccgtgatcacatctctgggcgccatcgtgtcctgctacggcaagacaaagtgtaccgccagcaacaagaaccggggcatcatcaagaccttcagcaacggctgcgactacgtgtccaacaaaggcgtggacaccgtgtctgtgggcaacaccctgtactacgtgaacaagctggaaggcaagaatctgtacgtgaagggcgagcccatcatcaactactacgaccctctggtgttccccagcagcgagtttgatgccagcatcagccaagtgaacgagaagatcaaccagagcctggccttcatccgcagatccgatgaactgctgcacaatgtgaacaccggcaagagcaccacaaacatcatgatcaccgccatcatcatcgtgatcatcgtcgtgctgctgagcctgatcgctatcggcctgctgctgtactgatga

SEQ ID NO: 275 - DNA, 1653 bp, synthetic construct
  source 1..1653: mol_type = other DNA
atggaactgctgattcacagaagcagcgccatctttctgaccctggccatcaatgccctgtacctgaccagcagccagaacatcaccgaagagttctaccagagcacctgtagcgccgtgtccagaggctacttttctgccctgagaaccggctggtatcacagcgtgatcaccatcgagctgagcaacatcaaagaaacaaagtgcaacggcaccgacaccaaagtgaagctgatcaagcaagagctggacaagtacaagaacgccgtgaccgaactgcagctgctgatgcagaatacccctgcctgcaacaaccgggccagaagagaagcccctcagtacatgaactacaccatcaacaccaccaagaacctgaacgtgtccatcagcaagaagcggaagcggagattcctgggctttctgctcggagtgggatgcgccattgcctctggaattgccgtgtctaaggtgctgcacctggaaggcgaagtgaacaagatcaagaatgccctgctgagcaccaacaaggccgtggtgtctctgtctaatggcgtgtccgtgctgaccatcaaggtgctggacctgaagaactacatcaacaaccagctgctgcccatcgtgaaccagcagagctgccggatcagcaacatcgagacagtgatcgagttccagcagaagaacagcagactgctggaaatcacccgcgagttttccgtgaatgccggcgtgacaacacccctgagcacctacatgctgaccaacagcgagctgctgtccctgatcaacgacatgcccatcaccaacgaccagaaaaagctgatgagcagcaacgtgcagatcgtgcggcagcagtcctacagcatcatgagcattatcaaagaagagatcctggcctacgtggtgcagctgcctatctacggcgtgatcgataccccttgctggaagctgcacacaagccctctgtgcaccaccaatatcaaagagggctccaacatctgcctgaccagaaccgatagaggctggtactgcgataatgccggcagcgtcagcttcttcccacaagccgatacctgcaaggtgcagagcaacagagtgttctgcgataccatgaacagcctgacactgcccagcgaggtgtccctgtgcaacaccgacatcttcaactctaagtacgactgcaagatcatgacctccaagaccgacatcagctcctccgtgatcacatctctgggcgccatcgtgtcctgctacggcaagacaaagtgtaccgccagcaacaagaaccggggcatcatcaagaccttcagcaacggctgcgactacgtgtccaacaaaggcgtggacaccgtgtctgtgggcaacaccctgtactacgtgaacaagctggaaggcaagaatctgtacgtgaagggcgagcccatcatcaactactacgaccctctggtgttccccagcagcgagtttgatgccagcatcagccaagtgaacgagaagatcaaccagagcctggccttcatccgcagatccgatgaactgctgcacaatgtgaacaccggcaagagcaccacaaacatcatgatcaccgccatcatcatcgtgatcatcgtcgtgctgctgagcctgatcgctatcggcctgctgctgtactgatga

SEQ ID NO: 276 - DNA, 1653 bp, synthetic construct
  source 1..1653: mol_type = other DNA
atggaactgcccatcctgaaaacaaacgccatcaccaccatcctggccgccgtgacactgtgttttgccagcagccagaacatcaccgaagagttctaccagagcacctgtagcgccgtgtctaagggctatctgtctgccctgagaaccggctggtatcacagcgtgatcaccatcgagctgagcaacatcaaagaaaacaagtgcaacggcaccgacgccaaagtgaagctgatcaagcaagagctggacaagtacaagaacgccgtgaccgaactgcagctgctgatgcagtctacccctgcctgcaatagcagagccagacgggaactgcctagattcatgaactacaccctgaacaacaccaagaacaccaacgtgaccctgagcaagaagcggaagcggagattcctgggctttctgctcggagtgggatgcgccattgcctctggaattgccgtgtccaaggtgctgcatctggaaggcgaagtgaacaagatcaagagcgccctgctgagcaccaacaaggccgtggtttctctgagcaatggcgtgtccgtgctgaccatcaaggtgctggacctgaagaactacatcgacaaacagctgctgcccatcgtcaacaagcagagctgcagcatcagcaacatcgagacagtgatcgagttccagcagaagaacaaccggctgctggaaatcacccgcgagttttctgtgaatgccggcgtgaccacacctgtgtccacctacatgctgaccaacagcgagctgctgtccctgatcaacgacatgcccatcaccaacgaccagaaaaagctgatgagcagcaacgtgcagatcgtgcggcagcagagctactccatcatgagcattatcaaagaagagatcctggcctacgtggtgcagctgcctctgtatggcgtgatcgataccccttgctggaagctgcacacaagccctctgtgcaccaccaacaccaaagagggctccaacatctgcctgaccagaaccgatagaggctggtactgcgataatgccggcagcgtcagcttcttcccacaagccgagacatgcaaggtgcagagcaacagagtgttctgcgataccatgaacagcctgacactgccctccgaagtgaatctgtgcaatatcgacatcttcaacccgaagtacgactgcaagatcatgaccagcaagaccgacgtgtcaagctccgtgatcacatctctgggcgccatcgtgtcctgctacggcaagacaaagtgcaccgccagcaacaagaaccggggcatcatcaagaccttcagcaacggctgcgactacgtgtccaacaaaggcgtggacaccgtgtctgtgggcaacaccctgtactacgtgaacaagcaagaaggcaagagcctgtacgtgaagggcgagcccatcatcaacttctacgaccctctggtgttccccagcagcgagtttgatgccagcatctcccaagtgaacgagaagatcaaccagagcctggccttcatcagaaagtccgatgagctgctgcacaacgtgaacgccggcaagtccaccaccaatatcatgatcaccacgatcatcatcgtgatcatcgtcatcctgctggctctgatcgctgtgggcctgctgctgtattgatga

SEQ ID NO: 277 - DNA, 1653 bp, synthetic construct
  source 1..1653: mol_type = other DNA
atggaactgctgattcacagaagcagcgccatctttctgaccctggccatcaatgccctgtacctgaccagcagccagaacatcaccgaagagttctaccagagcacctgtagcgccgtgtccagaggctacttttctgccctgagaaccggctggtatcacagcgtgatcaccatcgagctgagcaacatcaaagaaacaaagtgcaacggcaccgacaccaaagtgaagctgatcaagcaagagctggacaagtacaagaacgccgtgaccgaactgcagctgctgatgcagaataccccttgcgccaacaaccgggccagaagagaagcccctcagtacatgaactacaccatcaacaccaccaagaacctgaacgtgtccatcagcaagaagcggaagcggagattcctgggctttctgctcggagtgggaagcgccattgcctctggaatttgtgtgtctaaggtgctgcacctggaaggcgaagtgaacaagatcaagaatgccctgctgagcaccaacaaggccgtggtgtctctgtctaatggcgtgtccgtgctgaccatcaaggtgctggacctgaagaactacatcaacaaccagctgctgcccatcgtgaaccagcagagctgccggatcagcaacatcgagacagtgatcgagttccagcagaagaacagcagactgctggaaatcacccgcgagttttccgtgaatgccggcgtgacaacacccctgagcacctacatgctgaccaacagcgagctgctgtccctgatcaacgacatgcccatcaccaacgaccagaaaaagctgatgagcagcaacgtgcagatcgtgcggcagcagtcctacagcatcatgagcattatcaaagaagagatcctggcctacgtggtgcagctgcctatctacggcgtgatcgataccccttgctggaagctgcacacaagccctctgtgcaccaccaatatcaaagagggctccaacatctgcctgaccagaaccgatagaggctggtactgcgataatgccggcagcgtcagcttcttcccacaagccgatacctgcaaggtgcagagcaacagagtgttctgcgataccatgaacagcctgacactgcccagcgaggtgtccctgtgcaacaccgacatcttcaactctaagtacgactgcaagatcatgacctccaagaccgacatcagctcctccgtgatcacatctctgggcgccatcgtgtcctgctacggcaagacaaagtgtaccgccagcaacaagaaccggggcatcatcaagaccttcagcaacggctgcgactacgtgtccaacaaaggcgtggacaccgtgtctgtgggcaacaccctgtactacgtgaacaagctggaaggcaagaatctgtacgtgaagggcgagcccatcatcaactactacgaccctctggtgttccccagcagcgagtttgatgccagcatcagccaagtgaacgagaagatcaaccagagcctggccttcatccgcagatccgatgaactgctgcacaatgtgaacaccggcaagagcaccacaaacatcatgatcaccgccatcatcatcgtgatcatcgtcgtgctgctgagcctgatcgctatcggcctgctgctgtactgatga

SEQ ID NO: 278 - DNA, 1653 bp, synthetic construct
  source 1..1653: mol_type = other DNA
atggaactgctgattcacagaagcagcgccatctttctgaccctggccatcaatgccctgtacctgaccagcagccagaacatcaccgaagagttctaccagagcacctgtagcgccgtgtccagaggctacttttctgccctgagaaccggctggtatcacagcgtgatcaccatcgagctgagcaacatcaaagaaacaaagtgcaacggcaccgacaccaaagtgaagctgatcaagcaagagctggacaagtacaagaacgccgtgaccgaactgcagctgctgatgcagaataccccttgcgccaacaaccgggccagaagagaagcccctcagtacatgaactacaccatcaacaccaccaagaacctgaacgtgtccatcagcaagaagcggaagcggagattcctgggctttctgctcggagtgggaagcgccattgcctgtggaattgccgtgtctaaggtgctgcacctggaaggcgaagtgaacaagatcaagaatgccctgctgagcaccaacaaggccgtggtgtctctgtctaatggcgtgtccgtgctgaccatcaaggtgctggacctgaagaactacatcaacaaccagctgctgcccatcgtgaaccagcagagctgccggatcagcaacatcgagacagtgatcgagttccagcagaagaacagcagactgctggaaatcacccgcgagttttccgtgaatgccggcgtgacaacacccctgagcacctacatgctgaccaacagcgagctgctgtccctgatcaacgacatgcccatcaccaacgaccagaaaaagctgatgagcagcaacgtgcagatcgtgcggcagcagtcctacagcatcatgagcattatcaaagaagagatcctggcctacgtggtgcagctgcctatctacggcgtgatcgataccccttgctggaagctgcacacaagccctctgtgcaccaccaatatcaaagagggctccaacatctgcctgaccagaaccgatagaggctggtactgcgataatgccggcagcgtcagcttcttcccacaagccgatacctgcaaggtgcagagcaacagagtgttctgcgataccatgaacagcctgacactgcccagcgaggtgtccctgtgcaacaccgacatcttcaactctaagtacgactgcaagatcatgacctccaagaccgacatcagctcctccgtgatcacatctctgggcgccatcgtgtcctgctacggcaagacaaagtgtaccgccagcaacaagaaccggggcatcatcaagaccttcagcaacggctgcgactacgtgtccaacaaaggcgtggacaccgtgtctgtgggcaacaccctgtactacgtgaacaagctggaaggcaagaatctgtacgtgaagggcgagcccatcatcaactactacgaccctctggtgttccccagcagcgagtttgatgccagcatcagccaagtgaacgagaagatcaaccagagcctggccttcatccgcagatccgatgaactgctgcacaatgtgaacaccggcaagagcaccacaaacatcatgatcaccgccatcatcatcgtgatcatcgtcgtgctgctgagcctgatcgctatcggcctgctgctgtactgatga

SEQ ID NO: 279 - DNA, 1653 bp, synthetic construct
  source 1..1653: mol_type = other DNA
atggaactgcccatcctgaaaacaaacgccatcaccaccatcctggccgccgtgacactgtgttttgccagcagccagaacatcaccgaagagttctaccagagcacctgtagcgccgtgtctaagggctatctgtctgccctgagaaccggctggtatcacagcgtgatcaccatcgagctgagcaacatcaaagaaaacaagtgcaacggcaccgacgccaaagtgaagctgatcaagcaagagctggacaagtacaagaacgccgtgaccgaactgcagctgctgatgcagtctaccccttgcgccaatagcagagccagacgggaactgcctagattcatgaactacaccctgaacaacaccaagaacaccaacgtgaccctgagcaagaagcggaagcggagattcctgggctttctgctcggagtgggaagcgccattgcctctggaatttgtgtgtccaaggtgctgcatctggaaggcgaagtgaacaagatcaagagcgccctgctgagcaccaacaaggccgtggtttctctgagcaatggcgtgtccgtgctgaccatcaaggtgctggacctgaagaactacatcgacaaacagctgctgcccatcgtcaacaagcagagctgcagcatcagcaacatcgagacagtgatcgagttccagcagaagaacaaccggctgctggaaatcacccgcgagttttctgtgaatgccggcgtgaccacacctgtgtccacctacatgctgaccaacagcgagctgctgtccctgatcaacgacatgcccatcaccaacgaccagaaaaagctgatgagcagcaacgtgcagatcgtgcggcagcagagctactccatcatgagcattatcaaagaagagatcctggcctacgtggtgcagctgcctctgtatggcgtgatcgataccccttgctggaagctgcacacaagccctctgtgcaccaccaacaccaaagagggctccaacatctgcctgaccagaaccgatagaggctggtactgcgataatgccggcagcgtcagcttcttcccacaagccgagacatgcaaggtgcagagcaacagagtgttctgcgataccatgaacagcctgacactgccctccgaagtgaatctgtgcaatatcgacatcttcaacccgaagtacgactgcaagatcatgaccagcaagaccgacgtgtcaagctccgtgatcacatctctgggcgccatcgtgtcctgctacggcaagacaaagtgcaccgccagcaacaagaaccggggcatcatcaagaccttcagcaacggctgcgactacgtgtccaacaaaggcgtggacaccgtgtctgtgggcaacaccctgtactacgtgaacaagcaagaaggcaagagcctgtacgtgaagggcgagcccatcatcaacttctacgaccctctggtgttccccagcagcgagtttgatgccagcatctcccaagtgaacgagaagatcaaccagagcctggccttcatcagaaagtccgatgagctgctgcacaacgtgaacgccggcaagtccaccaccaatatcatgatcaccacgatcatcatcgtgatcatcgtcatcctgctggctctgatcgctgtgggcctgctgctgtattgatga

SEQ ID NO: 280 - DNA, 1653 bp, synthetic construct
  source 1..1653: mol_type = other DNA
atggaactgcccatcctgaaaacaaacgccatcaccaccatcctggccgccgtgacactgtgttttgccagcagccagaacatcaccgaagagttctaccagagcacctgtagcgccgtgtctaagggctatctgtctgccctgagaaccggctggtatcacagcgtgatcaccatcgagctgagcaacatcaaagaaaacaagtgcaacggcaccgacgccaaagtgaagctgatcaagcaagagctggacaagtacaagaacgccgtgaccgaactgcagctgctgatgcagtctaccccttgcgccaatagcagagccagacgggaactgcctagattcatgaactacaccctgaacaacaccaagaacaccaacgtgaccctgagcaagaagcggaagcggagattcctgggctttctgctcggagtgggaagcgccattgcctgtggaattgccgtgtccaaggtgctgcatctggaaggcgaagtgaacaagatcaagagcgccctgctgagcaccaacaaggccgtggtttctctgagcaatggcgtgtccgtgctgaccatcaaggtgctggacctgaagaactacatcgacaaacagctgctgcccatcgtcaacaagcagagctgcagcatcagcaacatcgagacagtgatcgagttccagcagaagaacaaccggctgctggaaatcacccgcgagttttctgtgaatgccggcgtgaccacacctgtgtccacctacatgctgaccaacagcgagctgctgtccctgatcaacgacatgcccatcaccaacgaccagaaaaagctgatgagcagcaacgtgcagatcgtgcggcagcagagctactccatcatgagcattatcaaagaagagatcctggcctacgtggtgcagctgcctctgtatggcgtgatcgataccccttgctggaagctgcacacaagccctctgtgcaccaccaacaccaaagagggctccaacatctgcctgaccagaaccgatagaggctggtactgcgataatgccggcagcgtcagcttcttcccacaagccgagacatgcaaggtgcagagcaacagagtgttctgcgataccatgaacagcctgacactgccctccgaagtgaatctgtgcaatatcgacatcttcaacccgaagtacgactgcaagatcatgaccagcaagaccgacgtgtcaagctccgtgatcacatctctgggcgccatcgtgtcctgctacggcaagacaaagtgcaccgccagcaacaagaaccggggcatcatcaagaccttcagcaacggctgcgactacgtgtccaacaaaggcgtggacaccgtgtctgtgggcaacaccctgtactacgtgaacaagcaagaaggcaagagcctgtacgtgaagggcgagcccatcatcaacttctacgaccctctggtgttccccagcagcgagtttgatgccagcatctcccaagtgaacgagaagatcaaccagagcctggccttcatcagaaagtccgatgagctgctgcacaacgtgaacgccggcaagtccaccaccaatatcatgatcaccacgatcatcatcgtgatcatcgtcatcctgctggctctgatcgctgtgggcctgctgctgtattgatga

SEQ ID NO: 281 - DNA, 1653 bp, synthetic construct
  source 1..1653: mol_type = other DNA
atggaactgcccatcctgaaaacaaacgccatcaccaccatcctggccgccgtgacactgtgttttgccagcagccagaacatcaccgaagagttctaccagagcacctgtagcgccgtgtctaagggctatctgtctgccctgagaaccggctggtatgccagcgtgatcaccatcgagctgagcaacatcaaagaaaacaagtgcaacggcaccgacgccaaagtgaagctgatcaagcaagagctggacaagtacaagaacgccgtgaccgaactgcagctgctgatgcagtctacccctgccgccaatagcagagccagacgggaactgcctagattcatgaactacaccctgaacaacaccaagaacaccaacgtgaccctgagcaagaagcggaagcggagattcctgggctttctgctcggagtgggaagcgccattgcctctggaattgccgtgtccaaggtgctgcatctggaaggcgaagtgaacaagatcaagagcgccctgctgagcaccaacaaggccgtggtttctctgagcaatggcgtgtccgtgctgacctctaaggtgctggacctgaagaactacatcgacaaacagctgctgcccatcgtcaacaagcagagctgcagcatcagcaacatcgagacagtgatcgagttccagcagaagaacaaccggctgctggaaatcacccgcgagttttctgtgaatgccggcgtgaccacacctgtgtccacctacatgctgaccaacagcgagctgctgtccctgatcaacgacatgcccatcaccaacgaccagaaaaagctgatgagcagcaacgtgcagatcgtgcggcagcagagctactccatcatgagcattatcaaagaagaggtgctggcctacgtggtgcagctgcctctgtatggcgtgatcgataccccttgctggaagctgcacacaagccctctgtgcaccaccaacaccaaagagggctccaacatctgcctgaccagaaccgatagaggctggtactgcgataatgccggcagcgtcagcttcttcccacaagccgagacatgcaaggtgcagagcaacagagtgttctgcgataccatgaacagcctgacactgccctccgaagtgaatctgtgcaatatcgacatcttcaacccgaagtacgactgcaagatcatgaccagcaagaccgacgtgtcaagctccgtgatcacatctctgggcgccatcgtgtcctgctacggcaagacaaagtgcaccgccagcaacaagaaccggggcatcatcaagaccttcagcaacggctgcgactacgtgtccaacaaaggcgtggacaccgtgtctgtgggcaacaccctgtactacgtgaacaagcaagaaggcaagagcctgtacgtgaagggcgagcccatcatcaacttctacgaccctctggtgttccccagcgacgagtttgatgccagcatctcccaagtgaacgagaagatcaaccagagcctggccttcatcagaaagtccgatgagctgctgcacaacgtgaacgccggcaagtccaccaccaatatcatgatcaccacgatcatcatcgtgatcatcgtcatcctgctggctctgatcgctgtgggcctgctgctgtattgatga

SEQ ID NO: 282 - DNA, 1653 bp, synthetic construct
  source 1..1653: mol_type = other DNA
atggaactgcccatcctgaaaacaaacgccatcaccaccatcctggccgccgtgacactgtgttttgccagcagccagaacatcaccgaagagttctaccagagcacctgtagcgccgtgtctaagggctatctgtctgccctgagaaccggctggtataccagcgtgatcaccatcgagctgagcaacatcaaagaaaacaagtgcaacggcaccgacgccaaagtgaagctgatcaagcaagagctggacaagtacaagaacgccgtgaccgaactgcagctgctgatgcagtctacctgcgccgccaatagcagagccagacgggaactgcctagattcatgaactacaccctgaacaacaccaagaacaccaacgtgaccctgagcaagaagcggaagcggagattcctgggctttctgctcggagtgggaagcgccattgcctctggatgcgccgtgtccaaggtgctgcatctggaaggcgaagtgaacaagatcaagagcgccctgctgagcaccaacaaggccgtggtttctctgagcaatggcgtgtccgtgctgacctctaaggtgctggacctgaagaactacatcgacaaacagctgctgcccatcgtcaacaagcagagctgcagcatcagcaacatcgagacagtgatcgagttccagcagaagaacaaccggctgctggaaatcacccgcgagttttctgtgaatgccggcgtgaccacacctgtgtccacctacatgctgaccaacagcgagctgctgtccctgatcaacgacatgcccatcaccaacgaccagaaaaagctgatgagcagcaacgtgcagatcgtgcggcagcagagctactccatcatgagcattatcaaagaagaggtgctggcctacgtggtgcagctgcctctgtatggcgtgatcgataccccttgctggaagctgcacacaagccctctgtgcaccaccaacaccaaagagggctccaacatctgcctgaccagaaccgatagaggctggtactgcgataatgccggcagcgtcagcttcttcccacaagccgagacatgcaaggtgcagagcaacagagtgttctgcgataccatgaacagcctgacactgccctccgaagtgaatctgtgcaatatcgacatcttcaacccgaagtacgactgcaagatcatgaccagcaagaccgacgtgtcaagctccgtgatcacatctctgggcgccatcgtgtcctgctacggcaagacaaagtgcaccgccagcaacaagaaccggggcatcatcaagaccttcagcaacggctgcgactacgtgtccaacaaaggcgtggacaccgtgtctgtgggcaacaccctgtactacgtgaacaagcaagaaggcaagagcctgtacgtgaagggcgagcccatcatcaacttctacgaccctctggtgttccccagcgacgagtttgatgccagcatctcccaagtgaacgagaagatcaaccagagcctggccttcatcagaaagtccgatgagctgctgcacaacgtgaacgccggcaagtccaccaccaatatcatgatcaccacgatcatcatcgtgatcatcgtcatcctgctggctctgatcgctgtgggcctgctgctgtattgatga

SEQ ID NO: 283 - DNA, 1653 bp, synthetic construct
  source 1..1653: mol_type = other DNA
atggaactgcccatcctgaaaacaaacgccatcaccaccatcctggccgccgtgacactgtgttttgccagcagccagaacatcaccgaagagttctaccagagcacctgtagcgccgtgtctaagggctatctgtctgccctgagaaccggctggtataccagcgtgatcaccatcgagctgagcaacatcaaagaaaacaagtgcaacggcaccgacgccaaagtgaagctgatcaagcaagagctggacaagtacaagaacgccgtgaccgaactgcagctgctgatgcagtctacccctgcctgcaatagcagagccagacgggaactgcctagattcatgaactacaccctgaacaacaccaagaacaccaacgtgaccctgagcaagaagcggaagcggagattcctgggctttctgctcggagtgggaagcgcctgcgcctctggaattgccgtgtccaaggtgctgcatctggaaggcgaagtgaacaagatcaagagcgccctgctgagcaccaacaaggccgtggtttctctgagcaatggcgtgtccgtgctgacctctaaggtgctggacctgaagaactacatcgacaaacagctgctgcccatcgtcaacaagcagagctgcagcatcagcaacatcgagacagtgatcgagttccagcagaagaacaaccggctgctggaaatcacccgcgagttttctgtgaatgccggcgtgaccacacctgtgtccacctacatgctgaccaacagcgagctgctgtccctgatcaacgacatgcccatcaccaacgaccagaaaaagctgatgagcagcaacgtgcagatcgtgcggcagcagagctactccatcatgagcattatcaaagaagaggtgctggcctacgtggtgcagctgcctctgtatggcgtgatcgataccccttgctggaagctgcacacaagccctctgtgcaccaccaacaccaaagagggctccaacatctgcctgaccagaaccgatagaggctggtactgcgataatgccggcagcgtcagcttcttcccacaagccgagacatgcaaggtgcagagcaacagagtgttctgcgataccatgaacagcctgacactgccctccgaagtgaatctgtgcaatatcgacatcttcaacccgaagtacgactgcaagatcatgaccagcaagaccgacgtgtcaagctccgtgatcacatctctgggcgccatcgtgtcctgctacggcaagacaaagtgcaccgccagcaacaagaaccggggcatcatcaagaccttcagcaacggctgcgactacgtgtccaacaaaggcgtggacaccgtgtctgtgggcaacaccctgtactacgtgaacaagcaagaaggcaagagcctgtacgtgaagggcgagcccatcatcaacttctacgaccctctggtgttccccagcgacgagtttgatgccagcatctcccaagtgaacgagaagatcaaccagagcctggccttcatcagaaagtccgatgagctgctgcacaacgtgaacgccggcaagtccaccaccaatatcatgatcaccacgatcatcatcgtgatcatcgtcatcctgctggctctgatcgctgtgggcctgctgctgtattgatga

SEQ ID NO: 284 - DNA, 1653 bp, synthetic construct
  source 1..1653: mol_type = other DNA
atggaactgcccatcctgaaaacaaacgccatcaccaccatcctggccgccgtgacactgtgttttgccagcagccagaacatcaccgaagagttctaccagagcacctgtagcgccgtgtctaagggctatctgtctgccctgagaaccggctggtataccagcgtgatcaccatcgagctgagcaacatcaaagaaaacaagtgcaacggcaccgacgccaaagtgaagctgatcaagcaagagctggacaagtacaagaacgccgtgaccgaactgcagctgctgatgcagtctacccctgccgccaatagcagagccagacgggaactgcctagattcatgaactacaccctgaacaacaccaagaacaccaacgtgaccctgagcaagaagcggaagcggagattcctgggctttctgctcggagtgggaagcgccattgcctctggaattgccgtgtccaaggtgctgcatctggaaggcgaagtgaacaagatcaagagcgccctgctgagcaccaacaaggccgtggtttctctgagcaatggcgtgtccgtgctgaccatgaaggtgctggacctgaagaactacatcgacaaacagctgctgcccatcgtcaacaagcagagctgcagcatcagcaacatcgagacagtgatcgagttccagcagaagaacaaccggctgctggaaatcacccgcgagttttctgtgaatgccggcgtgaccacacctgtgtccacctacatgctgaccaacagcgagctgctgtccctgatcaacgacatgcccatcaccaacgaccagaaaaagctgatgagcagcaacgtgcagatcgtgcggcagcagagctactccatcatgagcattatcaaagaagaggtgctggcctacgtggtgcagctgcctctgtatggcgtgatcgataccccttgctggaagctgcacacaagccctctgtgcaccaccaacaccaaagagggctccaacatctgcctgaccagaaccgatagaggctggtactgcgataatgccggcagcgtcagcttcttcccacaagccgagacatgcaaggtgcagagcaacagagtgttctgcgataccatgaacagcctgacactgccctccgaagtgaatctgtgcaatatcgacatcttcaacccgaagtacgactgcaagatcatgaccagcaagaccgacgtgtcaagctccgtgatcacatctctgggcgccatcgtgtcctgctacggcaagacaaagtgcaccgccagcaacaagaaccggggcatcatcaagaccttcagcaacggctgcgactacgtgtccaacaaaggcgtggacaccgtgtctgtgggcaacaccctgtactacgtgaacaagcaagaaggcaagagcctgtacgtgaagggcgagcccatcatcaacttctacgaccctctggtgttccccagcgacgagtttgatgccagcatctcccaagtgaacgagaagatcaaccagagcctggccttcatcagaaagtccgatgagctgctgcacaacgtgaacgccggcaagtccaccaccaatatcatgatcaccacgatcatcatcgtgatcatcgtcatcctgctggctctgatcgctgtgggcctgctgctgtattgatga

SEQ ID NO: 285 - DNA, 1653 bp, synthetic construct
  source 1..1653: mol_type = other DNA
atggaactgcccatcctgaaaacaaacgccatcaccaccatcctggccgccgtgacactgtgttttgccagcagccagaacatcaccgaagagttctaccagagcacctgtagcgccgtgtctaagggctatctgtctgccctgagaaccggctggtataccagcgtgatcaccatcgagctgagcaacatcaaagaaaacaagtgcaacggcaccgacgccaaagtgaagctgatcaagcaagagctggacaagtacaagaacgccgtgaccgaactgcagctgctgatgcagtctacccctgccgccaatagcagagccagacgggaactgcctagattcatgaactacaccctgaacaacaccaagaacaccaacgtgaccctgagcaagaagcggaagcggagattcctgggctttctgctcggagtgggaagcgccattgcctctggaattgccgtgtccaaggtgctgcatctggaaggcgaagtgaacaagatcaagagcgccctgctgagcaccaacaaggccgtggtttctctgagcaatggcgtgtccgtgctgaccatcaaggtgctggacctgaagaactacatcgacaaacagctgctgcccatcgtcaacaagcagagctgcagcatcagcaacatcgagacagtgatcgagttccagcagaagaacaaccggctgctggaaatcacccgcgagttttctgtgaatgccggcgtgaccacacctgtgtccacctacatgctgaccaacagcgagctgctgtccctgatcaacgacatgcccatcaccaacgaccagaaaaagctgatgagcagcaacgtgcagatcgtgcggcagcagagctactccatcatgagcattatcaaagaagaggtgctggcctacgtggtgcagctgcctctgtatggcgtgatcgataccccttgctggaagctgcacacaagccctctgtgcaccaccaacaccaaagagggctccaacatctgcctgaccagaaccgatagaggctggtactgcgataatgccggcagcgtcagcttcttcccacaagccgagacatgcaaggtgcagagcaacagagtgttctgcgataccatgaacagcctgacactgccctccgaagtgaatctgtgcaatatcgacatcttcaacccgaagtacgactgcaagatcatgaccagcaagaccgacgtgtcaagctccgtgatcacatctctgggcgccatcgtgtcctgctacggcaagacaaagtgcaccgccagcaacaagaaccggggcatcatcaagaccttcagcaacggctgcgactacgtgtccaacaaaggcgtggacaccgtgtctgtgggcaacaccctgtactacgtgaacaagcaagaaggcaagagcctgtacgtgaagggcgagcccatcatcaacttctacgaccctctggtgttccccagcgacgagtttgatgccagcatctcccaagtgaacgagaagatcaaccagagcctggccttcatcagaaagtccgatgagctgctgcacaacgtgaacgccggcaagtccaccaccaatatcatgatcaccacgatcatcatcgtgatcatcgtcatcctgctggctctgatcgctgtgggcctgctgctgtattgatga

SEQ ID NO: 286 - DNA, 1653 bp, synthetic construct
  source 1..1653: mol_type = other DNA
atggaactgcccatcctgaaaacaaacgccatcaccaccatcctggccgccgtgacactgtgttttgccagcagccagaacatcaccgaagagttctaccagagcacctgtagcgccgtgtctaagggctatctgtctgccctgagaaccggctggtataccagcgtgatcaccatcgagctgagcaacatcaaagaaaacaagtgcaacggcaccgacgccaaagtgaagctgatcaagcaagagctggacaagtacaagaacgccgtgaccgaactgcagctgctgatgcagtctacccctgccgccaatagcagagccagacgggaactgcctagattcatgaactacaccctgaacaacaccaagaacaccaacgtgaccctgagcaagaagcggaagcggagattcctgggctttctgctcggagtgggaagcgccattgcctctggaattgccgtgtccaaggtgctgcatctggaaggcgaagtgaacaagatcaagagcgccctgctgagcaccaacaaggccgtggtttctctgagcaatggcgtgtccgtgctgacctctaaggtgctggacctgaagaactacatcgacaaacagctgctgcccatcgtcaacaagcagagctgcagcatcagcaacatcgagacagtgatcgagttccagcagaagaacaaccggctgctggaaatcacccgcgagttttctgtgaatgccggcgtgaccacacctgtgtccacctacatgctgaccaacagcgagctgctgtccctgatcaacgacatgcccatcaccaacgaccagaaaaagctgatgagcagcaacgtgcagatcgtgcggcagcagagctactccatcatgagcattatcaaagaagagctgctggcctacgtggtgcagctgcctctgtatggcgtgatcgataccccttgctggaagctgcacacaagccctctgtgcaccaccaacaccaaagagggctccaacatctgcctgaccagaaccgatagaggctggtactgcgataatgccggcagcgtcagcttcttcccacaagccgagacatgcaaggtgcagagcaacagagtgttctgcgataccatgaacagcctgacactgccctccgaagtgaatctgtgcaatatcgacatcttcaacccgaagtacgactgcaagatcatgaccagcaagaccgacgtgtcaagctccgtgatcacatctctgggcgccatcgtgtcctgctacggcaagacaaagtgcaccgccagcaacaagaaccggggcatcatcaagaccttcagcaacggctgcgactacgtgtccaacaaaggcgtggacaccgtgtctgtgggcaacaccctgtactacgtgaacaagcaagaaggcaagagcctgtacgtgaagggcgagcccatcatcaacttctacgaccctctggtgttccccagcgacgagtttgatgccagcatctcccaagtgaacgagaagatcaaccagagcctggccttcatcagaaagtccgatgagctgctgcacaacgtgaacgccggcaagtccaccaccaatatcatgatcaccacgatcatcatcgtgatcatcgtcatcctgctggctctgatcgctgtgggcctgctgctgtattgatga

SEQ ID NO: 287 - DNA, 1653 bp, synthetic construct
  source 1..1653: mol_type = other DNA
atggaactgcccatcctgaaaacaaacgccatcaccaccatcctggccgccgtgacactgtgttttgccagcagccagaacatcaccgaagagttctaccagagcacctgtagcgccgtgtctaagggctatctgtctgccctgagaaccggctggtatgccagcgtgatcaccatcgagctgagcaacatcaaagaaaacaagtgcaacggcaccgacgccaaagtgaagctgatcaagcaagagctggacaagtacaagaacgccgtgaccgaactgcagctgctgatgcagtctacccctgccgccaatagcagagccagacgggaactgcctagattcatgaactacaccctgaacaacaccaagaacaccaacgtgaccctgagcaagaagcggaagcggagattcctgggctttctgctcggagtgggaagcgccattgcctctggaattgccgtgtccaaggtgctgcatctggaaggcgaagtgaacaagatcaagagcgccctgctgagcaccaacaaggccgtggtttctctgagcaatggcgtgtccgtgctgaccatgaaggtgctggacctgaagaactacatcgacaaacagctgctgcccatcgtcaacaagcagagctgcagcatcagcaacatcgagacagtgatcgagttccagcagaagaacaaccggctgctggaaatcacccgcgagttttctgtgaatgccggcgtgaccacacctgtgtccacctacatgctgaccaacagcgagctgctgtccctgatcaacgacatgcccatcaccaacgaccagaaaaagctgatgagcagcaacgtgcagatcgtgcggcagcagagctactccatcatgagcattatcaaagaagaggtgctggcctacgtggtgcagctgcctctgtatggcgtgatcgataccccttgctggaagctgcacacaagccctctgtgcaccaccaacaccaaagagggctccaacatctgcctgaccagaaccgatagaggctggtactgcgataatgccggcagcgtcagcttcttcccacaagccgagacatgcaaggtgcagagcaacagagtgttctgcgataccatgaacagcctgacactgccctccgaagtgaatctgtgcaatatcgacatcttcaacccgaagtacgactgcaagatcatgaccagcaagaccgacgtgtcaagctccgtgatcacatctctgggcgccatcgtgtcctgctacggcaagacaaagtgcaccgccagcaacaagaaccggggcatcatcaagaccttcagcaacggctgcgactacgtgtccaacaaaggcgtggacaccgtgtctgtgggcaacaccctgtactacgtgaacaagcaagaaggcaagagcctgtacgtgaagggcgagcccatcatcaacttctacgaccctctggtgttccccagcgacgagtttgatgccagcatctcccaagtgaacgagaagatcaaccagagcctggccttcatcagaaagtccgatgagctgctgcacaacgtgaacgccggcaagtccaccaccaatatcatgatcaccacgatcatcatcgtgatcatcgtcatcctgctggctctgatcgctgtgggcctgctgctgtattgatga

SEQ ID NO: 288 - DNA, 1653 bp, synthetic construct
  source 1..1653: mol_type = other DNA
atggaactgcccatcctgaaaacaaacgccatcaccaccatcctggccgccgtgacactgtgttttgccagcagccagaacatcaccgaagagttctaccagagcacctgtagcgccgtgtctaagggctatctgtctgccctgagaaccggctggtatgccagcgtgatcaccatcgagctgagcaacatcaaagaaaacaagtgcaacggcaccgacgccaaagtgaagctgatcaagcaagagctggacaagtacaagaacgccgtgaccgaactgcagctgctgatgcagtctacccctgccgccaatagcagagccagacgggaactgcctagattcatgaactacaccctgaacaacaccaagaacaccaacgtgaccctgagcaagaagcggaagcggagattcctgggctttctgctcggagtgggaagcgccattgcctctggaattgccgtgtccaaggtgctgcatctggaaggcgaagtgaacaagatcaagagcgccctgctgagcaccaacaaggccgtggtttctctgagcaatggcgtgtccgtgctgacctctaaggtgctggacctgaagaactacatcgacaaacagctgctgcccatcgtcaacaagcagagctgcagcatcagcaacatcgagacagtgatcgagttccagcagaagaacaaccggctgctggaaatcacccgcgagttttctgtgaatgccggcgtgaccacacctgtgtccacctacatgctgaccaacagcgagctgctgtccctgatcaacgacatgcccatcaccaacgaccagaaaaagctgatgagcagcaacgtgcagatcgtgcggcagcagagctactccatcatgagcattatcaaagaagagctgctggcctacgtggtgcagctgcctctgtatggcgtgatcgataccccttgctggaagctgcacacaagccctctgtgcaccaccaacaccaaagagggctccaacatctgcctgaccagaaccgatagaggctggtactgcgataatgccggcagcgtcagcttcttcccacaagccgagacatgcaaggtgcagagcaacagagtgttctgcgataccatgaacagcctgacactgccctccgaagtgaatctgtgcaatatcgacatcttcaacccgaagtacgactgcaagatcatgaccagcaagaccgacgtgtcaagctccgtgatcacatctctgggcgccatcgtgtcctgctacggcaagacaaagtgcaccgccagcaacaagaaccggggcatcatcaagaccttcagcaacggctgcgactacgtgtccaacaaaggcgtggacaccgtgtctgtgggcaacaccctgtactacgtgaacaagcaagaaggcaagagcctgtacgtgaagggcgagcccatcatcaacttctacgaccctctggtgttccccagcgacgagtttgatgccagcatctcccaagtgaacgagaagatcaaccagagcctggccttcatcagaaagtccgatgagctgctgcacaacgtgaacgccggcaagtccaccaccaatatcatgatcaccacgatcatcatcgtgatcatcgtcatcctgctggctctgatcgctgtgggcctgctgctgtattgatga

SEQ ID NO: 289 - DNA, 1653 bp, synthetic construct
  source 1..1653: mol_type = other DNA
atggaactgcccatcctgaaaacaaacgccatcaccaccatcctggccgccgtgacactgtgttttgccagcagccagaacatcaccgaagagttctaccagagcacctgtagcgccgtgtctaagggctatctgtctgccctgagaaccggctggtataccagcgtgatcaccatcgagctgagcaacatcaaagaaaacaagtgcaacggcaccgacgccaaagtgaagctgatcaagcaagagctggacaagtacaagaacgccgtgaccgaactgcagctgctgatgcagtctacccctgccgccaatagcagagccagacgggaactgcctagattcatgaactacaccctgaacaacaccaagaacaccaacgtgaccctgagcaagaagcggaagcggagattcctgggctttctgctcggagtgggaagcgccattgcctctggaattgccgtgtccaaggtgctgcatctggaaggcgaagtgaacaagatcaagagcgccctgctgagcaccaacaaggccgtggtttctctgagcaatggcgtgtccgtgctgaccatgaaggtgctggacctgaagaactacatcgacaaacagctgctgcccatcgtcaacaagcagagctgcagcatcagcaacatcgagacagtgatcgagttccagcagaagaacaaccggctgctggaaatcacccgcgagttttctgtgaatgccggcgtgaccacacctgtgtccacctacatgctgaccaacagcgagctgctgtccctgatcaacgacatgcccatcaccaacgaccagaaaaagctgatgagcagcaacgtgcagatcgtgcggcagcagagctactccatcatgagcattatcaaagaagagctgctggcctacgtggtgcagctgcctctgtatggcgtgatcgataccccttgctggaagctgcacacaagccctctgtgcaccaccaacaccaaagagggctccaacatctgcctgaccagaaccgatagaggctggtactgcgataatgccggcagcgtcagcttcttcccacaagccgagacatgcaaggtgcagagcaacagagtgttctgcgataccatgaacagcctgacactgccctccgaagtgaatctgtgcaatatcgacatcttcaacccgaagtacgactgcaagatcatgaccagcaagaccgacgtgtcaagctccgtgatcacatctctgggcgccatcgtgtcctgctacggcaagacaaagtgcaccgccagcaacaagaaccggggcatcatcaagaccttcagcaacggctgcgactacgtgtccaacaaaggcgtggacaccgtgtctgtgggcaacaccctgtactacgtgaacaagcaagaaggcaagagcctgtacgtgaagggcgagcccatcatcaacttctacgaccctctggtgttccccagcgacgagtttgatgccagcatctcccaagtgaacgagaagatcaaccagagcctggccttcatcagaaagtccgatgagctgctgcacaacgtgaacgccggcaagtccaccaccaatatcatgatcaccacgatcatcatcgtgatcatcgtcatcctgctggctctgatcgctgtgggcctgctgctgtattgatga

SEQ ID NO: 290 - DNA, 1653 bp, synthetic construct
  source 1..1653: mol_type = other DNA
atggaactgcccatcctgaaaacaaacgccatcaccaccatcctggccgccgtgacactgtgttttgccagcagccagaacatcaccgaagagttctaccagagcacctgtagcgccgtgtctaagggctatctgtctgccctgagaaccggctggtatgccagcgtgatcaccatcgagctgagcaacatcaaagaaaacaagtgcaacggcaccgacgccaaagtgaagctgatcaagcaagagctggacaagtacaagaacgccgtgaccgaactgcagctgctgatgcagtctacccctgccgccaatagcagagccagacgggaactgcctagattcatgaactacaccctgaacaacaccaagaacaccaacgtgaccctgagcaagaagcggaagcggagattcctgggctttctgctcggagtgggaagcgccattgcctctggaattgccgtgtccaaggtgctgcatctggaaggcgaagtgaacaagatcaagagcgccctgctgagcaccaacaaggccgtggtttctctgagcaatggcgtgtccgtgctgaccatgaaggtgctggacctgaagaactacatcgacaaacagctgctgcccatcgtcaacaagcagagctgcagcatcagcaacatcgagacagtgatcgagttccagcagaagaacaaccggctgctggaaatcacccgcgagttttctgtgaatgccggcgtgaccacacctgtgtccacctacatgctgaccaacagcgagctgctgtccctgatcaacgacatgcccatcaccaacgaccagaaaaagctgatgagcagcaacgtgcagatcgtgcggcagcagagctactccatcatgagcattatcaaagaagagctgctggcctacgtggtgcagctgcctctgtatggcgtgatcgataccccttgctggaagctgcacacaagccctctgtgcaccaccaacaccaaagagggctccaacatctgcctgaccagaaccgatagaggctggtactgcgataatgccggcagcgtcagcttcttcccacaagccgagacatgcaaggtgcagagcaacagagtgttctgcgataccatgaacagcctgacactgccctccgaagtgaatctgtgcaatatcgacatcttcaacccgaagtacgactgcaagatcatgaccagcaagaccgacgtgtcaagctccgtgatcacatctctgggcgccatcgtgtcctgctacggcaagacaaagtgcaccgccagcaacaagaaccggggcatcatcaagaccttcagcaacggctgcgactacgtgtccaacaaaggcgtggacaccgtgtctgtgggcaacaccctgtactacgtgaacaagcaagaaggcaagagcctgtacgtgaagggcgagcccatcatcaacttctacgaccctctggtgttccccagcgacgagtttgatgccagcatctcccaagtgaacgagaagatcaaccagagcctggccttcatcagaaagtccgatgagctgctgcacaacgtgaacgccggcaagtccaccaccaatatcatgatcaccacgatcatcatcgtgatcatcgtcatcctgctggctctgatcgctgtgggcctgctgctgtattgatga

SEQ ID NO: 291 - DNA, 1653 bp, synthetic construct
  source 1..1653: mol_type = other DNA
atggaactgcccatcctgaaaacaaacgccatcaccaccatcctggccgccgtgacactgtgttttgccagcagccagaacatcaccgaagagttctaccagagcacctgtagcgccgtgtctaagggctatctgtctgccctgagaaccggctggtataccagcgtgatcaccatcgagctgagcaacatcaaagaaaacaagtgcaacggcaccgacgccaaagtgaagctgatcaagcaagagctggacaagtacaagaacgccgtgaccgaactgcagctgctgatgcagtctaccccttgcgccaatagcagagccagacgggaactgcctagattcatgaactacaccctgaacaacaccaagaacaccaacgtgaccctgagcaagaagcggaagcggagattcctgggctttctgctcggagtgggaagcgccattgcctctggatgcgccgtgtccaaggtgctgcatctggaaggcgaagtgaacaagatcaagagcgccctgctgagcaccaacaaggccgtggtttctctgagcaatggcgtgtccgtgctgacctctaaggtgctggacctgaagaactacatcgacaaacagctgctgcccatcgtcaacaagcagagctgcagcatcagcaacatcgagacagtgatcgagttccagcagaagaacaaccggctgctggaaatcacccgcgagttttctgtgaatgccggcgtgaccacacctgtgtccacctacatgctgaccaacagcgagctgctgtccctgatcaacgacatgcccatcaccaacgaccagaaaaagctgatgagcagcaacgtgcagatcgtgcggcagcagagctactccatcatgagcattatcaaagaagaggtgctggcctacgtggtgcagctgcctctgtatggcgtgatcgataccccttgctggaagctgcacacaagccctctgtgcaccaccaacaccaaagagggctccaacatctgcctgaccagaaccgatagaggctggtactgcgataatgccggcagcgtcagcttcttcccacaagccgagacatgcaaggtgcagagcaacagagtgttctgcgataccatgaacagcctgacactgccctccgaagtgaatctgtgcaatatcgacatcttcaacccgaagtacgactgcaagatcatgaccagcaagaccgacgtgtcaagctccgtgatcacatctctgggcgccatcgtgtcctgctacggcaagacaaagtgcaccgccagcaacaagaaccggggcatcatcaagaccttcagcaacggctgcgactacgtgtccaacaaaggcgtggacaccgtgtctgtgggcaacaccctgtactacgtgaacaagcaagaaggcaagagcctgtacgtgaagggcgagcccatcatcaacttctacgaccctctggtgttccccagcgacgagtttgatgccagcatctcccaagtgaacgagaagatcaaccagagcctggccttcatcagaaagtccgatgagctgctgcacaacgtgaacgccggcaagtccaccaccaatatcatgatcaccacgatcatcatcgtgatcatcgtcatcctgctggctctgatcgctgtgggcctgctgctgtattgatga

SEQ ID NO: 292 - DNA, 1653 bp, synthetic construct
  source 1..1653: mol_type = other DNA
atggaactgcccatcctgaaaacaaacgccatcaccaccatcctggccgccgtgacactgtgttttgccagcagccagaacatcaccgaagagttctaccagagcacctgtagcgccgtgtctaagggctatctgtctgccctgagaaccggctggtataccagcgtgatcaccatcgagctgagcaacatcaaagaaaacaagtgcaacggcaccgacgccaaagtgaagctgatcaagcaagagctggacaagtacaagaacgccgtgaccgaactgcagctgctgatgcagtctaccccttgcgccaatagcagagccagacgggaactgcctagattcatgaactacaccctgaacaacaccaagaacaccaacgtgaccctgagcaagaagcggaagcggagattcctgggctttctgctcggagtgggaagcgccattgcctctggaatttgcgtgtccaaggtgctgcatctggaaggcgaagtgaacaagatcaagagcgccctgctgagcaccaacaaggccgtggtttctctgagcaatggcgtgtccgtgctgacctctaaggtgctggacctgaagaactacatcgacaaacagctgctgcccatcgtcaacaagcagagctgcagcatcagcaacatcgagacagtgatcgagttccagcagaagaacaaccggctgctggaaatcacccgcgagttttctgtgaatgccggcgtgaccacacctgtgtccacctacatgctgaccaacagcgagctgctgtccctgatcaacgacatgcccatcaccaacgaccagaaaaagctgatgagcagcaacgtgcagatcgtgcggcagcagagctactccatcatgagcattatcaaagaagaggtgctggcctacgtggtgcagctgcctctgtatggcgtgatcgataccccttgctggaagctgcacacaagccctctgtgcaccaccaacaccaaagagggctccaacatctgcctgaccagaaccgatagaggctggtactgcgataatgccggcagcgtcagcttcttcccacaagccgagacatgcaaggtgcagagcaacagagtgttctgcgataccatgaacagcctgacactgccctccgaagtgaatctgtgcaatatcgacatcttcaacccgaagtacgactgcaagatcatgaccagcaagaccgacgtgtcaagctccgtgatcacatctctgggcgccatcgtgtcctgctacggcaagacaaagtgcaccgccagcaacaagaaccggggcatcatcaagaccttcagcaacggctgcgactacgtgtccaacaaaggcgtggacaccgtgtctgtgggcaacaccctgtactacgtgaacaagcaagaaggcaagagcctgtacgtgaagggcgagcccatcatcaacttctacgaccctctggtgttccccagcgacgagtttgatgccagcatctcccaagtgaacgagaagatcaaccagagcctggccttcatcagaaagtccgatgagctgctgcacaacgtgaacgccggcaagtccaccaccaatatcatgatcaccacgatcatcatcgtgatcatcgtcatcctgctggctctgatcgctgtgggcctgctgctgtattgatga

SEQ ID NO: 293 - DNA, 1653 bp, synthetic construct
  source 1..1653: mol_type = other DNA
atggaactgcccatcctgaaaacaaacgccatcaccaccatcctggccgccgtgacactgtgttttgccagcagccagaacatcaccgaagagttctaccagagcacctgtagcgccgtgtctaagggctatctgtctgccctgagaaccggctggtataccagcgtgatcaccatcgagctgagcaacatcaaagaaaacaagtgcaacggcaccgacgccaaagtgaagctgatcaagcaagagctggacaagtacaagaacgccgtgaccgaactgcagctgctgatgcagtctaccccttgcgccaatagcagagccagacgggaactgcctagattcatgaactacaccctgaacaacaccaagaacaccaacgtgaccctgagcaagaagcggaagcggagattcctgggctttctgctcggagtgggaagcgccattgcctgcggaattgccgtgtccaaggtgctgcatctggaaggcgaagtgaacaagatcaagagcgccctgctgagcaccaacaaggccgtggtttctctgagcaatggcgtgtccgtgctgacctctaaggtgctggacctgaagaactacatcgacaaacagctgctgcccatcgtcaacaagcagagctgcagcatcagcaacatcgagacagtgatcgagttccagcagaagaacaaccggctgctggaaatcacccgcgagttttctgtgaatgccggcgtgaccacacctgtgtccacctacatgctgaccaacagcgagctgctgtccctgatcaacgacatgcccatcaccaacgaccagaaaaagctgatgagcagcaacgtgcagatcgtgcggcagcagagctactccatcatgagcattatcaaagaagaggtgctggcctacgtggtgcagctgcctctgtatggcgtgatcgataccccttgctggaagctgcacacaagccctctgtgcaccaccaacaccaaagagggctccaacatctgcctgaccagaaccgatagaggctggtactgcgataatgccggcagcgtcagcttcttcccacaagccgagacatgcaaggtgcagagcaacagagtgttctgcgataccatgaacagcctgacactgccctccgaagtgaatctgtgcaatatcgacatcttcaacccgaagtacgactgcaagatcatgaccagcaagaccgacgtgtcaagctccgtgatcacatctctgggcgccatcgtgtcctgctacggcaagacaaagtgcaccgccagcaacaagaaccggggcatcatcaagaccttcagcaacggctgcgactacgtgtccaacaaaggcgtggacaccgtgtctgtgggcaacaccctgtactacgtgaacaagcaagaaggcaagagcctgtacgtgaagggcgagcccatcatcaacttctacgaccctctggtgttccccagcgacgagtttgatgccagcatctcccaagtgaacgagaagatcaaccagagcctggccttcatcagaaagtccgatgagctgctgcacaacgtgaacgccggcaagtccaccaccaatatcatgatcaccacgatcatcatcgtgatcatcgtcatcctgctggctctgatcgctgtgggcctgctgctgtattgatga